European Patent Application EP 4 711 452 A2, published March 18, 2026. Title: Klotho mRNA. Applicant: ADvantage Therapeutics, Inc. Application WO, filed March 21, 2024. The sequence listing filed with the application follows.

SEQUENCE LISTING (138 sequences)

SEQ ID NO: 1 - RNA, 1353 nt, synthetic construct
  source 1..1353: mol_type = other RNA
ctgttccagggcaccttccccgacggatttctgtgggccgtgggaagcgctgcctaccagaccgagggcggctggcaacagcacggcaagggcgccagcatctgggacaccttcacccaccatcctctggctcctcccggagacagcagaaacgccagcctgcctctgggagcccccagccccctgcagcccgccactggagacgtggccagcgactcctacaacaacgtgttccgcgacaccgaggccctgcgcgagctgggcgtgacccactaccgctttagcatcagctgggccagagtgctgcccaacggcagcgccggcgtgcccaaccgggaaggcctgagatactatcgccgcctgctggagaggctgagagagttgggcgtgcagcccgtggtgaccctgtaccactgggacctgccccagcgcctgcaggacgcctacggcggctgggccaacagggcactcgccgaccacttccgcgactacgccgagctgtgcttccgccacttcggcgggcaggtgaagtactggatcaccatcgacaacccctacgtggtggcctggcacggctacgctacaggaaggctggcccccgggatccgcggcagccccaggctgggctacctggtggcccacaacctgctgctggcacacgccaaagtgtggcacctgtataacaccagctttcgccccacccagggtggacaggtgagcattgccctgagttctcattggatcaaccccaggcgcatgaccgatcacagcatcaaggaatgccagaagagcctggacttcgtgctgggctggttcgccaagcccgtgtttatcgacggcgactaccccgagtctatgaagaacaacctcagcagcatcctgcctgacttcaccgagagcgagaagaagttcatcaagggcaccgccgacttcttcgccctgtgcttcggccccaccctgagcttccagctgctggatccccatatgaagttcagacaactcgagagtcctaacctgcgccagctgctgagctggatcgacctggaattcaaccacccacagatcttcatcgtggagaacggctggtttgtgagcggcaccactaagcgcgacgacgcaaagtatatgtattatctgaagaaattcatcatggaaaccctgaaggccatcaagctggacggcgtggacgtgatcggatacaccgcatggagcctgatggacggcttcgagtggcaccgcggttacagcatccgccggggcctgttctacgttgacttcctgagccaggacaagatgttgctgcccaagagctccgccctgttctaccagaagttgatcgagaagaacggcttc

SEQ ID NO: 2 - RNA, 1353 nt, synthetic construct
  source 1..1353: mol_type = other RNA
ttgtttcagggaacctttcctgacggtttcctgtgggctgtgggcagcgccgcctatcagaccgagggcggctggcaacagcacggaaaaggagccagcatctgggataccttcacccaccaccccctggccccccccggcgattcccgcaatgccagcctccctctgggagcccctagccccctgcaacctgccacaggagacgtggcctcagacagctataacaacgtgttccgcgacaccgaggcactgcgcgagctgggcgtgacccattaccgctttagcatcagctgggccagagtgctgcccaatggctctgccggcgtgcccaaccgggagggcctgaggtactaccgccgcctgctggagaggctgcgggagctgggcgtgcagcccgtggtaaccctgtaccactgggacctgccccagcgcctgcaggacgcttacggcggctgggccaaccgcgctctcgcagaccacttccgcgactacgccgagctgtgctttcgccactttggcggccaggtgaagtattggatcaccatcgataacccttacgtggtggcctggcacggatacgctacaggccgcctggcccccggcatccgcggcagccccagactgggctacctggtggcccacaacctgctgctggcccacgccaaggtgtggcacctgtacaacaccagcttccgccccacccagggtggacaggtctctattgccctgagctctcactggattaaccccaggaggatgaccgatcacagcatcaaggaatgccagaagagcctggacttcgttctgggctggttcgccaagcccgtgtttatcgacggcgactaccccgagagcatgaagaacaacctgtctagcatcctgcccgacttcaccgagagcgaaaaaaaattcatcaagggcaccgccgatttcttcgccctgtgtttcggcccaaccctgagcttccaactgctggatccccacatgaagttcagacaactcgagagtcccaacctgcgccagctgctgagctggatcgatctggaattcaaccacccccagatattcatagtggagaacggctggtttgtaagcggcactactaagcgcgatgatgcaaagtacatgtactatctgaagaagttcatcatggaaaccctgaaggccatcaagctggatggcgtggacgtgatcggatacaccgcatggagcctgatggacggcttcgagtggcaccgcggttactcaatccgcagggggttgttctacgtcgacttcctgagtcaggacaagatgttgctgccaaagagtagcgcccttttctaccagaagttgattgagaagaacggcttc

SEQ ID NO: 3 - RNA, 1353 nt, synthetic construct
  source 1..1353: mol_type = other RNA
ctgttccagggcaccttccccgacggatttctgtgggccgtgggaagcgctgcctaccagaccgagggcggctggcaacagcacggcaagggcgccagcatctgggacaccttcacccaccatcctctggctcctcccggagacagcagaaacgccagcctgcctctgggagcccccagccccctgcagcccgccactggagacgtggccagcgactcctacaacaacgtgttccgcgacaccgaggccctgcgcgagctgggcgtgacccactaccgctttagcatcagctgggccagagtgctgcccaacggcagcgccggcgtgcccaaccgggaaggcctgagatactatcgccgcctgctggagaggctgagagagttgggcgtgcagcccgtggtgaccctgtaccactgggacctgccccagcgcctgcaggacgcctacggcggctgggccaacagggcactcgccgaccacttccgcgactacgccgagctgtgcttccgccacttcggcgggcaggtgaagtactggatcaccatcgacaacccctacgtggtggcctggcacggctacgctacaggaaggctggcccccgggatccgcggcagccccaggctgggctacctggtggcccacaacctgctgctggcacacgccaaagtgtggcacctgtataacaccagctttcgccccacccagggtggacaggtgagcattgccctgagttctcattggatcaaccccaggcgcatgaccgatcacagcatcaaggaatgccagaagagcctggacttcgtgctgggctggttcgccaagcccgtgtttatcgacggcgactaccccgagtctatgaagaacaacctcagcagcatcctgcctgacgtcaccgagagcgagaagaagttcatcaagggcaccgccgacttcttcgccctgagcttcggccccaccctgagcttccagctgctggatccccatatgaagttcagacaactcgagagtcctaacctgcgccagctgctgagctggatcgacctggaattcaaccacccacagatcttcatcgtggagaacggctggtttgtgagcggcaccactaagcgcgacgacgcaaagtatatgtattatctgaagaaattcatcatggaaaccctgaaggccatcaagctggacggcgtggacgtgatcggatacaccgcatggagcctgatggacggcttcgagtggcaccgcggttacagcatccgccggggcctgttctacgttgacttcctgagccaggacaagatgttgctgcccaagagctccgccctgttctaccagaagttgatcgagaagaacggcttc

SEQ ID NO: 4 - RNA, 1353 nt, synthetic construct
  source 1..1353: mol_type = other RNA
ttgtttcagggaacctttcctgacggtttcctgtgggctgtgggcagcgccgcctatcagaccgagggcggctggcaacagcacggaaaaggagccagcatctgggataccttcacccaccaccccctggccccccccggcgattcccgcaatgccagcctccctctgggagcccctagccccctgcaacctgccacaggagacgtggcctcagacagctataacaacgtgttccgcgacaccgaggcactgcgcgagctgggcgtgacccattaccgctttagcatcagctgggccagagtgctgcccaatggctctgccggcgtgcccaaccgggagggcctgaggtactaccgccgcctgctggagaggctgcgggagctgggcgtgcagcccgtggtaaccctgtaccactgggacctgccccagcgcctgcaggacgcttacggcggctgggccaaccgcgctctcgcagaccacttccgcgactacgccgagctgtgctttcgccactttggcggccaggtgaagtattggatcaccatcgataacccttacgtggtggcctggcacggatacgctacaggccgcctggcccccggcatccgcggcagccccagactgggctacctggtggcccacaacctgctgctggcccacgccaaggtgtggcacctgtacaacaccagcttccgccccacccagggtggacaggtctctattgccctgagctctcactggattaaccccaggaggatgaccgatcacagcatcaaggaatgccagaagagcctggacttcgttctgggctggttcgccaagcccgtgtttatcgacggcgactaccccgagagcatgaagaacaacctgtctagcatcctgcccgacgtcaccgagagcgaaaaaaaattcatcaagggcaccgccgatttcttcgccctgagcttcggcccaaccctgagcttccaactgctggatccccacatgaagttcagacaactcgagagtcccaacctgcgccagctgctgagctggatcgatctggaattcaaccacccccagatattcatagtggagaacggctggtttgtaagcggcactactaagcgcgatgatgcaaagtacatgtactatctgaagaagttcatcatggaaaccctgaaggccatcaagctggatggcgtggacgtgatcggatacaccgcatggagcctgatggacggcttcgagtggcaccgcggttactcaatccgcagggggttgttctacgtcgacttcctgagtcaggacaagatgttgctgccaaagagtagcgcccttttctaccagaagttgattgagaagaacggcttc

SEQ ID NO: 5 - RNA, 1521 nt, synthetic construct
  source 1..1521: mol_type = other RNA
atgcccgctagcgccccaccgagaagaccgcggccgccaccgccatcgctgtcgctgctgctggtgctgctgggactgggcggaagaagactgcgtgcggagcctggcgacggggcccagacctgggccagattcagcagaccccccgcacccgaggccgccggcctgttccagggcaccttccccgacggatttctgtgggccgtgggaagcgctgcctaccagaccgagggcggctggcaacagcacggcaagggcgccagcatctgggacaccttcacccaccatcctctggctcctcccggagacagcagaaacgccagcctgcctctgggagcccccagccccctgcagcccgccactggagacgtggccagcgactcctacaacaacgtgttccgcgacaccgaggccctgcgcgagctgggcgtgacccactaccgctttagcatcagctgggccagagtgctgcccaacggcagcgccggcgtgcccaaccgggaaggcctgagatactatcgccgcctgctggagaggctgagagagttgggcgtgcagcccgtggtgaccctgtaccactgggacctgccccagcgcctgcaggacgcctacggcggctgggccaacagggcactcgccgaccacttccgcgactacgccgagctgtgcttccgccacttcggcgggcaggtgaagtactggatcaccatcgacaacccctacgtggtggcctggcacggctacgctacaggaaggctggcccccgggatccgcggcagccccaggctgggctacctggtggcccacaacctgctgctggcacacgccaaagtgtggcacctgtataacaccagctttcgccccacccagggtggacaggtgagcattgccctgagttctcattggatcaaccccaggcgcatgaccgatcacagcatcaaggaatgccagaagagcctggacttcgtgctgggctggttcgccaagcccgtgtttatcgacggcgactaccccgagtctatgaagaacaacctcagcagcatcctgcctgacttcaccgagagcgagaagaagttcatcaagggcaccgccgacttcttcgccctgtgcttcggccccaccctgagcttccagctgctggatccccatatgaagttcagacaactcgagagtcctaacctgcgccagctgctgagctggatcgacctggaattcaaccacccacagatcttcatcgtggagaacggctggtttgtgagcggcaccactaagcgcgacgacgcaaagtatatgtattatctgaagaaattcatcatggaaaccctgaaggccatcaagctggacggcgtggacgtgatcggatacaccgcatggagcctgatggacggcttcgagtggcaccgcggttacagcatccgccggggcctgttctacgttgacttcctgagccaggacaagatgttgctgcccaagagctccgccctgttctaccagaagttgatcgagaagaacggcttctga

SEQ ID NO: 6 - RNA, 1521 nt, synthetic construct
  source 1..1521: mol_type = other RNA
atgcccgctagcgccccaccgagaagaccgcggccgccaccgccatcgctgtcgctgctgctggtgctgctgggactgggcggaagaagactgcgtgcggagcctggagatggagcccaaacatgggccagattcagcagacctcccgctcctgaagccgccggcttgtttcagggaacctttcctgacggtttcctgtgggctgtgggcagcgccgcctatcagaccgagggcggctggcaacagcacggaaaaggagccagcatctgggataccttcacccaccaccccctggccccccccggcgattcccgcaatgccagcctccctctgggagcccctagccccctgcaacctgccacaggagacgtggcctcagacagctataacaacgtgttccgcgacaccgaggcactgcgcgagctgggcgtgacccattaccgctttagcatcagctgggccagagtgctgcccaatggctctgccggcgtgcccaaccgggagggcctgaggtactaccgccgcctgctggagaggctgcgggagctgggcgtgcagcccgtggtaaccctgtaccactgggacctgccccagcgcctgcaggacgcttacggcggctgggccaaccgcgctctcgcagaccacttccgcgactacgccgagctgtgctttcgccactttggcggccaggtgaagtattggatcaccatcgataacccttacgtggtggcctggcacggatacgctacaggccgcctggcccccggcatccgcggcagccccagactgggctacctggtggcccacaacctgctgctggcccacgccaaggtgtggcacctgtacaacaccagcttccgccccacccagggtggacaggtctctattgccctgagctctcactggattaaccccaggaggatgaccgatcacagcatcaaggaatgccagaagagcctggacttcgttctgggctggttcgccaagcccgtgtttatcgacggcgactaccccgagagcatgaagaacaacctgtctagcatcctgcccgacttcaccgagagcgaaaaaaaattcatcaagggcaccgccgatttcttcgccctgtgtttcggcccaaccctgagcttccaactgctggatccccacatgaagttcagacaactcgagagtcccaacctgcgccagctgctgagctggatcgatctggaattcaaccacccccagatattcatagtggagaacggctggtttgtaagcggcactactaagcgcgatgatgcaaagtacatgtactatctgaagaagttcatcatggaaaccctgaaggccatcaagctggatggcgtggacgtgatcggatacaccgcatggagcctgatggacggcttcgagtggcaccgcggttactcaatccgcagggggttgttctacgtcgacttcctgagtcaggacaagatgttgctgccaaagagtagcgcccttttctaccagaagttgattgagaagaacggcttctga

SEQ ID NO: 7 - RNA, 1521 nt, synthetic construct
  source 1..1521: mol_type = other RNA
atgcccgctagcgccccaccgagaagaccgcggccgccaccgccatcgctgtcgctgctgctggtgctgctgggactgggcggaagaagactgcgtgcggagcctggcgacggggcccagacctgggccagattcagcagaccccccgcacccgaggccgccggcctgttccagggcaccttccccgacggatttctgtgggccgtgggaagcgctgcctaccagaccgagggcggctggcaacagcacggcaagggcgccagcatctgggacaccttcacccaccatcctctggctcctcccggagacagcagaaacgccagcctgcctctgggagcccccagccccctgcagcccgccactggagacgtggccagcgactcctacaacaacgtgttccgcgacaccgaggccctgcgcgagctgggcgtgacccactaccgctttagcatcagctgggccagagtgctgcccaacggcagcgccggcgtgcccaaccgggaaggcctgagatactatcgccgcctgctggagaggctgagagagttgggcgtgcagcccgtggtgaccctgtaccactgggacctgccccagcgcctgcaggacgcctacggcggctgggccaacagggcactcgccgaccacttccgcgactacgccgagctgtgcttccgccacttcggcgggcaggtgaagtactggatcaccatcgacaacccctacgtggtggcctggcacggctacgctacaggaaggctggcccccgggatccgcggcagccccaggctgggctacctggtggcccacaacctgctgctggcacacgccaaagtgtggcacctgtataacaccagctttcgccccacccagggtggacaggtgagcattgccctgagttctcattggatcaaccccaggcgcatgaccgatcacagcatcaaggaatgccagaagagcctggacttcgtgctgggctggttcgccaagcccgtgtttatcgacggcgactaccccgagtctatgaagaacaacctcagcagcatcctgcctgacgtcaccgagagcgagaagaagttcatcaagggcaccgccgacttcttcgccctgagcttcggccccaccctgagcttccagctgctggatccccatatgaagttcagacaactcgagagtcctaacctgcgccagctgctgagctggatcgacctggaattcaaccacccacagatcttcatcgtggagaacggctggtttgtgagcggcaccactaagcgcgacgacgcaaagtatatgtattatctgaagaaattcatcatggaaaccctgaaggccatcaagctggacggcgtggacgtgatcggatacaccgcatggagcctgatggacggcttcgagtggcaccgcggttacagcatccgccggggcctgttctacgttgacttcctgagccaggacaagatgttgctgcccaagagctccgccctgttctaccagaagttgatcgagaagaacggcttctga

SEQ ID NO: 8 - RNA, 1521 nt, synthetic construct
  source 1..1521: mol_type = other RNA
atgcccgctagcgccccaccgagaagaccgcggccgccaccgccatcgctgtcgctgctgctggtgctgctgggactgggcggaagaagactgcgtgcggagcctggagatggagcccaaacatgggccagattcagcagacctcccgctcctgaagccgccggcttgtttcagggaacctttcctgacggtttcctgtgggctgtgggcagcgccgcctatcagaccgagggcggctggcaacagcacggaaaaggagccagcatctgggataccttcacccaccaccccctggccccccccggcgattcccgcaatgccagcctccctctgggagcccctagccccctgcaacctgccacaggagacgtggcctcagacagctataacaacgtgttccgcgacaccgaggcactgcgcgagctgggcgtgacccattaccgctttagcatcagctgggccagagtgctgcccaatggctctgccggcgtgcccaaccgggagggcctgaggtactaccgccgcctgctggagaggctgcgggagctgggcgtgcagcccgtggtaaccctgtaccactgggacctgccccagcgcctgcaggacgcttacggcggctgggccaaccgcgctctcgcagaccacttccgcgactacgccgagctgtgctttcgccactttggcggccaggtgaagtattggatcaccatcgataacccttacgtggtggcctggcacggatacgctacaggccgcctggcccccggcatccgcggcagccccagactgggctacctggtggcccacaacctgctgctggcccacgccaaggtgtggcacctgtacaacaccagcttccgccccacccagggtggacaggtctctattgccctgagctctcactggattaaccccaggaggatgaccgatcacagcatcaaggaatgccagaagagcctggacttcgttctgggctggttcgccaagcccgtgtttatcgacggcgactaccccgagagcatgaagaacaacctgtctagcatcctgcccgacgtcaccgagagcgaaaaaaaattcatcaagggcaccgccgatttcttcgccctgagcttcggcccaaccctgagcttccaactgctggatccccacatgaagttcagacaactcgagagtcccaacctgcgccagctgctgagctggatcgatctggaattcaaccacccccagatattcatagtggagaacggctggtttgtaagcggcactactaagcgcgatgatgcaaagtacatgtactatctgaagaagttcatcatggaaaccctgaaggccatcaagctggatggcgtggacgtgatcggatacaccgcatggagcctgatggacggcttcgagtggcaccgcggttactcaatccgcagggggttgttctacgtcgacttcctgagtcaggacaagatgttgctgccaaagagtagcgcccttttctaccagaagttgattgagaagaacggcttctga

SEQ ID NO: 9 - RNA, 2691 nt, synthetic construct
  source 1..2691: mol_type = other RNA
ctgttccagggcaccttccccgacggatttctgtgggccgtgggaagcgctgcctaccagaccgagggcggctggcaacagcacggcaagggcgccagcatctgggacaccttcacccaccatcctctggctcctcccggagacagcagaaacgccagcctgcctctgggagcccccagccccctgcagcccgccactggagacgtggccagcgactcctacaacaacgtgttccgcgacaccgaggccctgcgcgagctgggcgtgacccactaccgctttagcatcagctgggccagagtgctgcccaacggcagcgccggcgtgcccaaccgggaaggcctgagatactatcgccgcctgctggagaggctgagagagttgggcgtgcagcccgtggtgaccctgtaccactgggacctgccccagcgcctgcaggacgcctacggcggctgggccaacagggcactcgccgaccacttccgcgactacgccgagctgtgcttccgccacttcggcgggcaggtgaagtactggatcaccatcgacaacccctacgtggtggcctggcacggctacgctacaggaaggctggcccccgggatccgcggcagccccaggctgggctacctggtggcccacaacctgctgctggcacacgccaaagtgtggcacctgtataacaccagctttcgccccacccagggtggacaggtgagcattgccctgagttctcattggatcaaccccaggcgcatgaccgatcacagcatcaaggaatgccagaagagcctggacttcgtgctgggctggttcgccaagcccgtgtttatcgacggcgactaccccgagtctatgaagaacaacctcagcagcatcctgcctgacttcaccgagagcgagaagaagttcatcaagggcaccgccgacttcttcgccctgtgcttcggccccaccctgagcttccagctgctggatccccatatgaagttcagacaactcgagagtcctaacctgcgccagctgctgagctggatcgacctggaattcaaccacccacagatcttcatcgtggagaacggctggtttgtgagcggcaccactaagcgcgacgacgcaaagtatatgtattatctgaagaaattcatcatggaaaccctgaaggccatcaagctggacggcgtggacgtgatcggatacaccgcatggagcctgatggacggcttcgagtggcaccgcggttacagcatccgccggggcctgttctacgttgacttcctgagccaggacaagatgttgctgcccaagagctccgccctgttctaccagaagttgatcgagaagaacggcttcccaccactccccgagaaccagcccctggagggcaccttcccctgcgatttcgcctggggcgtggtggacaactacatccaggtggacaccaccctgagtcagttcactgacctgaacgtgtacctttgggacgtgcaccacagcaagcgcctgataaaggtcgacggcgtggtgaccaagaagcgcaaaagctactgcgtggactttgccgccatccagccccagatcgccctgctgcaggagatgcacgtgactcacttccgcttcagcctcgactgggccctgattctgcccctgggcaaccagtcacaagtgaaccacaccattctgcagtactaccgctgtatggccagcgagctggtacgcgtgaacatcacccccgttgtggccctttggcagcccatggcccccaaccagggcctgcctcgcctgctggcccgccagggagcctgggagaatccctacaccgcactggccttcgctgaatacgcccgcctgtgcttccaggagctggggcaccacgtgaaactctggatcaccatgaacgagccctacaccagaaacatgacctacagcgccggacacaatctgctgaaggcccacgctctggcctggcacgtgtacaacgagaagtttcgccacgcccagaacggcaagatcagcatcgccctgcaggccgattggatcgagcccgcctgccccttcagccagaaggacaaggaggtggctgagcgggtgctggagttcgacatcgggtggctggctgagcctatcttcggcagcggagactacccctgggtgatgcgcgattggcttaaccagaggaacaatttcctgctgccctacttcaccgaggacgagaagaagctgatccagggcacctttgacttcctggctttgagccactataccactatcctggtggacagcgagaaggaggaccccatcaagtacaacgactacttggaggtgcaggagatgaccgacatcacctggctgaacagccctagccaggtggctgtggtgccttggggcctgcgcaaggtgctgaactggctgaagttcaagtacggcgacctgcccatgtatatcatcagcaacggcatcgacgacggcctgcacgccgaggacgaccagctgagagtgtactacatgcagaactacatcaacgaggccctcaaggcccacatcctggacggcatcaacctgtgtggctactttgcctacagcttcaacgacagaaccgccccccgcttcggcctgtacaggtacgccgccgaccagttcgaacccaaggccagcatgaagcactaccgcaaaatcatcgacagcaacgga

SEQ ID NO: 10 - RNA, 2691 nt, synthetic construct
  source 1..2691: mol_type = other RNA
ttgtttcagggaacctttcctgacggtttcctgtgggctgtgggcagcgccgcctatcagaccgagggcggctggcaacagcacggaaaaggagccagcatctgggataccttcacccaccaccccctggccccccccggcgattcccgcaatgccagcctccctctgggagcccctagccccctgcaacctgccacaggagacgtggcctcagacagctataacaacgtgttccgcgacaccgaggcactgcgcgagctgggcgtgacccattaccgctttagcatcagctgggccagagtgctgcccaatggctctgccggcgtgcccaaccgggagggcctgaggtactaccgccgcctgctggagaggctgcgggagctgggcgtgcagcccgtggtaaccctgtaccactgggacctgccccagcgcctgcaggacgcttacggcggctgggccaaccgcgctctcgcagaccacttccgcgactacgccgagctgtgctttcgccactttggcggccaggtgaagtattggatcaccatcgataacccttacgtggtggcctggcacggatacgctacaggccgcctggcccccggcatccgcggcagccccagactgggctacctggtggcccacaacctgctgctggcccacgccaaggtgtggcacctgtacaacaccagcttccgccccacccagggtggacaggtctctattgccctgagctctcactggattaaccccaggaggatgaccgatcacagcatcaaggaatgccagaagagcctggacttcgttctgggctggttcgccaagcccgtgtttatcgacggcgactaccccgagagcatgaagaacaacctgtctagcatcctgcccgacttcaccgagagcgaaaaaaaattcatcaagggcaccgccgatttcttcgccctgtgtttcggcccaaccctgagcttccaactgctggatccccacatgaagttcagacaactcgagagtcccaacctgcgccagctgctgagctggatcgatctggaattcaaccacccccagatattcatagtggagaacggctggtttgtaagcggcactactaagcgcgatgatgcaaagtacatgtactatctgaagaagttcatcatggaaaccctgaaggccatcaagctggatggcgtggacgtgatcggatacaccgcatggagcctgatggacggcttcgagtggcaccgcggttactcaatccgcagggggttgttctacgtcgacttcctgagtcaggacaagatgttgctgccaaagagtagcgcccttttctaccagaagttgattgagaagaacggcttcccaccactccccgagaaccagcccctggagggcacctttccctgcgatttcgcttggggcgtggtggataattatattcaggtggacaccaccctgtcacagttcactgacctgaacgtgtacctgtgggacgtgcaccattccaagcgcctgatcaaggtggacggcgtggtgaccaagaagcgcaaatcctactgcgttgactttgccgccattcagccacagatcgccctgctgcaggagatgcacgtcacccacttccgcttcagcctggactgggccctcatcctgccactgggcaaccagtcccaggtgaaccacaccattctgcagtactaccgctgtatggccagcgagctggtacgcgtgaacatcacccccgtggtggccctgtggcagcccatggcccccaaccagggcctgccacgcctgctggccaggcagggggcctgggagaacccctacaccgcactcgctttcgccgaatatgccaggctgtgcttccaggagctggggcaccacgtgaagctctggatcaccatgaacgaaccctacaccagaaacatgacctactctgccggacacaatctgctgaaggcccacgccctggcctggcacgtctacaacgagaagttccgccacgcccaaaatggaaagatctctatagccctgcaggccgattggatcgagcccgcctgccccttctcacagaaggacaaggaggtggccgagcgcgtgctggagttcgacatcggctggctggccgagcccatcttcggcagcggagactacccctgggtgatgcgcgattggcttaaccagcgcaacaactttctgctgccctacttcaccgaggacgagaagaagctgatccagggcaccttcgacttcctggccctgagccactatactaccatcctggtcgacagcgagaaggaggacccaatcaagtacaacgactacctggaggtgcaggagatgaccgacatcacctggctgaacagccctagccaggtcgccgtggtgccttggggcctgcgcaaggtgctgaactggctgaagttcaagtatggcgacctgccaatgtacatcatcagcaacggcattgatgacggcctgcacgccgaggacgatcagctgagagtgtactatatgcagaactacatcaacgaggcactgaaggcccacatcctggacggcatcaacctgtgtggctactttgcatactccttcaacgacagaaccgccccccgcttcggcctgtacaggtacgctgccgatcagttcgagcccaaggccagcatgaagcactacagaaaaatcattgatagcaacggg

SEQ ID NO: 11 - RNA, 2691 nt, synthetic construct
  source 1..2691: mol_type = other RNA
ctgttccagggcaccttccccgacggatttctgtgggccgtgggaagcgctgcctaccagaccgagggcggctggcaacagcacggcaagggcgccagcatctgggacaccttcacccaccatcctctggctcctcccggagacagcagaaacgccagcctgcctctgggagcccccagccccctgcagcccgccactggagacgtggccagcgactcctacaacaacgtgttccgcgacaccgaggccctgcgcgagctgggcgtgacccactaccgctttagcatcagctgggccagagtgctgcccaacggcagcgccggcgtgcccaaccgggaaggcctgagatactatcgccgcctgctggagaggctgagagagttgggcgtgcagcccgtggtgaccctgtaccactgggacctgccccagcgcctgcaggacgcctacggcggctgggccaacagggcactcgccgaccacttccgcgactacgccgagctgtgcttccgccacttcggcgggcaggtgaagtactggatcaccatcgacaacccctacgtggtggcctggcacggctacgctacaggaaggctggcccccgggatccgcggcagccccaggctgggctacctggtggcccacaacctgctgctggcacacgccaaagtgtggcacctgtataacaccagctttcgccccacccagggtggacaggtgagcattgccctgagttctcattggatcaaccccaggcgcatgaccgatcacagcatcaaggaatgccagaagagcctggacttcgtgctgggctggttcgccaagcccgtgtttatcgacggcgactaccccgagtctatgaagaacaacctcagcagcatcctgcctgacgtcaccgagagcgagaagaagttcatcaagggcaccgccgacttcttcgccctgagcttcggccccaccctgagcttccagctgctggatccccatatgaagttcagacaactcgagagtcctaacctgcgccagctgctgagctggatcgacctggaattcaaccacccacagatcttcatcgtggagaacggctggtttgtgagcggcaccactaagcgcgacgacgcaaagtatatgtattatctgaagaaattcatcatggaaaccctgaaggccatcaagctggacggcgtggacgtgatcggatacaccgcatggagcctgatggacggcttcgagtggcaccgcggttacagcatccgccggggcctgttctacgttgacttcctgagccaggacaagatgttgctgcccaagagctccgccctgttctaccagaagttgatcgagaagaacggcttcccaccactccccgagaaccagcccctggagggcaccttcccctgcgatttcgcctggggcgtggtggacaactacatccaggtggacaccaccctgagtcagttcactgacctgaacgtgtacctttgggacgtgcaccacagcaagcgcctgataaaggtcgacggcgtggtgaccaagaagcgcaaaagctactgcgtggactttgccgccatccagccccagatcgccctgctgcaggagatgcacgtgactcacttccgcttcagcctcgactgggccctgattctgcccctgggcaaccagtcacaagtgaaccacaccattctgcagtactaccgctgtatggccagcgagctggtacgcgtgaacatcacccccgttgtggccctttggcagcccatggcccccaaccagggcctgcctcgcctgctggcccgccagggagcctgggagaatccctacaccgcactggccttcgctgaatacgcccgcctgtgcttccaggagctggggcaccacgtgaaactctggatcaccatgaacgagccctacaccagaaacatgacctacagcgccggacacaatctgctgaaggcccacgctctggcctggcacgtgtacaacgagaagtttcgccacgcccagaacggcaagatcagcatcgccctgcaggccgattggatcgagcccgcctgccccttcagccagaaggacaaggaggtggctgagcgggtgctggagttcgacatcgggtggctggctgagcctatcttcggcagcggagactacccctgggtgatgcgcgattggcttaaccagaggaacaatttcctgctgccctacttcaccgaggacgagaagaagctgatccagggcacctttgacttcctggctttgagccactataccactatcctggtggacagcgagaaggaggaccccatcaagtacaacgactacttggaggtgcaggagatgaccgacatcacctggctgaacagccctagccaggtggctgtggtgccttggggcctgcgcaaggtgctgaactggctgaagttcaagtacggcgacctgcccatgtatatcatcagcaacggcatcgacgacggcctgcacgccgaggacgaccagctgagagtgtactacatgcagaactacatcaacgaggccctcaaggcccacatcctggacggcatcaacctgtgtggctactttgcctacagcttcaacgacagaaccgccccccgcttcggcctgtacaggtacgccgccgaccagttcgaacccaaggccagcatgaagcactaccgcaaaatcatcgacagcaacgga

SEQ ID NO: 12 - RNA, 2691 nt, synthetic construct
  source 1..2691: mol_type = other RNA
ttgtttcagggaacctttcctgacggtttcctgtgggctgtgggcagcgccgcctatcagaccgagggcggctggcaacagcacggaaaaggagccagcatctgggataccttcacccaccaccccctggccccccccggcgattcccgcaatgccagcctccctctgggagcccctagccccctgcaacctgccacaggagacgtggcctcagacagctataacaacgtgttccgcgacaccgaggcactgcgcgagctgggcgtgacccattaccgctttagcatcagctgggccagagtgctgcccaatggctctgccggcgtgcccaaccgggagggcctgaggtactaccgccgcctgctggagaggctgcgggagctgggcgtgcagcccgtggtaaccctgtaccactgggacctgccccagcgcctgcaggacgcttacggcggctgggccaaccgcgctctcgcagaccacttccgcgactacgccgagctgtgctttcgccactttggcggccaggtgaagtattggatcaccatcgataacccttacgtggtggcctggcacggatacgctacaggccgcctggcccccggcatccgcggcagccccagactgggctacctggtggcccacaacctgctgctggcccacgccaaggtgtggcacctgtacaacaccagcttccgccccacccagggtggacaggtctctattgccctgagctctcactggattaaccccaggaggatgaccgatcacagcatcaaggaatgccagaagagcctggacttcgttctgggctggttcgccaagcccgtgtttatcgacggcgactaccccgagagcatgaagaacaacctgtctagcatcctgcccgacgtcaccgagagcgaaaaaaaattcatcaagggcaccgccgatttcttcgccctgagcttcggcccaaccctgagcttccaactgctggatccccacatgaagttcagacaactcgagagtcccaacctgcgccagctgctgagctggatcgatctggaattcaaccacccccagatattcatagtggagaacggctggtttgtaagcggcactactaagcgcgatgatgcaaagtacatgtactatctgaagaagttcatcatggaaaccctgaaggccatcaagctggatggcgtggacgtgatcggatacaccgcatggagcctgatggacggcttcgagtggcaccgcggttactcaatccgcagggggttgttctacgtcgacttcctgagtcaggacaagatgttgctgccaaagagtagcgcccttttctaccagaagttgattgagaagaacggcttcccaccactccccgagaaccagcccctggagggcacctttccctgcgatttcgcttggggcgtggtggataattatattcaggtggacaccaccctgtcacagttcactgacctgaacgtgtacctgtgggacgtgcaccattccaagcgcctgatcaaggtggacggcgtggtgaccaagaagcgcaaatcctactgcgttgactttgccgccattcagccacagatcgccctgctgcaggagatgcacgtcacccacttccgcttcagcctggactgggccctcatcctgccactgggcaaccagtcccaggtgaaccacaccattctgcagtactaccgctgtatggccagcgagctggtacgcgtgaacatcacccccgtggtggccctgtggcagcccatggcccccaaccagggcctgccacgcctgctggccaggcagggggcctgggagaacccctacaccgcactcgctttcgccgaatatgccaggctgtgcttccaggagctggggcaccacgtgaagctctggatcaccatgaacgaaccctacaccagaaacatgacctactctgccggacacaatctgctgaaggcccacgccctggcctggcacgtctacaacgagaagttccgccacgcccaaaatggaaagatctctatagccctgcaggccgattggatcgagcccgcctgccccttctcacagaaggacaaggaggtggccgagcgcgtgctggagttcgacatcggctggctggccgagcccatcttcggcagcggagactacccctgggtgatgcgcgattggcttaaccagcgcaacaactttctgctgccctacttcaccgaggacgagaagaagctgatccagggcaccttcgacttcctggccctgagccactatactaccatcctggtcgacagcgagaaggaggacccaatcaagtacaacgactacctggaggtgcaggagatgaccgacatcacctggctgaacagccctagccaggtcgccgtggtgccttggggcctgcgcaaggtgctgaactggctgaagttcaagtatggcgacctgccaatgtacatcatcagcaacggcattgatgacggcctgcacgccgaggacgatcagctgagagtgtactatatgcagaactacatcaacgaggcactgaaggcccacatcctggacggcatcaacctgtgtggctactttgcatactccttcaacgacagaaccgccccccgcttcggcctgtacaggtacgctgccgatcagttcgagcccaaggccagcatgaagcactacagaaaaatcattgatagcaacggg

SEQ ID NO: 13 - RNA, 2844 nt, synthetic construct
  source 1..2844: mol_type = other RNA
gagcctggcgacggggcccagacctgggccagattcagcagaccccccgcacccgaggccgccggcctgttccagggcaccttccccgacggatttctgtgggccgtgggaagcgctgcctaccagaccgagggcggctggcaacagcacggcaagggcgccagcatctgggacaccttcacccaccatcctctggctcctcccggagacagcagaaacgccagcctgcctctgggagcccccagccccctgcagcccgccactggagacgtggccagcgactcctacaacaacgtgttccgcgacaccgaggccctgcgcgagctgggcgtgacccactaccgctttagcatcagctgggccagagtgctgcccaacggcagcgccggcgtgcccaaccgggaaggcctgagatactatcgccgcctgctggagaggctgagagagttgggcgtgcagcccgtggtgaccctgtaccactgggacctgccccagcgcctgcaggacgcctacggcggctgggccaacagggcactcgccgaccacttccgcgactacgccgagctgtgcttccgccacttcggcgggcaggtgaagtactggatcaccatcgacaacccctacgtggtggcctggcacggctacgctacaggaaggctggcccccgggatccgcggcagccccaggctgggctacctggtggcccacaacctgctgctggcacacgccaaagtgtggcacctgtataacaccagctttcgccccacccagggtggacaggtgagcattgccctgagttctcattggatcaaccccaggcgcatgaccgatcacagcatcaaggaatgccagaagagcctggacttcgtgctgggctggttcgccaagcccgtgtttatcgacggcgactaccccgagtctatgaagaacaacctcagcagcatcctgcctgacttcaccgagagcgagaagaagttcatcaagggcaccgccgacttcttcgccctgtgcttcggccccaccctgagcttccagctgctggatccccatatgaagttcagacaactcgagagtcctaacctgcgccagctgctgagctggatcgacctggaattcaaccacccacagatcttcatcgtggagaacggctggtttgtgagcggcaccactaagcgcgacgacgcaaagtatatgtattatctgaagaaattcatcatggaaaccctgaaggccatcaagctggacggcgtggacgtgatcggatacaccgcatggagcctgatggacggcttcgagtggcaccgcggttacagcatccgccggggcctgttctacgttgacttcctgagccaggacaagatgttgctgcccaagagctccgccctgttctaccagaagttgatcgagaagaacggcttcccaccactccccgagaaccagcccctggagggcaccttcccctgcgatttcgcctggggcgtggtggacaactacatccaggtggacaccaccctgagtcagttcactgacctgaacgtgtacctttgggacgtgcaccacagcaagcgcctgataaaggtcgacggcgtggtgaccaagaagcgcaaaagctactgcgtggactttgccgccatccagccccagatcgccctgctgcaggagatgcacgtgactcacttccgcttcagcctcgactgggccctgattctgcccctgggcaaccagtcacaagtgaaccacaccattctgcagtactaccgctgtatggccagcgagctggtacgcgtgaacatcacccccgttgtggccctttggcagcccatggcccccaaccagggcctgcctcgcctgctggcccgccagggagcctgggagaatccctacaccgcactggccttcgctgaatacgcccgcctgtgcttccaggagctggggcaccacgtgaaactctggatcaccatgaacgagccctacaccagaaacatgacctacagcgccggacacaatctgctgaaggcccacgctctggcctggcacgtgtacaacgagaagtttcgccacgcccagaacggcaagatcagcatcgccctgcaggccgattggatcgagcccgcctgccccttcagccagaaggacaaggaggtggctgagcgggtgctggagttcgacatcgggtggctggctgagcctatcttcggcagcggagactacccctgggtgatgcgcgattggcttaaccagaggaacaatttcctgctgccctacttcaccgaggacgagaagaagctgatccagggcacctttgacttcctggctttgagccactataccactatcctggtggacagcgagaaggaggaccccatcaagtacaacgactacttggaggtgcaggagatgaccgacatcacctggctgaacagccctagccaggtggctgtggtgccttggggcctgcgcaaggtgctgaactggctgaagttcaagtacggcgacctgcccatgtatatcatcagcaacggcatcgacgacggcctgcacgccgaggacgaccagctgagagtgtactacatgcagaactacatcaacgaggccctcaaggcccacatcctggacggcatcaacctgtgtggctactttgcctacagcttcaacgacagaaccgccccccgcttcggcctgtacaggtacgccgccgaccagttcgaacccaaggccagcatgaagcactaccgcaaaatcatcgacagcaacggattccctggacccgagacactggagcgcttctgcccagaggagttcaccgtgtgcaccgagtgcagtttcttccacacccgcaagagc

SEQ ID NO: 14 - RNA, 2844 nt, synthetic construct
  source 1..2844: mol_type = other RNA
gagcctggagatggagcccaaacatgggccagattcagcagacctcccgctcctgaagccgccggcttgtttcagggaacctttcctgacggtttcctgtgggctgtgggcagcgccgcctatcagaccgagggcggctggcaacagcacggaaaaggagccagcatctgggataccttcacccaccaccccctggccccccccggcgattcccgcaatgccagcctccctctgggagcccctagccccctgcaacctgccacaggagacgtggcctcagacagctataacaacgtgttccgcgacaccgaggcactgcgcgagctgggcgtgacccattaccgctttagcatcagctgggccagagtgctgcccaatggctctgccggcgtgcccaaccgggagggcctgaggtactaccgccgcctgctggagaggctgcgggagctgggcgtgcagcccgtggtaaccctgtaccactgggacctgccccagcgcctgcaggacgcttacggcggctgggccaaccgcgctctcgcagaccacttccgcgactacgccgagctgtgctttcgccactttggcggccaggtgaagtattggatcaccatcgataacccttacgtggtggcctggcacggatacgctacaggccgcctggcccccggcatccgcggcagccccagactgggctacctggtggcccacaacctgctgctggcccacgccaaggtgtggcacctgtacaacaccagcttccgccccacccagggtggacaggtctctattgccctgagctctcactggattaaccccaggaggatgaccgatcacagcatcaaggaatgccagaagagcctggacttcgttctgggctggttcgccaagcccgtgtttatcgacggcgactaccccgagagcatgaagaacaacctgtctagcatcctgcccgacttcaccgagagcgaaaaaaaattcatcaagggcaccgccgatttcttcgccctgtgtttcggcccaaccctgagcttccaactgctggatccccacatgaagttcagacaactcgagagtcccaacctgcgccagctgctgagctggatcgatctggaattcaaccacccccagatattcatagtggagaacggctggtttgtaagcggcactactaagcgcgatgatgcaaagtacatgtactatctgaagaagttcatcatggaaaccctgaaggccatcaagctggatggcgtggacgtgatcggatacaccgcatggagcctgatggacggcttcgagtggcaccgcggttactcaatccgcagggggttgttctacgtcgacttcctgagtcaggacaagatgttgctgccaaagagtagcgcccttttctaccagaagttgattgagaagaacggcttcccaccactccccgagaaccagcccctggagggcacctttccctgcgatttcgcttggggcgtggtggataattatattcaggtggacaccaccctgtcacagttcactgacctgaacgtgtacctgtgggacgtgcaccattccaagcgcctgatcaaggtggacggcgtggtgaccaagaagcgcaaatcctactgcgttgactttgccgccattcagccacagatcgccctgctgcaggagatgcacgtcacccacttccgcttcagcctggactgggccctcatcctgccactgggcaaccagtcccaggtgaaccacaccattctgcagtactaccgctgtatggccagcgagctggtacgcgtgaacatcacccccgtggtggccctgtggcagcccatggcccccaaccagggcctgccacgcctgctggccaggcagggggcctgggagaacccctacaccgcactcgctttcgccgaatatgccaggctgtgcttccaggagctggggcaccacgtgaagctctggatcaccatgaacgaaccctacaccagaaacatgacctactctgccggacacaatctgctgaaggcccacgccctggcctggcacgtctacaacgagaagttccgccacgcccaaaatggaaagatctctatagccctgcaggccgattggatcgagcccgcctgccccttctcacagaaggacaaggaggtggccgagcgcgtgctggagttcgacatcggctggctggccgagcccatcttcggcagcggagactacccctgggtgatgcgcgattggcttaaccagcgcaacaactttctgctgccctacttcaccgaggacgagaagaagctgatccagggcaccttcgacttcctggccctgagccactatactaccatcctggtcgacagcgagaaggaggacccaatcaagtacaacgactacctggaggtgcaggagatgaccgacatcacctggctgaacagccctagccaggtcgccgtggtgccttggggcctgcgcaaggtgctgaactggctgaagttcaagtatggcgacctgccaatgtacatcatcagcaacggcattgatgacggcctgcacgccgaggacgatcagctgagagtgtactatatgcagaactacatcaacgaggcactgaaggcccacatcctggacggcatcaacctgtgtggctactttgcatactccttcaacgacagaaccgccccccgcttcggcctgtacaggtacgctgccgatcagttcgagcccaaggccagcatgaagcactacagaaaaatcattgatagcaacgggttcccaggccccgagaccctggagcgcttctgccccgaggagttcaccgtgtgcaccgagtgcagttttttccacacccgcaagagc

SEQ ID NO: 15 - RNA, 2844 nt, synthetic construct
  source 1..2844: mol_type = other RNA
gagcctggcgacggggcccagacctgggccagattcagcagaccccccgcacccgaggccgccggcctgttccagggcaccttccccgacggatttctgtgggccgtgggaagcgctgcctaccagaccgagggcggctggcaacagcacggcaagggcgccagcatctgggacaccttcacccaccatcctctggctcctcccggagacagcagaaacgccagcctgcctctgggagcccccagccccctgcagcccgccactggagacgtggccagcgactcctacaacaacgtgttccgcgacaccgaggccctgcgcgagctgggcgtgacccactaccgctttagcatcagctgggccagagtgctgcccaacggcagcgccggcgtgcccaaccgggaaggcctgagatactatcgccgcctgctggagaggctgagagagttgggcgtgcagcccgtggtgaccctgtaccactgggacctgccccagcgcctgcaggacgcctacggcggctgggccaacagggcactcgccgaccacttccgcgactacgccgagctgtgcttccgccacttcggcgggcaggtgaagtactggatcaccatcgacaacccctacgtggtggcctggcacggctacgctacaggaaggctggcccccgggatccgcggcagccccaggctgggctacctggtggcccacaacctgctgctggcacacgccaaagtgtggcacctgtataacaccagctttcgccccacccagggtggacaggtgagcattgccctgagttctcattggatcaaccccaggcgcatgaccgatcacagcatcaaggaatgccagaagagcctggacttcgtgctgggctggttcgccaagcccgtgtttatcgacggcgactaccccgagtctatgaagaacaacctcagcagcatcctgcctgacgtcaccgagagcgagaagaagttcatcaagggcaccgccgacttcttcgccctgagcttcggccccaccctgagcttccagctgctggatccccatatgaagttcagacaactcgagagtcctaacctgcgccagctgctgagctggatcgacctggaattcaaccacccacagatcttcatcgtggagaacggctggtttgtgagcggcaccactaagcgcgacgacgcaaagtatatgtattatctgaagaaattcatcatggaaaccctgaaggccatcaagctggacggcgtggacgtgatcggatacaccgcatggagcctgatggacggcttcgagtggcaccgcggttacagcatccgccggggcctgttctacgttgacttcctgagccaggacaagatgttgctgcccaagagctccgccctgttctaccagaagttgatcgagaagaacggcttcccaccactccccgagaaccagcccctggagggcaccttcccctgcgatttcgcctggggcgtggtggacaactacatccaggtggacaccaccctgagtcagttcactgacctgaacgtgtacctttgggacgtgcaccacagcaagcgcctgataaaggtcgacggcgtggtgaccaagaagcgcaaaagctactgcgtggactttgccgccatccagccccagatcgccctgctgcaggagatgcacgtgactcacttccgcttcagcctcgactgggccctgattctgcccctgggcaaccagtcacaagtgaaccacaccattctgcagtactaccgctgtatggccagcgagctggtacgcgtgaacatcacccccgttgtggccctttggcagcccatggcccccaaccagggcctgcctcgcctgctggcccgccagggagcctgggagaatccctacaccgcactggccttcgctgaatacgcccgcctgtgcttccaggagctggggcaccacgtgaaactctggatcaccatgaacgagccctacaccagaaacatgacctacagcgccggacacaatctgctgaaggcccacgctctggcctggcacgtgtacaacgagaagtttcgccacgcccagaacggcaagatcagcatcgccctgcaggccgattggatcgagcccgcctgccccttcagccagaaggacaaggaggtggctgagcgggtgctggagttcgacatcgggtggctggctgagcctatcttcggcagcggagactacccctgggtgatgcgcgattggcttaaccagaggaacaatttcctgctgccctacttcaccgaggacgagaagaagctgatccagggcacctttgacttcctggctttgagccactataccactatcctggtggacagcgagaaggaggaccccatcaagtacaacgactacttggaggtgcaggagatgaccgacatcacctggctgaacagccctagccaggtggctgtggtgccttggggcctgcgcaaggtgctgaactggctgaagttcaagtacggcgacctgcccatgtatatcatcagcaacggcatcgacgacggcctgcacgccgaggacgaccagctgagagtgtactacatgcagaactacatcaacgaggccctcaaggcccacatcctggacggcatcaacctgtgtggctactttgcctacagcttcaacgacagaaccgccccccgcttcggcctgtacaggtacgccgccgaccagttcgaacccaaggccagcatgaagcactaccgcaaaatcatcgacagcaacggattccctggacccgagacactggagcgcttctgcccagaggagttcaccgtgtgcaccgagtgcagtttcttccacacccgcaagagc

SEQ ID NO: 16 - RNA, 2844 nt, synthetic construct
  source 1..2844: mol_type = other RNA
gagcctggagatggagcccaaacatgggccagattcagcagacctcccgctcctgaagccgccggcttgtttcagggaacctttcctgacggtttcctgtgggctgtgggcagcgccgcctatcagaccgagggcggctggcaacagcacggaaaaggagccagcatctgggataccttcacccaccaccccctggccccccccggcgattcccgcaatgccagcctccctctgggagcccctagccccctgcaacctgccacaggagacgtggcctcagacagctataacaacgtgttccgcgacaccgaggcactgcgcgagctgggcgtgacccattaccgctttagcatcagctgggccagagtgctgcccaatggctctgccggcgtgcccaaccgggagggcctgaggtactaccgccgcctgctggagaggctgcgggagctgggcgtgcagcccgtggtaaccctgtaccactgggacctgccccagcgcctgcaggacgcttacggcggctgggccaaccgcgctctcgcagaccacttccgcgactacgccgagctgtgctttcgccactttggcggccaggtgaagtattggatcaccatcgataacccttacgtggtggcctggcacggatacgctacaggccgcctggcccccggcatccgcggcagccccagactgggctacctggtggcccacaacctgctgctggcccacgccaaggtgtggcacctgtacaacaccagcttccgccccacccagggtggacaggtctctattgccctgagctctcactggattaaccccaggaggatgaccgatcacagcatcaaggaatgccagaagagcctggacttcgttctgggctggttcgccaagcccgtgtttatcgacggcgactaccccgagagcatgaagaacaacctgtctagcatcctgcccgacgtcaccgagagcgaaaaaaaattcatcaagggcaccgccgatttcttcgccctgagcttcggcccaaccctgagcttccaactgctggatccccacatgaagttcagacaactcgagagtcccaacctgcgccagctgctgagctggatcgatctggaattcaaccacccccagatattcatagtggagaacggctggtttgtaagcggcactactaagcgcgatgatgcaaagtacatgtactatctgaagaagttcatcatggaaaccctgaaggccatcaagctggatggcgtggacgtgatcggatacaccgcatggagcctgatggacggcttcgagtggcaccgcggttactcaatccgcagggggttgttctacgtcgacttcctgagtcaggacaagatgttgctgccaaagagtagcgcccttttctaccagaagttgattgagaagaacggcttcccaccactccccgagaaccagcccctggagggcacctttccctgcgatttcgcttggggcgtggtggataattatattcaggtggacaccaccctgtcacagttcactgacctgaacgtgtacctgtgggacgtgcaccattccaagcgcctgatcaaggtggacggcgtggtgaccaagaagcgcaaatcctactgcgttgactttgccgccattcagccacagatcgccctgctgcaggagatgcacgtcacccacttccgcttcagcctggactgggccctcatcctgccactgggcaaccagtcccaggtgaaccacaccattctgcagtactaccgctgtatggccagcgagctggtacgcgtgaacatcacccccgtggtggccctgtggcagcccatggcccccaaccagggcctgccacgcctgctggccaggcagggggcctgggagaacccctacaccgcactcgctttcgccgaatatgccaggctgtgcttccaggagctggggcaccacgtgaagctctggatcaccatgaacgaaccctacaccagaaacatgacctactctgccggacacaatctgctgaaggcccacgccctggcctggcacgtctacaacgagaagttccgccacgcccaaaatggaaagatctctatagccctgcaggccgattggatcgagcccgcctgccccttctcacagaaggacaaggaggtggccgagcgcgtgctggagttcgacatcggctggctggccgagcccatcttcggcagcggagactacccctgggtgatgcgcgattggcttaaccagcgcaacaactttctgctgccctacttcaccgaggacgagaagaagctgatccagggcaccttcgacttcctggccctgagccactatactaccatcctggtcgacagcgagaaggaggacccaatcaagtacaacgactacctggaggtgcaggagatgaccgacatcacctggctgaacagccctagccaggtcgccgtggtgccttggggcctgcgcaaggtgctgaactggctgaagttcaagtatggcgacctgccaatgtacatcatcagcaacggcattgatgacggcctgcacgccgaggacgatcagctgagagtgtactatatgcagaactacatcaacgaggcactgaaggcccacatcctggacggcatcaacctgtgtggctactttgcatactccttcaacgacagaaccgccccccgcttcggcctgtacaggtacgctgccgatcagttcgagcccaaggccagcatgaagcactacagaaaaatcattgatagcaacgggttcccaggccccgagaccctggagcgcttctgccccgaggagttcaccgtgtgcaccgagtgcagttttttccacacccgcaagagc

SEQ ID NO: 17 - RNA, 2946 nt, Homo sapiens
  source 1..2946: mol_type = other RNA
atgcccgccagcgccccgccgcgccgcccgcggccgccgccgccgtcgctgtcgctgctgctggtgctgctgggcctgggcggccgccgcctgcgtgcggagccgggcgacggcgcgcagacctgggcccgtttctcgcggcctcctgcccccgaggccgcgggcctcttccagggcaccttccccgacggcttcctctgggccgtgggcagcgccgcctaccagaccgagggcggctggcagcagcacggcaagggtgcgtccatctgggatacgttcacccaccaccccctggcacccccgggagactcccggaacgccagtctgccgttgggcgccccgtcgccgctgcagcccgccaccggggacgtagccagcgacagctacaacaacgtcttccgcgacacggaggcgctgcgcgagctcggggtcactcactaccgcttctccatctcgtgggcgcgagtgctccccaatggcagcgcgggcgtccccaaccgcgaggggctgcgctactaccggcgcctgctggagcggctgcgggagctgggcgtgcagcccgtggtcaccctgtaccactgggacctgccccagcgcctgcaggacgcctacggcggctgggccaaccgcgccctggccgaccacttcagggattacgcggagctctgcttccgccacttcggcggtcaggtcaagtactggatcaccatcgacaacccctacgtggtggcctggcacggctacgccaccgggcgcctggcccccggcatccggggcagcccgcggctcgggtacctggtggcgcacaacctcctcctggctcatgccaaagtctggcatctctacaatacttctttccgtcccactcagggaggtcaggtgtccattgccctaagctctcactggatcaatcctcgaagaatgaccgaccacagcatcaaagaatgtcaaaaatctctggactttgtactaggttggtttgccaaacccgtatttattgatggtgactatcccgagagcatgaagaataacctttcatctattctgcctgattttactgaatctgagaaaaagttcatcaaaggaactgctgacttttttgctctttgctttggacccaccttgagttttcaacttttggaccctcacatgaagttccgccaattggaatctcccaacctgaggcaactgctttcctggattgaccttgaatttaaccatcctcaaatatttattgtggaaaatggctggtttgtctcagggaccaccaagagagatgatgccaaatatatgtattacctcaaaaagttcatcatggaaaccttaaaagccatcaagctggatggggtggatgtcatcgggtataccgcatggtccctcatggatggtttcgagtggcacagaggttacagcatcaggcgtggactcttctatgttgactttctaagccaggacaagatgttgttgccaaagtcttcagccttgttctaccaaaagctgatagagaaaaatggcttccctcctttacctgaaaatcagcccctagaagggacatttccctgtgactttgcttggggagttgttgacaactacattcaagtagataccactctgtctcagtttaccgacctgaatgtttacctgtgggatgtccaccacagtaaaaggcttattaaagtggatggggttgtgaccaagaagaggaaatcctactgtgttgactttgctgccatccagccccagatcgctttactccaggaaatgcacgttacacattttcgcttctccctggactgggccctgattctccctctgggtaaccagtcccaggtgaaccacaccatcctgcagtactatcgctgcatggccagcgagcttgtccgtgtcaacatcaccccagtggtggccctgtggcagcctatggccccgaaccaaggactgccgcgcctcctggccaggcagggcgcctgggagaacccctacactgccctggcctttgcagagtatgcccgactgtgctttcaagagctcggccatcacgtcaagctttggataacgatgaatgagccgtatacaaggaatatgacatacagtgctggccacaaccttctgaaggcccatgccctggcttggcatgtgtacaatgaaaagtttaggcatgctcagaatgggaaaatatccatagccttgcaggctgattggatagaacctgcctgccctttctcccaaaaggacaaagaggtggctgagagagttttggaatttgacattggctggctggctgagcccattttcggctctggagattatccatgggtgatgagggactggctgaaccaaagaaacaattttcttcttccttatttcactgaagatgaaaaaaagctaatccagggtacctttgactttttggctttaagccattataccaccatccttgtagactcagaaaaagaagatccaataaaatacaatgattacctagaagtgcaagaaatgaccgacatcacgtggctcaactcccccagtcaggtggcggtagtgccctgggggttgcgcaaagtgctgaactggctgaagttcaagtacggagacctccccatgtacataatatccaatggaatcgatgacgggctgcatgctgaggacgaccagctgagggtgtattatatgcagaattacataaacgaagctctcaaagcccacatactggatggtatcaatctttgcggatactttgcttattcgtttaacgaccgcacagctccgaggtttggcctctatcgttatgctgcagatcagtttgagcccaaggcatccatgaaacattacaggaaaattattgacagcaatggtttcccgggcccagaaactctggaaagattttgtccagaagaattcaccgtgtgtactgagtgcagtttttttcacacccgaaagtcttga

SEQ ID NO: 18 - RNA, 2946 nt, synthetic construct
  source 1..2946: mol_type = other RNA
atgcccgctagcgccccaccgagaagaccgcggccgccaccgccatcgctgtcgctgctgctggtgctgctgggactgggcggaagaagactgcgtgcggagcctggcgacggggcccagacctgggccagattcagcagaccccccgcacccgaggccgccggcctgttccagggcaccttccccgacggatttctgtgggccgtgggaagcgctgcctaccagaccgagggcggctggcaacagcacggcaagggcgccagcatctgggacaccttcacccaccatcctctggctcctcccggagacagcagaaacgccagcctgcctctgggagcccccagccccctgcagcccgccactggagacgtggccagcgactcctacaacaacgtgttccgcgacaccgaggccctgcgcgagctgggcgtgacccactaccgctttagcatcagctgggccagagtgctgcccaacggcagcgccggcgtgcccaaccgggaaggcctgagatactatcgccgcctgctggagaggctgagagagttgggcgtgcagcccgtggtgaccctgtaccactgggacctgccccagcgcctgcaggacgcctacggcggctgggccaacagggcactcgccgaccacttccgcgactacgccgagctgtgcttccgccacttcggcgggcaggtgaagtactggatcaccatcgacaacccctacgtggtggcctggcacggctacgctacaggaaggctggcccccgggatccgcggcagccccaggctgggctacctggtggcccacaacctgctgctggcacacgccaaagtgtggcacctgtataacaccagctttcgccccacccagggtggacaggtgagcattgccctgagttctcattggatcaaccccaggcgcatgaccgatcacagcatcaaggaatgccagaagagcctggacttcgtgctgggctggttcgccaagcccgtgtttatcgacggcgactaccccgagtctatgaagaacaacctcagcagcatcctgcctgacttcaccgagagcgagaagaagttcatcaagggcaccgccgacttcttcgccctgtgcttcggccccaccctgagcttccagctgctggatccccatatgaagttcagacaactcgagagtcctaacctgcgccagctgctgagctggatcgacctggaattcaaccacccacagatcttcatcgtggagaacggctggtttgtgagcggcaccactaagcgcgacgacgcaaagtatatgtattatctgaagaaattcatcatggaaaccctgaaggccatcaagctggacggcgtggacgtgatcggatacaccgcatggagcctgatggacggcttcgagtggcaccgcggttacagcatccgccggggcctgttctacgttgacttcctgagccaggacaagatgttgctgcccaagagctccgccctgttctaccagaagttgatcgagaagaacggcttcccaccactccccgagaaccagcccctggagggcaccttcccctgcgatttcgcctggggcgtggtggacaactacatccaggtggacaccaccctgagtcagttcactgacctgaacgtgtacctttgggacgtgcaccacagcaagcgcctgataaaggtcgacggcgtggtgaccaagaagcgcaaaagctactgcgtggactttgccgccatccagccccagatcgccctgctgcaggagatgcacgtgactcacttccgcttcagcctcgactgggccctgattctgcccctgggcaaccagtcacaagtgaaccacaccattctgcagtactaccgctgtatggccagcgagctggtacgcgtgaacatcacccccgttgtggccctttggcagcccatggcccccaaccagggcctgcctcgcctgctggcccgccagggagcctgggagaatccctacaccgcactggccttcgctgaatacgcccgcctgtgcttccaggagctggggcaccacgtgaaactctggatcaccatgaacgagccctacaccagaaacatgacctacagcgccggacacaatctgctgaaggcccacgctctggcctggcacgtgtacaacgagaagtttcgccacgcccagaacggcaagatcagcatcgccctgcaggccgattggatcgagcccgcctgccccttcagccagaaggacaaggaggtggctgagcgggtgctggagttcgacatcgggtggctggctgagcctatcttcggcagcggagactacccctgggtgatgcgcgattggcttaaccagaggaacaatttcctgctgccctacttcaccgaggacgagaagaagctgatccagggcacctttgacttcctggctttgagccactataccactatcctggtggacagcgagaaggaggaccccatcaagtacaacgactacttggaggtgcaggagatgaccgacatcacctggctgaacagccctagccaggtggctgtggtgccttggggcctgcgcaaggtgctgaactggctgaagttcaagtacggcgacctgcccatgtatatcatcagcaacggcatcgacgacggcctgcacgccgaggacgaccagctgagagtgtactacatgcagaactacatcaacgaggccctcaaggcccacatcctggacggcatcaacctgtgtggctactttgcctacagcttcaacgacagaaccgccccccgcttcggcctgtacaggtacgccgccgaccagttcgaacccaaggccagcatgaagcactaccgcaaaatcatcgacagcaacggattccctggacccgagacactggagcgcttctgcccagaggagttcaccgtgtgcaccgagtgcagtttcttccacacccgcaagagctga

SEQ ID NO: 19 - RNA, 2946 nt, synthetic construct
  source 1..2946: mol_type = other RNA
atgcccgctagcgccccaccgagaagaccgcggccgccaccgccatcgctgtcgctgctgctggtgctgctgggactgggcggaagaagactgcgtgcggagcctggagatggagcccaaacatgggccagattcagcagacctcccgctcctgaagccgccggcttgtttcagggaacctttcctgacggtttcctgtgggctgtgggcagcgccgcctatcagaccgagggcggctggcaacagcacggaaaaggagccagcatctgggataccttcacccaccaccccctggccccccccggcgattcccgcaatgccagcctccctctgggagcccctagccccctgcaacctgccacaggagacgtggcctcagacagctataacaacgtgttccgcgacaccgaggcactgcgcgagctgggcgtgacccattaccgctttagcatcagctgggccagagtgctgcccaatggctctgccggcgtgcccaaccgggagggcctgaggtactaccgccgcctgctggagaggctgcgggagctgggcgtgcagcccgtggtaaccctgtaccactgggacctgccccagcgcctgcaggacgcttacggcggctgggccaaccgcgctctcgcagaccacttccgcgactacgccgagctgtgctttcgccactttggcggccaggtgaagtattggatcaccatcgataacccttacgtggtggcctggcacggatacgctacaggccgcctggcccccggcatccgcggcagccccagactgggctacctggtggcccacaacctgctgctggcccacgccaaggtgtggcacctgtacaacaccagcttccgccccacccagggtggacaggtctctattgccctgagctctcactggattaaccccaggaggatgaccgatcacagcatcaaggaatgccagaagagcctggacttcgttctgggctggttcgccaagcccgtgtttatcgacggcgactaccccgagagcatgaagaacaacctgtctagcatcctgcccgacttcaccgagagcgaaaaaaaattcatcaagggcaccgccgatttcttcgccctgtgtttcggcccaaccctgagcttccaactgctggatccccacatgaagttcagacaactcgagagtcccaacctgcgccagctgctgagctggatcgatctggaattcaaccacccccagatattcatagtggagaacggctggtttgtaagcggcactactaagcgcgatgatgcaaagtacatgtactatctgaagaagttcatcatggaaaccctgaaggccatcaagctggatggcgtggacgtgatcggatacaccgcatggagcctgatggacggcttcgagtggcaccgcggttactcaatccgcagggggttgttctacgtcgacttcctgagtcaggacaagatgttgctgccaaagagtagcgcccttttctaccagaagttgattgagaagaacggcttcccaccactccccgagaaccagcccctggagggcacctttccctgcgatttcgcttggggcgtggtggataattatattcaggtggacaccaccctgtcacagttcactgacctgaacgtgtacctgtgggacgtgcaccattccaagcgcctgatcaaggtggacggcgtggtgaccaagaagcgcaaatcctactgcgttgactttgccgccattcagccacagatcgccctgctgcaggagatgcacgtcacccacttccgcttcagcctggactgggccctcatcctgccactgggcaaccagtcccaggtgaaccacaccattctgcagtactaccgctgtatggccagcgagctggtacgcgtgaacatcacccccgtggtggccctgtggcagcccatggcccccaaccagggcctgccacgcctgctggccaggcagggggcctgggagaacccctacaccgcactcgctttcgccgaatatgccaggctgtgcttccaggagctggggcaccacgtgaagctctggatcaccatgaacgaaccctacaccagaaacatgacctactctgccggacacaatctgctgaaggcccacgccctggcctggcacgtctacaacgagaagttccgccacgcccaaaatggaaagatctctatagccctgcaggccgattggatcgagcccgcctgccccttctcacagaaggacaaggaggtggccgagcgcgtgctggagttcgacatcggctggctggccgagcccatcttcggcagcggagactacccctgggtgatgcgcgattggcttaaccagcgcaacaactttctgctgccctacttcaccgaggacgagaagaagctgatccagggcaccttcgacttcctggccctgagccactatactaccatcctggtcgacagcgagaaggaggacccaatcaagtacaacgactacctggaggtgcaggagatgaccgacatcacctggctgaacagccctagccaggtcgccgtggtgccttggggcctgcgcaaggtgctgaactggctgaagttcaagtatggcgacctgccaatgtacatcatcagcaacggcattgatgacggcctgcacgccgaggacgatcagctgagagtgtactatatgcagaactacatcaacgaggcactgaaggcccacatcctggacggcatcaacctgtgtggctactttgcatactccttcaacgacagaaccgccccccgcttcggcctgtacaggtacgctgccgatcagttcgagcccaaggccagcatgaagcactacagaaaaatcattgatagcaacgggttcccaggccccgagaccctggagcgcttctgccccgaggagttcaccgtgtgcaccgagtgcagttttttccacacccgcaagagctga

SEQ ID NO: 20 - RNA, 2946 nt, synthetic construct
  source 1..2946: mol_type = other RNA
atgcccgctagcgccccaccgagaagaccgcggccgccaccgccatcgctgtcgctgctgctggtgctgctgggactgggcggaagaagactgcgtgcggagcctggcgacggggcccagacctgggccagattcagcagaccccccgcacccgaggccgccggcctgttccagggcaccttccccgacggatttctgtgggccgtgggaagcgctgcctaccagaccgagggcggctggcaacagcacggcaagggcgccagcatctgggacaccttcacccaccatcctctggctcctcccggagacagcagaaacgccagcctgcctctgggagcccccagccccctgcagcccgccactggagacgtggccagcgactcctacaacaacgtgttccgcgacaccgaggccctgcgcgagctgggcgtgacccactaccgctttagcatcagctgggccagagtgctgcccaacggcagcgccggcgtgcccaaccgggaaggcctgagatactatcgccgcctgctggagaggctgagagagttgggcgtgcagcccgtggtgaccctgtaccactgggacctgccccagcgcctgcaggacgcctacggcggctgggccaacagggcactcgccgaccacttccgcgactacgccgagctgtgcttccgccacttcggcgggcaggtgaagtactggatcaccatcgacaacccctacgtggtggcctggcacggctacgctacaggaaggctggcccccgggatccgcggcagccccaggctgggctacctggtggcccacaacctgctgctggcacacgccaaagtgtggcacctgtataacaccagctttcgccccacccagggtggacaggtgagcattgccctgagttctcattggatcaaccccaggcgcatgaccgatcacagcatcaaggaatgccagaagagcctggacttcgtgctgggctggttcgccaagcccgtgtttatcgacggcgactaccccgagtctatgaagaacaacctcagcagcatcctgcctgacgtcaccgagagcgagaagaagttcatcaagggcaccgccgacttcttcgccctgagcttcggccccaccctgagcttccagctgctggatccccatatgaagttcagacaactcgagagtcctaacctgcgccagctgctgagctggatcgacctggaattcaaccacccacagatcttcatcgtggagaacggctggtttgtgagcggcaccactaagcgcgacgacgcaaagtatatgtattatctgaagaaattcatcatggaaaccctgaaggccatcaagctggacggcgtggacgtgatcggatacaccgcatggagcctgatggacggcttcgagtggcaccgcggttacagcatccgccggggcctgttctacgttgacttcctgagccaggacaagatgttgctgcccaagagctccgccctgttctaccagaagttgatcgagaagaacggcttcccaccactccccgagaaccagcccctggagggcaccttcccctgcgatttcgcctggggcgtggtggacaactacatccaggtggacaccaccctgagtcagttcactgacctgaacgtgtacctttgggacgtgcaccacagcaagcgcctgataaaggtcgacggcgtggtgaccaagaagcgcaaaagctactgcgtggactttgccgccatccagccccagatcgccctgctgcaggagatgcacgtgactcacttccgcttcagcctcgactgggccctgattctgcccctgggcaaccagtcacaagtgaaccacaccattctgcagtactaccgctgtatggccagcgagctggtacgcgtgaacatcacccccgttgtggccctttggcagcccatggcccccaaccagggcctgcctcgcctgctggcccgccagggagcctgggagaatccctacaccgcactggccttcgctgaatacgcccgcctgtgcttccaggagctggggcaccacgtgaaactctggatcaccatgaacgagccctacaccagaaacatgacctacagcgccggacacaatctgctgaaggcccacgctctggcctggcacgtgtacaacgagaagtttcgccacgcccagaacggcaagatcagcatcgccctgcaggccgattggatcgagcccgcctgccccttcagccagaaggacaaggaggtggctgagcgggtgctggagttcgacatcgggtggctggctgagcctatcttcggcagcggagactacccctgggtgatgcgcgattggcttaaccagaggaacaatttcctgctgccctacttcaccgaggacgagaagaagctgatccagggcacctttgacttcctggctttgagccactataccactatcctggtggacagcgagaaggaggaccccatcaagtacaacgactacttggaggtgcaggagatgaccgacatcacctggctgaacagccctagccaggtggctgtggtgccttggggcctgcgcaaggtgctgaactggctgaagttcaagtacggcgacctgcccatgtatatcatcagcaacggcatcgacgacggcctgcacgccgaggacgaccagctgagagtgtactacatgcagaactacatcaacgaggccctcaaggcccacatcctggacggcatcaacctgtgtggctactttgcctacagcttcaacgacagaaccgccccccgcttcggcctgtacaggtacgccgccgaccagttcgaacccaaggccagcatgaagcactaccgcaaaatcatcgacagcaacggattccctggacccgagacactggagcgcttctgcccagaggagttcaccgtgtgcaccgagtgcagtttcttccacacccgcaagagctga

SEQ ID NO: 21 - RNA, 2946 nt, synthetic construct
  source 1..2946: mol_type = other RNA
atgcccgctagcgccccaccgagaagaccgcggccgccaccgccatcgctgtcgctgctgctggtgctgctgggactgggcggaagaagactgcgtgcggagcctggagatggagcccaaacatgggccagattcagcagacctcccgctcctgaagccgccggcttgtttcagggaacctttcctgacggtttcctgtgggctgtgggcagcgccgcctatcagaccgagggcggctggcaacagcacggaaaaggagccagcatctgggataccttcacccaccaccccctggccccccccggcgattcccgcaatgccagcctccctctgggagcccctagccccctgcaacctgccacaggagacgtggcctcagacagctataacaacgtgttccgcgacaccgaggcactgcgcgagctgggcgtgacccattaccgctttagcatcagctgggccagagtgctgcccaatggctctgccggcgtgcccaaccgggagggcctgaggtactaccgccgcctgctggagaggctgcgggagctgggcgtgcagcccgtggtaaccctgtaccactgggacctgccccagcgcctgcaggacgcttacggcggctgggccaaccgcgctctcgcagaccacttccgcgactacgccgagctgtgctttcgccactttggcggccaggtgaagtattggatcaccatcgataacccttacgtggtggcctggcacggatacgctacaggccgcctggcccccggcatccgcggcagccccagactgggctacctggtggcccacaacctgctgctggcccacgccaaggtgtggcacctgtacaacaccagcttccgccccacccagggtggacaggtctctattgccctgagctctcactggattaaccccaggaggatgaccgatcacagcatcaaggaatgccagaagagcctggacttcgttctgggctggttcgccaagcccgtgtttatcgacggcgactaccccgagagcatgaagaacaacctgtctagcatcctgcccgacgtcaccgagagcgaaaaaaaattcatcaagggcaccgccgatttcttcgccctgagcttcggcccaaccctgagcttccaactgctggatccccacatgaagttcagacaactcgagagtcccaacctgcgccagctgctgagctggatcgatctggaattcaaccacccccagatattcatagtggagaacggctggtttgtaagcggcactactaagcgcgatgatgcaaagtacatgtactatctgaagaagttcatcatggaaaccctgaaggccatcaagctggatggcgtggacgtgatcggatacaccgcatggagcctgatggacggcttcgagtggcaccgcggttactcaatccgcagggggttgttctacgtcgacttcctgagtcaggacaagatgttgctgccaaagagtagcgcccttttctaccagaagttgattgagaagaacggcttcccaccactccccgagaaccagcccctggagggcacctttccctgcgatttcgcttggggcgtggtggataattatattcaggtggacaccaccctgtcacagttcactgacctgaacgtgtacctgtgggacgtgcaccattccaagcgcctgatcaaggtggacggcgtggtgaccaagaagcgcaaatcctactgcgttgactttgccgccattcagccacagatcgccctgctgcaggagatgcacgtcacccacttccgcttcagcctggactgggccctcatcctgccactgggcaaccagtcccaggtgaaccacaccattctgcagtactaccgctgtatggccagcgagctggtacgcgtgaacatcacccccgtggtggccctgtggcagcccatggcccccaaccagggcctgccacgcctgctggccaggcagggggcctgggagaacccctacaccgcactcgctttcgccgaatatgccaggctgtgcttccaggagctggggcaccacgtgaagctctggatcaccatgaacgaaccctacaccagaaacatgacctactctgccggacacaatctgctgaaggcccacgccctggcctggcacgtctacaacgagaagttccgccacgcccaaaatggaaagatctctatagccctgcaggccgattggatcgagcccgcctgccccttctcacagaaggacaaggaggtggccgagcgcgtgctggagttcgacatcggctggctggccgagcccatcttcggcagcggagactacccctgggtgatgcgcgattggcttaaccagcgcaacaactttctgctgccctacttcaccgaggacgagaagaagctgatccagggcaccttcgacttcctggccctgagccactatactaccatcctggtcgacagcgagaaggaggacccaatcaagtacaacgactacctggaggtgcaggagatgaccgacatcacctggctgaacagccctagccaggtcgccgtggtgccttggggcctgcgcaaggtgctgaactggctgaagttcaagtatggcgacctgccaatgtacatcatcagcaacggcattgatgacggcctgcacgccgaggacgatcagctgagagtgtactatatgcagaactacatcaacgaggcactgaaggcccacatcctggacggcatcaacctgtgtggctactttgcatactccttcaacgacagaaccgccccccgcttcggcctgtacaggtacgctgccgatcagttcgagcccaaggccagcatgaagcactacagaaaaatcattgatagcaacgggttcccaggccccgagaccctggagcgcttctgccccgaggagttcaccgtgtgcaccgagtgcagttttttccacacccgcaagagctga

SEQ ID NO: 22 - RNA, 2946 nt, synthetic construct
  source 1..2946: mol_type = other RNA
atgcccgctagcgccccaccgagaagaccgcggccgccaccgccatcgctgtcgctgctgctggtgctgctgggactgggcggaagaagactgcgtgcggagccaggcgatggcgcccagacttgggcccgcttcagcagacctcccgcccccgaggccgccggattgttccagggaaccttccctgacggtttcctgtgggccgtgggtagcgccgcctaccagaccgagggcggctggcagcagcacggcaagggcgcaagcatctgggacacctttacccaccaccccctggccccccccggcgacagtagaaatgctagtctccccctgggcgcccccagcccccttcagcccgccaccggagacgtggcctcagacagctacaacaacgtgttcagagacaccgaagctctgagggagctcggcgtgacccactatcggtttagcattagctgggccagagtgctgcccaacggcagcgccggcgtgcccaaccgcgaaggcctcagatactatcgcagactgctggagaggctgcgggagctgggcgtgcagcccgtggtaactctgtaccactgggatctgccccagagattgcaagacgcttacggcggatgggccaaccgcgctctcgccgaccacttccgggactacgcagagctgtgcttccgccacttcggcggtcaggtgaaatattggattacaatcgacaacccctacgttgtggcctggcacgggtacgctactgggcgcctggcacccggcatccgcggcagccccagactgggctaccttgttgctcacaacctcctgctggctcatgcaaaggtgtggcacttgtacaacacaagtttccgccccacccagggtggacaggtgtcaatcgcactgtcttcacactggattaacccccggcgcatgactgaccactcaattaaggaatgccagaagagcctggacttcgttctgggctggttcgccaagcccgtgtttatcgacggggactaccccgagagcatgaagaataatctgagcagcatcttgcccgactttaccgagagcgaaaagaaattcatcaagggcaccgccgactttttcgcactgtgtttcggccccactctgagctttcaactgctcgatccccacatgaagtttagacaactggagtcccctaatctgcgccagcttctgagctggattgatctggaatttaaccatccccagatttttatagttgagaatgggtggtttgttagcggcaccactaagcgcgatgacgcaaagtacatgtattatctgaagaaatttatcatggaaactctgaaggccataaaactcgacggcgttgacgtgatcggttataccgcatggagccttatggacgggttcgagtggcaccgcgggtactccatcaggaggggcttgttctacgtcgacttcctcagtcaggacaagatgttgctgcctaagagcagcgccttgttctaccagaagttgatcgaaaagaacggctttccaccactccccgagaaccaacccctggagggcacctttccctgcgatttcgcttggggcgtggtggacaactacatccaggtggataccactctgtctcagttcactgatctcaacgtgtatctgtgggacgtccaccactccaagaggctgatcaaggtggacggcgtcgtgaccaagaagagaaagtcctactgcgtggactttgccgccattcagccccagatcgccctgctgcaggagatgcatgtcacacacttccgcttttctctggactgggccctgattctgcccctggggaaccagtcccaggtcaaccacaccattctccagtactaccgctgtatggccagtgagctggtacgcgtgaacatcacccccgtcgtggccctctggcagcccatggcccccaatcagggcctgccacgcctgctcgcccggcagggagcctgggaaaatccatacactgcactcgccttcgctgagtacgccaggctgtgcttccaggagctgggacatcacgtgaagctgtggattaccatgaacgaaccatacactagaaatatgacctactccgccggacacaatctcctgaaggcccacgcactggcttggcacgtgtacaacgagaagttcaggcacgcccagaatggaaagattagcatcgccctgcaggccgactggatcgagcccgcctgtcccttcagccagaaagacaaagaggtggctgagcgcgtgctggagtttgatattggctggcttgctgagccaatattcggcagtggagactacccctgggtgatgagagattggcttaaccagagaaacaactttctcctgccctacttcaccgaggacgaaaagaaactgatccagggtaccttcgatttccttgctctgagccactatactaccatcctggtcgacagcgagaaggaggaccccatcaaatataacgactacctggaggtgcaagagatgactgacatcacatggctgaatagccctagccaggtcgccgtggtgccttggggcctgcgcaaggtgctcaactggctgaagttcaagtatggcgacctgcccatgtacatcatcagcaacggcattgatgacggactgcacgccgaggatgatcaactcagagtatactatatgcagaactatatcaacgaggcattgaaggcccacatcctggacggcatcaacctgtgtgggtactttgcatactccttcaacgacagaaccgctccccgctttggtctgtataggtacgctgccgaccagttcgagcccaaggccagcatgaagcactaccgcaagattatcgatagcaatggcttccctggccccgagacccttgagcgcttttgccccgaggagttcaccgtgtgtaccgaatgttccttcttccacacacgcaagtcatga

SEQ ID NO: 23 - RNA, 2946 nt, synthetic construct
  source 1..2946: mol_type = other RNA
atgcccgctagcgccccaccgagaagaccgcggccgccaccgccatcgctgtcgctgctgctggtgctgctgggactgggcggaagaagactgcgtgcggagcctggcgatggcgctcagacttgggctcgcttcagcagacccccagcccccgaagcagccggattgttccagggaaccttccccgatggtttcctgtgggccgtaggtagcgccgcctaccagactgagggcggatggcagcagcacggcaagggcgcaagcatctgggacaccttcacccaccaccccctggccccccctggcgactcccgcaatgctagtctccccctgggcgcccctagcccccttcagcccgccactggcgacgtggcctcagacagctacaacaatgtgttccgggacacagaagctctgagggagcttggcgtgacccattataggtttagcatctcatgggcccgcgtgctgccaaatggcagcgccggcgtgcctaaccgcgaaggacttcgctactatcgcagactgctggagaggctgcgggaactgggggtgcaacctgtggtgacattgtaccactgggatctgcctcagcgcttgcaagacgcttacggtggatgggccaaccgcgctctggccgaccatttccgggactacgcagagctttgcttccgccacttcgggggtcaagtgaaatattggattacaatcgataacccctacgtggttgcatggcatggctacgccacagggcgccttgctcccggcatcagaggaagccccaggctgggttatcttgtggcacacaacctcctgctggcacacgcaaaagtgtggcacttgtataacacaagtttccgccccacccagggtggacaggtgtcaatagcactgtcttcacactggattaatcctcggaggatgacagatcactccatcaaggaatgccagaagagcctggacttcgtcctgggctggtttgctaagcccgtgtttatcgacggggactaccccgagagcatgaagaataatctgagcagcatattgccagattttaccgagtccgagaagaaatttatcaaagggaccgctgactttttcgctctgtgtttcggccccactctgagctttcaattgctggatccacacatgaagtttagacaactggaaagtcccaatctgcggcagttgctgagctggattgatctggaattcaaccatccccagatttttattgttgagaatgggtggtttgttagtggcactacaaagagggatgacgccaagtacatgtactatctgaagaaattcatcatggagaccctgaaggccataaagctcgacggagttgacgtgatcggttataccgcatggagcctgatggacgggttcgagtggcaccgcgggtacagcatcaggagaggcttgttctacgtcgacttcttgtcacaggacaaaatgttgttgcctaagtcaagtgccttgttttaccagaaactgattgaaaaaaacggctttcctcctttgcccgagaaccaacctctggagggaacctttccctgcgattttgcttggggcgtggtggacaactacatccaggtggacacaaccctgtctcagttcaccgatttgaatgtgtatctctgggatgtccaccactccaagcgcctgatcaaggtggatggcgtcgtgaccaagaaaagaaagagctactgcgtggactttgccgccattcagccccagattgccctgctccaggagatgcacgtcacacactttaggttctccctggactgggccctgatactgcccctgggtaaccagtcacaagtgaaccataccattttgcagtactaccgctgtatggcttcagagctggtacgcgtgaacatcacccccgtagttgccctctggcagcccatggcccccaatcagggcctgcctcgcctgctcgcccggcagggagcctgggaaaacccatacaccgcacttgccttcgctgagtacgccaggttgtgcttccaggagctgggacatcacgtgaagctttggattaccatgaacgagccatacaccaggaacatgacatactccgccggacataatctgctgaaggctcacgcactggcctggcacgtgtacaacgagaagtttcggcatgcccagaatggaaagatcagcatcgctctgcaggcagactggatcgagcctgcctgtcctttcagtcagaaagataaagaggtggccgagcgggtgctggaattcgatatcggatggctggctgaaccaatcttcggcagtggggactacccctgggtgatgagagattggctgaaccagcgcaacaattttctgctgccctactttaccgaggacgaaaagaagcttatccagggtaccttcgatttccttgccctgtcccactatactaccatacttgtcgactctgagaaagaggaccccatcaaatacaatgactacctggaggtgcaagaaatgacagacataacctggctgaatagccctagtcaggtcgctgtggtgccttggggcctccgcaaagtgttgaactggctgaagtttaagtatggcgacctgcccatgtacatcattagcaacgggattgatgacggactgcacgctgaggatgatcaactgagagtatactatatgcagaattacatcaatgaggctttgaaggcccacatcctggatggaattaacctgtgcgggtactttgcatactccttcaacgatagaaccgctccccgctttggtctgtataggtacgctgccgatcagttcgagcccaaagccagcatgaagcactaccgcaagatcatcgatagcaacggcttccctgggcccgagactctcgagaggttttgccccgaggagttcaccgtgtgtaccgaatgcagttttttccacacaaggaaatcatga

SEQ ID NO: 24 - RNA, 2946 nt, synthetic construct
  source 1..2946: mol_type = other RNA
atgcccgctagcgccccaccgagaagaccgcggccgccaccgccatcgctgtcgctgctgctggtgctgctgggactgggcggaagaagactgcgtgcggagcctggagacggcgctcagacatgggcccggttcagccggccaccagcccccgaagctgctggattgttccagggaacctttcctgacgggttcctgtgggcagtaggctctgctgcctatcagactgagggtggatggcagcagcacggtaaaggcgcaagcatttgggatacattcacccaccacccactggcacccccaggcgacagccgcaacgcttctcttccactgggagcccccagtcctcttcagcccgccacaggcgacgttgcatcagatagctataacaatgtgttccgggacaccgaagctctgagggagctcggcgtgacacactatcggttcagcatcagttgggccagggtgctgccaaacggcagtgctggtgtgcccaaccgcgaaggtctcagatactatcgccgccttctggagaggctgagagaactgggcgtgcagccagtggtgactctgtatcactgggatctgccacagagactgcaagatgcttatggtggttgggccaaccgcgccctggcagatcatttccgggactatgcagaactgtgcttccggcactttggaggacaggttaaatattggattactatcgacaacccctatgttgtggcctggcacgggtacgccactgggcgcctcgctcccggcataaggggctcccccaggctgggttaccttgtcgcccacaacctcttgctcgctcacgccaaggtctggcatctgtacaatacttctttccgccccacccagggtggtcaggtgtcaatcgcactgagcagccactggattaaccccaggcgcatgaccgatcattctattaaggagtgccagaagagccttgatttcgttctgggctggtttgctaaaccagtctttattgacggtgactaccctgagagcatgaaaaataatctgtccagcatcttgccagattttaccgagagcgaaaagaaatttatcaagggtaccgctgattttttcgctttgtgtttcggccccacattgagcttccagctgctggacccacacatgaagtttcgccagctggagtcacccaacttgcggcagctgctgtcatggatcgacctggaatttaatcacccccagatctttattgttgagaatgggtggtttgtttctggcactactaagagggatgacgcaaagtatatgtattatctgaagaagtttattatggagaccctgaaagcaatcaagctcgatggagtggatgtgatcggttataccgcttggagccttatggatggatttgagtggcacagggggtattcaataaggagaggcttgttctacgtggactttctgtcacaggataaaatgttgctgcccaaatcaagcgcccttttttaccagaaattgatagaaaagaacggcttccctcctctcccagagaaccagccactggagggaacatttccttgcgatttcgcatggggagtggtggataactacatacaggtggacaccactctgtctcagtttaccgatctcaatgtgtatctgtgggacgttcaccattccaagcgcctcattaaagtggatggcgttgtcactaagaaaagaaagagctactgtgtggactttgctgccattcagccacagatcgctctgctccaggagatgcacgtgacccacttccggttctccctggactgggccttgatactgcccttgggcaaccagagtcaggtcaatcataccatcctgcagtactatcgctgtatggcctcagagctggttcgcgtgaacataacccccgtggtggcactgtggcagcccatggcaccaaatcagggcctgcccagactgctggctagacagggcgcctgggaaaatccctacactgcactggcatttgctgagtacgccaggttgtgttttcaggagctgggacatcacgttaagctttggattaccatgaacgaaccatatactagaaacatgacctattccgccggacacaatctgctgaaagcccacgccctggcatggcatgtgtataacgagaaattcaggcacgcccagaacggaaagatcagcattgccctgcaagcagactggattgagccagcctgtcctttctcacaaaaagacaaagaggtggccgaacgggtcctggagttcgacatcggctggctcgctgaaccaatctttggcagtggcgactacccttgggttatgagggactggctcaaccagagaaacaactttcttcttccctattttacagaggatgagaagaaactgattcagggcaccttcgattttcttgctctcagccattatactactatccttgtggatagtgaaaaagaggacccaattaagtacaatgactatctcgaagtgcaagagatgaccgacatcacctggctgaatagcccatcccaggtcgcagtggtgccttggggcctgcggaaggtgctgaactggctgaagtttaagtatggcgacctgcccatgtacattattagcaacgggatagacgatggactgcacgcagaagatgatcagctgcgcgtgtattatatgcaaaattatatcaacgaagccttgaaggcccacatcctggatggaatcaacctgtgtggctattttgcatactcattcaacgaccgcaccgcaccacggtttggtctgtataggtacgctgccgaccagtttgagccaaaagccagtatgaagcactaccggaaaatcatcgattctaatggcttccctggccctgagaccctggagagattttgccccgaggaattcaccgtgtgtacagaatgttcattttttcacacccggaaaagttga

SEQ ID NO: 25 - RNA, 2946 nt, synthetic construct
  source 1..2946: mol_type = other RNA
atgcccgctagcgccccaccgagaagaccgcggccgccaccgccatcgctgtcgctgctgctggtgctgctgggactgggcggaagaagactgcgtgcggaacccggcgatggagcccaaacatgggccagattcagcagacctcccgctccagaagctgctggtctgtttcagggtacgtttcctgacggttttctctgggcagtcggctctgctgcctatcagactgagggaggttggcaacaacatggcaaaggtgctagcatatgggacactttcacgcatcacccactggccccgcctggggatagtcgcaacgcaagtctgccactgggagcaccctctcctctgcaaccggctaccggggatgtggcttccgactcttacaacaacgtgttcagggatactgaagcgcttagggaattgggcgtgacgcattaccgctttagcattagctgggccagagtcttgcctaatggatcagccggtgtgccaaatcgcgaagggctgcgatactataggcggctgttggagaggctccgggaactgggtgttcagcctgtggtgacactctatcactgggacctcccacagagacttcaagacgcgtacggaggctgggcaaatcgggccttggctgatcatttccgggactatgcagagctgtgtttccgtcactttggcggccaggtaaagtattggattaccatagataacccttatgtcgtagcttggcatggctatgcgacagggagacttgctcctgggattcgcggatctcccaggctgggatatctggtcgctcacaatctgttgctggcccatgccaaagtatggcacctgtacaacacctcattccggccgacccaaggcggccaggtgtcaattgcccttagcagccactggattaatccccgccgaatgaccgatcacagcattaaggagtgccagaaatccctggactttgttttggggtggtttgcgaaaccggtgttcatcgatggggactaccccgagtccatgaagaacaatctgagttctatcctgccagacttcacagaatccgagaagaagttcatcaaggggactgccgacttcttcgcactgtgctttggccccacactctcctttcagctgctcgatcctcacatgaaatttcgccagcttgagagcccaaatctccgtcagctgctttcatggatagacctggagttcaaccatccccagatctttatcgtcgaaaacggttggttcgtgagtggaaccacaaagagggacgatgccaaatacatgtattacctcaagaagttcattatggagactctgaaggccatcaaactcgacggagttgacgtgatcggctatactgcatggtccttgatggatggattcgaatggcatagagggtacagcatccgaagaggcctgttttacgtggactttctgagccaggacaagatgctgctccccaaaagctcagccctcttctaccagaaactgatcgagaagaacggctttccacccttgcccgagaatcagcctctggagggcacattcccctgtgactttgcctggggcgttgtggacaattacattcaggtggataccaccctgtctcagttcaccgatctgaacgtgtacctctgggatgttcaccacagtaaacgtctgatcaaggtcgatggggtggttacaaagaaacgcaagagttattgcgtcgattttgcagccatccagccgcagattgccctgctccaagagatgcacgtgacacacttcagattttccctggattgggccctgattctccctctgggaaaccagagccaggtaaaccacaccattctgcagtactaccgttgcatggcaagtgaactggtgagagtgaacattactccagtggtagctttgtggcagcctatggcccctaatcaaggactgccaagactgctcgcccgtcaaggcgcatgggaaaatccctatacggctcttgcctttgctgagtatgcaaggctgtgctttcaggaactgggacatcacgtgaagttgtggattaccatgaatgagccttatactcgaaacatgacctattcagctggccataatctcctcaaagcccatgcattggcttggcacgtctacaacgagaagtttcgccatgcccaaaatggcaagatcagcattgccctccaagcagactggatcgagccagcatgtcccttttctcagaaagacaaggaagtcgccgaacgggtgctggagtttgacatcggatggctggctgagcccatatttgggagtggcgattacccctgggtgatgagggactggttgaaccagaggaacaactttcttctcccgtatttcacagaggacgagaagaagctgatccagggtacatttgacttcctggctctgtcccattacaccaccattctggttgattctgagaaggaggatcccatcaagtacaatgactacctggaagtacaggagatgacggacattacctggctgaattccccatcacaggttgctgtggttccatggggtttgcgcaaagtgctgaactggctcaagttcaaatatggggatctcccgatgtatattatctctaatggcatagacgatgggcttcatgcagaagatgatcagctgagagtctactatatgcagaactacatcaacgaagcgcttaaagcgcacatattggacggaattaatctgtgtgggtacttcgcctatagcttcaatgatcggactgctccccggtttggcctgtatcgctatgccgcggaccagttcgagcctaaagcgagcatgaagcactacaggaaaatcatcgactcaaacggcttcccaggtcctgaaactcttgaacggttttgtcccgaggaattcaccgtctgcactgagtgtagcttcttccacacacgaaaatcctga

SEQ ID NO: 26 - RNA, 2946 nt, synthetic construct
  source 1..2946: mol_type = other RNA
atgcccgctagcgccccaccgagaagaccgcggccgccaccgccatcgctgtcgctgctgctggtgctgctgggactgggcggaagaagactgcgtgcggagcccggcgatggggcccaaacctgggctcggttcagtagaccgcctgcacctgaagctgcagggttgttccagggcacttttccggatgggtttctctgggcggtagggtccgcggcatatcagaccgagggggggtggcaacaacacgggaagggtgcgtcaatatgggacacttttactcatcacccacttgcgcctcccggagattcaaggaatgcctctctgcctctgggagcacccagtcctctccaacccgcaactggcgatgtcgcatcagacagttacaacaacgtttttagggacacagaagcgctccgagaactgggggttactcattatcggttttccatttcatgggcccgagtactcccaaatgggtccgctggagtaccgaaccgcgagggcctccgctattatagaagactcctcgagcgcctgcgcgaactcggtgttcaaccggttgtcaccctgtaccattgggatctcccgcaacgcctgcaagatgcttacgggggctgggcaaaccgcgcactggcggatcattttcgagattacgccgagctgtgcttccggcattttggtgggcaagtcaagtattggatcaccattgacaacccatatgtcgttgcatggcatggatatgcaaccgggaggcttgcaccggggattagggggagccctagacttggatacctggtcgcccataatctgttgctcgctcatgcgaaggtctggcatctgtataacactagcttccggccgacgcaagggggccaagtatccattgcactgtcttcccactggattaatcccagacgcatgaccgatcacagcataaaggagtgtcaaaagtccctggattttgtcctgggctggtttgcaaagcccgtcttcatagacggcgactaccctgagagcatgaagaataacctgtcttctattcttccggatttcacggagtcagaaaaaaagtttatcaagggcaccgccgacttcttcgcactgtgtttcggaccgacattgtcctttcagcttttggaccctcatatgaaattcaggcagctcgagtcccccaatctgcgacagctgttgtcatggattgatttggaatttaaccacccacaaatttttattgtcgaaaatggttggtttgttagtgggactaccaaacgcgacgatgcgaagtacatgtactatttgaagaagtttataatggagacccttaaagccatcaaattggatggcgtggatgtgataggttatactgcatggagcttgatggacggcttcgagtggcatcgagggtacagcataaggaggggtcttttctacgttgatttcttgtctcaggataagatgcttctgccaaaaagttcagcgcttttttatcagaaattgatagaaaagaatggttttccgccgcttccagaaaatcagcccctcgaaggtacgtttccgtgcgactttgcctggggcgtggtcgacaactacatacaggtagacactactttgtcccaattcactgatctcaatgtgtatctctgggatgttcatcacagcaagcgactgataaaggtagatggggtcgttactaaaaagaggaagtcatactgcgtcgattttgcagccatccagcctcagatagcgttgctccaggagatgcacgtgacacattttcggttttcactggactgggcccttattctgccgctcgggaaccaatctcaagttaatcatactattctgcaatattacaggtgcatggcgagcgagcttgttcgagtaaatattacgcctgtggttgcactctggcagccgatggcgcctaatcaggggcttccgagacttcttgctcgacaaggtgcttgggagaacccatatacagcattggcctttgcagaatacgcgcgcttgtgtttccaagagctgggccatcatgtgaaactttggataaccatgaatgagccttatacacggaacatgacatactcagcagggcacaacttgctgaaggctcatgctcttgcatggcatgtttataatgaaaaatttcgacacgcacaaaacgggaaaatcagcattgctctgcaggctgattggatagaacccgcatgtccattttcacaaaaagacaaggaagtagcggagcgcgtacttgagttcgacataggctggcttgccgagcccatatttggttccggtgattatccgtgggtaatgcgggattggcttaatcaacgcaacaacttcctcctgccttactttacagaggacgagaaaaaactcattcagggcacctttgatttcctcgctcttagccattatacaactatactcgttgacagtgaaaaggaagaccctatcaagtacaacgattatcttgaagtccaggaaatgacagatataacctggcttaacagcccgtcccaggtagctgttgttccttgggggttgcggaaagttttgaattggctgaaattcaagtatggggatcttcccatgtatattatttcaaacggcatcgatgatggtttgcatgccgaagatgaccaacttagggtatattacatgcaaaactacatcaacgaggcgctcaaggcccatatccttgacggtatcaacttgtgcggttattttgcctattcctttaatgatagaacagcccctaggttcggtttgtaccgctacgcagcggaccaatttgagccgaaagcgtcaatgaaacactataggaagataatagatagcaatggatttcctgggcccgagactctcgagaggttctgtccagaggaattcacagtctgcacagaatgtagcttttttcatacgagaaagtcctga

SEQ ID NO: 27 - RNA, 2946 nt, synthetic construct
  source 1..2946: mol_type = other RNA
atgcccgctagcgccccaccgagaagaccgcggccgccaccgccatcgctgtcgctgctgctggtgctgctgggactgggcggaagaagactgcgtgcggaaccgggggatggagctcagacttgggctaggttctctagacctccagctcccgaagctgcaggactgtttcagggaactttccccgatgggtttctgtgggccgtgggatctgctgcctaccaaaccgagggcggatggcaacagcatggaaaaggtgcatccatttgggataccttcacccaccatcctctggcaccccccggagattcaagaaatgcttctctccctctcggtgctccatcaccactgcagcctgctacaggagatgttgccagtgattcatacaacaatgtgtttagggacaccgaagctttgcgagagctcggggtcactcattaccgcttttctatttcatgggcccgcgtacttccaaatggatctgcgggagtcccaaatagagagggcttgagatattaccgaaggttgctggaacgcctgagggaacttggagtgcaacccgtagtgacattgtaccactgggatctcccccagaggcttcaggatgcttacggtggttgggctaacagagctctcgcagaccacttcagagattatgcagaactgtgctttcgacatttcggcggccaggtaaaatactggatcaccatagacaatccctatgtggttgcgtggcatggttatgccacaggaagactggctcccggtatccgggggagtcctagacttggctacctcgtggcccacaatctgctgttggcgcacgctaaggtgtggcatctgtataatactagctttagaccgacccagggaggtcaagtgagcatcgccctgtcctctcactggataaatccccgcagaatgaccgaccactccattaaggagtgtcaaaagtctctcgacttcgtgctcggatggtttgctaagccggttttcattgatggagactaccccgagagcatgaaaaacaacttgagctccattctgcctgactttacagaaagcgaaaaaaaatttatcaagggtactgccgactttttcgcactctgctttggccccactcttagctttcagttgctcgatccacacatgaagttccgccaactggagagtcctaatctgcgccaactcctttcttggattgacttggagttcaatcacccgcagatcttcatcgtggaaaacggctggttcgtgtcaggaaccacgaagcgcgacgatgccaagtacatgtactacctcaaaaagttcatcatggaaactctcaaagcaattaaactggacggcgtcgacgtgatcggctataccgcgtggtctctgatggacggtttcgagtggcataggggctattccataaggcgagggttgttttacgttgattttctcagccaagataaaatgctgctgcccaagtcttcagccttgttttatcagaaattgattgagaagaatggcttcccgccactccccgagaatcaacccctcgaggggacatttccatgtgacttcgcctggggggtagtcgataattacatccaagtggatacaaccctcagccagtttaccgacctgaacgtttacttgtgggacgtgcaccacagtaagagactgattaaagtggatggagtggttactaaaaagcggaagagttattgtgtagattttgccgcaatccagccacaaatcgccctgctgcaggagatgcacgtgacccatttcagatttagtctcgactgggctctgattttgcccttgggcaatcagagccaggtgaatcatacaatcctccagtactatcggtgtatggccagtgaattggtccgagtcaacatcaccccagtggtggcactctggcagccaatggctcctaaccaagggctgccaagactgctggcaaggcagggtgcctgggagaatccttacactgctctggcctttgccgagtacgctcgcctttgttttcaggagctcgggcatcatgtgaaactgtggattacaatgaatgaaccatatactcgcaacatgacctattccgcaggtcacaatctcctcaaggctcatgcactcgcatggcacgtctacaatgaaaaattccgacacgcccagaatgggaagattagtatcgccctgcaggctgattggatcgagcccgcatgtccattttcacaaaaggacaaagaggtagccgagagagtgctggagttcgatatcggctggcttgccgaacctattttcggctctggcgattacccctgggtgatgagggattggttgaaccagaggaacaatttcctcctgccgtattttaccgaggacgaaaagaagttgatccaaggcacattcgatttcctcgccctttctcactacacaaccatacttgtggatagcgagaaggaggacccaattaaatataatgactatctggaagttcaggagatgactgatatcacatggctgaattcccccagccaagtagcagtcgtgccctggggtctgagaaaggtgcttaattggttgaagtttaagtacggtgatctgcctatgtatataatttctaacggcatagatgatgggctgcacgctgaggacgatcaactgcgagtgtactacatgcagaattatatcaacgaagccttgaaagcccacattctggacggcatcaatctttgtggctacttcgcttattcattcaatgatagaacagccccccgctttggattgtatcggtatgccgccgaccaattcgagccaaaggcttctatgaagcactaccggaagattatcgactccaacgggtttccagggccagagacactggaaaggttttgcccagaggagttcaccgtgtgtacagagtgcagctttttccacacccggaaatcatga

SEQ ID NO: 28 - RNA, 2946 nt, synthetic construct
  source 1..2946: mol_type = other RNA
atgcccgctagcgccccaccgagaagaccgcggccgccaccgccatcgctgtcgctgctgctggtgctgctgggactgggcggaagaagactgcgtgcggaaccaggagatggtgcccaaacttgggctaggttctctcgtccacccgcacctgaagctgctgggctgtttcaaggtacttttcctgatggatttctttgggctgtcgggtccgctgcttatcaaactgaaggtggatggcaacaacatgggaaaggcgcttcaatttgggacacctttacacatcatcctctcgccccacctggtgatagtcgcaatgcgagcttacctctcggagcaccatctcccttgcaaccagcaacaggcgatgtggcttcagattcctataataatgtgtttagagatactgaagctctcagagaattgggagtgacccattatagattttctatttcttgggcccgggtcctgcctaacgggtccgccggggttcctaatcgagaaggtttgcggtattatagaaggcttctcgaaaggttgcgagaacttggagtacaacctgtcgtgactttgtatcattgggatcttccgcaaagacttcaagatgcatatggtggatgggcaaatcgtgcactcgctgatcattttcgggactatgccgaactttgttttaggcattttggcggccaagttaaatattggattacaatagataatccttatgtagttgcatggcatggttatgcaacaggccggttggcaccagggattcgaggttcaccacgacttggatatttagtcgcccataatcttcttttggcccacgcgaaggtatggcacttatataacacctcttttaggccgacgcaaggtggacaagtctctatcgcattgtcctcacattggattaaccccaggcgtatgacagatcattctattaaggaatgccagaagagtctcgatttcgtgttaggctggttcgcaaagccagtcttcatcgacggagattacccggaatcaatgaagaacaatctgagcagtatccttcccgacttcaccgagagtgaaaagaaatttattaagggcaccgcagatttcttcgccctgtgtttcggcccgactctctccttccagctgctcgatccacatatgaaatttcggcagctcgagtcacctaatttaagacagctcctgagttggatcgatctggagttcaatcacccacagatcttcatcgttgagaacgggtggttcgtgtctggcacgactaaacgcgacgacgctaagtacatgtactatctgaagaaatttataatggagacacttaaggctataaaattggacggcgtagacgtgattggttacactgcttggagcctgatggacggctttgaatggcatcgtgggtattcaatacggcggggcttattttacgtggatttcttgtctcaagataaaatgctgctgcccaaaagcagtgcacttttctatcagaaactcatcgaaaagaacggatttccacccttgccagagaaccaacctctggaaggaaccttcccatgcgatttcgcgtggggtgtggtggataattatatccaggtggacactaccttaagtcaattcacagatctcaacgtgtatttatgggacgtgcatcatagcaagagactgatcaaggtcgacggtgtggttactaagaagcgcaagagctattgcgtcgatttcgcagcaattcaaccacaaattgccctgctgcaagagatgcatgtgacccacttcagatttagtctcgattgggcattgatcctgcccctcggaaatcaatcacaagtaaatcatactatactccaatattacaggtgtatggcttccgaactggttcgagtaaatattacacctgtcgttgctttgtggcaaccgatggcacctaatcaggggcttccaaggctgctcgcaagacaaggagcgtgggaaaatccatatacagcgttagctttcgctgaatacgctaggctctgtttccaggaattgggtcaccatgtgaaattgtggatcactatgaacgaaccttacactcggaacatgacctattctgcaggacataatctcctcaaagctcacgcattagcctggcacgtttataacgagaaattccgacacgcccaaaacggtaagatttctattgcgcttcaagccgactggattgagcccgcttgtccctttagccagaaagataaggaagtagcagaacgagtactggagttcgatataggatggctcgcggaaccgatatttggatccggcgactacccgtgggtcatgcgagattggctcaatcagcgcaataacttcctgctcccatactttacagaggacgagaagaaactcattcaaggcacgttcgatttccttgccctgtcccactacacgacgattctcgtggattccgagaaagaggaccctatcaagtataacgactatttggaagtccaggagatgactgatataacttggctgaattcaccttcccaagtcgccgttgtcccgtggggtctgagaaaggtacttaattggttgaaatttaaatatggcgatcttcctatgtatatcattagcaacgggattgacgatggcttgcacgcagaagatgatcaattgcgtgtctactacatgcaaaactatatcaatgaggccctgaaggctcatatcctcgacggcattaacttgtgtgggtatttcgcatactcattcaatgatagaaccgcacctcgcttcgggctttaccgctacgccgctgaccaattcgaacctaaagcctcaatgaagcactatagaaagatcatcgattccaacgggtttcccgggcctgagacacttgagaggttctgccccgaggagtttacggtctgcacagaatgtagcttcttccatacacggaaatcctga

SEQ ID NO: 29 - RNA, 3249 nt, synthetic construct
  source 1..3249: mol_type = other RNA
gggagacataaaccctggcgcgctcgcggcccggcactcttctggtccccacagactcagagagaacccaccatgcccgctagcgccccaccgagaagaccgcggccgccaccgccatcgctgtcgctgctgctggtgctgctgggactgggcggaagaagactgcgtgcggagcctggcgacggggcccagacctgggccagattcagcagaccccccgcacccgaggccgccggcctgttccagggcaccttccccgacggatttctgtgggccgtgggaagcgctgcctaccagaccgagggcggctggcaacagcacggcaagggcgccagcatctgggacaccttcacccaccatcctctggctcctcccggagacagcagaaacgccagcctgcctctgggagcccccagccccctgcagcccgccactggagacgtggccagcgactcctacaacaacgtgttccgcgacaccgaggccctgcgcgagctgggcgtgacccactaccgctttagcatcagctgggccagagtgctgcccaacggcagcgccggcgtgcccaaccgggaaggcctgagatactatcgccgcctgctggagaggctgagagagttgggcgtgcagcccgtggtgaccctgtaccactgggacctgccccagcgcctgcaggacgcctacggcggctgggccaacagggcactcgccgaccacttccgcgactacgccgagctgtgcttccgccacttcggcgggcaggtgaagtactggatcaccatcgacaacccctacgtggtggcctggcacggctacgctacaggaaggctggcccccgggatccgcggcagccccaggctgggctacctggtggcccacaacctgctgctggcacacgccaaagtgtggcacctgtataacaccagctttcgccccacccagggtggacaggtgagcattgccctgagttctcattggatcaaccccaggcgcatgaccgatcacagcatcaaggaatgccagaagagcctggacttcgtgctgggctggttcgccaagcccgtgtttatcgacggcgactaccccgagtctatgaagaacaacctcagcagcatcctgcctgacttcaccgagagcgagaagaagttcatcaagggcaccgccgacttcttcgccctgtgcttcggccccaccctgagcttccagctgctggatccccatatgaagttcagacaactcgagagtcctaacctgcgccagctgctgagctggatcgacctggaattcaaccacccacagatcttcatcgtggagaacggctggtttgtgagcggcaccactaagcgcgacgacgcaaagtatatgtattatctgaagaaattcatcatggaaaccctgaaggccatcaagctggacggcgtggacgtgatcggatacaccgcatggagcctgatggacggcttcgagtggcaccgcggttacagcatccgccggggcctgttctacgttgacttcctgagccaggacaagatgttgctgcccaagagctccgccctgttctaccagaagttgatcgagaagaacggcttcccaccactccccgagaaccagcccctggagggcaccttcccctgcgatttcgcctggggcgtggtggacaactacatccaggtggacaccaccctgagtcagttcactgacctgaacgtgtacctttgggacgtgcaccacagcaagcgcctgataaaggtcgacggcgtggtgaccaagaagcgcaaaagctactgcgtggactttgccgccatccagccccagatcgccctgctgcaggagatgcacgtgactcacttccgcttcagcctcgactgggccctgattctgcccctgggcaaccagtcacaagtgaaccacaccattctgcagtactaccgctgtatggccagcgagctggtacgcgtgaacatcacccccgttgtggccctttggcagcccatggcccccaaccagggcctgcctcgcctgctggcccgccagggagcctgggagaatccctacaccgcactggccttcgctgaatacgcccgcctgtgcttccaggagctggggcaccacgtgaaactctggatcaccatgaacgagccctacaccagaaacatgacctacagcgccggacacaatctgctgaaggcccacgctctggcctggcacgtgtacaacgagaagtttcgccacgcccagaacggcaagatcagcatcgccctgcaggccgattggatcgagcccgcctgccccttcagccagaaggacaaggaggtggctgagcgggtgctggagttcgacatcgggtggctggctgagcctatcttcggcagcggagactacccctgggtgatgcgcgattggcttaaccagaggaacaatttcctgctgccctacttcaccgaggacgagaagaagctgatccagggcacctttgacttcctggctttgagccactataccactatcctggtggacagcgagaaggaggaccccatcaagtacaacgactacttggaggtgcaggagatgaccgacatcacctggctgaacagccctagccaggtggctgtggtgccttggggcctgcgcaaggtgctgaactggctgaagttcaagtacggcgacctgcccatgtatatcatcagcaacggcatcgacgacggcctgcacgccgaggacgaccagctgagagtgtactacatgcagaactacatcaacgaggccctcaaggcccacatcctggacggcatcaacctgtgtggctactttgcctacagcttcaacgacagaaccgccccccgcttcggcctgtacaggtacgccgccgaccagttcgaacccaaggccagcatgaagcactaccgcaaaatcatcgacagcaacggattccctggacccgagacactggagcgcttctgcccagaggagttcaccgtgtgcaccgagtgcagtttcttccacacccgcaagagctgagctggagcctcggtggccatgcttcttgccccttgggcctccccccagcccctcctccccttcctgcacccgtacccccgtggtctttgaataaagtctgagtgggcggcaaaaaaaaaaaaaaaaaaaaaaaaaaaaaaaaaaaaaaaaaaaaaaaaaaaaaaaaaaaaaaaaaaaaaaaaaaaaaaaaaaaaaaaaaaaaaaaaaaaaaaaaaaaaaaaaaaaaaaaaa

SEQ ID NO: 30 - RNA, 3249 nt, synthetic construct
  source 1..3249: mol_type = other RNA
gggagacataaaccctggcgcgctcgcggcccggcactcttctggtccccacagactcagagagaacccaccatgcccgctagcgccccaccgagaagaccgcggccgccaccgccatcgctgtcgctgctgctggtgctgctgggactgggcggaagaagactgcgtgcggagcctggagatggagcccaaacatgggccagattcagcagacctcccgctcctgaagccgccggcttgtttcagggaacctttcctgacggtttcctgtgggctgtgggcagcgccgcctatcagaccgagggcggctggcaacagcacggaaaaggagccagcatctgggataccttcacccaccaccccctggccccccccggcgattcccgcaatgccagcctccctctgggagcccctagccccctgcaacctgccacaggagacgtggcctcagacagctataacaacgtgttccgcgacaccgaggcactgcgcgagctgggcgtgacccattaccgctttagcatcagctgggccagagtgctgcccaatggctctgccggcgtgcccaaccgggagggcctgaggtactaccgccgcctgctggagaggctgcgggagctgggcgtgcagcccgtggtaaccctgtaccactgggacctgccccagcgcctgcaggacgcttacggcggctgggccaaccgcgctctcgcagaccacttccgcgactacgccgagctgtgctttcgccactttggcggccaggtgaagtattggatcaccatcgataacccttacgtggtggcctggcacggatacgctacaggccgcctggcccccggcatccgcggcagccccagactgggctacctggtggcccacaacctgctgctggcccacgccaaggtgtggcacctgtacaacaccagcttccgccccacccagggtggacaggtctctattgccctgagctctcactggattaaccccaggaggatgaccgatcacagcatcaaggaatgccagaagagcctggacttcgttctgggctggttcgccaagcccgtgtttatcgacggcgactaccccgagagcatgaagaacaacctgtctagcatcctgcccgacttcaccgagagcgaaaaaaaattcatcaagggcaccgccgatttcttcgccctgtgtttcggcccaaccctgagcttccaactgctggatccccacatgaagttcagacaactcgagagtcccaacctgcgccagctgctgagctggatcgatctggaattcaaccacccccagatattcatagtggagaacggctggtttgtaagcggcactactaagcgcgatgatgcaaagtacatgtactatctgaagaagttcatcatggaaaccctgaaggccatcaagctggatggcgtggacgtgatcggatacaccgcatggagcctgatggacggcttcgagtggcaccgcggttactcaatccgcagggggttgttctacgtcgacttcctgagtcaggacaagatgttgctgccaaagagtagcgcccttttctaccagaagttgattgagaagaacggcttcccaccactccccgagaaccagcccctggagggcacctttccctgcgatttcgcttggggcgtggtggataattatattcaggtggacaccaccctgtcacagttcactgacctgaacgtgtacctgtgggacgtgcaccattccaagcgcctgatcaaggtggacggcgtggtgaccaagaagcgcaaatcctactgcgttgactttgccgccattcagccacagatcgccctgctgcaggagatgcacgtcacccacttccgcttcagcctggactgggccctcatcctgccactgggcaaccagtcccaggtgaaccacaccattctgcagtactaccgctgtatggccagcgagctggtacgcgtgaacatcacccccgtggtggccctgtggcagcccatggcccccaaccagggcctgccacgcctgctggccaggcagggggcctgggagaacccctacaccgcactcgctttcgccgaatatgccaggctgtgcttccaggagctggggcaccacgtgaagctctggatcaccatgaacgaaccctacaccagaaacatgacctactctgccggacacaatctgctgaaggcccacgccctggcctggcacgtctacaacgagaagttccgccacgcccaaaatggaaagatctctatagccctgcaggccgattggatcgagcccgcctgccccttctcacagaaggacaaggaggtggccgagcgcgtgctggagttcgacatcggctggctggccgagcccatcttcggcagcggagactacccctgggtgatgcgcgattggcttaaccagcgcaacaactttctgctgccctacttcaccgaggacgagaagaagctgatccagggcaccttcgacttcctggccctgagccactatactaccatcctggtcgacagcgagaaggaggacccaatcaagtacaacgactacctggaggtgcaggagatgaccgacatcacctggctgaacagccctagccaggtcgccgtggtgccttggggcctgcgcaaggtgctgaactggctgaagttcaagtatggcgacctgccaatgtacatcatcagcaacggcattgatgacggcctgcacgccgaggacgatcagctgagagtgtactatatgcagaactacatcaacgaggcactgaaggcccacatcctggacggcatcaacctgtgtggctactttgcatactccttcaacgacagaaccgccccccgcttcggcctgtacaggtacgctgccgatcagttcgagcccaaggccagcatgaagcactacagaaaaatcattgatagcaacgggttcccaggccccgagaccctggagcgcttctgccccgaggagttcaccgtgtgcaccgagtgcagttttttccacacccgcaagagctgagctggagcctcggtggccatgcttcttgccccttgggcctccccccagcccctcctccccttcctgcacccgtacccccgtggtctttgaataaagtctgagtgggcggcaaaaaaaaaaaaaaaaaaaaaaaaaaaaaaaaaaaaaaaaaaaaaaaaaaaaaaaaaaaaaaaaaaaaaaaaaaaaaaaaaaaaaaaaaaaaaaaaaaaaaaaaaaaaaaaaaaaaaaaaa

SEQ ID NO: 31 - RNA, 3249 nt, synthetic construct
  source 1..3249: mol_type = other RNA
gggagacataaaccctggcgcgctcgcggcccggcactcttctggtccccacagactcagagagaacccaccatgcccgctagcgccccaccgagaagaccgcggccgccaccgccatcgctgtcgctgctgctggtgctgctgggactgggcggaagaagactgcgtgcggagcctggcgacggggcccagacctgggccagattcagcagaccccccgcacccgaggccgccggcctgttccagggcaccttccccgacggatttctgtgggccgtgggaagcgctgcctaccagaccgagggcggctggcaacagcacggcaagggcgccagcatctgggacaccttcacccaccatcctctggctcctcccggagacagcagaaacgccagcctgcctctgggagcccccagccccctgcagcccgccactggagacgtggccagcgactcctacaacaacgtgttccgcgacaccgaggccctgcgcgagctgggcgtgacccactaccgctttagcatcagctgggccagagtgctgcccaacggcagcgccggcgtgcccaaccgggaaggcctgagatactatcgccgcctgctggagaggctgagagagttgggcgtgcagcccgtggtgaccctgtaccactgggacctgccccagcgcctgcaggacgcctacggcggctgggccaacagggcactcgccgaccacttccgcgactacgccgagctgtgcttccgccacttcggcgggcaggtgaagtactggatcaccatcgacaacccctacgtggtggcctggcacggctacgctacaggaaggctggcccccgggatccgcggcagccccaggctgggctacctggtggcccacaacctgctgctggcacacgccaaagtgtggcacctgtataacaccagctttcgccccacccagggtggacaggtgagcattgccctgagttctcattggatcaaccccaggcgcatgaccgatcacagcatcaaggaatgccagaagagcctggacttcgtgctgggctggttcgccaagcccgtgtttatcgacggcgactaccccgagtctatgaagaacaacctcagcagcatcctgcctgacgtcaccgagagcgagaagaagttcatcaagggcaccgccgacttcttcgccctgagcttcggccccaccctgagcttccagctgctggatccccatatgaagttcagacaactcgagagtcctaacctgcgccagctgctgagctggatcgacctggaattcaaccacccacagatcttcatcgtggagaacggctggtttgtgagcggcaccactaagcgcgacgacgcaaagtatatgtattatctgaagaaattcatcatggaaaccctgaaggccatcaagctggacggcgtggacgtgatcggatacaccgcatggagcctgatggacggcttcgagtggcaccgcggttacagcatccgccggggcctgttctacgttgacttcctgagccaggacaagatgttgctgcccaagagctccgccctgttctaccagaagttgatcgagaagaacggcttcccaccactccccgagaaccagcccctggagggcaccttcccctgcgatttcgcctggggcgtggtggacaactacatccaggtggacaccaccctgagtcagttcactgacctgaacgtgtacctttgggacgtgcaccacagcaagcgcctgataaaggtcgacggcgtggtgaccaagaagcgcaaaagctactgcgtggactttgccgccatccagccccagatcgccctgctgcaggagatgcacgtgactcacttccgcttcagcctcgactgggccctgattctgcccctgggcaaccagtcacaagtgaaccacaccattctgcagtactaccgctgtatggccagcgagctggtacgcgtgaacatcacccccgttgtggccctttggcagcccatggcccccaaccagggcctgcctcgcctgctggcccgccagggagcctgggagaatccctacaccgcactggccttcgctgaatacgcccgcctgtgcttccaggagctggggcaccacgtgaaactctggatcaccatgaacgagccctacaccagaaacatgacctacagcgccggacacaatctgctgaaggcccacgctctggcctggcacgtgtacaacgagaagtttcgccacgcccagaacggcaagatcagcatcgccctgcaggccgattggatcgagcccgcctgccccttcagccagaaggacaaggaggtggctgagcgggtgctggagttcgacatcgggtggctggctgagcctatcttcggcagcggagactacccctgggtgatgcgcgattggcttaaccagaggaacaatttcctgctgccctacttcaccgaggacgagaagaagctgatccagggcacctttgacttcctggctttgagccactataccactatcctggtggacagcgagaaggaggaccccatcaagtacaacgactacttggaggtgcaggagatgaccgacatcacctggctgaacagccctagccaggtggctgtggtgccttggggcctgcgcaaggtgctgaactggctgaagttcaagtacggcgacctgcccatgtatatcatcagcaacggcatcgacgacggcctgcacgccgaggacgaccagctgagagtgtactacatgcagaactacatcaacgaggccctcaaggcccacatcctggacggcatcaacctgtgtggctactttgcctacagcttcaacgacagaaccgccccccgcttcggcctgtacaggtacgccgccgaccagttcgaacccaaggccagcatgaagcactaccgcaaaatcatcgacagcaacggattccctggacccgagacactggagcgcttctgcccagaggagttcaccgtgtgcaccgagtgcagtttcttccacacccgcaagagctgagctggagcctcggtggccatgcttcttgccccttgggcctccccccagcccctcctccccttcctgcacccgtacccccgtggtctttgaataaagtctgagtgggcggcaaaaaaaaaaaaaaaaaaaaaaaaaaaaaaaaaaaaaaaaaaaaaaaaaaaaaaaaaaaaaaaaaaaaaaaaaaaaaaaaaaaaaaaaaaaaaaaaaaaaaaaaaaaaaaaaaaaaaaaaa

SEQ ID NO: 32 - RNA, 3249 nt, synthetic construct
  source 1..3249: mol_type = other RNA
gggagacataaaccctggcgcgctcgcggcccggcactcttctggtccccacagactcagagagaacccaccatgcccgctagcgccccaccgagaagaccgcggccgccaccgccatcgctgtcgctgctgctggtgctgctgggactgggcggaagaagactgcgtgcggagcctggagatggagcccaaacatgggccagattcagcagacctcccgctcctgaagccgccggcttgtttcagggaacctttcctgacggtttcctgtgggctgtgggcagcgccgcctatcagaccgagggcggctggcaacagcacggaaaaggagccagcatctgggataccttcacccaccaccccctggccccccccggcgattcccgcaatgccagcctccctctgggagcccctagccccctgcaacctgccacaggagacgtggcctcagacagctataacaacgtgttccgcgacaccgaggcactgcgcgagctgggcgtgacccattaccgctttagcatcagctgggccagagtgctgcccaatggctctgccggcgtgcccaaccgggagggcctgaggtactaccgccgcctgctggagaggctgcgggagctgggcgtgcagcccgtggtaaccctgtaccactgggacctgccccagcgcctgcaggacgcttacggcggctgggccaaccgcgctctcgcagaccacttccgcgactacgccgagctgtgctttcgccactttggcggccaggtgaagtattggatcaccatcgataacccttacgtggtggcctggcacggatacgctacaggccgcctggcccccggcatccgcggcagccccagactgggctacctggtggcccacaacctgctgctggcccacgccaaggtgtggcacctgtacaacaccagcttccgccccacccagggtggacaggtctctattgccctgagctctcactggattaaccccaggaggatgaccgatcacagcatcaaggaatgccagaagagcctggacttcgttctgggctggttcgccaagcccgtgtttatcgacggcgactaccccgagagcatgaagaacaacctgtctagcatcctgcccgacgtcaccgagagcgaaaaaaaattcatcaagggcaccgccgatttcttcgccctgagcttcggcccaaccctgagcttccaactgctggatccccacatgaagttcagacaactcgagagtcccaacctgcgccagctgctgagctggatcgatctggaattcaaccacccccagatattcatagtggagaacggctggtttgtaagcggcactactaagcgcgatgatgcaaagtacatgtactatctgaagaagttcatcatggaaaccctgaaggccatcaagctggatggcgtggacgtgatcggatacaccgcatggagcctgatggacggcttcgagtggcaccgcggttactcaatccgcagggggttgttctacgtcgacttcctgagtcaggacaagatgttgctgccaaagagtagcgcccttttctaccagaagttgattgagaagaacggcttcccaccactccccgagaaccagcccctggagggcacctttccctgcgatttcgcttggggcgtggtggataattatattcaggtggacaccaccctgtcacagttcactgacctgaacgtgtacctgtgggacgtgcaccattccaagcgcctgatcaaggtggacggcgtggtgaccaagaagcgcaaatcctactgcgttgactttgccgccattcagccacagatcgccctgctgcaggagatgcacgtcacccacttccgcttcagcctggactgggccctcatcctgccactgggcaaccagtcccaggtgaaccacaccattctgcagtactaccgctgtatggccagcgagctggtacgcgtgaacatcacccccgtggtggccctgtggcagcccatggcccccaaccagggcctgccacgcctgctggccaggcagggggcctgggagaacccctacaccgcactcgctttcgccgaatatgccaggctgtgcttccaggagctggggcaccacgtgaagctctggatcaccatgaacgaaccctacaccagaaacatgacctactctgccggacacaatctgctgaaggcccacgccctggcctggcacgtctacaacgagaagttccgccacgcccaaaatggaaagatctctatagccctgcaggccgattggatcgagcccgcctgccccttctcacagaaggacaaggaggtggccgagcgcgtgctggagttcgacatcggctggctggccgagcccatcttcggcagcggagactacccctgggtgatgcgcgattggcttaaccagcgcaacaactttctgctgccctacttcaccgaggacgagaagaagctgatccagggcaccttcgacttcctggccctgagccactatactaccatcctggtcgacagcgagaaggaggacccaatcaagtacaacgactacctggaggtgcaggagatgaccgacatcacctggctgaacagccctagccaggtcgccgtggtgccttggggcctgcgcaaggtgctgaactggctgaagttcaagtatggcgacctgccaatgtacatcatcagcaacggcattgatgacggcctgcacgccgaggacgatcagctgagagtgtactatatgcagaactacatcaacgaggcactgaaggcccacatcctggacggcatcaacctgtgtggctactttgcatactccttcaacgacagaaccgccccccgcttcggcctgtacaggtacgctgccgatcagttcgagcccaaggccagcatgaagcactacagaaaaatcattgatagcaacgggttcccaggccccgagaccctggagcgcttctgccccgaggagttcaccgtgtgcaccgagtgcagttttttccacacccgcaagagctgagctggagcctcggtggccatgcttcttgccccttgggcctccccccagcccctcctccccttcctgcacccgtacccccgtggtctttgaataaagtctgagtgggcggcaaaaaaaaaaaaaaaaaaaaaaaaaaaaaaaaaaaaaaaaaaaaaaaaaaaaaaaaaaaaaaaaaaaaaaaaaaaaaaaaaaaaaaaaaaaaaaaaaaaaaaaaaaaaaaaaaaaaaaaaa

SEQ ID NO: 33 - RNA, 1482 nt, synthetic construct
  source 1..1482: mol_type = other RNA
ctgttccagggcaccttccccgacggatttctgtgggccgtgggaagcgctgcctaccagaccgagggcggctggcaacagcacggcaagggcgccagcatctgggacaccttcacccaccatcctctggctcctcccggagacagcagaaacgccagcctgcctctgggagcccccagccccctgcagcccgccactggagacgtggccagcgactcctacaacaacgtgttccgcgacaccgaggccctgcgcgagctgggcgtgacccactaccgctttagcatcagctgggccagagtgctgcccaacggcagcgccggcgtgcccaaccgggaaggcctgagatactatcgccgcctgctggagaggctgagagagttgggcgtgcagcccgtggtgaccctgtaccactgggacctgccccagcgcctgcaggacgcctacggcggctgggccaacagggcactcgccgaccacttccgcgactacgccgagctgtgcttccgccacttcggcgggcaggtgaagtactggatcaccatcgacaacccctacgtggtggcctggcacggctacgctacaggaaggctggcccccgggatccgcggcagccccaggctgggctacctggtggcccacaacctgctgctggcacacgccaaagtgtggcacctgtataacaccagctttcgccccacccagggtggacaggtgagcattgccctgagttctcattggatcaaccccaggcgcatgaccgatcacagcatcaaggaatgccagaagagcctggacttcgtgctgggctggttcgccaagcccgtgtttatcgacggcgactaccccgagtctatgaagaacaacctcagcagcatcctgcctgacttcaccgagagcgagaagaagttcatcaagggcaccgccgacttcttcgccctgtgcttcggccccaccctgagcttccagctgctggatccccatatgaagttcagacaactcgagagtcctaacctgcgccagctgctgagctggatcgacctggaattcaaccacccacagatcttcatcgtggagaacggctggtttgtgagcggcaccactaagcgcgacgacgcaaagtatatgtattatctgaagaaattcatcatggaaaccctgaaggccatcaagctggacggcgtggacgtgatcggatacaccgcatggagcctgatggacggcttcgagtggcaccgcggttacagcatccgccggggcctgttctacgttgacttcctgagccaggacaagatgttgctgcccaagagctccgccctgttctaccagaagttgatcgagaagaacggcttcccaccactccccgagaaccagcccctggagggcaccttcccctgcgatttcgcctggggcgtggtggacaactacatccaggtgagccagctgacaaaacctatcagcagcctgacaaagccttaccat

SEQ ID NO: 34 - RNA, 1482 nt, synthetic construct
  source 1..1482: mol_type = other RNA
ttgtttcagggaacctttcctgacggtttcctgtgggctgtgggcagcgccgcctatcagaccgagggcggctggcaacagcacggaaaaggagccagcatctgggataccttcacccaccaccccctggccccccccggcgattcccgcaatgccagcctccctctgggagcccctagccccctgcaacctgccacaggagacgtggcctcagacagctataacaacgtgttccgcgacaccgaggcactgcgcgagctgggcgtgacccattaccgctttagcatcagctgggccagagtgctgcccaatggctctgccggcgtgcccaaccgggagggcctgaggtactaccgccgcctgctggagaggctgcgggagctgggcgtgcagcccgtggtaaccctgtaccactgggacctgccccagcgcctgcaggacgcttacggcggctgggccaaccgcgctctcgcagaccacttccgcgactacgccgagctgtgctttcgccactttggcggccaggtgaagtattggatcaccatcgataacccttacgtggtggcctggcacggatacgctacaggccgcctggcccccggcatccgcggcagccccagactgggctacctggtggcccacaacctgctgctggcccacgccaaggtgtggcacctgtacaacaccagcttccgccccacccagggtggacaggtctctattgccctgagctctcactggattaaccccaggaggatgaccgatcacagcatcaaggaatgccagaagagcctggacttcgttctgggctggttcgccaagcccgtgtttatcgacggcgactaccccgagagcatgaagaacaacctgtctagcatcctgcccgacttcaccgagagcgaaaaaaaattcatcaagggcaccgccgatttcttcgccctgtgtttcggcccaaccctgagcttccaactgctggatccccacatgaagttcagacaactcgagagtcccaacctgcgccagctgctgagctggatcgatctggaattcaaccacccccagatattcatagtggagaacggctggtttgtaagcggcactactaagcgcgatgatgcaaagtacatgtactatctgaagaagttcatcatggaaaccctgaaggccatcaagctggatggcgtggacgtgatcggatacaccgcatggagcctgatggacggcttcgagtggcaccgcggttactcaatccgcagggggttgttctacgtcgacttcctgagtcaggacaagatgttgctgccaaagagtagcgcccttttctaccagaagttgattgagaagaacggcttcccaccactccccgagaaccagcccctggagggcacctttccctgcgatttcgcttggggcgtggtggataattatattcaggtgagccagctgacaaaacctatcagcagcctgacaaagccttaccat

SEQ ID NO: 35 - RNA, 1482 nt, synthetic construct
  source 1..1482: mol_type = other RNA
ctgttccagggcaccttccccgacggatttctgtgggccgtgggaagcgctgcctaccagaccgagggcggctggcaacagcacggcaagggcgccagcatctgggacaccttcacccaccatcctctggctcctcccggagacagcagaaacgccagcctgcctctgggagcccccagccccctgcagcccgccactggagacgtggccagcgactcctacaacaacgtgttccgcgacaccgaggccctgcgcgagctgggcgtgacccactaccgctttagcatcagctgggccagagtgctgcccaacggcagcgccggcgtgcccaaccgggaaggcctgagatactatcgccgcctgctggagaggctgagagagttgggcgtgcagcccgtggtgaccctgtaccactgggacctgccccagcgcctgcaggacgcctacggcggctgggccaacagggcactcgccgaccacttccgcgactacgccgagctgtgcttccgccacttcggcgggcaggtgaagtactggatcaccatcgacaacccctacgtggtggcctggcacggctacgctacaggaaggctggcccccgggatccgcggcagccccaggctgggctacctggtggcccacaacctgctgctggcacacgccaaagtgtggcacctgtataacaccagctttcgccccacccagggtggacaggtgagcattgccctgagttctcattggatcaaccccaggcgcatgaccgatcacagcatcaaggaatgccagaagagcctggacttcgtgctgggctggttcgccaagcccgtgtttatcgacggcgactaccccgagtctatgaagaacaacctcagcagcatcctgcctgacgtcaccgagagcgagaagaagttcatcaagggcaccgccgacttcttcgccctgagcttcggccccaccctgagcttccagctgctggatccccatatgaagttcagacaactcgagagtcctaacctgcgccagctgctgagctggatcgacctggaattcaaccacccacagatcttcatcgtggagaacggctggtttgtgagcggcaccactaagcgcgacgacgcaaagtatatgtattatctgaagaaattcatcatggaaaccctgaaggccatcaagctggacggcgtggacgtgatcggatacaccgcatggagcctgatggacggcttcgagtggcaccgcggttacagcatccgccggggcctgttctacgttgacttcctgagccaggacaagatgttgctgcccaagagctccgccctgttctaccagaagttgatcgagaagaacggcttcccaccactccccgagaaccagcccctggagggcaccttcccctgcgatttcgcctggggcgtggtggacaactacatccaggtgagccagctgacaaaacctatcagcagcctgacaaagccttaccat

SEQ ID NO: 36 - RNA, 1482 nt, synthetic construct
  source 1..1482: mol_type = other RNA
ttgtttcagggaacctttcctgacggtttcctgtgggctgtgggcagcgccgcctatcagaccgagggcggctggcaacagcacggaaaaggagccagcatctgggataccttcacccaccaccccctggccccccccggcgattcccgcaatgccagcctccctctgggagcccctagccccctgcaacctgccacaggagacgtggcctcagacagctataacaacgtgttccgcgacaccgaggcactgcgcgagctgggcgtgacccattaccgctttagcatcagctgggccagagtgctgcccaatggctctgccggcgtgcccaaccgggagggcctgaggtactaccgccgcctgctggagaggctgcgggagctgggcgtgcagcccgtggtaaccctgtaccactgggacctgccccagcgcctgcaggacgcttacggcggctgggccaaccgcgctctcgcagaccacttccgcgactacgccgagctgtgctttcgccactttggcggccaggtgaagtattggatcaccatcgataacccttacgtggtggcctggcacggatacgctacaggccgcctggcccccggcatccgcggcagccccagactgggctacctggtggcccacaacctgctgctggcccacgccaaggtgtggcacctgtacaacaccagcttccgccccacccagggtggacaggtctctattgccctgagctctcactggattaaccccaggaggatgaccgatcacagcatcaaggaatgccagaagagcctggacttcgttctgggctggttcgccaagcccgtgtttatcgacggcgactaccccgagagcatgaagaacaacctgtctagcatcctgcccgacgtcaccgagagcgaaaaaaaattcatcaagggcaccgccgatttcttcgccctgagcttcggcccaaccctgagcttccaactgctggatccccacatgaagttcagacaactcgagagtcccaacctgcgccagctgctgagctggatcgatctggaattcaaccacccccagatattcatagtggagaacggctggtttgtaagcggcactactaagcgcgatgatgcaaagtacatgtactatctgaagaagttcatcatggaaaccctgaaggccatcaagctggatggcgtggacgtgatcggatacaccgcatggagcctgatggacggcttcgagtggcaccgcggttactcaatccgcagggggttgttctacgtcgacttcctgagtcaggacaagatgttgctgccaaagagtagcgcccttttctaccagaagttgattgagaagaacggcttcccaccactccccgagaaccagcccctggagggcacctttccctgcgatttcgcttggggcgtggtggataattatattcaggtgagccagctgacaaaacctatcagcagcctgacaaagccttaccat

SEQ ID NO: 37 - RNA, 1548 nt, synthetic construct
  source 1..1548: mol_type = other RNA
gagcctggcgacggggcccagacctgggccagattcagcagaccccccgcacccgaggccgccggcctgttccagggcaccttccccgacggatttctgtgggccgtgggaagcgctgcctaccagaccgagggcggctggcaacagcacggcaagggcgccagcatctgggacaccttcacccaccatcctctggctcctcccggagacagcagaaacgccagcctgcctctgggagcccccagccccctgcagcccgccactggagacgtggccagcgactcctacaacaacgtgttccgcgacaccgaggccctgcgcgagctgggcgtgacccactaccgctttagcatcagctgggccagagtgctgcccaacggcagcgccggcgtgcccaaccgggaaggcctgagatactatcgccgcctgctggagaggctgagagagttgggcgtgcagcccgtggtgaccctgtaccactgggacctgccccagcgcctgcaggacgcctacggcggctgggccaacagggcactcgccgaccacttccgcgactacgccgagctgtgcttccgccacttcggcgggcaggtgaagtactggatcaccatcgacaacccctacgtggtggcctggcacggctacgctacaggaaggctggcccccgggatccgcggcagccccaggctgggctacctggtggcccacaacctgctgctggcacacgccaaagtgtggcacctgtataacaccagctttcgccccacccagggtggacaggtgagcattgccctgagttctcattggatcaaccccaggcgcatgaccgatcacagcatcaaggaatgccagaagagcctggacttcgtgctgggctggttcgccaagcccgtgtttatcgacggcgactaccccgagtctatgaagaacaacctcagcagcatcctgcctgacttcaccgagagcgagaagaagttcatcaagggcaccgccgacttcttcgccctgtgcttcggccccaccctgagcttccagctgctggatccccatatgaagttcagacaactcgagagtcctaacctgcgccagctgctgagctggatcgacctggaattcaaccacccacagatcttcatcgtggagaacggctggtttgtgagcggcaccactaagcgcgacgacgcaaagtatatgtattatctgaagaaattcatcatggaaaccctgaaggccatcaagctggacggcgtggacgtgatcggatacaccgcatggagcctgatggacggcttcgagtggcaccgcggttacagcatccgccggggcctgttctacgttgacttcctgagccaggacaagatgttgctgcccaagagctccgccctgttctaccagaagttgatcgagaagaacggcttcccaccactccccgagaaccagcccctggagggcaccttcccctgcgatttcgcctggggcgtggtggacaactacatccaggtgagccagctgacaaaacctatcagcagcctgacaaagccttaccat

SEQ ID NO: 38 - RNA, 1548 nt, synthetic construct
  source 1..1548: mol_type = other RNA
gagcctggagatggagcccaaacatgggccagattcagcagacctcccgctcctgaagccgccggcttgtttcagggaacctttcctgacggtttcctgtgggctgtgggcagcgccgcctatcagaccgagggcggctggcaacagcacggaaaaggagccagcatctgggataccttcacccaccaccccctggccccccccggcgattcccgcaatgccagcctccctctgggagcccctagccccctgcaacctgccacaggagacgtggcctcagacagctataacaacgtgttccgcgacaccgaggcactgcgcgagctgggcgtgacccattaccgctttagcatcagctgggccagagtgctgcccaatggctctgccggcgtgcccaaccgggagggcctgaggtactaccgccgcctgctggagaggctgcgggagctgggcgtgcagcccgtggtaaccctgtaccactgggacctgccccagcgcctgcaggacgcttacggcggctgggccaaccgcgctctcgcagaccacttccgcgactacgccgagctgtgctttcgccactttggcggccaggtgaagtattggatcaccatcgataacccttacgtggtggcctggcacggatacgctacaggccgcctggcccccggcatccgcggcagccccagactgggctacctggtggcccacaacctgctgctggcccacgccaaggtgtggcacctgtacaacaccagcttccgccccacccagggtggacaggtctctattgccctgagctctcactggattaaccccaggaggatgaccgatcacagcatcaaggaatgccagaagagcctggacttcgttctgggctggttcgccaagcccgtgtttatcgacggcgactaccccgagagcatgaagaacaacctgtctagcatcctgcccgacttcaccgagagcgaaaaaaaattcatcaagggcaccgccgatttcttcgccctgtgtttcggcccaaccctgagcttccaactgctggatccccacatgaagttcagacaactcgagagtcccaacctgcgccagctgctgagctggatcgatctggaattcaaccacccccagatattcatagtggagaacggctggtttgtaagcggcactactaagcgcgatgatgcaaagtacatgtactatctgaagaagttcatcatggaaaccctgaaggccatcaagctggatggcgtggacgtgatcggatacaccgcatggagcctgatggacggcttcgagtggcaccgcggttactcaatccgcagggggttgttctacgtcgacttcctgagtcaggacaagatgttgctgccaaagagtagcgcccttttctaccagaagttgattgagaagaacggcttcccaccactccccgagaaccagcccctggagggcacctttccctgcgatttcgcttggggcgtggtggataattatattcaggtgagccagctgacaaaacctatcagcagcctgacaaagccttaccat

SEQ ID NO: 39 - RNA, 1548 nt, synthetic construct
  source 1..1548: mol_type = other RNA
gagcctggcgacggggcccagacctgggccagattcagcagaccccccgcacccgaggccgccggcctgttccagggcaccttccccgacggatttctgtgggccgtgggaagcgctgcctaccagaccgagggcggctggcaacagcacggcaagggcgccagcatctgggacaccttcacccaccatcctctggctcctcccggagacagcagaaacgccagcctgcctctgggagcccccagccccctgcagcccgccactggagacgtggccagcgactcctacaacaacgtgttccgcgacaccgaggccctgcgcgagctgggcgtgacccactaccgctttagcatcagctgggccagagtgctgcccaacggcagcgccggcgtgcccaaccgggaaggcctgagatactatcgccgcctgctggagaggctgagagagttgggcgtgcagcccgtggtgaccctgtaccactgggacctgccccagcgcctgcaggacgcctacggcggctgggccaacagggcactcgccgaccacttccgcgactacgccgagctgtgcttccgccacttcggcgggcaggtgaagtactggatcaccatcgacaacccctacgtggtggcctggcacggctacgctacaggaaggctggcccccgggatccgcggcagccccaggctgggctacctggtggcccacaacctgctgctggcacacgccaaagtgtggcacctgtataacaccagctttcgccccacccagggtggacaggtgagcattgccctgagttctcattggatcaaccccaggcgcatgaccgatcacagcatcaaggaatgccagaagagcctggacttcgtgctgggctggttcgccaagcccgtgtttatcgacggcgactaccccgagtctatgaagaacaacctcagcagcatcctgcctgacgtcaccgagagcgagaagaagttcatcaagggcaccgccgacttcttcgccctgagcttcggccccaccctgagcttccagctgctggatccccatatgaagttcagacaactcgagagtcctaacctgcgccagctgctgagctggatcgacctggaattcaaccacccacagatcttcatcgtggagaacggctggtttgtgagcggcaccactaagcgcgacgacgcaaagtatatgtattatctgaagaaattcatcatggaaaccctgaaggccatcaagctggacggcgtggacgtgatcggatacaccgcatggagcctgatggacggcttcgagtggcaccgcggttacagcatccgccggggcctgttctacgttgacttcctgagccaggacaagatgttgctgcccaagagctccgccctgttctaccagaagttgatcgagaagaacggcttcccaccactccccgagaaccagcccctggagggcaccttcccctgcgatttcgcctggggcgtggtggacaactacatccaggtgagccagctgacaaaacctatcagcagcctgacaaagccttaccat

SEQ ID NO: 40 - RNA, 1548 nt, synthetic construct
  source 1..1548: mol_type = other RNA
gagcctggagatggagcccaaacatgggccagattcagcagacctcccgctcctgaagccgccggcttgtttcagggaacctttcctgacggtttcctgtgggctgtgggcagcgccgcctatcagaccgagggcggctggcaacagcacggaaaaggagccagcatctgggataccttcacccaccaccccctggccccccccggcgattcccgcaatgccagcctccctctgggagcccctagccccctgcaacctgccacaggagacgtggcctcagacagctataacaacgtgttccgcgacaccgaggcactgcgcgagctgggcgtgacccattaccgctttagcatcagctgggccagagtgctgcccaatggctctgccggcgtgcccaaccgggagggcctgaggtactaccgccgcctgctggagaggctgcgggagctgggcgtgcagcccgtggtaaccctgtaccactgggacctgccccagcgcctgcaggacgcttacggcggctgggccaaccgcgctctcgcagaccacttccgcgactacgccgagctgtgctttcgccactttggcggccaggtgaagtattggatcaccatcgataacccttacgtggtggcctggcacggatacgctacaggccgcctggcccccggcatccgcggcagccccagactgggctacctggtggcccacaacctgctgctggcccacgccaaggtgtggcacctgtacaacaccagcttccgccccacccagggtggacaggtctctattgccctgagctctcactggattaaccccaggaggatgaccgatcacagcatcaaggaatgccagaagagcctggacttcgttctgggctggttcgccaagcccgtgtttatcgacggcgactaccccgagagcatgaagaacaacctgtctagcatcctgcccgacgtcaccgagagcgaaaaaaaattcatcaagggcaccgccgatttcttcgccctgagcttcggcccaaccctgagcttccaactgctggatccccacatgaagttcagacaactcgagagtcccaacctgcgccagctgctgagctggatcgatctggaattcaaccacccccagatattcatagtggagaacggctggtttgtaagcggcactactaagcgcgatgatgcaaagtacatgtactatctgaagaagttcatcatggaaaccctgaaggccatcaagctggatggcgtggacgtgatcggatacaccgcatggagcctgatggacggcttcgagtggcaccgcggttactcaatccgcagggggttgttctacgtcgacttcctgagtcaggacaagatgttgctgccaaagagtagcgcccttttctaccagaagttgattgagaagaacggcttcccaccactccccgagaaccagcccctggagggcacctttccctgcgatttcgcttggggcgtggtggataattatattcaggtgagccagctgacaaaacctatcagcagcctgacaaagccttaccat

SEQ ID NO: 41 - RNA, 1650 nt, synthetic construct
  source 1..1650: mol_type = other RNA
atgcccgctagcgccccaccgagaagaccgcggccgccaccgccatcgctgtcgctgctgctggtgctgctgggactgggcggaagaagactgcgtgcggagcctggcgacggggcccagacctgggccagattcagcagaccccccgcacccgaggccgccggcctgttccagggcaccttccccgacggatttctgtgggccgtgggaagcgctgcctaccagaccgagggcggctggcaacagcacggcaagggcgccagcatctgggacaccttcacccaccatcctctggctcctcccggagacagcagaaacgccagcctgcctctgggagcccccagccccctgcagcccgccactggagacgtggccagcgactcctacaacaacgtgttccgcgacaccgaggccctgcgcgagctgggcgtgacccactaccgctttagcatcagctgggccagagtgctgcccaacggcagcgccggcgtgcccaaccgggaaggcctgagatactatcgccgcctgctggagaggctgagagagttgggcgtgcagcccgtggtgaccctgtaccactgggacctgccccagcgcctgcaggacgcctacggcggctgggccaacagggcactcgccgaccacttccgcgactacgccgagctgtgcttccgccacttcggcgggcaggtgaagtactggatcaccatcgacaacccctacgtggtggcctggcacggctacgctacaggaaggctggcccccgggatccgcggcagccccaggctgggctacctggtggcccacaacctgctgctggcacacgccaaagtgtggcacctgtataacaccagctttcgccccacccagggtggacaggtgagcattgccctgagttctcattggatcaaccccaggcgcatgaccgatcacagcatcaaggaatgccagaagagcctggacttcgtgctgggctggttcgccaagcccgtgtttatcgacggcgactaccccgagtctatgaagaacaacctcagcagcatcctgcctgacttcaccgagagcgagaagaagttcatcaagggcaccgccgacttcttcgccctgtgcttcggccccaccctgagcttccagctgctggatccccatatgaagttcagacaactcgagagtcctaacctgcgccagctgctgagctggatcgacctggaattcaaccacccacagatcttcatcgtggagaacggctggtttgtgagcggcaccactaagcgcgacgacgcaaagtatatgtattatctgaagaaattcatcatggaaaccctgaaggccatcaagctggacggcgtggacgtgatcggatacaccgcatggagcctgatggacggcttcgagtggcaccgcggttacagcatccgccggggcctgttctacgttgacttcctgagccaggacaagatgttgctgcccaagagctccgccctgttctaccagaagttgatcgagaagaacggcttcccaccactccccgagaaccagcccctggagggcaccttcccctgcgatttcgcctggggcgtggtggacaactacatccaggtgagccagctgacaaaacctatcagcagcctgacaaagccttaccattga

SEQ ID NO: 42 - RNA, 1650 nt, synthetic construct
  source 1..1650: mol_type = other RNA
atgcccgctagcgccccaccgagaagaccgcggccgccaccgccatcgctgtcgctgctgctggtgctgctgggactgggcggaagaagactgcgtgcggagcctggagatggagcccaaacatgggccagattcagcagacctcccgctcctgaagccgccggcttgtttcagggaacctttcctgacggtttcctgtgggctgtgggcagcgccgcctatcagaccgagggcggctggcaacagcacggaaaaggagccagcatctgggataccttcacccaccaccccctggccccccccggcgattcccgcaatgccagcctccctctgggagcccctagccccctgcaacctgccacaggagacgtggcctcagacagctataacaacgtgttccgcgacaccgaggcactgcgcgagctgggcgtgacccattaccgctttagcatcagctgggccagagtgctgcccaatggctctgccggcgtgcccaaccgggagggcctgaggtactaccgccgcctgctggagaggctgcgggagctgggcgtgcagcccgtggtaaccctgtaccactgggacctgccccagcgcctgcaggacgcttacggcggctgggccaaccgcgctctcgcagaccacttccgcgactacgccgagctgtgctttcgccactttggcggccaggtgaagtattggatcaccatcgataacccttacgtggtggcctggcacggatacgctacaggccgcctggcccccggcatccgcggcagccccagactgggctacctggtggcccacaacctgctgctggcccacgccaaggtgtggcacctgtacaacaccagcttccgccccacccagggtggacaggtctctattgccctgagctctcactggattaaccccaggaggatgaccgatcacagcatcaaggaatgccagaagagcctggacttcgttctgggctggttcgccaagcccgtgtttatcgacggcgactaccccgagagcatgaagaacaacctgtctagcatcctgcccgacttcaccgagagcgaaaaaaaattcatcaagggcaccgccgatttcttcgccctgtgtttcggcccaaccctgagcttccaactgctggatccccacatgaagttcagacaactcgagagtcccaacctgcgccagctgctgagctggatcgatctggaattcaaccacccccagatattcatagtggagaacggctggtttgtaagcggcactactaagcgcgatgatgcaaagtacatgtactatctgaagaagttcatcatggaaaccctgaaggccatcaagctggatggcgtggacgtgatcggatacaccgcatggagcctgatggacggcttcgagtggcaccgcggttactcaatccgcagggggttgttctacgtcgacttcctgagtcaggacaagatgttgctgccaaagagtagcgcccttttctaccagaagttgattgagaagaacggcttcccaccactccccgagaaccagcccctggagggcacctttccctgcgatttcgcttggggcgtggtggataattatattcaggtgagccagctgacaaaacctatcagcagcctgacaaagccttaccattga

SEQ ID NO: 43 - RNA, 1650 nt, synthetic construct
  source 1..1650: mol_type = other RNA
atgcccgctagcgccccaccgagaagaccgcggccgccaccgccatcgctgtcgctgctgctggtgctgctgggactgggcggaagaagactgcgtgcggagcctggcgacggggcccagacctgggccagattcagcagaccccccgcacccgaggccgccggcctgttccagggcaccttccccgacggatttctgtgggccgtgggaagcgctgcctaccagaccgagggcggctggcaacagcacggcaagggcgccagcatctgggacaccttcacccaccatcctctggctcctcccggagacagcagaaacgccagcctgcctctgggagcccccagccccctgcagcccgccactggagacgtggccagcgactcctacaacaacgtgttccgcgacaccgaggccctgcgcgagctgggcgtgacccactaccgctttagcatcagctgggccagagtgctgcccaacggcagcgccggcgtgcccaaccgggaaggcctgagatactatcgccgcctgctggagaggctgagagagttgggcgtgcagcccgtggtgaccctgtaccactgggacctgccccagcgcctgcaggacgcctacggcggctgggccaacagggcactcgccgaccacttccgcgactacgccgagctgtgcttccgccacttcggcgggcaggtgaagtactggatcaccatcgacaacccctacgtggtggcctggcacggctacgctacaggaaggctggcccccgggatccgcggcagccccaggctgggctacctggtggcccacaacctgctgctggcacacgccaaagtgtggcacctgtataacaccagctttcgccccacccagggtggacaggtgagcattgccctgagttctcattggatcaaccccaggcgcatgaccgatcacagcatcaaggaatgccagaagagcctggacttcgtgctgggctggttcgccaagcccgtgtttatcgacggcgactaccccgagtctatgaagaacaacctcagcagcatcctgcctgacgtcaccgagagcgagaagaagttcatcaagggcaccgccgacttcttcgccctgagcttcggccccaccctgagcttccagctgctggatccccatatgaagttcagacaactcgagagtcctaacctgcgccagctgctgagctggatcgacctggaattcaaccacccacagatcttcatcgtggagaacggctggtttgtgagcggcaccactaagcgcgacgacgcaaagtatatgtattatctgaagaaattcatcatggaaaccctgaaggccatcaagctggacggcgtggacgtgatcggatacaccgcatggagcctgatggacggcttcgagtggcaccgcggttacagcatccgccggggcctgttctacgttgacttcctgagccaggacaagatgttgctgcccaagagctccgccctgttctaccagaagttgatcgagaagaacggcttcccaccactccccgagaaccagcccctggagggcaccttcccctgcgatttcgcctggggcgtggtggacaactacatccaggtgagccagctgacaaaacctatcagcagcctgacaaagccttaccattga

SEQ ID NO: 44 - RNA, 1650 nt, synthetic construct
  source 1..1650: mol_type = other RNA
atgcccgctagcgccccaccgagaagaccgcggccgccaccgccatcgctgtcgctgctgctggtgctgctgggactgggcggaagaagactgcgtgcggagcctggagatggagcccaaacatgggccagattcagcagacctcccgctcctgaagccgccggcttgtttcagggaacctttcctgacggtttcctgtgggctgtgggcagcgccgcctatcagaccgagggcggctggcaacagcacggaaaaggagccagcatctgggataccttcacccaccaccccctggccccccccggcgattcccgcaatgccagcctccctctgggagcccctagccccctgcaacctgccacaggagacgtggcctcagacagctataacaacgtgttccgcgacaccgaggcactgcgcgagctgggcgtgacccattaccgctttagcatcagctgggccagagtgctgcccaatggctctgccggcgtgcccaaccgggagggcctgaggtactaccgccgcctgctggagaggctgcgggagctgggcgtgcagcccgtggtaaccctgtaccactgggacctgccccagcgcctgcaggacgcttacggcggctgggccaaccgcgctctcgcagaccacttccgcgactacgccgagctgtgctttcgccactttggcggccaggtgaagtattggatcaccatcgataacccttacgtggtggcctggcacggatacgctacaggccgcctggcccccggcatccgcggcagccccagactgggctacctggtggcccacaacctgctgctggcccacgccaaggtgtggcacctgtacaacaccagcttccgccccacccagggtggacaggtctctattgccctgagctctcactggattaaccccaggaggatgaccgatcacagcatcaaggaatgccagaagagcctggacttcgttctgggctggttcgccaagcccgtgtttatcgacggcgactaccccgagagcatgaagaacaacctgtctagcatcctgcccgacgtcaccgagagcgaaaaaaaattcatcaagggcaccgccgatttcttcgccctgagcttcggcccaaccctgagcttccaactgctggatccccacatgaagttcagacaactcgagagtcccaacctgcgccagctgctgagctggatcgatctggaattcaaccacccccagatattcatagtggagaacggctggtttgtaagcggcactactaagcgcgatgatgcaaagtacatgtactatctgaagaagttcatcatggaaaccctgaaggccatcaagctggatggcgtggacgtgatcggatacaccgcatggagcctgatggacggcttcgagtggcaccgcggttactcaatccgcagggggttgttctacgtcgacttcctgagtcaggacaagatgttgctgccaaagagtagcgcccttttctaccagaagttgattgagaagaacggcttcccaccactccccgagaaccagcccctggagggcacctttccctgcgatttcgcttggggcgtggtggataattatattcaggtgagccagctgacaaaacctatcagcagcctgacaaagccttaccattga

SEQ ID NO: 45 - RNA, 1953 nt, synthetic construct
  source 1..1953: mol_type = other RNA
gggagacataaaccctggcgcgctcgcggcccggcactcttctggtccccacagactcagagagaacccaccatgcccgctagcgccccaccgagaagaccgcggccgccaccgccatcgctgtcgctgctgctggtgctgctgggactgggcggaagaagactgcgtgcggagcctggcgacggggcccagacctgggccagattcagcagaccccccgcacccgaggccgccggcctgttccagggcaccttccccgacggatttctgtgggccgtgggaagcgctgcctaccagaccgagggcggctggcaacagcacggcaagggcgccagcatctgggacaccttcacccaccatcctctggctcctcccggagacagcagaaacgccagcctgcctctgggagcccccagccccctgcagcccgccactggagacgtggccagcgactcctacaacaacgtgttccgcgacaccgaggccctgcgcgagctgggcgtgacccactaccgctttagcatcagctgggccagagtgctgcccaacggcagcgccggcgtgcccaaccgggaaggcctgagatactatcgccgcctgctggagaggctgagagagttgggcgtgcagcccgtggtgaccctgtaccactgggacctgccccagcgcctgcaggacgcctacggcggctgggccaacagggcactcgccgaccacttccgcgactacgccgagctgtgcttccgccacttcggcgggcaggtgaagtactggatcaccatcgacaacccctacgtggtggcctggcacggctacgctacaggaaggctggcccccgggatccgcggcagccccaggctgggctacctggtggcccacaacctgctgctggcacacgccaaagtgtggcacctgtataacaccagctttcgccccacccagggtggacaggtgagcattgccctgagttctcattggatcaaccccaggcgcatgaccgatcacagcatcaaggaatgccagaagagcctggacttcgtgctgggctggttcgccaagcccgtgtttatcgacggcgactaccccgagtctatgaagaacaacctcagcagcatcctgcctgacttcaccgagagcgagaagaagttcatcaagggcaccgccgacttcttcgccctgtgcttcggccccaccctgagcttccagctgctggatccccatatgaagttcagacaactcgagagtcctaacctgcgccagctgctgagctggatcgacctggaattcaaccacccacagatcttcatcgtggagaacggctggtttgtgagcggcaccactaagcgcgacgacgcaaagtatatgtattatctgaagaaattcatcatggaaaccctgaaggccatcaagctggacggcgtggacgtgatcggatacaccgcatggagcctgatggacggcttcgagtggcaccgcggttacagcatccgccggggcctgttctacgttgacttcctgagccaggacaagatgttgctgcccaagagctccgccctgttctaccagaagttgatcgagaagaacggcttcccaccactccccgagaaccagcccctggagggcaccttcccctgcgatttcgcctggggcgtggtggacaactacatccaggtgagccagctgacaaaacctatcagcagcctgacaaagccttaccattgagctggagcctcggtggccatgcttcttgccccttgggcctccccccagcccctcctccccttcctgcacccgtacccccgtggtctttgaataaagtctgagtgggcggcaaaaaaaaaaaaaaaaaaaaaaaaaaaaaaaaaaaaaaaaaaaaaaaaaaaaaaaaaaaaaaaaaaaaaaaaaaaaaaaaaaaaaaaaaaaaaaaaaaaaaaaaaaaaaaaaaaaaaaaaa

SEQ ID NO: 46 - RNA, 1953 nt, synthetic construct
  source 1..1953: mol_type = other RNA
gggagacataaaccctggcgcgctcgcggcccggcactcttctggtccccacagactcagagagaacccaccatgcccgctagcgccccaccgagaagaccgcggccgccaccgccatcgctgtcgctgctgctggtgctgctgggactgggcggaagaagactgcgtgcggagcctggagatggagcccaaacatgggccagattcagcagacctcccgctcctgaagccgccggcttgtttcagggaacctttcctgacggtttcctgtgggctgtgggcagcgccgcctatcagaccgagggcggctggcaacagcacggaaaaggagccagcatctgggataccttcacccaccaccccctggccccccccggcgattcccgcaatgccagcctccctctgggagcccctagccccctgcaacctgccacaggagacgtggcctcagacagctataacaacgtgttccgcgacaccgaggcactgcgcgagctgggcgtgacccattaccgctttagcatcagctgggccagagtgctgcccaatggctctgccggcgtgcccaaccgggagggcctgaggtactaccgccgcctgctggagaggctgcgggagctgggcgtgcagcccgtggtaaccctgtaccactgggacctgccccagcgcctgcaggacgcttacggcggctgggccaaccgcgctctcgcagaccacttccgcgactacgccgagctgtgctttcgccactttggcggccaggtgaagtattggatcaccatcgataacccttacgtggtggcctggcacggatacgctacaggccgcctggcccccggcatccgcggcagccccagactgggctacctggtggcccacaacctgctgctggcccacgccaaggtgtggcacctgtacaacaccagcttccgccccacccagggtggacaggtctctattgccctgagctctcactggattaaccccaggaggatgaccgatcacagcatcaaggaatgccagaagagcctggacttcgttctgggctggttcgccaagcccgtgtttatcgacggcgactaccccgagagcatgaagaacaacctgtctagcatcctgcccgacttcaccgagagcgaaaaaaaattcatcaagggcaccgccgatttcttcgccctgtgtttcggcccaaccctgagcttccaactgctggatccccacatgaagttcagacaactcgagagtcccaacctgcgccagctgctgagctggatcgatctggaattcaaccacccccagatattcatagtggagaacggctggtttgtaagcggcactactaagcgcgatgatgcaaagtacatgtactatctgaagaagttcatcatggaaaccctgaaggccatcaagctggatggcgtggacgtgatcggatacaccgcatggagcctgatggacggcttcgagtggcaccgcggttactcaatccgcagggggttgttctacgtcgacttcctgagtcaggacaagatgttgctgccaaagagtagcgcccttttctaccagaagttgattgagaagaacggcttcccaccactccccgagaaccagcccctggagggcacctttccctgcgatttcgcttggggcgtggtggataattatattcaggtgagccagctgacaaaacctatcagcagcctgacaaagccttaccattgagctggagcctcggtggccatgcttcttgccccttgggcctccccccagcccctcctccccttcctgcacccgtacccccgtggtctttgaataaagtctgagtgggcggcaaaaaaaaaaaaaaaaaaaaaaaaaaaaaaaaaaaaaaaaaaaaaaaaaaaaaaaaaaaaaaaaaaaaaaaaaaaaaaaaaaaaaaaaaaaaaaaaaaaaaaaaaaaaaaaaaaaaaaaaa

SEQ ID NO: 47 - RNA, 1953 nt, synthetic construct
  source 1..1953: mol_type = other RNA
gggagacataaaccctggcgcgctcgcggcccggcactcttctggtccccacagactcagagagaacccaccatgcccgctagcgccccaccgagaagaccgcggccgccaccgccatcgctgtcgctgctgctggtgctgctgggactgggcggaagaagactgcgtgcggagcctggcgacggggcccagacctgggccagattcagcagaccccccgcacccgaggccgccggcctgttccagggcaccttccccgacggatttctgtgggccgtgggaagcgctgcctaccagaccgagggcggctggcaacagcacggcaagggcgccagcatctgggacaccttcacccaccatcctctggctcctcccggagacagcagaaacgccagcctgcctctgggagcccccagccccctgcagcccgccactggagacgtggccagcgactcctacaacaacgtgttccgcgacaccgaggccctgcgcgagctgggcgtgacccactaccgctttagcatcagctgggccagagtgctgcccaacggcagcgccggcgtgcccaaccgggaaggcctgagatactatcgccgcctgctggagaggctgagagagttgggcgtgcagcccgtggtgaccctgtaccactgggacctgccccagcgcctgcaggacgcctacggcggctgggccaacagggcactcgccgaccacttccgcgactacgccgagctgtgcttccgccacttcggcgggcaggtgaagtactggatcaccatcgacaacccctacgtggtggcctggcacggctacgctacaggaaggctggcccccgggatccgcggcagccccaggctgggctacctggtggcccacaacctgctgctggcacacgccaaagtgtggcacctgtataacaccagctttcgccccacccagggtggacaggtgagcattgccctgagttctcattggatcaaccccaggcgcatgaccgatcacagcatcaaggaatgccagaagagcctggacttcgtgctgggctggttcgccaagcccgtgtttatcgacggcgactaccccgagtctatgaagaacaacctcagcagcatcctgcctgacgtcaccgagagcgagaagaagttcatcaagggcaccgccgacttcttcgccctgagcttcggccccaccctgagcttccagctgctggatccccatatgaagttcagacaactcgagagtcctaacctgcgccagctgctgagctggatcgacctggaattcaaccacccacagatcttcatcgtggagaacggctggtttgtgagcggcaccactaagcgcgacgacgcaaagtatatgtattatctgaagaaattcatcatggaaaccctgaaggccatcaagctggacggcgtggacgtgatcggatacaccgcatggagcctgatggacggcttcgagtggcaccgcggttacagcatccgccggggcctgttctacgttgacttcctgagccaggacaagatgttgctgcccaagagctccgccctgttctaccagaagttgatcgagaagaacggcttcccaccactccccgagaaccagcccctggagggcaccttcccctgcgatttcgcctggggcgtggtggacaactacatccaggtgagccagctgacaaaacctatcagcagcctgacaaagccttaccattgagctggagcctcggtggccatgcttcttgccccttgggcctccccccagcccctcctccccttcctgcacccgtacccccgtggtctttgaataaagtctgagtgggcggcaaaaaaaaaaaaaaaaaaaaaaaaaaaaaaaaaaaaaaaaaaaaaaaaaaaaaaaaaaaaaaaaaaaaaaaaaaaaaaaaaaaaaaaaaaaaaaaaaaaaaaaaaaaaaaaaaaaaaaaaa

SEQ ID NO: 48 - RNA, 1953 nt, synthetic construct
  source 1..1953: mol_type = other RNA
gggagacataaaccctggcgcgctcgcggcccggcactcttctggtccccacagactcagagagaacccaccatgcccgctagcgccccaccgagaagaccgcggccgccaccgccatcgctgtcgctgctgctggtgctgctgggactgggcggaagaagactgcgtgcggagcctggagatggagcccaaacatgggccagattcagcagacctcccgctcctgaagccgccggcttgtttcagggaacctttcctgacggtttcctgtgggctgtgggcagcgccgcctatcagaccgagggcggctggcaacagcacggaaaaggagccagcatctgggataccttcacccaccaccccctggccccccccggcgattcccgcaatgccagcctccctctgggagcccctagccccctgcaacctgccacaggagacgtggcctcagacagctataacaacgtgttccgcgacaccgaggcactgcgcgagctgggcgtgacccattaccgctttagcatcagctgggccagagtgctgcccaatggctctgccggcgtgcccaaccgggagggcctgaggtactaccgccgcctgctggagaggctgcgggagctgggcgtgcagcccgtggtaaccctgtaccactgggacctgccccagcgcctgcaggacgcttacggcggctgggccaaccgcgctctcgcagaccacttccgcgactacgccgagctgtgctttcgccactttggcggccaggtgaagtattggatcaccatcgataacccttacgtggtggcctggcacggatacgctacaggccgcctggcccccggcatccgcggcagccccagactgggctacctggtggcccacaacctgctgctggcccacgccaaggtgtggcacctgtacaacaccagcttccgccccacccagggtggacaggtctctattgccctgagctctcactggattaaccccaggaggatgaccgatcacagcatcaaggaatgccagaagagcctggacttcgttctgggctggttcgccaagcccgtgtttatcgacggcgactaccccgagagcatgaagaacaacctgtctagcatcctgcccgacgtcaccgagagcgaaaaaaaattcatcaagggcaccgccgatttcttcgccctgagcttcggcccaaccctgagcttccaactgctggatccccacatgaagttcagacaactcgagagtcccaacctgcgccagctgctgagctggatcgatctggaattcaaccacccccagatattcatagtggagaacggctggtttgtaagcggcactactaagcgcgatgatgcaaagtacatgtactatctgaagaagttcatcatggaaaccctgaaggccatcaagctggatggcgtggacgtgatcggatacaccgcatggagcctgatggacggcttcgagtggcaccgcggttactcaatccgcagggggttgttctacgtcgacttcctgagtcaggacaagatgttgctgccaaagagtagcgcccttttctaccagaagttgattgagaagaacggcttcccaccactccccgagaaccagcccctggagggcacctttccctgcgatttcgcttggggcgtggtggataattatattcaggtgagccagctgacaaaacctatcagcagcctgacaaagccttaccattgagctggagcctcggtggccatgcttcttgccccttgggcctccccccagcccctcctccccttcctgcacccgtacccccgtggtctttgaataaagtctgagtgggcggcaaaaaaaaaaaaaaaaaaaaaaaaaaaaaaaaaaaaaaaaaaaaaaaaaaaaaaaaaaaaaaaaaaaaaaaaaaaaaaaaaaaaaaaaaaaaaaaaaaaaaaaaaaaaaaaaaaaaaaaaa

SEQ ID NO: 49 - protein, 1012 aa, Homo sapiens
MPASAPPRRPRPPPPSLSLLLVLLGLGGRRLRAEPGDGAQTWARFSRPPAPEAAGLFQGTFPDGFLWAVGSAAYQTEGGWQQHGKGASIWDTFTHHPLAPPGDSRNASLPLGAPSPLQPATGDVASDSYNNVFRDTEALRELGVTHYRFSISWARVLPNGSAGVPNREGLRYYRRLLERLRELGVQPVVTLYHWDLPQRLQDAYGGWANRALADHFRDYAELCFRHFGGQVKYWITIDNPYVVAWHGYATGRLAPGIRGSPRLGYLVAHNLLLAHAKVWHLYNTSFRPTQGGQVSIALSSHWINPRRMTDHSIKECQKSLDFVLGWFAKPVFIDGDYPESMKNNLSSILPDFTESEKKFIKGTADFFALCFGPTLSFQLLDPHMKFRQLESPNLRQLLSWIDLEFNHPQIFIVENGWFVSGTTKRDDAKYMYYLKKFIMETLKAIKLDGVDVIGYTAWSLMDGFEWHRGYSIRRGLFYVDFLSQDKMLLPKSSALFYQKLIEKNGFPPLPENQPLEGTFPCDFAWGVVDNYIQVDTTLSQFTDLNVYLWDVHHSKRLIKVDGVVTKKRKSYCVDFAAIQPQIALLQEMHVTHFRFSLDWALILPLGNQSQVNHTILQYYRCMASELVRVNITPVVALWQPMAPNQGLPRLLARQGAWENPYTALAFAEYARLCFQELGHHVKLWITMNEPYTRNMTYSAGHNLLKAHALAWHVYNEKFRHAQNGKISIALQADWIEPACPFSQKDKEVAERVLEFDIGWLAEPIFGSGDYPWVMRDWLNQRNNFLLPYFTEDEKKLIQGTFDFLALSHYTTILVDSEKEDPIKYNDYLEVQEMTDITWLNSPSQVAVVPWGLRKVLNWLKFKYGDLPMYIISNGIDDGLHAEDDQLRVYYMQNYINEALKAHILDGINLCGYFAYSFNDRTAPRFGLYRYAADQFEPKASMKHYRKIIDSNGFPGPETLERFCPEEFTVCTECSFFHTRKSLLAFIAFLFFASIISLSLIFYYSKKGRRSYK

SEQ ID NO: 50 - protein, 549 aa, Homo sapiens
MPASAPPRRPRPPPPSLSLLLVLLGLGGRRLRAEPGDGAQTWARFSRPPAPEAAGLFQGTFPDGFLWAVGSAAYQTEGGWQQHGKGASIWDTFTHHPLAPPGDSRNASLPLGAPSPLQPATGDVASDSYNNVFRDTEALRELGVTHYRFSISWARVLPNGSAGVPNREGLRYYRRLLERLRELGVQPVVTLYHWDLPQRLQDAYGGWANRALADHFRDYAELCFRHFGGQVKYWITIDNPYVVAWHGYATGRLAPGIRGSPRLGYLVAHNLLLAHAKVWHLYNTSFRPTQGGQVSIALSSHWINPRRMTDHSIKECQKSLDFVLGWFAKPVFIDGDYPESMKNNLSSILPDFTESEKKFIKGTADFFALCFGPTLSFQLLDPHMKFRQLESPNLRQLLSWIDLEFNHPQIFIVENGWFVSGTTKRDDAKYMYYLKKFIMETLKAIKLDGVDVIGYTAWSLMDGFEWHRGYSIRRGLFYVDFLSQDKMLLPKSSALFYQKLIEKNGFPPLPENQPLEGTFPCDFAWGVVDNYIQVSQLTKPISSLTKPYH

SEQ ID NO: 51 - protein, 33 aa, Homo sapiens
MPASAPPRRPRPPPPSLSLLLVLLGLGGRRLRA

SEQ ID NO: 52 - protein, 451 aa, Homo sapiens
LFQGTFPDGFLWAVGSAAYQTEGGWQQHGKGASIWDTFTHHPLAPPGDSRNASLPLGAPSPLQPATGDVASDSYNNVFRDTEALRELGVTHYRFSISWARVLPNGSAGVPNREGLRYYRRLLERLRELGVQPVVTLYHWDLPQRLQDAYGGWANRALADHFRDYAELCFRHFGGQVKYWITIDNPYVVAWHGYATGRLAPGIRGSPRLGYLVAHNLLLAHAKVWHLYNTSFRPTQGGQVSIALSSHWINPRRMTDHSIKECQKSLDFVLGWFAKPVFIDGDYPESMKNNLSSILPDFTESEKKFIKGTADFFALCFGPTLSFQLLDPHMKFRQLESPNLRQLLSWIDLEFNHPQIFIVENGWFVSGTTKRDDAKYMYYLKKFIMETLKAIKLDGVDVIGYTAWSLMDGFEWHRGYSIRRGLFYVDFLSQDKMLLPKSSALFYQKLIEKNGF

SEQ ID NO: 53 - protein, 451 aa, synthetic construct
LFQGTFPDGFLWAVGSAAYQTEGGWQQHGKGASIWDTFTHHPLAPPGDSRNASLPLGAPSPLQPATGDVASDSYNNVFRDTEALRELGVTHYRFSISWARVLPNGSAGVPNREGLRYYRRLLERLRELGVQPVVTLYHWDLPQRLQDAYGGWANRALADHFRDYAELCFRHFGGQVKYWITIDNPYVVAWHGYATGRLAPGIRGSPRLGYLVAHNLLLAHAKVWHLYNTSFRPTQGGQVSIALSSHWINPRRMTDHSIKECQKSLDFVLGWFAKPVFIDGDYPESMKNNLSSILPDVTESEKKFIKGTADFFALSFGPTLSFQLLDPHMKFRQLESPNLRQLLSWIDLEFNHPQIFIVENGWFVSGTTKRDDAKYMYYLKKFIMETLKAIKLDGVDVIGYTAWSLMDGFEWHRGYSIRRGLFYVDFLSQDKMLLPKSSALFYQKLIEKNGF

SEQ ID NO: 54 - protein, 438 aa, Homo sapiens
LEGTFPCDFAWGVVDNYIQVDTTLSQFTDLNVYLWDVHHSKRLIKVDGVVTKKRKSYCVDFAAIQPQIALLQEMHVTHFRFSLDWALILPLGNQSQVNHTILQYYRCMASELVRVNITPVVALWQPMAPNQGLPRLLARQGAWENPYTALAFAEYARLCFQELGHHVKLWITMNEPYTRNMTYSAGHNLLKAHALAWHVYNEKFRHAQNGKISIALQADWIEPACPFSQKDKEVAERVLEFDIGWLAEPIFGSGDYPWVMRDWLNQRNNFLLPYFTEDEKKLIQGTFDFLALSHYTTILVDSEKEDPIKYNDYLEVQEMTDITWLNSPSQVAVVPWGLRKVLNWLKFKYGDLPMYIISNGIDDGLHAEDDQLRVYYMQNYINEALKAHILDGINLCGYFAYSFNDRTAPRFGLYRYAADQFEPKASMKHYRKIIDSNG

SEQ ID NO: 55 - protein, 506 aa, Homo sapiens
MPASAPPRRPRPPPPSLSLLLVLLGLGGRRLRAEPGDGAQTWARFSRPPAPEAAGLFQGTFPDGFLWAVGSAAYQTEGGWQQHGKGASIWDTFTHHPLAPPGDSRNASLPLGAPSPLQPATGDVASDSYNNVFRDTEALRELGVTHYRFSISWARVLPNGSAGVPNREGLRYYRRLLERLRELGVQPVVTLYHWDLPQRLQDAYGGWANRALADHFRDYAELCFRHFGGQVKYWITIDNPYVVAWHGYATGRLAPGIRGSPRLGYLVAHNLLLAHAKVWHLYNTSFRPTQGGQVSIALSSHWINPRRMTDHSIKECQKSLDFVLGWFAKPVFIDGDYPESMKNNLSSILPDFTESEKKFIKGTADFFALCFGPTLSFQLLDPHMKFRQLESPNLRQLLSWIDLEFNHPQIFIVENGWFVSGTTKRDDAKYMYYLKKFIMETLKAIKLDGVDVIGYTAWSLMDGFEWHRGYSIRRGLFYVDFLSQDKMLLPKSSALFYQKLIEKNGF

SEQ ID NO: 56 - protein, 506 aa, synthetic construct
MPASAPPRRPRPPPPSLSLLLVLLGLGGRRLRAEPGDGAQTWARFSRPPAPEAAGLFQGTFPDGFLWAVGSAAYQTEGGWQQHGKGASIWDTFTHHPLAPPGDSRNASLPLGAPSPLQPATGDVASDSYNNVFRDTEALRELGVTHYRFSISWARVLPNGSAGVPNREGLRYYRRLLERLRELGVQPVVTLYHWDLPQRLQDAYGGWANRALADHFRDYAELCFRHFGGQVKYWITIDNPYVVAWHGYATGRLAPGIRGSPRLGYLVAHNLLLAHAKVWHLYNTSFRPTQGGQVSIALSSHWINPRRMTDHSIKECQKSLDFVLGWFAKPVFIDGDYPESMKNNLSSILPDVTESEKKFIKGTADFFALSFGPTLSFQLLDPHMKFRQLESPNLRQLLSWIDLEFNHPQIFIVENGWFVSGTTKRDDAKYMYYLKKFIMETLKAIKLDGVDVIGYTAWSLMDGFEWHRGYSIRRGLFYVDFLSQDKMLLPKSSALFYQKLIEKNGF

SEQ ID NO: 57 - protein, 981 aa, Homo sapiens
MPASAPPRRPRPPPPSLSLLLVLLGLGGRRLRAEPGDGAQTWARFSRPPAPEAAGLFQGTFPDGFLWAVGSAAYQTEGGWQQHGKGASIWDTFTHHPLAPPGDSRNASLPLGAPSPLQPATGDVASDSYNNVFRDTEALRELGVTHYRFSISWARVLPNGSAGVPNREGLRYYRRLLERLRELGVQPVVTLYHWDLPQRLQDAYGGWANRALADHFRDYAELCFRHFGGQVKYWITIDNPYVVAWHGYATGRLAPGIRGSPRLGYLVAHNLLLAHAKVWHLYNTSFRPTQGGQVSIALSSHWINPRRMTDHSIKECQKSLDFVLGWFAKPVFIDGDYPESMKNNLSSILPDFTESEKKFIKGTADFFALCFGPTLSFQLLDPHMKFRQLESPNLRQLLSWIDLEFNHPQIFIVENGWFVSGTTKRDDAKYMYYLKKFIMETLKAIKLDGVDVIGYTAWSLMDGFEWHRGYSIRRGLFYVDFLSQDKMLLPKSSALFYQKLIEKNGFPPLPENQPLEGTFPCDFAWGVVDNYIQVDTTLSQFTDLNVYLWDVHHSKRLIKVDGVVTKKRKSYCVDFAAIQPQIALLQEMHVTHFRFSLDWALILPLGNQSQVNHTILQYYRCMASELVRVNITPVVALWQPMAPNQGLPRLLARQGAWENPYTALAFAEYARLCFQELGHHVKLWITMNEPYTRNMTYSAGHNLLKAHALAWHVYNEKFRHAQNGKISIALQADWIEPACPFSQKDKEVAERVLEFDIGWLAEPIFGSGDYPWVMRDWLNQRNNFLLPYFTEDEKKLIQGTFDFLALSHYTTILVDSEKEDPIKYNDYLEVQEMTDITWLNSPSQVAVVPWGLRKVLNWLKFKYGDLPMYIISNGIDDGLHAEDDQLRVYYMQNYINEALKAHILDGINLCGYFAYSFNDRTAPRFGLYRYAADQFEPKASMKHYRKIIDSNGFPGPETLERFCPEEFTVCTECSFFHTRKS

SEQ ID NO: 58 - protein, 981 aa, synthetic construct
MPASAPPRRPRPPPPSLSLLLVLLGLGGRRLRAEPGDGAQTWARFSRPPAPEAAGLFQGTFPDGFLWAVGSAAYQTEGGWQQHGKGASIWDTFTHHPLAPPGDSRNASLPLGAPSPLQPATGDVASDSYNNVFRDTEALRELGVTHYRFSISWARVLPNGSAGVPNREGLRYYRRLLERLRELGVQPVVTLYHWDLPQRLQDAYGGWANRALADHFRDYAELCFRHFGGQVKYWITIDNPYVVAWHGYATGRLAPGIRGSPRLGYLVAHNLLLAHAKVWHLYNTSFRPTQGGQVSIALSSHWINPRRMTDHSIKECQKSLDFVLGWFAKPVFIDGDYPESMKNNLSSILPDVTESEKKFIKGTADFFALSFGPTLSFQLLDPHMKFRQLESPNLRQLLSWIDLEFNHPQIFIVENGWFVSGTTKRDDAKYMYYLKKFIMETLKAIKLDGVDVIGYTAWSLMDGFEWHRGYSIRRGLFYVDFLSQDKMLLPKSSALFYQKLIEKNGFPPLPENQPLEGTFPCDFAWGVVDNYIQVDTTLSQFTDLNVYLWDVHHSKRLIKVDGVVTKKRKSYCVDFAAIQPQIALLQEMHVTHFRFSLDWALILPLGNQSQVNHTILQYYRCMASELVRVNITPVVALWQPMAPNQGLPRLLARQGAWENPYTALAFAEYARLCFQELGHHVKLWITMNEPYTRNMTYSAGHNLLKAHALAWHVYNEKFRHAQNGKISIALQADWIEPACPFSQKDKEVAERVLEFDIGWLAEPIFGSGDYPWVMRDWLNQRNNFLLPYFTEDEKKLIQGTFDFLALSHYTTILVDSEKEDPIKYNDYLEVQEMTDITWLNSPSQVAVVPWGLRKVLNWLKFKYGDLPMYIISNGIDDGLHAEDDQLRVYYMQNYINEALKAHILDGINLCGYFAYSFNDRTAPRFGLYRYAADQFEPKASMKHYRKIIDSNGFPGPETLERFCPEEFTVCTECSFFHTRKS

SEQ ID NO: 59 - protein, 549 aa, Homo sapiens; identical to SEQ ID NO: 50

SEQ ID NO: 60 - protein, 549 aa, synthetic construct
MPASAPPRRPRPPPPSLSLLLVLLGLGGRRLRAEPGDGAQTWARFSRPPAPEAAGLFQGTFPDGFLWAVGSAAYQTEGGWQQHGKGASIWDTFTHHPLAPPGDSRNASLPLGAPSPLQPATGDVASDSYNNVFRDTEALRELGVTHYRFSISWARVLPNGSAGVPNREGLRYYRRLLERLRELGVQPVVTLYHWDLPQRLQDAYGGWANRALADHFRDYAELCFRHFGGQVKYWITIDNPYVVAWHGYATGRLAPGIRGSPRLGYLVAHNLLLAHAKVWHLYNTSFRPTQGGQVSIALSSHWINPRRMTDHSIKECQKSLDFVLGWFAKPVFIDGDYPESMKNNLSSILPDVTESEKKFIKGTADFFALSFGPTLSFQLLDPHMKFRQLESPNLRQLLSWIDLEFNHPQIFIVENGWFVSGTTKRDDAKYMYYLKKFIMETLKAIKLDGVDVIGYTAWSLMDGFEWHRGYSIRRGLFYVDFLSQDKMLLPKSSALFYQKLIEKNGFPPLPENQPLEGTFPCDFAWGVVDNYIQVSQLTKPISSLTKPYH

SEQ ID NO: 61 - RNA, 72 nt, synthetic construct
  source 1..72: mol_type = other RNA
gggagacataaaccctggcgcgctcgcggcccggcactcttctggtccccacagactcagagagaacccacc

SEQ ID NO: 62 - RNA, 111 nt, synthetic construct
  source 1..111: mol_type = other RNA
gctggagcctcggtggccatgcttcttgccccttgggcctccccccagcccctcctccccttcctgcacccgtacccccgtggtctttgaataaagtctgagtgggcggca

SEQ ID NO: 63 - RNA, 15 nt, synthetic construct
  source 1..15: mol_type = other RNA
  misc_feature 5: note = any 0 to 10 nucleotides
  misc_feature 10: note = any 0 to 10 pyrimidine (y) nucleotides
yccancccwntcycc

SEQ ID NO: 64 - RNA, 2937 nt, synthetic construct
  source 1..2937: mol_type = other RNA
gagcctggcgacggggcccagacctgggccagattcagcagaccccccgcacccgaggccgccggcctgttccagggcaccttccccgacggatttctgtgggccgtgggaagcgctgcctaccagaccgagggcggctggcaacagcacggcaagggcgccagcatctgggacaccttcacccaccatcctctggctcctcccggagacagcagaaacgccagcctgcctctgggagcccccagccccctgcagcccgccactggagacgtggccagcgactcctacaacaacgtgttccgcgacaccgaggccctgcgcgagctgggcgtgacccactaccgctttagcatcagctgggccagagtgctgcccaacggcagcgccggcgtgcccaaccgggaaggcctgagatactatcgccgcctgctggagaggctgagagagttgggcgtgcagcccgtggtgaccctgtaccactgggacctgccccagcgcctgcaggacgcctacggcggctgggccaacagggcactcgccgaccacttccgcgactacgccgagctgtgcttccgccacttcggcgggcaggtgaagtactggatcaccatcgacaacccctacgtggtggcctggcacggctacgctacaggaaggctggcccccgggatccgcggcagccccaggctgggctacctggtggcccacaacctgctgctggcacacgccaaagtgtggcacctgtataacaccagctttcgccccacccagggtggacaggtgagcattgccctgagttctcattggatcaaccccaggcgcatgaccgatcacagcatcaaggaatgccagaagagcctggacttcgtgctgggctggttcgccaagcccgtgtttatcgacggcgactaccccgagtctatgaagaacaacctcagcagcatcctgcctgacttcaccgagagcgagaagaagttcatcaagggcaccgccgacttcttcgccctgtgcttcggccccaccctgagcttccagctgctggatccccatatgaagttcagacaactcgagagtcctaacctgcgccagctgctgagctggatcgacctggaattcaaccacccacagatcttcatcgtggagaacggctggtttgtgagcggcaccactaagcgcgacgacgcaaagtatatgtattatctgaagaaattcatcatggaaaccctgaaggccatcaagctggacggcgtggacgtgatcggatacaccgcatggagcctgatggacggcttcgagtggcaccgcggttacagcatccgccggggcctgttctacgttgacttcctgagccaggacaagatgttgctgcccaagagctccgccctgttctaccagaagttgatcgagaagaacggcttcccaccactccccgagaaccagcccctggagggcaccttcccctgcgatttcgcctggggcgtggtggacaactacatccaggtggacaccaccctgagtcagttcactgacctgaacgtgtacctttgggacgtgcaccacagcaagcgcctgataaaggtcgacggcgtggtgaccaagaagcgcaaaagctactgcgtggactttgccgccatccagccccagatcgccctgctgcaggagatgcacgtgactcacttccgcttcagcctcgactgggccctgattctgcccctgggcaaccagtcacaagtgaaccacaccattctgcagtactaccgctgtatggccagcgagctggtacgcgtgaacatcacccccgttgtggccctttggcagcccatggcccccaaccagggcctgcctcgcctgctggcccgccagggagcctgggagaatccctacaccgcactggccttcgctgaatacgcccgcctgtgcttccaggagctggggcaccacgtgaaactctggatcaccatgaacgagccctacaccagaaacatgacctacagcgccggacacaatctgctgaaggcccacgctctggcctggcacgtgtacaacgagaagtttcgccacgcccagaacggcaagatcagcatcgccctgcaggccgattggatcgagcccgcctgccccttcagccagaaggacaaggaggtggctgagcgggtgctggagttcgacatcgggtggctggctgagcctatcttcggcagcggagactacccctgggtgatgcgcgattggcttaaccagaggaacaatttcctgctgccctacttcaccgaggacgagaagaagctgatccagggcacctttgacttcctggctttgagccactataccactatcctggtggacagcgagaaggaggaccccatcaagtacaacgactacttggaggtgcaggagatgaccgacatcacctggctgaacagccctagccaggtggctgtggtgccttggggcctgcgcaaggtgctgaactggctgaagttcaagtacggcgacctgcccatgtatatcatcagcaacggcatcgacgacggcctgcacgccgaggacgaccagctgagagtgtactacatgcagaactacatcaacgaggccctcaaggcccacatcctggacggcatcaacctgtgtggctactttgcctacagcttcaacgacagaaccgccccccgcttcggcctgtacaggtacgccgccgaccagttcgaacccaaggccagcatgaagcactaccgcaaaatcatcgacagcaacggattccctggacccgagacactggagcgcttctgcccagaggagttcaccgtgtgcaccgagtgcagtttcttccacacccgcaagagcctgctggctttcattgcttttctgttttttgcttccattatttctctctccctcatcttttactacagcaagaaaggaagaagaagctacaaa

SEQ ID NO: 65 - RNA, 2937 nt, synthetic construct
  source 1..2937: mol_type = other RNA
gagcctggagatggagcccaaacatgggccagattcagcagacctcccgctcctgaagccgccggcttgtttcagggaacctttcctgacggtttcctgtgggctgtgggcagcgccgcctatcagaccgagggcggctggcaacagcacggaaaaggagccagcatctgggataccttcacccaccaccccctggccccccccggcgattcccgcaatgccagcctccctctgggagcccctagccccctgcaacctgccacaggagacgtggcctcagacagctataacaacgtgttccgcgacaccgaggcactgcgcgagctgggcgtgacccattaccgctttagcatcagctgggccagagtgctgcccaatggctctgccggcgtgcccaaccgggagggcctgaggtactaccgccgcctgctggagaggctgcgggagctgggcgtgcagcccgtggtaaccctgtaccactgggacctgccccagcgcctgcaggacgcttacggcggctgggccaaccgcgctctcgcagaccacttccgcgactacgccgagctgtgctttcgccactttggcggccaggtgaagtattggatcaccatcgataacccttacgtggtggcctggcacggatacgctacaggccgcctggcccccggcatccgcggcagccccagactgggctacctggtggcccacaacctgctgctggcccacgccaaggtgtggcacctgtacaacaccagcttccgccccacccagggtggacaggtctctattgccctgagctctcactggattaaccccaggaggatgaccgatcacagcatcaaggaatgccagaagagcctggacttcgttctgggctggttcgccaagcccgtgtttatcgacggcgactaccccgagagcatgaagaacaacctgtctagcatcctgcccgacttcaccgagagcgaaaaaaaattcatcaagggcaccgccgatttcttcgccctgtgtttcggcccaaccctgagcttccaactgctggatccccacatgaagttcagacaactcgagagtcccaacctgcgccagctgctgagctggatcgatctggaattcaaccacccccagatattcatagtggagaacggctggtttgtaagcggcactactaagcgcgatgatgcaaagtacatgtactatctgaagaagttcatcatggaaaccctgaaggccatcaagctggatggcgtggacgtgatcggatacaccgcatggagcctgatggacggcttcgagtggcaccgcggttactcaatccgcagggggttgttctacgtcgacttcctgagtcaggacaagatgttgctgccaaagagtagcgcccttttctaccagaagttgattgagaagaacggcttcccaccactccccgagaaccagcccctggagggcacctttccctgcgatttcgcttggggcgtggtggataattatattcaggtggacaccaccctgtcacagttcactgacctgaacgtgtacctgtgggacgtgcaccattccaagcgcctgatcaaggtggacggcgtggtgaccaagaagcgcaaatcctactgcgttgactttgccgccattcagccacagatcgccctgctgcaggagatgcacgtcacccacttccgcttcagcctggactgggccctcatcctgccactgggcaaccagtcccaggtgaaccacaccattctgcagtactaccgctgtatggccagcgagctggtacgcgtgaacatcacccccgtggtggccctgtggcagcccatggcccccaaccagggcctgccacgcctgctggccaggcagggggcctgggagaacccctacaccgcactcgctttcgccgaatatgccaggctgtgcttccaggagctggggcaccacgtgaagctctggatcaccatgaacgaaccctacaccagaaacatgacctactctgccggacacaatctgctgaaggcccacgccctggcctggcacgtctacaacgagaagttccgccacgcccaaaatggaaagatctctatagccctgcaggccgattggatcgagcccgcctgccccttctcacagaaggacaaggaggtggccgagcgcgtgctggagttcgacatcggctggctggccgagcccatcttcggcagcggagactacccctgggtgatgcgcgattggcttaaccagcgcaacaactttctgctgccctacttcaccgaggacgagaagaagctgatccagggcaccttcgacttcctggccctgagccactatactaccatcctggtcgacagcgagaaggaggacccaatcaagtacaacgactacctggaggtgcaggagatgaccgacatcacctggctgaacagccctagccaggtcgccgtggtgccttggggcctgcgcaaggtgctgaactggctgaagttcaagtatggcgacctgccaatgtacatcatcagcaacggcattgatgacggcctgcacgccgaggacgatcagctgagagtgtactatatgcagaactacatcaacgaggcactgaaggcccacatcctggacggcatcaacctgtgtggctactttgcatactccttcaacgacagaaccgccccccgcttcggcctgtacaggtacgctgccgatcagttcgagcccaaggccagcatgaagcactacagaaaaatcattgatagcaacgggttcccaggccccgagaccctggagcgcttctgccccgaggagttcaccgtgtgcaccgagtgcagttttttccacacccgcaagagcctgctggctttcattgcttttctgttttttgcttccattatttctctctccctcatcttttactacagcaagaaaggaagaagaagctacaaa

SEQ ID NO: 66 - RNA, 2937 nt, synthetic construct
  source 1..2937: mol_type = other RNA
gagcctggcgacggggcccagacctgggccagattcagcagaccccccgcacccgaggccgccggcctgttccagggcaccttccccgacggatttctgtgggccgtgggaagcgctgcctaccagaccgagggcggctggcaacagcacggcaagggcgccagcatctgggacaccttcacccaccatcctctggctcctcccggagacagcagaaacgccagcctgcctctgggagcccccagccccctgcagcccgccactggagacgtggccagcgactcctacaacaacgtgttccgcgacaccgaggccctgcgcgagctgggcgtgacccactaccgctttagcatcagctgggccagagtgctgcccaacggcagcgccggcgtgcccaaccgggaaggcctgagatactatcgccgcctgctggagaggctgagagagttgggcgtgcagcccgtggtgaccctgtaccactgggacctgccccagcgcctgcaggacgcctacggcggctgggccaacagggcactcgccgaccacttccgcgactacgccgagctgtgcttccgccacttcggcgggcaggtgaagtactggatcaccatcgacaacccctacgtggtggcctggcacggctacgctacaggaaggctggcccccgggatccgcggcagccccaggctgggctacctggtggcccacaacctgctgctggcacacgccaaagtgtggcacctgtataacaccagctttcgccccacccagggtggacaggtgagcattgccctgagttctcattggatcaaccccaggcgcatgaccgatcacagcatcaaggaatgccagaagagcctggacttcgtgctgggctggttcgccaagcccgtgtttatcgacggcgactaccccgagtctatgaagaacaacctcagcagcatcctgcctgacgtcaccgagagcgagaagaagttcatcaagggcaccgccgacttcttcgccctgagcttcggccccaccctgagcttccagctgctggatccccatatgaagttcagacaactcgagagtcctaacctgcgccagctgctgagctggatcgacctggaattcaaccacccacagatcttcatcgtggagaacggctggtttgtgagcggcaccactaagcgcgacgacgcaaagtatatgtattatctgaagaaattcatcatggaaaccctgaaggccatcaagctggacggcgtggacgtgatcggatacaccgcatggagcctgatggacggcttcgagtggcaccgcggttacagcatccgccggggcctgttctacgttgacttcctgagccaggacaagatgttgctgcccaagagctccgccctgttctaccagaagttgatcgagaagaacggcttcccaccactccccgagaaccagcccctggagggcaccttcccctgcgatttcgcctggggcgtggtggacaactacatccaggtggacaccaccctgagtcagttcactgacctgaacgtgtacctttgggacgtgcaccacagcaagcgcctgataaaggtcgacggcgtggtgaccaagaagcgcaaaagctactgcgtggactttgccgccatccagccccagatcgccctgctgcaggagatgcacgtgactcacttccgcttcagcctcgactgggccctgattctgcccctgggcaaccagtcacaagtgaaccacaccattctgcagtactaccgctgtatggccagcgagctggtacgcgtgaacatcacccccgttgtggccctttggcagcccatggcccccaaccagggcctgcctcgcctgctggcccgccagggagcctgggagaatccctacaccgcactggccttcgctgaatacgcccgcctgtgcttccaggagctggggcaccacgtgaaactctggatcaccatgaacgagccctacaccagaaacatgacctacagcgccggacacaatctgctgaaggcccacgctctggcctggcacgtgtacaacgagaagtttcgccacgcccagaacggcaagatcagcatcgccctgcaggccgattggatcgagcccgcctgccccttcagccagaaggacaaggaggtggctgagcgggtgctggagttcgacatcgggtggctggctgagcctatcttcggcagcggagactacccctgggtgatgcgcgattggcttaaccagaggaacaatttcctgctgccctacttcaccgaggacgagaagaagctgatccagggcacctttgacttcctggctttgagccactataccactatcctggtggacagcgagaaggaggaccccatcaagtacaacgactacttggaggtgcaggagatgaccgacatcacctggctgaacagccctagccaggtggctgtggtgccttggggcctgcgcaaggtgctgaactggctgaagttcaagtacggcgacctgcccatgtatatcatcagcaacggcatcgacgacggcctgcacgccgaggacgaccagctgagagtgtactacatgcagaactacatcaacgaggccctcaaggcccacatcctggacggcatcaacctgtgtggctactttgcctacagcttcaacgacagaaccgccccccgcttcggcctgtacaggtacgccgccgaccagttcgaacccaaggccagcatgaagcactaccgcaaaatcatcgacagcaacggattccctggacccgagacactggagcgcttctgcccagaggagttcaccgtgtgcaccgagtgcagtttcttccacacccgcaagagcctgctggctttcattgcttttctgttttttgcttccattatttctctctccctcatcttttactacagcaagaaaggaagaagaagctacaaa

SEQ ID NO: 67 - RNA, 2937 nt, synthetic construct
  source 1..2937: mol_type = other RNA
gagcctggagatggagcccaaacatgggccagattcagcagacctcccgctcctgaagccgccggcttgtttcagggaacctttcctgacggtttcctgtgggctgtgggcagcgccgcctatcagaccgagggcggctggcaacagcacggaaaaggagccagcatctgggataccttcacccaccaccccctggccccccccggcgattcccgcaatgccagcctccctctgggagcccctagccccctgcaacctgccacaggagacgtggcctcagacagctataacaacgtgttccgcgacaccgaggcactgcgcgagctgggcgtgacccattaccgctttagcatcagctgggccagagtgctgcccaatggctctgccggcgtgcccaaccgggagggcctgaggtactaccgccgcctgctggagaggctgcgggagctgggcgtgcagcccgtggtaaccctgtaccactgggacctgccccagcgcctgcaggacgcttacggcggctgggccaaccgcgctctcgcagaccacttccgcgactacgccgagctgtgctttcgccactttggcggccaggtgaagtattggatcaccatcgataacccttacgtggtggcctggcacggatacgctacaggccgcctggcccccggcatccgcggcagccccagactgggctacctggtggcccacaacctgctgctggcccacgccaaggtgtggcacctgtacaacaccagcttccgccccacccagggtggacaggtctctattgccctgagctctcactggattaaccccaggaggatgaccgatcacagcatcaaggaatgccagaagagcctggacttcgttctgggctggttcgccaagcccgtgtttatcgacggcgactaccccgagagcatgaagaacaacctgtctagcatcctgcccgacgtcaccgagagcgaaaaaaaattcatcaagggcaccgccgatttcttcgccctgagcttcggcccaaccctgagcttccaactgctggatccccacatgaagttcagacaactcgagagtcccaacctgcgccagctgctgagctggatcgatctggaattcaaccacccccagatattcatagtggagaacggctggtttgtaagcggcactactaagcgcgatgatgcaaagtacatgtactatctgaagaagttcatcatggaaaccctgaaggccatcaagctggatggcgtggacgtgatcggatacaccgcatggagcctgatggacggcttcgagtggcaccgcggttactcaatccgcagggggttgttctacgtcgacttcctgagtcaggacaagatgttgctgccaaagagtagcgcccttttctaccagaagttgattgagaagaacggcttcccaccactccccgagaaccagcccctggagggcacctttccctgcgatttcgcttggggcgtggtggataattatattcaggtggacaccaccctgtcacagttcactgacctgaacgtgtacctgtgggacgtgcaccattccaagcgcctgatcaaggtggacggcgtggtgaccaagaagcgcaaatcctactgcgttgactttgccgccattcagccacagatcgccctgctgcaggagatgcacgtcacccacttccgcttcagcctggactgggccctcatcctgccactgggcaaccagtcccaggtgaaccacaccattctgcagtactaccgctgtatggccagcgagctggtacgcgtgaacatcacccccgtggtggccctgtggcagcccatggcccccaaccagggcctgccacgcctgctggccaggcagggggcctgggagaacccctacaccgcactcgctttcgccgaatatgccaggctgtgcttccaggagctggggcaccacgtgaagctctggatcaccatgaacgaaccctacaccagaaacatgacctactctgccggacacaatctgctgaaggcccacgccctggcctggcacgtctacaacgagaagttccgccacgcccaaaatggaaagatctctatagccctgcaggccgattggatcgagcccgcctgccccttctcacagaaggacaaggaggtggccgagcgcgtgctggagttcgacatcggctggctggccgagcccatcttcggcagcggagactacccctgggtgatgcgcgattggcttaaccagcgcaacaactttctgctgccctacttcaccgaggacgagaagaagctgatccagggcaccttcgacttcctggccctgagccactatactaccatcctggtcgacagcgagaaggaggacccaatcaagtacaacgactacctggaggtgcaggagatgaccgacatcacctggctgaacagccctagccaggtcgccgtggtgccttggggcctgcgcaaggtgctgaactggctgaagttcaagtatggcgacctgccaatgtacatcatcagcaacggcattgatgacggcctgcacgccgaggacgatcagctgagagtgtactatatgcagaactacatcaacgaggcactgaaggcccacatcctggacggcatcaacctgtgtggctactttgcatactccttcaacgacagaaccgccccccgcttcggcctgtacaggtacgctgccgatcagttcgagcccaaggccagcatgaagcactacagaaaaatcattgatagcaacgggttcccaggccccgagaccctggagcgcttctgccccgaggagttcaccgtgtgcaccgagtgcagttttttccacacccgcaagagcctgctggctttcattgcttttctgttttttgcttccattatttctctctccctcatcttttactacagcaagaaaggaagaagaagctacaaa

SEQ ID NO: 68 - RNA, 3039 nt, synthetic construct
  source 1..3039: mol_type = other RNA
atgcccgctagcgccccaccgagaagaccgcggccgccaccgccatcgctgtcgctgctgctggtgctgctgggactgggcggaagaagactgcgtgcggagcctggcgacggggcccagacctgggccagattcagcagaccccccgcacccgaggccgccggcctgttccagggcaccttccccgacggatttctgtgggccgtgggaagcgctgcctaccagaccgagggcggctggcaacagcacggcaagggcgccagcatctgggacaccttcacccaccatcctctggctcctcccggagacagcagaaacgccagcctgcctctgggagcccccagccccctgcagcccgccactggagacgtggccagcgactcctacaacaacgtgttccgcgacaccgaggccctgcgcgagctgggcgtgacccactaccgctttagcatcagctgggccagagtgctgcccaacggcagcgccggcgtgcccaaccgggaaggcctgagatactatcgccgcctgctggagaggctgagagagttgggcgtgcagcccgtggtgaccctgtaccactgggacctgccccagcgcctgcaggacgcctacggcggctgggccaacagggcactcgccgaccacttccgcgactacgccgagctgtgcttccgccacttcggcgggcaggtgaagtactggatcaccatcgacaacccctacgtggtggcctggcacggctacgctacaggaaggctggcccccgggatccgcggcagccccaggctgggctacctggtggcccacaacctgctgctggcacacgccaaagtgtggcacctgtataacaccagctttcgccccacccagggtggacaggtgagcattgccctgagttctcattggatcaaccccaggcgcatgaccgatcacagcatcaaggaatgccagaagagcctggacttcgtgctgggctggttcgccaagcccgtgtttatcgacggcgactaccccgagtctatgaagaacaacctcagcagcatcctgcctgacttcaccgagagcgagaagaagttcatcaagggcaccgccgacttcttcgccctgtgcttcggccccaccctgagcttccagctgctggatccccatatgaagttcagacaactcgagagtcctaacctgcgccagctgctgagctggatcgacctggaattcaaccacccacagatcttcatcgtggagaacggctggtttgtgagcggcaccactaagcgcgacgacgcaaagtatatgtattatctgaagaaattcatcatggaaaccctgaaggccatcaagctggacggcgtggacgtgatcggatacaccgcatggagcctgatggacggcttcgagtggcaccgcggttacagcatccgccggggcctgttctacgttgacttcctgagccaggacaagatgttgctgcccaagagctccgccctgttctaccagaagttgatcgagaagaacggcttcccaccactccccgagaaccagcccctggagggcaccttcccctgcgatttcgcctggggcgtggtggacaactacatccaggtggacaccaccctgagtcagttcactgacctgaacgtgtacctttgggacgtgcaccacagcaagcgcctgataaaggtcgacggcgtggtgaccaagaagcgcaaaagctactgcgtggactttgccgccatccagccccagatcgccctgctgcaggagatgcacgtgactcacttccgcttcagcctcgactgggccctgattctgcccctgggcaaccagtcacaagtgaaccacaccattctgcagtactaccgctgtatggccagcgagctggtacgcgtgaacatcacccccgttgtggccctttggcagcccatggcccccaaccagggcctgcctcgcctgctggcccgccagggagcctgggagaatccctacaccgcactggccttcgctgaatacgcccgcctgtgcttccaggagctggggcaccacgtgaaactctggatcaccatgaacgagccctacaccagaaacatgacctacagcgccggacacaatctgctgaaggcccacgctctggcctggcacgtgtacaacgagaagtttcgccacgcccagaacggcaagatcagcatcgccctgcaggccgattggatcgagcccgcctgccccttcagccagaaggacaaggaggtggctgagcgggtgctggagttcgacatcgggtggctggctgagcctatcttcggcagcggagactacccctgggtgatgcgcgattggcttaaccagaggaacaatttcctgctgccctacttcaccgaggacgagaagaagctgatccagggcacctttgacttcctggctttgagccactataccactatcctggtggacagcgagaaggaggaccccatcaagtacaacgactacttggaggtgcaggagatgaccgacatcacctggctgaacagccctagccaggtggctgtggtgccttggggcctgcgcaaggtgctgaactggctgaagttcaagtacggcgacctgcccatgtatatcatcagcaacggcatcgacgacggcctgcacgccgaggacgaccagctgagagtgtactacatgcagaactacatcaacgaggccctcaaggcccacatcctggacggcatcaacctgtgtggctactttgcctacagcttcaacgacagaaccgccccccgcttcggcctgtacaggtacgccgccgaccagttcgaacccaaggccagcatgaagcactaccgcaaaatcatcgacagcaacggattccctggacccgagacactggagcgcttctgcccagaggagttcaccgtgtgcaccgagtgcagtttcttccacacccgcaagagcctgctggctttcattgcttttctgttttttgcttccattatttctctctccctcatcttttactacagcaagaaaggaagaagaagctacaaatga

SEQ ID NO: 69 - RNA, 3039 nt, synthetic construct
  source 1..3039: mol_type = other RNA
atgcccgctagcgccccaccgagaagaccgcggccgccaccgccatcgctgtcgctgctgctggtgctgctgggactgggcggaagaagactgcgtgcggagcctggagatggagcccaaacatgggccagattcagcagacctcccgctcctgaagccgccggcttgtttcagggaacctttcctgacggtttcctgtgggctgtgggcagcgccgcctatcagaccgagggcggctggcaacagcacggaaaaggagccagcatctgggataccttcacccaccaccccctggccccccccggcgattcccgcaatgccagcctccctctgggagcccctagccccctgcaacctgccacaggagacgtggcctcagacagctataacaacgtgttccgcgacaccgaggcactgcgcgagctgggcgtgacccattaccgctttagcatcagctgggccagagtgctgcccaatggctctgccggcgtgcccaaccgggagggcctgaggtactaccgccgcctgctggagaggctgcgggagctgggcgtgcagcccgtggtaaccctgtaccactgggacctgccccagcgcctgcaggacgcttacggcggctgggccaaccgcgctctcgcagaccacttccgcgactacgccgagctgtgctttcgccactttggcggccaggtgaagtattggatcaccatcgataacccttacgtggtggcctggcacggatacgctacaggccgcctggcccccggcatccgcggcagccccagactgggctacctggtggcccacaacctgctgctggcccacgccaaggtgtggcacctgtacaacaccagcttccgccccacccagggtggacaggtctctattgccctgagctctcactggattaaccccaggaggatgaccgatcacagcatcaaggaatgccagaagagcctggacttcgttctgggctggttcgccaagcccgtgtttatcgacggcgactaccccgagagcatgaagaacaacctgtctagcatcctgcccgacttcaccgagagcgaaaaaaaattcatcaagggcaccgccgatttcttcgccctgtgtttcggcccaaccctgagcttccaactgctggatccccacatgaagttcagacaactcgagagtcccaacctgcgccagctgctgagctggatcgatctggaattcaaccacccccagatattcatagtggagaacggctggtttgtaagcggcactactaagcgcgatgatgcaaagtacatgtactatctgaagaagttcatcatggaaaccctgaaggccatcaagctggatggcgtggacgtgatcggatacaccgcatggagcctgatggacggcttcgagtggcaccgcggttactcaatccgcagggggttgttctacgtcgacttcctgagtcaggacaagatgttgctgccaaagagtagcgcccttttctaccagaagttgattgagaagaacggcttcccaccactccccgagaaccagcccctggagggcacctttccctgcgatttcgcttggggcgtggtggataattatattcaggtggacaccaccctgtcacagttcactgacctgaacgtgtacctgtgggacgtgcaccattccaagcgcctgatcaaggtggacggcgtggtgaccaagaagcgcaaatcctactgcgttgactttgccgccattcagccacagatcgccctgctgcaggagatgcacgtcacccacttccgcttcagcctggactgggccctcatcctgccactgggcaaccagtcccaggtgaaccacaccattctgcagtactaccgctgtatggccagcgagctggtacgcgtgaacatcacccccgtggtggccctgtggcagcccatggcccccaaccagggcctgccacgcctgctggccaggcagggggcctgggagaacccctacaccgcactcgctttcgccgaatatgccaggctgtgcttccaggagctggggcaccacgtgaagctctggatcaccatgaacgaaccctacaccagaaacatgacctactctgccggacacaatctgctgaaggcccacgccctggcctggcacgtctacaacgagaagttccgccacgcccaaaatggaaagatctctatagccctgcaggccgattggatcgagcccgcctgccccttctcacagaaggacaaggaggtggccgagcgcgtgctggagttcgacatcggctggctggccgagcccatcttcggcagcggagactacccctgggtgatgcgcgattggcttaaccagcgcaacaactttctgctgccctacttcaccgaggacgagaagaagctgatccagggcaccttcgacttcctggccctgagccactatactaccatcctggtcgacagcgagaaggaggacccaatcaagtacaacgactacctggaggtgcaggagatgaccgacatcacctggctgaacagccctagccaggtcgccgtggtgccttggggcctgcgcaaggtgctgaactggctgaagttcaagtatggcgacctgccaatgtacatcatcagcaacggcattgatgacggcctgcacgccgaggacgatcagctgagagtgtactatatgcagaactacatcaacgaggcactgaaggcccacatcctggacggcatcaacctgtgtggctactttgcatactccttcaacgacagaaccgccccccgcttcggcctgtacaggtacgctgccgatcagttcgagcccaaggccagcatgaagcactacagaaaaatcattgatagcaacgggttcccaggccccgagaccctggagcgcttctgccccgaggagttcaccgtgtgcaccgagtgcagttttttccacacccgcaagagcctgctggctttcattgcttttctgttttttgcttccattatttctctctccctcatcttttactacagcaagaaaggaagaagaagctacaaatga

SEQ ID NO: 70 - RNA, 3039 nt, synthetic construct
  source 1..3039: mol_type = other RNA
atgcccgctagcgccccaccgagaagaccgcggccgccaccgccatcgctgtcgctgctgctggtgctgctgggactgggcggaagaagactgcgtgcggagcctggcgacggggcccagacctgggccagattcagcagaccccccgcacccgaggccgccggcctgttccagggcaccttccccgacggatttctgtgggccgtgggaagcgctgcctaccagaccgagggcggctggcaacagcacggcaagggcgccagcatctgggacaccttcacccaccatcctctggctcctcccggagacagcagaaacgccagcctgcctctgggagcccccagccccctgcagcccgccactggagacgtggccagcgactcctacaacaacgtgttccgcgacaccgaggccctgcgcgagctgggcgtgacccactaccgctttagcatcagctgggccagagtgctgcccaacggcagcgccggcgtgcccaaccgggaaggcctgagatactatcgccgcctgctggagaggctgagagagttgggcgtgcagcccgtggtgaccctgtaccactgggacctgccccagcgcctgcaggacgcctacggcggctgggccaacagggcactcgccgaccacttccgcgactacgccgagctgtgcttccgccacttcggcgggcaggtgaagtactggatcaccatcgacaacccctacgtggtggcctggcacggctacgctacaggaaggctggcccccgggatccgcggcagccccaggctgggctacctggtggcccacaacctgctgctggcacacgccaaagtgtggcacctgtataacaccagctttcgccccacccagggtggacaggtgagcattgccctgagttctcattggatcaaccccaggcgcatgaccgatcacagcatcaaggaatgccagaagagcctggacttcgtgctgggctggttcgccaagcccgtgtttatcgacggcgactaccccgagtctatgaagaacaacctcagcagcatcctgcctgacgtcaccgagagcgagaagaagttcatcaagggcaccgccgacttcttcgccctgagcttcggccccaccctgagcttccagctgctggatccccatatgaagttcagacaactcgagagtcctaacctgcgccagctgctgagctggatcgacctggaattcaaccacccacagatcttcatcgtggagaacggctggtttgtgagcggcaccactaagcgcgacgacgcaaagtatatgtattatctgaagaaattcatcatggaaaccctgaaggccatcaagctggacggcgtggacgtgatcggatacaccgcatggagcctgatggacggcttcgagtggcaccgcggttacagcatccgccggggcctgttctacgttgacttcctgagccaggacaagatgttgctgcccaagagctccgccctgttctaccagaagttgatcgagaagaacggcttcccaccactccccgagaaccagcccctggagggcaccttcccctgcgatttcgcctggggcgtggtggacaactacatccaggtggacaccaccctgagtcagttcactgacctgaacgtgtacctttgggacgtgcaccacagcaagcgcctgataaaggtcgacggcgtggtgaccaagaagcgcaaaagctactgcgtggactttgccgccatccagccccagatcgccctgctgcaggagatgcacgtgactcacttccgcttcagcctcgactgggccctgattctgcccctgggcaaccagtcacaagtgaaccacaccattctgcagtactaccgctgtatggccagcgagctggtacgcgtgaacatcacccccgttgtggccctttggcagcccatggcccccaaccagggcctgcctcgcctgctggcccgccagggagcctgggagaatccctacaccgcactggccttcgctgaatacgcccgcctgtgcttccaggagctggggcaccacgtgaaactctggatcaccatgaacgagccctacaccagaaacatgacctacagcgccggacacaatctgctgaaggcccacgctctggcctggcacgtgtacaacgagaagtttcgccacgcccagaacggcaagatcagcatcgccctgcaggccgattggatcgagcccgcctgccccttcagccagaaggacaaggaggtggctgagcgggtgctggagttcgacatcgggtggctggctgagcctatcttcggcagcggagactacccctgggtgatgcgcgattggcttaaccagaggaacaatttcctgctgccctacttcaccgaggacgagaagaagctgatccagggcacctttgacttcctggctttgagccactataccactatcctggtggacagcgagaaggaggaccccatcaagtacaacgactacttggaggtgcaggagatgaccgacatcacctggctgaacagccctagccaggtggctgtggtgccttggggcctgcgcaaggtgctgaactggctgaagttcaagtacggcgacctgcccatgtatatcatcagcaacggcatcgacgacggcctgcacgccgaggacgaccagctgagagtgtactacatgcagaactacatcaacgaggccctcaaggcccacatcctggacggcatcaacctgtgtggctactttgcctacagcttcaacgacagaaccgccccccgcttcggcctgtacaggtacgccgccgaccagttcgaacccaaggccagcatgaagcactaccgcaaaatcatcgacagcaacggattccctggacccgagacactggagcgcttctgcccagaggagttcaccgtgtgcaccgagtgcagtttcttccacacccgcaagagcctgctggctttcattgcttttctgttttttgcttccattatttctctctccctcatcttttactacagcaagaaaggaagaagaagctacaaatga

SEQ ID NO: 71 - RNA, 3039 nt, synthetic construct
  source 1..3039: mol_type = other RNA
atgcccgctagcgccccaccgagaagaccgcggccgccaccgccatcgctgtcgctgctgctggtgctgctgggactgggcggaagaagactgcgtgcggagcctggagatggagcccaaacatgggccagattcagcagacctcccgctcctgaagccgccggcttgtttcagggaacctttcctgacggtttcctgtgggctgtgggcagcgccgcctatcagaccgagggcggctggcaacagcacggaaaaggagccagcatctgggataccttcacccaccaccccctggccccccccggcgattcccgcaatgccagcctccctctgggagcccctagccccctgcaacctgccacaggagacgtggcctcagacagctataacaacgtgttccgcgacaccgaggcactgcgcgagctgggcgtgacccattaccgctttagcatcagctgggccagagtgctgcccaatggctctgccggcgtgcccaaccgggagggcctgaggtactaccgccgcctgctggagaggctgcgggagctgggcgtgcagcccgtggtaaccctgtaccactgggacctgccccagcgcctgcaggacgcttacggcggctgggccaaccgcgctctcgcagaccacttccgcgactacgccgagctgtgctttcgccactttggcggccaggtgaagtattggatcaccatcgataacccttacgtggtggcctggcacggatacgctacaggccgcctggcccccggcatccgcggcagccccagactgggctacctggtggcccacaacctgctgctggcccacgccaaggtgtggcacctgtacaacaccagcttccgccccacccagggtggacaggtctctattgccctgagctctcactggattaaccccaggaggatgaccgatcacagcatcaaggaatgccagaagagcctggacttcgttctgggctggttcgccaagcccgtgtttatcgacggcgactaccccgagagcatgaagaacaacctgtctagcatcctgcccgacgtcaccgagagcgaaaaaaaattcatcaagggcaccgccgatttcttcgccctgagcttcggcccaaccctgagcttccaactgctggatccccacatgaagttcagacaactcgagagtcccaacctgcgccagctgctgagctggatcgatctggaattcaaccacccccagatattcatagtggagaacggctggtttgtaagcggcactactaagcgcgatgatgcaaagtacatgtactatctgaagaagttcatcatggaaaccctgaaggccatcaagctggatggcgtggacgtgatcggatacaccgcatggagcctgatggacggcttcgagtggcaccgcggttactcaatccgcagggggttgttctacgtcgacttcctgagtcaggacaagatgttgctgccaaagagtagcgcccttttctaccagaagttgattgagaagaacggcttcccaccactccccgagaaccagcccctggagggcacctttccctgcgatttcgcttggggcgtggtggataattatattcaggtggacaccaccctgtcacagttcactgacctgaacgtgtacctgtgggacgtgcaccattccaagcgcctgatcaaggtggacggcgtggtgaccaagaagcgcaaatcctactgcgttgactttgccgccattcagccacagatcgccctgctgcaggagatgcacgtcacccacttccgcttcagcctggactgggccctcatcctgccactgggcaaccagtcccaggtgaaccacaccattctgcagtactaccgctgtatggccagcgagctggtacgcgtgaacatcacccccgtggtggccctgtggcagcccatggcccccaaccagggcctgccacgcctgctggccaggcagggggcctgggagaacccctacaccgcactcgctttcgccgaatatgccaggctgtgcttccaggagctggggcaccacgtgaagctctggatcaccatgaacgaaccctacaccagaaacatgacctactctgccggacacaatctgctgaaggcccacgccctggcctggcacgtctacaacgagaagttccgccacgcccaaaatggaaagatctctatagccctgcaggccgattggatcgagcccgcctgccccttctcacagaaggacaaggaggtggccgagcgcgtgctggagttcgacatcggctggctggccgagcccatcttcggcagcggagactacccctgggtgatgcgcgattggcttaaccagcgcaacaactttctgctgccctacttcaccgaggacgagaagaagctgatccagggcaccttcgacttcctggccctgagccactatactaccatcctggtcgacagcgagaaggaggacccaatcaagtacaacgactacctggaggtgcaggagatgaccgacatcacctggctgaacagccctagccaggtcgccgtggtgccttggggcctgcgcaaggtgctgaactggctgaagttcaagtatggcgacctgccaatgtacatcatcagcaacggcattgatgacggcctgcacgccgaggacgatcagctgagagtgtactatatgcagaactacatcaacgaggcactgaaggcccacatcctggacggcatcaacctgtgtggctactttgcatactccttcaacgacagaaccgccccccgcttcggcctgtacaggtacgctgccgatcagttcgagcccaaggccagcatgaagcactacagaaaaatcattgatagcaacgggttcccaggccccgagaccctggagcgcttctgccccgaggagttcaccgtgtgcaccgagtgcagttttttccacacccgcaagagcctgctggctttcattgcttttctgttttttgcttccattatttctctctccctcatcttttactacagcaagaaaggaagaagaagctacaaatga

SEQ ID NO: 72 - RNA, 3342 nt, synthetic construct
  source 1..3342: mol_type = other RNA
gggagacataaaccctggcgcgctcgcggcccggcactcttctggtccccacagactcagagagaacccaccatgcccgctagcgccccaccgagaagaccgcggccgccaccgccatcgctgtcgctgctgctggtgctgctgggactgggcggaagaagactgcgtgcggagcctggcgacggggcccagacctgggccagattcagcagaccccccgcacccgaggccgccggcctgttccagggcaccttccccgacggatttctgtgggccgtgggaagcgctgcctaccagaccgagggcggctggcaacagcacggcaagggcgccagcatctgggacaccttcacccaccatcctctggctcctcccggagacagcagaaacgccagcctgcctctgggagcccccagccccctgcagcccgccactggagacgtggccagcgactcctacaacaacgtgttccgcgacaccgaggccctgcgcgagctgggcgtgacccactaccgctttagcatcagctgggccagagtgctgcccaacggcagcgccggcgtgcccaaccgggaaggcctgagatactatcgccgcctgctggagaggctgagagagttgggcgtgcagcccgtggtgaccctgtaccactgggacctgccccagcgcctgcaggacgcctacggcggctgggccaacagggcactcgccgaccacttccgcgactacgccgagctgtgcttccgccacttcggcgggcaggtgaagtactggatcaccatcgacaacccctacgtggtggcctggcacggctacgctacaggaaggctggcccccgggatccgcggcagccccaggctgggctacctggtggcccacaacctgctgctggcacacgccaaagtgtggcacctgtataacaccagctttcgccccacccagggtggacaggtgagcattgccctgagttctcattggatcaaccccaggcgcatgaccgatcacagcatcaaggaatgccagaagagcctggacttcgtgctgggctggttcgccaagcccgtgtttatcgacggcgactaccccgagtctatgaagaacaacctcagcagcatcctgcctgacttcaccgagagcgagaagaagttcatcaagggcaccgccgacttcttcgccctgtgcttcggccccaccctgagcttccagctgctggatccccatatgaagttcagacaactcgagagtcctaacctgcgccagctgctgagctggatcgacctggaattcaaccacccacagatcttcatcgtggagaacggctggtttgtgagcggcaccactaagcgcgacgacgcaaagtatatgtattatctgaagaaattcatcatggaaaccctgaaggccatcaagctggacggcgtggacgtgatcggatacaccgcatggagcctgatggacggcttcgagtggcaccgcggttacagcatccgccggggcctgttctacgttgacttcctgagccaggacaagatgttgctgcccaagagctccgccctgttctaccagaagttgatcgagaagaacggcttcccaccactccccgagaaccagcccctggagggcaccttcccctgcgatttcgcctggggcgtggtggacaactacatccaggtggacaccaccctgagtcagttcactgacctgaacgtgtacctttgggacgtgcaccacagcaagcgcctgataaaggtcgacggcgtggtgaccaagaagcgcaaaagctactgcgtggactttgccgccatccagccccagatcgccctgctgcaggagatgcacgtgactcacttccgcttcagcctcgactgggccctgattctgcccctgggcaaccagtcacaagtgaaccacaccattctgcagtactaccgctgtatggccagcgagctggtacgcgtgaacatcacccccgttgtggccctttggcagcccatggcccccaaccagggcctgcctcgcctgctggcccgccagggagcctgggagaatccctacaccgcactggccttcgctgaatacgcccgcctgtgcttccaggagctggggcaccacgtgaaactctggatcaccatgaacgagccctacaccagaaacatgacctacagcgccggacacaatctgctgaaggcccacgctctggcctggcacgtgtacaacgagaagtttcgccacgcccagaacggcaagatcagcatcgccctgcaggccgattggatcgagcccgcctgccccttcagccagaaggacaaggaggtggctgagcgggtgctggagttcgacatcgggtggctggctgagcctatcttcggcagcggagactacccctgggtgatgcgcgattggcttaaccagaggaacaatttcctgctgccctacttcaccgaggacgagaagaagctgatccagggcacctttgacttcctggctttgagccactataccactatcctggtggacagcgagaaggaggaccccatcaagtacaacgactacttggaggtgcaggagatgaccgacatcacctggctgaacagccctagccaggtggctgtggtgccttggggcctgcgcaaggtgctgaactggctgaagttcaagtacggcgacctgcccatgtatatcatcagcaacggcatcgacgacggcctgcacgccgaggacgaccagctgagagtgtactacatgcagaactacatcaacgaggccctcaaggcccacatcctggacggcatcaacctgtgtggctactttgcctacagcttcaacgacagaaccgccccccgcttcggcctgtacaggtacgccgccgaccagttcgaacccaaggccagcatgaagcactaccgcaaaatcatcgacagcaacggattccctggacccgagacactggagcgcttctgcccagaggagttcaccgtgtgcaccgagtgcagtttcttccacacccgcaagagcctgctggctttcattgcttttctgttttttgcttccattatttctctctccctcatcttttactacagcaagaaaggaagaagaagctacaaatgagctggagcctcggtggccatgcttcttgccccttgggcctccccccagcccctcctccccttcctgcacccgtacccccgtggtctttgaataaagtctgagtgggcggcaaaaaaaaaaaaaaaaaaaaaaaaaaaaaaaaaaaaaaaaaaaaaaaaaaaaaaaaaaaaaaaaaaaaaaaaaaaaaaaaaaaaaaaaaaaaaaaaaaaaaaaaaaaaaaaaaaaaaaaaa

SEQ ID NO: 73 - RNA, 3342 nt, synthetic construct
  source 1..3342: mol_type = other RNA
gggagacataaaccctggcgcgctcgcggcccggcactcttctggtccccacagactcagagagaacccaccatgcccgctagcgccccaccgagaagaccgcggccgccaccgccatcgctgtcgctgctgctggtgctgctgggactgggcggaagaagactgcgtgcggagcctggagatggagcccaaacatgggccagattcagcagacctcccgctcctgaagccgccggcttgtttcagggaacctttcctgacggtttcctgtgggctgtgggcagcgccgcctatcagaccgagggcggctggcaacagcacggaaaaggagccagcatctgggataccttcacccaccaccccctggccccccccggcgattcccgcaatgccagcctccctctgggagcccctagccccctgcaacctgccacaggagacgtggcctcagacagctataacaacgtgttccgcgacaccgaggcactgcgcgagctgggcgtgacccattaccgctttagcatcagctgggccagagtgctgcccaatggctctgccggcgtgcccaaccgggagggcctgaggtactaccgccgcctgctggagaggctgcgggagctgggcgtgcagcccgtggtaaccctgtaccactgggacctgccccagcgcctgcaggacgcttacggcggctgggccaaccgcgctctcgcagaccacttccgcgactacgccgagctgtgctttcgccactttggcggccaggtgaagtattggatcaccatcgataacccttacgtggtggcctggcacggatacgctacaggccgcctggcccccggcatccgcggcagccccagactgggctacctggtggcccacaacctgctgctggcccacgccaaggtgtggcacctgtacaacaccagcttccgccccacccagggtggacaggtctctattgccctgagctctcactggattaaccccaggaggatgaccgatcacagcatcaaggaatgccagaagagcctggacttcgttctgggctggttcgccaagcccgtgtttatcgacggcgactaccccgagagcatgaagaacaacctgtctagcatcctgcccgacttcaccgagagcgaaaaaaaattcatcaagggcaccgccgatttcttcgccctgtgtttcggcccaaccctgagcttccaactgctggatccccacatgaagttcagacaactcgagagtcccaacctgcgccagctgctgagctggatcgatctggaattcaaccacccccagatattcatagtggagaacggctggtttgtaagcggcactactaagcgcgatgatgcaaagtacatgtactatctgaagaagttcatcatggaaaccctgaaggccatcaagctggatggcgtggacgtgatcggatacaccgcatggagcctgatggacggcttcgagtggcaccgcggttactcaatccgcagggggttgttctacgtcgacttcctgagtcaggacaagatgttgctgccaaagagtagcgcccttttctaccagaagttgattgagaagaacggcttcccaccactccccgagaaccagcccctggagggcacctttccctgcgatttcgcttggggcgtggtggataattatattcaggtggacaccaccctgtcacagttcactgacctgaacgtgtacctgtgggacgtgcaccattccaagcgcctgatcaaggtggacggcgtggtgaccaagaagcgcaaatcctactgcgttgactttgccgccattcagccacagatcgccctgctgcaggagatgcacgtcacccacttccgcttcagcctggactgggccctcatcctgccactgggcaaccagtcccaggtgaaccacaccattctgcagtactaccgctgtatggccagcgagctggtacgcgtgaacatcacccccgtggtggccctgtggcagcccatggcccccaaccagggcctgccacgcctgctggccaggcagggggcctgggagaacccctacaccgcactcgctttcgccgaatatgccaggctgtgcttccaggagctggggcaccacgtgaagctctggatcaccatgaacgaaccctacaccagaaacatgacctactctgccggacacaatctgctgaaggcccacgccctggcctggcacgtctacaacgagaagttccgccacgcccaaaatggaaagatctctatagccctgcaggccgattggatcgagcccgcctgccccttctcacagaaggacaaggaggtggccgagcgcgtgctggagttcgacatcggctggctggccgagcccatcttcggcagcggagactacccctgggtgatgcgcgattggcttaaccagcgcaacaactttctgctgccctacttcaccgaggacgagaagaagctgatccagggcaccttcgacttcctggccctgagccactatactaccatcctggtcgacagcgagaaggaggacccaatcaagtacaacgactacctggaggtgcaggagatgaccgacatcacctggctgaacagccctagccaggtcgccgtggtgccttggggcctgcgcaaggtgctgaactggctgaagttcaagtatggcgacctgccaatgtacatcatcagcaacggcattgatgacggcctgcacgccgaggacgatcagctgagagtgtactatatgcagaactacatcaacgaggcactgaaggcccacatcctggacggcatcaacctgtgtggctactttgcatactccttcaacgacagaaccgccccccgcttcggcctgtacaggtacgctgccgatcagttcgagcccaaggccagcatgaagcactacagaaaaatcattgatagcaacgggttcccaggccccgagaccctggagcgcttctgccccgaggagttcaccgtgtgcaccgagtgcagttttttccacacccgcaagagcctgctggctttcattgcttttctgttttttgcttccattatttctctctccctcatcttttactacagcaagaaaggaagaagaagctacaaatgagctggagcctcggtggccatgcttcttgccccttgggcctccccccagcccctcctccccttcctgcacccgtacccccgtggtctttgaataaagtctgagtgggcggcaaaaaaaaaaaaaaaaaaaaaaaaaaaaaaaaaaaaaaaaaaaaaaaaaaaaaaaaaaaaaaaaaaaaaaaaaaaaaaaaaaaaaaaaaaaaaaaaaaaaaaaaaaaaaaaaaaaaaaaaa

SEQ ID NO: 74 - RNA, 3342 nt, synthetic construct
  source 1..3342: mol_type = other RNA
gggagacataaaccctggcgcgctcgcggcccggcactcttctggtccccacagactcagagagaacccaccatgcccgctagcgccccaccgagaagaccgcggccgccaccgccatcgctgtcgctgctgctggtgctgctgggactgggcggaagaagactgcgtgcggagcctggcgacggggcccagacctgggccagattcagcagaccccccgcacccgaggccgccggcctgttccagggcaccttccccgacggatttctgtgggccgtgggaagcgctgcctaccagaccgagggcggctggcaacagcacggcaagggcgccagcatctgggacaccttcacccaccatcctctggctcctcccggagacagcagaaacgccagcctgcctctgggagcccccagccccctgcagcccgccactggagacgtggccagcgactcctacaacaacgtgttccgcgacaccgaggccctgcgcgagctgggcgtgacccactaccgctttagcatcagctgggccagagtgctgcccaacggcagcgccggcgtgcccaaccgggaaggcctgagatactatcgccgcctgctggagaggctgagagagttgggcgtgcagcccgtggtgaccctgtaccactgggacctgccccagcgcctgcaggacgcctacggcggctgggccaacagggcactcgccgaccacttccgcgactacgccgagctgtgcttccgccacttcggcgggcaggtgaagtactggatcaccatcgacaacccctacgtggtggcctggcacggctacgctacaggaaggctggcccccgggatccgcggcagccccaggctgggctacctggtggcccacaacctgctgctggcacacgccaaagtgtggcacctgtataacaccagctttcgccccacccagggtggacaggtgagcattgccctgagttctcattggatcaaccccaggcgcatgaccgatcacagcatcaaggaatgccagaagagcctggacttcgtgctgggctggttcgccaagcccgtgtttatcgacggcgactaccccgagtctatgaagaacaacctcagcagcatcctgcctgacgtcaccgagagcgagaagaagttcatcaagggcaccgccgacttcttcgccctgagcttcggccccaccctgagcttccagctgctggatccccatatgaagttcagacaactcgagagtcctaacctgcgccagctgctgagctggatcgacctggaattcaaccacccacagatcttcatcgtggagaacggctggtttgtgagcggcaccactaagcgcgacgacgcaaagtatatgtattatctgaagaaattcatcatggaaaccctgaaggccatcaagctggacggcgtggacgtgatcggatacaccgcatggagcctgatggacggcttcgagtggcaccgcggttacagcatccgccggggcctgttctacgttgacttcctgagccaggacaagatgttgctgcccaagagctccgccctgttctaccagaagttgatcgagaagaacggcttcccaccactccccgagaaccagcccctggagggcaccttcccctgcgatttcgcctggggcgtggtggacaactacatccaggtggacaccaccctgagtcagttcactgacctgaacgtgtacctttgggacgtgcaccacagcaagcgcctgataaaggtcgacggcgtggtgaccaagaagcgcaaaagctactgcgtggactttgccgccatccagccccagatcgccctgctgcaggagatgcacgtgactcacttccgcttcagcctcgactgggccctgattctgcccctgggcaaccagtcacaagtgaaccacaccattctgcagtactaccgctgtatggccagcgagctggtacgcgtgaacatcacccccgttgtggccctttggcagcccatggcccccaaccagggcctgcctcgcctgctggcccgccagggagcctgggagaatccctacaccgcactggccttcgctgaatacgcccgcctgtgcttccaggagctggggcaccacgtgaaactctggatcaccatgaacgagccctacaccagaaacatgacctacagcgccggacacaatctgctgaaggcccacgctctggcctggcacgtgtacaacgagaagtttcgccacgcccagaacggcaagatcagcatcgccctgcaggccgattggatcgagcccgcctgccccttcagccagaaggacaaggaggtggctgagcgggtgctggagttcgacatcgggtggctggctgagcctatcttcggcagcggagactacccctgggtgatgcgcgattggcttaaccagaggaacaatttcctgctgccctacttcaccgaggacgagaagaagctgatccagggcacctttgacttcctggctttgagccactataccactatcctggtggacagcgagaaggaggaccccatcaagtacaacgactacttggaggtgcaggagatgaccgacatcacctggctgaacagccctagccaggtggctgtggtgccttggggcctgcgcaaggtgctgaactggctgaagttcaagtacggcgacctgcccatgtatatcatcagcaacggcatcgacgacggcctgcacgccgaggacgaccagctgagagtgtactacatgcagaactacatcaacgaggccctcaaggcccacatcctggacggcatcaacctgtgtggctactttgcctacagcttcaacgacagaaccgccccccgcttcggcctgtacaggtacgccgccgaccagttcgaacccaaggccagcatgaagcactaccgcaaaatcatcgacagcaacggattccctggacccgagacactggagcgcttctgcccagaggagttcaccgtgtgcaccgagtgcagtttcttccacacccgcaagagcctgctggctttcattgcttttctgttttttgcttccattatttctctctccctcatcttttactacagcaagaaaggaagaagaagctacaaatgagctggagcctcggtggccatgcttcttgccccttgggcctccccccagcccctcctccccttcctgcacccgtacccccgtggtctttgaataaagtctgagtgggcggcaaaaaaaaaaaaaaaaaaaaaaaaaaaaaaaaaaaaaaaaaaaaaaaaaaaaaaaaaaaaaaaaaaaaaaaaaaaaaaaaaaaaaaaaaaaaaaaaaaaaaaaaaaaaaaaaaaaaaaaaa

SEQ ID NO: 75 - RNA, 3342 nt, synthetic construct
  source 1..3342: mol_type = other RNA
gggagacataaaccctggcgcgctcgcggcccggcactcttctggtccccacagactcagagagaacccaccatgcccgctagcgccccaccgagaagaccgcggccgccaccgccatcgctgtcgctgctgctggtgctgctgggactgggcggaagaagactgcgtgcggagcctggagatggagcccaaacatgggccagattcagcagacctcccgctcctgaagccgccggcttgtttcagggaacctttcctgacggtttcctgtgggctgtgggcagcgccgcctatcagaccgagggcggctggcaacagcacggaaaaggagccagcatctgggataccttcacccaccaccccctggccccccccggcgattcccgcaatgccagcctccctctgggagcccctagccccctgcaacctgccacaggagacgtggcctcagacagctataacaacgtgttccgcgacaccgaggcactgcgcgagctgggcgtgacccattaccgctttagcatcagctgggccagagtgctgcccaatggctctgccggcgtgcccaaccgggagggcctgaggtactaccgccgcctgctggagaggctgcgggagctgggcgtgcagcccgtggtaaccctgtaccactgggacctgccccagcgcctgcaggacgcttacggcggctgggccaaccgcgctctcgcagaccacttccgcgactacgccgagctgtgctttcgccactttggcggccaggtgaagtattggatcaccatcgataacccttacgtggtggcctggcacggatacgctacaggccgcctggcccccggcatccgcggcagccccagactgggctacctggtggcccacaacctgctgctggcccacgccaaggtgtggcacctgtacaacaccagcttccgccccacccagggtggacaggtctctattgccctgagctctcactggattaaccccaggaggatgaccgatcacagcatcaaggaatgccagaagagcctggacttcgttctgggctggttcgccaagcccgtgtttatcgacggcgactaccccgagagcatgaagaacaacctgtctagcatcctgcccgacgtcaccgagagcgaaaaaaaattcatcaagggcaccgccgatttcttcgccctgagcttcggcccaaccctgagcttccaactgctggatccccacatgaagttcagacaactcgagagtcccaacctgcgccagctgctgagctggatcgatctggaattcaaccacccccagatattcatagtggagaacggctggtttgtaagcggcactactaagcgcgatgatgcaaagtacatgtactatctgaagaagttcatcatggaaaccctgaaggccatcaagctggatggcgtggacgtgatcggatacaccgcatggagcctgatggacggcttcgagtggcaccgcggttactcaatccgcagggggttgttctacgtcgacttcctgagtcaggacaagatgttgctgccaaagagtagcgcccttttctaccagaagttgattgagaagaacggcttcccaccactccccgagaaccagcccctggagggcacctttccctgcgatttcgcttggggcgtggtggataattatattcaggtggacaccaccctgtcacagttcactgacctgaacgtgtacctgtgggacgtgcaccattccaagcgcctgatcaaggtggacggcgtggtgaccaagaagcgcaaatcctactgcgttgactttgccgccattcagccacagatcgccctgctgcaggagatgcacgtcacccacttccgcttcagcctggactgggccctcatcctgccactgggcaaccagtcccaggtgaaccacaccattctgcagtactaccgctgtatggccagcgagctggtacgcgtgaacatcacccccgtggtggccctgtggcagcccatggcccccaaccagggcctgccacgcctgctggccaggcagggggcctgggagaacccctacaccgcactcgctttcgccgaatatgccaggctgtgcttccaggagctggggcaccacgtgaagctctggatcaccatgaacgaaccctacaccagaaacatgacctactctgccggacacaatctgctgaaggcccacgccctggcctggcacgtctacaacgagaagttccgccacgcccaaaatggaaagatctctatagccctgcaggccgattggatcgagcccgcctgccccttctcacagaaggacaaggaggtggccgagcgcgtgctggagttcgacatcggctggctggccgagcccatcttcggcagcggagactacccctgggtgatgcgcgattggcttaaccagcgcaacaactttctgctgccctacttcaccgaggacgagaagaagctgatccagggcaccttcgacttcctggccctgagccactatactaccatcctggtcgacagcgagaaggaggacccaatcaagtacaacgactacctggaggtgcaggagatgaccgacatcacctggctgaacagccctagccaggtcgccgtggtgccttggggcctgcgcaaggtgctgaactggctgaagttcaagtatggcgacctgccaatgtacatcatcagcaacggcattgatgacggcctgcacgccgaggacgatcagctgagagtgtactatatgcagaactacatcaacgaggcactgaaggcccacatcctggacggcatcaacctgtgtggctactttgcatactccttcaacgacagaaccgccccccgcttcggcctgtacaggtacgctgccgatcagttcgagcccaaggccagcatgaagcactacagaaaaatcattgatagcaacgggttcccaggccccgagaccctggagcgcttctgccccgaggagttcaccgtgtgcaccgagtgcagttttttccacacccgcaagagcctgctggctttcattgcttttctgttttttgcttccattatttctctctccctcatcttttactacagcaagaaaggaagaagaagctacaaatgagctggagcctcggtggccatgcttcttgccccttgggcctccccccagcccctcctccccttcctgcacccgtacccccgtggtctttgaataaagtctgagtgggcggcaaaaaaaaaaaaaaaaaaaaaaaaaaaaaaaaaaaaaaaaaaaaaaaaaaaaaaaaaaaaaaaaaaaaaaaaaaaaaaaaaaaaaaaaaaaaaaaaaaaaaaaaaaaaaaaaaaaaaaaaa

SEQ ID NO: 76 - protein, 1012 aa, synthetic construct
MPASAPPRRPRPPPPSLSLLLVLLGLGGRRLRAEPGDGAQTWARFSRPPAPEAAGLFQGTFPDGFLWAVGSAAYQTEGGWQQHGKGASIWDTFTHHPLAPPGDSRNASLPLGAPSPLQPATGDVASDSYNNVFRDTEALRELGVTHYRFSISWARVLPNGSAGVPNREGLRYYRRLLERLRELGVQPVVTLYHWDLPQRLQDAYGGWANRALADHFRDYAELCFRHFGGQVKYWITIDNPYVVAWHGYATGRLAPGIRGSPRLGYLVAHNLLLAHAKVWHLYNTSFRPTQGGQVSIALSSHWINPRRMTDHSIKECQKSLDFVLGWFAKPVFIDGDYPESMKNNLSSILPDVTESEKKFIKGTADFFALSFGPTLSFQLLDPHMKFRQLESPNLRQLLSWIDLEFNHPQIFIVENGWFVSGTTKRDDAKYMYYLKKFIMETLKAIKLDGVDVIGYTAWSLMDGFEWHRGYSIRRGLFYVDFLSQDKMLLPKSSALFYQKLIEKNGFPPLPENQPLEGTFPCDFAWGVVDNYIQVDTTLSQFTDLNVYLWDVHHSKRLIKVDGVVTKKRKSYCVDFAAIQPQIALLQEMHVTHFRFSLDWALILPLGNQSQVNHTILQYYRCMASELVRVNITPVVALWQPMAPNQGLPRLLARQGAWENPYTALAFAEYARLCFQELGHHVKLWITMNEPYTRNMTYSAGHNLLKAHALAWHVYNEKFRHAQNGKISIALQADWIEPACPFSQKDKEVAERVLEFDIGWLAEPIFGSGDYPWVMRDWLNQRNNFLLPYFTEDEKKLIQGTFDFLALSHYTTILVDSEKEDPIKYNDYLEVQEMTDITWLNSPSQVAVVPWGLRKVLNWLKFKYGDLPMYIISNGIDDGLHAEDDQLRVYYMQNYINEALKAHILDGINLCGYFAYSFNDRTAPRFGLYRYAADQFEPKASMKHYRKIIDSNGFPGPETLERFCPEEFTVCTECSFFHTRKSLLAFIAFLFFASIISLSLIFYYSKKGRRSYK

SEQ ID NO: 77 - DNA, 28 bp, synthetic construct
  source 1..28: mol_type = other DNA
tgctgccgtaatacgactcactataagg

SEQ ID NO: 78 - DNA, 143 bp, synthetic construct
  source 1..143: mol_type = other DNA
tttttttttttttttttttttttttttttttttttttttttttttttttttttttttttttttttttttttttttttttttttttttttttttttttttttttttttttttttttttttttgccgcccactcagactttattc

SEQ ID NO: 79 - RNA, 1353 nt, synthetic construct
  source 1..1353: mol_type = other RNA
ctgttccagggcaccttccccgacggatttctgtgggccgtgggaagcgctgcctaccagaccgagggcggctggcaacagcacggcaagggcgccagcatctgggacaccttcacccaccatcctctggctcctcccggagacagcagaaacgccagcctgcctctgggagcccccagccccctgcagcccgccactggagacgtggccagcgactcctacaacaacgtgttccgcgacaccgaggccctgcgcgagctgggcgtgacccactaccgctttagcatcagctgggccagagtgctgcccaacggcagcgccggcgtgcccaaccgggaaggcctgagatactatcgccgcctgctggagaggctgagagagttgggcgtgcagcccgtggtgaccctgtaccactgggatctgccccagcgcctgcaggacgcctacggcggctgggccaacagggcactcgccgaccacttccgcgactacgccgagctgtgcttccgccacttcggcggccaggtgaagtactggatcaccatcgacaacccctacgtggtggcctggcacggctacgctacaggaaggctggcccccgggatccgcggcagccccaggctgggctacctggtggcccacaatctgctgctggcacacgccaaagtgtggcacctgtataacaccagctttcgccccacccagggtggacaggtgagcattgccctgagttctcattggatcaaccccaggcgcatgaccgatcacagcatcaaggaatgccagaagagcctggacttcgtgctgggctggttcgccaagcccgtgtttatcgacggcgactaccccgagtctatgaagaacaacctcagcagcatcctgcctgacttcaccgagagcgagaagaagttcatcaagggcaccgccgacttcttcgccctgtgcttcggccccaccctgagcttccagctgctggatccccatatgaagttcagacaactcgagagtcctaatctgcgccagctgctgagctggatcgacctggaattcaaccacccacagatcttcatcgtggagaacggctggtttgtgagcggcaccactaagcgcgacgacgcaaagtatatgtattatctgaagaaattcatcatggaaaccctgaaggccatcaagctggacggcgtggacgtgatcggatacaccgcatggagcctgatggacggcttcgagtggcaccgcggttacagcatccgccggggcctgttctacgttgacttcctgagccaggacaagatgttgctgcccaagagctccgccctgttctaccagaagttgatcgagaagaacggcttc

SEQ ID NO: 80 - RNA, 1353 nt, synthetic construct
  source 1..1353: mol_type = other RNA
ttgtttcagggaacctttcctgacggtttcctgtgggctgtgggcagcgccgcctatcagaccgagggcggctggcaacagcacggaaaaggagccagcatctgggataccttcacccaccaccccctggccccccccggcgattcccgcaatgccagcctccctctgggagcccctagccccctgcagcctgccacaggagacgtggcctcagacagctataacaacgtgttccgcgacaccgaggcactgcgcgagctgggcgtgacccattaccgctttagcatcagctgggccagagtgctgcccaatggctctgccggcgtgcccaaccgggagggcctgaggtactaccgccgcctgctggagaggctgcgggagctgggcgtgcagcccgtggtaaccctgtaccactgggatctgccccagcgcctgcaggacgcttacggcggctgggccaaccgcgctctcgcagaccacttccgcgactacgccgagctgtgctttcgccactttggcggccaggtgaagtattggatcaccatcgataacccttacgtggtggcctggcacggatacgctacaggccgcctggcccccggcatccgcggcagccccagactgggctacctggtggcccacaatctgctgctggcccacgccaaggtgtggcacctgtacaacaccagcttccgccccacccagggtggacaggtctctattgccctgagctctcactggattaaccccaggaggatgaccgatcacagcatcaaggaatgccagaagagcctggacttcgttctgggctggttcgccaagcccgtgtttatcgacggcgactaccccgagagcatgaagaacaacctgtctagcatcctgcccgacttcaccgagagcgaaaaaaaattcatcaagggcaccgccgatttcttcgccctgtgtttcggcccaaccctgagcttccaactgctggatccccacatgaagttcagacaactcgagagtcccaatctgcgccagctgctgagctggatcgatctggaattcaaccacccccagatattcatagtggagaacggctggtttgtaagcggcactactaagcgcgatgatgcaaagtacatgtactatctgaagaagttcatcatggaaaccctgaaggccatcaagctggatggcgtggacgtgatcggatacaccgcatggagcctgatggacggcttcgagtggcaccgcggttactcaatccgcagggggttgttctacgtcgacttcctgagtcaggacaagatgttgctgccaaagagtagcgcccttttctaccagaagttgattgagaagaacggcttc

SEQ ID NO: 81 - RNA, 1353 nt, synthetic construct
  source 1..1353: mol_type = other RNA
ctgttccagggcaccttccccgacggatttctgtgggccgtgggaagcgctgcctaccagaccgagggcggctggcaacagcacggcaagggcgccagcatctgggacaccttcacccaccatcctctggctcctcccggagacagcagaaacgccagcctgcctctgggagcccccagccccctgcagcccgccactggagacgtggccagcgactcctacaacaacgtgttccgcgacaccgaggccctgcgcgagctgggcgtgacccactaccgctttagcatcagctgggccagagtgctgcccaacggcagcgccggcgtgcccaaccgggaaggcctgagatactatcgccgcctgctggagaggctgagagagttgggcgtgcagcccgtggtgaccctgtaccactgggatctgccccagcgcctgcaggacgcctacggcggctgggccaacagggcactcgccgaccacttccgcgactacgccgagctgtgcttccgccacttcggcggccaggtgaagtactggatcaccatcgacaacccctacgtggtggcctggcacggctacgctacaggaaggctggcccccgggatccgcggcagccccaggctgggctacctggtggcccacaatctgctgctggcacacgccaaagtgtggcacctgtataacaccagctttcgccccacccagggtggacaggtgagcattgccctgagttctcattggatcaaccccaggcgcatgaccgatcacagcatcaaggaatgccagaagagcctggacttcgtgctgggctggttcgccaagcccgtgtttatcgacggcgactaccccgagtctatgaagaacaacctcagcagcatcctgcctgacgtcaccgagagcgagaagaagttcatcaagggcaccgccgacttcttcgccctgagcttcggccccaccctgagcttccagctgctggatccccatatgaagttcagacaactcgagagtcctaatctgcgccagctgctgagctggatcgacctggaattcaaccacccacagatcttcatcgtggagaacggctggtttgtgagcggcaccactaagcgcgacgacgcaaagtatatgtattatctgaagaaattcatcatggaaaccctgaaggccatcaagctggacggcgtggacgtgatcggatacaccgcatggagcctgatggacggcttcgagtggcaccgcggttacagcatccgccggggcctgttctacgttgacttcctgagccaggacaagatgttgctgcccaagagctccgccctgttctaccagaagttgatcgagaagaacggcttc

SEQ ID NO: 82 - RNA, 1353 nt, synthetic construct
  source 1..1353: mol_type = other RNA
ttgtttcagggaacctttcctgacggtttcctgtgggctgtgggcagcgccgcctatcagaccgagggcggctggcaacagcacggaaaaggagccagcatctgggataccttcacccaccaccccctggccccccccggcgattcccgcaatgccagcctccctctgggagcccctagccccctgcagcctgccacaggagacgtggcctcagacagctataacaacgtgttccgcgacaccgaggcactgcgcgagctgggcgtgacccattaccgctttagcatcagctgggccagagtgctgcccaatggctctgccggcgtgcccaaccgggagggcctgaggtactaccgccgcctgctggagaggctgcgggagctgggcgtgcagcccgtggtaaccctgtaccactgggatctgccccagcgcctgcaggacgcttacggcggctgggccaaccgcgctctcgcagaccacttccgcgactacgccgagctgtgctttcgccactttggcggccaggtgaagtattggatcaccatcgataacccttacgtggtggcctggcacggatacgctacaggccgcctggcccccggcatccgcggcagccccagactgggctacctggtggcccacaatctgctgctggcccacgccaaggtgtggcacctgtacaacaccagcttccgccccacccagggtggacaggtctctattgccctgagctctcactggattaaccccaggaggatgaccgatcacagcatcaaggaatgccagaagagcctggacttcgttctgggctggttcgccaagcccgtgtttatcgacggcgactaccccgagagcatgaagaacaacctgtctagcatcctgcccgacgtcaccgagagcgaaaaaaaattcatcaagggcaccgccgatttcttcgccctgagcttcggcccaaccctgagcttccaactgctggatccccacatgaagttcagacaactcgagagtcccaatctgcgccagctgctgagctggatcgatctggaattcaaccacccccagatattcatagtggagaacggctggtttgtaagcggcactactaagcgcgatgatgcaaagtacatgtactatctgaagaagttcatcatggaaaccctgaaggccatcaagctggatggcgtggacgtgatcggatacaccgcatggagcctgatggacggcttcgagtggcaccgcggttactcaatccgcagggggttgttctacgtcgacttcctgagtcaggacaagatgttgctgccaaagagtagcgcccttttctaccagaagttgattgagaagaacggcttc

SEQ ID NO: 83 - RNA, 1521 nt, synthetic construct
  source 1..1521: mol_type = other RNA
atgcccgctagcgccccaccgagaagaccgcggccgccaccgccatcgctgtcgctgctgctggtgctgctgggactgggcggaagaagactgcgtgcggagcctggcgacggggcccagacctgggccagattcagcagaccccccgcacccgaggccgccggcctgttccagggcaccttccccgacggatttctgtgggccgtgggaagcgctgcctaccagaccgagggcggctggcaacagcacggcaagggcgccagcatctgggacaccttcacccaccatcctctggctcctcccggagacagcagaaacgccagcctgcctctgggagcccccagccccctgcagcccgccactggagacgtggccagcgactcctacaacaacgtgttccgcgacaccgaggccctgcgcgagctgggcgtgacccactaccgctttagcatcagctgggccagagtgctgcccaacggcagcgccggcgtgcccaaccgggaaggcctgagatactatcgccgcctgctggagaggctgagagagttgggcgtgcagcccgtggtgaccctgtaccactgggatctgccccagcgcctgcaggacgcctacggcggctgggccaacagggcactcgccgaccacttccgcgactacgccgagctgtgcttccgccacttcggcggccaggtgaagtactggatcaccatcgacaacccctacgtggtggcctggcacggctacgctacaggaaggctggcccccgggatccgcggcagccccaggctgggctacctggtggcccacaatctgctgctggcacacgccaaagtgtggcacctgtataacaccagctttcgccccacccagggtggacaggtgagcattgccctgagttctcattggatcaaccccaggcgcatgaccgatcacagcatcaaggaatgccagaagagcctggacttcgtgctgggctggttcgccaagcccgtgtttatcgacggcgactaccccgagtctatgaagaacaacctcagcagcatcctgcctgacttcaccgagagcgagaagaagttcatcaagggcaccgccgacttcttcgccctgtgcttcggccccaccctgagcttccagctgctggatccccatatgaagttcagacaactcgagagtcctaatctgcgccagctgctgagctggatcgacctggaattcaaccacccacagatcttcatcgtggagaacggctggtttgtgagcggcaccactaagcgcgacgacgcaaagtatatgtattatctgaagaaattcatcatggaaaccctgaaggccatcaagctggacggcgtggacgtgatcggatacaccgcatggagcctgatggacggcttcgagtggcaccgcggttacagcatccgccggggcctgttctacgttgacttcctgagccaggacaagatgttgctgcccaagagctccgccctgttctaccagaagttgatcgagaagaacggcttctga

SEQ ID NO: 84 - RNA, 1521 nt, synthetic construct
  source 1..1521: mol_type = other RNA
atgcccgctagcgccccaccgagaagaccgcggccgccaccgccatcgctgtcgctgctgctggtgctgctgggactgggcggaagaagactgcgtgcggagcctggagatggagcccaaacatgggccagattcagcagacctcccgctcctgaagccgccggcttgtttcagggaacctttcctgacggtttcctgtgggctgtgggcagcgccgcctatcagaccgagggcggctggcaacagcacggaaaaggagccagcatctgggataccttcacccaccaccccctggccccccccggcgattcccgcaatgccagcctccctctgggagcccctagccccctgcagcctgccacaggagacgtggcctcagacagctataacaacgtgttccgcgacaccgaggcactgcgcgagctgggcgtgacccattaccgctttagcatcagctgggccagagtgctgcccaatggctctgccggcgtgcccaaccgggagggcctgaggtactaccgccgcctgctggagaggctgcgggagctgggcgtgcagcccgtggtaaccctgtaccactgggatctgccccagcgcctgcaggacgcttacggcggctgggccaaccgcgctctcgcagaccacttccgcgactacgccgagctgtgctttcgccactttggcggccaggtgaagtattggatcaccatcgataacccttacgtggtggcctggcacggatacgctacaggccgcctggcccccggcatccgcggcagccccagactgggctacctggtggcccacaatctgctgctggcccacgccaaggtgtggcacctgtacaacaccagcttccgccccacccagggtggacaggtctctattgccctgagctctcactggattaaccccaggaggatgaccgatcacagcatcaaggaatgccagaagagcctggacttcgttctgggctggttcgccaagcccgtgtttatcgacggcgactaccccgagagcatgaagaacaacctgtctagcatcctgcccgacttcaccgagagcgaaaaaaaattcatcaagggcaccgccgatttcttcgccctgtgtttcggcccaaccctgagcttccaactgctggatccccacatgaagttcagacaactcgagagtcccaatctgcgccagctgctgagctggatcgatctggaattcaaccacccccagatattcatagtggagaacggctggtttgtaagcggcactactaagcgcgatgatgcaaagtacatgtactatctgaagaagttcatcatggaaaccctgaaggccatcaagctggatggcgtggacgtgatcggatacaccgcatggagcctgatggacggcttcgagtggcaccgcggttactcaatccgcagggggttgttctacgtcgacttcctgagtcaggacaagatgttgctgccaaagagtagcgcccttttctaccagaagttgattgagaagaacggcttctga

SEQ ID NO: 85 - RNA, 1521 nt, synthetic construct
  source 1..1521: mol_type = other RNA
atgcccgctagcgccccaccgagaagaccgcggccgccaccgccatcgctgtcgctgctgctggtgctgctgggactgggcggaagaagactgcgtgcggagcctggcgacggggcccagacctgggccagattcagcagaccccccgcacccgaggccgccggcctgttccagggcaccttccccgacggatttctgtgggccgtgggaagcgctgcctaccagaccgagggcggctggcaacagcacggcaagggcgccagcatctgggacaccttcacccaccatcctctggctcctcccggagacagcagaaacgccagcctgcctctgggagcccccagccccctgcagcccgccactggagacgtggccagcgactcctacaacaacgtgttccgcgacaccgaggccctgcgcgagctgggcgtgacccactaccgctttagcatcagctgggccagagtgctgcccaacggcagcgccggcgtgcccaaccgggaaggcctgagatactatcgccgcctgctggagaggctgagagagttgggcgtgcagcccgtggtgaccctgtaccactgggatctgccccagcgcctgcaggacgcctacggcggctgggccaacagggcactcgccgaccacttccgcgactacgccgagctgtgcttccgccacttcggcggccaggtgaagtactggatcaccatcgacaacccctacgtggtggcctggcacggctacgctacaggaaggctggcccccgggatccgcggcagccccaggctgggctacctggtggcccacaatctgctgctggcacacgccaaagtgtggcacctgtataacaccagctttcgccccacccagggtggacaggtgagcattgccctgagttctcattggatcaaccccaggcgcatgaccgatcacagcatcaaggaatgccagaagagcctggacttcgtgctgggctggttcgccaagcccgtgtttatcgacggcgactaccccgagtctatgaagaacaacctcagcagcatcctgcctgacgtcaccgagagcgagaagaagttcatcaagggcaccgccgacttcttcgccctgagcttcggccccaccctgagcttccagctgctggatccccatatgaagttcagacaactcgagagtcctaatctgcgccagctgctgagctggatcgacctggaattcaaccacccacagatcttcatcgtggagaacggctggtttgtgagcggcaccactaagcgcgacgacgcaaagtatatgtattatctgaagaaattcatcatggaaaccctgaaggccatcaagctggacggcgtggacgtgatcggatacaccgcatggagcctgatggacggcttcgagtggcaccgcggttacagcatccgccggggcctgttctacgttgacttcctgagccaggacaagatgttgctgcccaagagctccgccctgttctaccagaagttgatcgagaagaacggcttctga

SEQ ID NO: 86 - RNA, 1521 nt, synthetic construct
  source 1..1521: mol_type = other RNA
atgcccgctagcgccccaccgagaagaccgcggccgccaccgccatcgctgtcgctgctgctggtgctgctgggactgggcggaagaagactgcgtgcggagcctggagatggagcccaaacatgggccagattcagcagacctcccgctcctgaagccgccggcttgtttcagggaacctttcctgacggtttcctgtgggctgtgggcagcgccgcctatcagaccgagggcggctggcaacagcacggaaaaggagccagcatctgggataccttcacccaccaccccctggccccccccggcgattcccgcaatgccagcctccctctgggagcccctagccccctgcagcctgccacaggagacgtggcctcagacagctataacaacgtgttccgcgacaccgaggcactgcgcgagctgggcgtgacccattaccgctttagcatcagctgggccagagtgctgcccaatggctctgccggcgtgcccaaccgggagggcctgaggtactaccgccgcctgctggagaggctgcgggagctgggcgtgcagcccgtggtaaccctgtaccactgggatctgccccagcgcctgcaggacgcttacggcggctgggccaaccgcgctctcgcagaccacttccgcgactacgccgagctgtgctttcgccactttggcggccaggtgaagtattggatcaccatcgataacccttacgtggtggcctggcacggatacgctacaggccgcctggcccccggcatccgcggcagccccagactgggctacctggtggcccacaatctgctgctggcccacgccaaggtgtggcacctgtacaacaccagcttccgccccacccagggtggacaggtctctattgccctgagctctcactggattaaccccaggaggatgaccgatcacagcatcaaggaatgccagaagagcctggacttcgttctgggctggttcgccaagcccgtgtttatcgacggcgactaccccgagagcatgaagaacaacctgtctagcatcctgcccgacgtcaccgagagcgaaaaaaaattcatcaagggcaccgccgatttcttcgccctgagcttcggcccaaccctgagcttccaactgctggatccccacatgaagttcagacaactcgagagtcccaatctgcgccagctgctgagctggatcgatctggaattcaaccacccccagatattcatagtggagaacggctggtttgtaagcggcactactaagcgcgatgatgcaaagtacatgtactatctgaagaagttcatcatggaaaccctgaaggccatcaagctggatggcgtggacgtgatcggatacaccgcatggagcctgatggacggcttcgagtggcaccgcggttactcaatccgcagggggttgttctacgtcgacttcctgagtcaggacaagatgttgctgccaaagagtagcgcccttttctaccagaagttgattgagaagaacggcttctga

SEQ ID NO: 87 - RNA, 2691 nt, synthetic construct
  source 1..2691: mol_type = other RNA
ctgttccagggcaccttccccgacggatttctgtgggccgtgggaagcgctgcctaccagaccgagggcggctggcaacagcacggcaagggcgccagcatctgggacaccttcacccaccatcctctggctcctcccggagacagcagaaacgccagcctgcctctgggagcccccagccccctgcagcccgccactggagacgtggccagcgactcctacaacaacgtgttccgcgacaccgaggccctgcgcgagctgggcgtgacccactaccgctttagcatcagctgggccagagtgctgcccaacggcagcgccggcgtgcccaaccgggaaggcctgagatactatcgccgcctgctggagaggctgagagagttgggcgtgcagcccgtggtgaccctgtaccactgggatctgccccagcgcctgcaggacgcctacggcggctgggccaacagggcactcgccgaccacttccgcgactacgccgagctgtgcttccgccacttcggcggccaggtgaagtactggatcaccatcgacaacccctacgtggtggcctggcacggctacgctacaggaaggctggcccccgggatccgcggcagccccaggctgggctacctggtggcccacaatctgctgctggcacacgccaaagtgtggcacctgtataacaccagctttcgccccacccagggtggacaggtgagcattgccctgagttctcattggatcaaccccaggcgcatgaccgatcacagcatcaaggaatgccagaagagcctggacttcgtgctgggctggttcgccaagcccgtgtttatcgacggcgactaccccgagtctatgaagaacaacctcagcagcatcctgcctgacttcaccgagagcgagaagaagttcatcaagggcaccgccgacttcttcgccctgtgcttcggccccaccctgagcttccagctgctggatccccatatgaagttcagacaactcgagagtcctaatctgcgccagctgctgagctggatcgacctggaattcaaccacccacagatcttcatcgtggagaacggctggtttgtgagcggcaccactaagcgcgacgacgcaaagtatatgtattatctgaagaaattcatcatggaaaccctgaaggccatcaagctggacggcgtggacgtgatcggatacaccgcatggagcctgatggacggcttcgagtggcaccgcggttacagcatccgccggggcctgttctacgttgacttcctgagccaggacaagatgttgctgcccaagagctccgccctgttctaccagaagttgatcgagaagaacggcttcccaccactccccgagaaccagcccctggagggcaccttcccctgcgatttcgcctggggcgtggtggacaactacatccaggtggacaccaccctgagtcagttcactgacctgaacgtgtacctttgggacgtgcaccacagcaagcgcctgataaaggtcgacggcgtggtgaccaagaagcgcaaaagctactgcgtggactttgccgccatccagccccagatcgccctgctgcaggagatgcacgtgactcacttccgcttcagcctcgactgggccctgattctgcccctgggcaaccagtcacaagtgaaccacaccattctgcagtactaccgctgtatggccagcgagctggtacgcgtgaacatcacccccgttgtggccctttggcagcccatggcccccaaccagggcctgcctcgcctgctggcccgccagggagcctgggagaatccctacaccgcactggccttcgctgaatacgcccgcctgtgcttccaggagctggggcaccacgtgaaactctggatcaccatgaacgagccctacaccagaaacatgacctacagcgccggacacaatctgctgaaggcccacgctctggcctggcacgtgtacaacgagaagtttcgccacgcccagaacggcaagatcagcatcgccctgcaggccgattggatcgagcccgcctgccccttcagccagaaggacaaggaggtggctgagcgggtgctggagttcgacatcgggtggctggctgagcctatcttcggcagcggagactacccctgggtgatgcgcgattggcttaaccagaggaacaatttcctgctgccctacttcaccgaggacgagaagaagctgatccagggcacctttgacttcctggctttgagccactataccactatcctggtggacagcgagaaggaggaccccatcaagtacaacgactacttggaggtgcaggagatgaccgacatcacctggctgaacagccctagccaggtggctgtggtgccttggggcctgcgcaaggtgctgaactggctgaagttcaagtacggcgatctgcccatgtatatcatcagcaacggcatcgacgacggcctgcacgccgaggacgaccagctgagagtgtactacatgcagaactacatcaacgaggccctcaaggcccacatcctggacggcatcaacctgtgtggctactttgcctacagcttcaacgacagaaccgccccccgcttcggcctgtacaggtacgccgccgaccagttcgaacccaaggccagcatgaagcactaccgcaaaatcatcgacagcaacgga

SEQ ID NO: 88 - RNA, 2691 nt, synthetic construct
  source 1..2691: mol_type = other RNA
ttgtttcagggaacctttcctgacggtttcctgtgggctgtgggcagcgccgcctatcagaccgagggcggctggcaacagcacggaaaaggagccagcatctgggataccttcacccaccaccccctggccccccccggcgattcccgcaatgccagcctccctctgggagcccctagccccctgcagcctgccacaggagacgtggcctcagacagctataacaacgtgttccgcgacaccgaggcactgcgcgagctgggcgtgacccattaccgctttagcatcagctgggccagagtgctgcccaatggctctgccggcgtgcccaaccgggagggcctgaggtactaccgccgcctgctggagaggctgcgggagctgggcgtgcagcccgtggtaaccctgtaccactgggatctgccccagcgcctgcaggacgcttacggcggctgggccaaccgcgctctcgcagaccacttccgcgactacgccgagctgtgctttcgccactttggcggccaggtgaagtattggatcaccatcgataacccttacgtggtggcctggcacggatacgctacaggccgcctggcccccggcatccgcggcagccccagactgggctacctggtggcccacaatctgctgctggcccacgccaaggtgtggcacctgtacaacaccagcttccgccccacccagggtggacaggtctctattgccctgagctctcactggattaaccccaggaggatgaccgatcacagcatcaaggaatgccagaagagcctggacttcgttctgggctggttcgccaagcccgtgtttatcgacggcgactaccccgagagcatgaagaacaacctgtctagcatcctgcccgacttcaccgagagcgaaaaaaaattcatcaagggcaccgccgatttcttcgccctgtgtttcggcccaaccctgagcttccaactgctggatccccacatgaagttcagacaactcgagagtcccaatctgcgccagctgctgagctggatcgatctggaattcaaccacccccagatattcatagtggagaacggctggtttgtaagcggcactactaagcgcgatgatgcaaagtacatgtactatctgaagaagttcatcatggaaaccctgaaggccatcaagctggatggcgtggacgtgatcggatacaccgcatggagcctgatggacggcttcgagtggcaccgcggttactcaatccgcagggggttgttctacgtcgacttcctgagtcaggacaagatgttgctgccaaagagtagcgcccttttctaccagaagttgattgagaagaacggcttcccaccactccccgagaaccagcccctggagggcacctttccctgcgatttcgcttggggcgtggtggataattatattcaggtggacaccaccctgtcacagttcactgacctgaacgtgtacctgtgggacgtgcaccattccaagcgcctgatcaaggtggacggcgtggtgaccaagaagcgcaaatcctactgcgttgactttgccgccattcagccacagatcgccctgctgcaggagatgcacgtcacccacttccgcttcagcctggactgggccctcatcctgccactgggcaaccagtcccaggtgaaccacaccattctgcagtactaccgctgtatggccagcgagctggtacgcgtgaacatcacccccgtggtggccctgtggcagcccatggcccccaaccagggcctgccacgcctgctggccaggcagggggcctgggagaacccctacaccgcactcgctttcgccgaatatgccaggctgtgcttccaggagctggggcaccacgtgaagctctggatcaccatgaacgaaccctacaccagaaacatgacctactctgccggacacaatctgctgaaggcccacgccctggcctggcacgtctacaacgagaagttccgccacgcccaaaatggaaagatctctatagccctgcaggccgattggatcgagcccgcctgccccttctcacagaaggacaaggaggtggccgagcgcgtgctggagttcgacatcggctggctggccgagcccatcttcggcagcggagactacccctgggtgatgcgcgattggcttaaccagcgcaacaactttctgctgccctacttcaccgaggacgagaagaagctgatccagggcaccttcgacttcctggccctgagccactatactaccatcctggtcgacagcgagaaggaggacccaatcaagtacaacgactacctggaggtgcaggagatgaccgacatcacctggctgaacagccctagccaggtcgccgtggtgccttggggcctgcgcaaggtgctgaactggctgaagttcaagtatggcgatctgccaatgtacatcatcagcaacggcattgatgacggcctgcacgccgaggacgatcagctgagagtgtactatatgcagaactacatcaacgaggcactgaaggcccacatcctggacggcatcaacctgtgtggctactttgcatactccttcaacgacagaaccgccccccgcttcggcctgtacaggtacgctgccgatcagttcgagcccaaggccagcatgaagcactacagaaaaatcattgatagcaacggg

SEQ ID NO: 89 - RNA, 2691 nt, synthetic construct
  source 1..2691: mol_type = other RNA
ctgttccagggcaccttccccgacggatttctgtgggccgtgggaagcgctgcctaccagaccgagggcggctggcaacagcacggcaagggcgccagcatctgggacaccttcacccaccatcctctggctcctcccggagacagcagaaacgccagcctgcctctgggagcccccagccccctgcagcccgccactggagacgtggccagcgactcctacaacaacgtgttccgcgacaccgaggccctgcgcgagctgggcgtgacccactaccgctttagcatcagctgggccagagtgctgcccaacggcagcgccggcgtgcccaaccgggaaggcctgagatactatcgccgcctgctggagaggctgagagagttgggcgtgcagcccgtggtgaccctgtaccactgggatctgccccagcgcctgcaggacgcctacggcggctgggccaacagggcactcgccgaccacttccgcgactacgccgagctgtgcttccgccacttcggcggccaggtgaagtactggatcaccatcgacaacccctacgtggtggcctggcacggctacgctacaggaaggctggcccccgggatccgcggcagccccaggctgggctacctggtggcccacaatctgctgctggcacacgccaaagtgtggcacctgtataacaccagctttcgccccacccagggtggacaggtgagcattgccctgagttctcattggatcaaccccaggcgcatgaccgatcacagcatcaaggaatgccagaagagcctggacttcgtgctgggctggttcgccaagcccgtgtttatcgacggcgactaccccgagtctatgaagaacaacctcagcagcatcctgcctgacgtcaccgagagcgagaagaagttcatcaagggcaccgccgacttcttcgccctgagcttcggccccaccctgagcttccagctgctggatccccatatgaagttcagacaactcgagagtcctaatctgcgccagctgctgagctggatcgacctggaattcaaccacccacagatcttcatcgtggagaacggctggtttgtgagcggcaccactaagcgcgacgacgcaaagtatatgtattatctgaagaaattcatcatggaaaccctgaaggccatcaagctggacggcgtggacgtgatcggatacaccgcatggagcctgatggacggcttcgagtggcaccgcggttacagcatccgccggggcctgttctacgttgacttcctgagccaggacaagatgttgctgcccaagagctccgccctgttctaccagaagttgatcgagaagaacggcttcccaccactccccgagaaccagcccctggagggcaccttcccctgcgatttcgcctggggcgtggtggacaactacatccaggtggacaccaccctgagtcagttcactgacctgaacgtgtacctttgggacgtgcaccacagcaagcgcctgataaaggtcgacggcgtggtgaccaagaagcgcaaaagctactgcgtggactttgccgccatccagccccagatcgccctgctgcaggagatgcacgtgactcacttccgcttcagcctcgactgggccctgattctgcccctgggcaaccagtcacaagtgaaccacaccattctgcagtactaccgctgtatggccagcgagctggtacgcgtgaacatcacccccgttgtggccctttggcagcccatggcccccaaccagggcctgcctcgcctgctggcccgccagggagcctgggagaatccctacaccgcactggccttcgctgaatacgcccgcctgtgcttccaggagctggggcaccacgtgaaactctggatcaccatgaacgagccctacaccagaaacatgacctacagcgccggacacaatctgctgaaggcccacgctctggcctggcacgtgtacaacgagaagtttcgccacgcccagaacggcaagatcagcatcgccctgcaggccgattggatcgagcccgcctgccccttcagccagaaggacaaggaggtggctgagcgggtgctggagttcgacatcgggtggctggctgagcctatcttcggcagcggagactacccctgggtgatgcgcgattggcttaaccagaggaacaatttcctgctgccctacttcaccgaggacgagaagaagctgatccagggcacctttgacttcctggctttgagccactataccactatcctggtggacagcgagaaggaggaccccatcaagtacaacgactacttggaggtgcaggagatgaccgacatcacctggctgaacagccctagccaggtggctgtggtgccttggggcctgcgcaaggtgctgaactggctgaagttcaagtacggcgatctgcccatgtatatcatcagcaacggcatcgacgacggcctgcacgccgaggacgaccagctgagagtgtactacatgcagaactacatcaacgaggccctcaaggcccacatcctggacggcatcaacctgtgtggctactttgcctacagcttcaacgacagaaccgccccccgcttcggcctgtacaggtacgccgccgaccagttcgaacccaaggccagcatgaagcactaccgcaaaatcatcgacagcaacgga

SEQ ID NO: 90 - RNA, 2691 nt, synthetic construct
  source 1..2691: mol_type = other RNA
ttgtttcagggaacctttcctgacggtttcctgtgggctgtgggcagcgccgcctatcagaccgagggcggctggcaacagcacggaaaaggagccagcatctgggataccttcacccaccaccccctggccccccccggcgattcccgcaatgccagcctccctctgggagcccctagccccctgcagcctgccacaggagacgtggcctcagacagctataacaacgtgttccgcgacaccgaggcactgcgcgagctgggcgtgacccattaccgctttagcatcagctgggccagagtgctgcccaatggctctgccggcgtgcccaaccgggagggcctgaggtactaccgccgcctgctggagaggctgcgggagctgggcgtgcagcccgtggtaaccctgtaccactgggatctgccccagcgcctgcaggacgcttacggcggctgggccaaccgcgctctcgcagaccacttccgcgactacgccgagctgtgctttcgccactttggcggccaggtgaagtattggatcaccatcgataacccttacgtggtggcctggcacggatacgctacaggccgcctggcccccggcatccgcggcagccccagactgggctacctggtggcccacaatctgctgctggcccacgccaaggtgtggcacctgtacaacaccagcttccgccccacccagggtggacaggtctctattgccctgagctctcactggattaaccccaggaggatgaccgatcacagcatcaaggaatgccagaagagcctggacttcgttctgggctggttcgccaagcccgtgtttatcgacggcgactaccccgagagcatgaagaacaacctgtctagcatcctgcccgacgtcaccgagagcgaaaaaaaattcatcaagggcaccgccgatttcttcgccctgagcttcggcccaaccctgagcttccaactgctggatccccacatgaagttcagacaactcgagagtcccaatctgcgccagctgctgagctggatcgatctggaattcaaccacccccagatattcatagtggagaacggctggtttgtaagcggcactactaagcgcgatgatgcaaagtacatgtactatctgaagaagttcatcatggaaaccctgaaggccatcaagctggatggcgtggacgtgatcggatacaccgcatggagcctgatggacggcttcgagtggcaccgcggttactcaatccgcagggggttgttctacgtcgacttcctgagtcaggacaagatgttgctgccaaagagtagcgcccttttctaccagaagttgattgagaagaacggcttcccaccactccccgagaaccagcccctggagggcacctttccctgcgatttcgcttggggcgtggtggataattatattcaggtggacaccaccctgtcacagttcactgacctgaacgtgtacctgtgggacgtgcaccattccaagcgcctgatcaaggtggacggcgtggtgaccaagaagcgcaaatcctactgcgttgactttgccgccattcagccacagatcgccctgctgcaggagatgcacgtcacccacttccgcttcagcctggactgggccctcatcctgccactgggcaaccagtcccaggtgaaccacaccattctgcagtactaccgctgtatggccagcgagctggtacgcgtgaacatcacccccgtggtggccctgtggcagcccatggcccccaaccagggcctgccacgcctgctggccaggcagggggcctgggagaacccctacaccgcactcgctttcgccgaatatgccaggctgtgcttccaggagctggggcaccacgtgaagctctggatcaccatgaacgaaccctacaccagaaacatgacctactctgccggacacaatctgctgaaggcccacgccctggcctggcacgtctacaacgagaagttccgccacgcccaaaatggaaagatctctatagccctgcaggccgattggatcgagcccgcctgccccttctcacagaaggacaaggaggtggccgagcgcgtgctggagttcgacatcggctggctggccgagcccatcttcggcagcggagactacccctgggtgatgcgcgattggcttaaccagcgcaacaactttctgctgccctacttcaccgaggacgagaagaagctgatccagggcaccttcgacttcctggccctgagccactatactaccatcctggtcgacagcgagaaggaggacccaatcaagtacaacgactacctggaggtgcaggagatgaccgacatcacctggctgaacagccctagccaggtcgccgtggtgccttggggcctgcgcaaggtgctgaactggctgaagttcaagtatggcgatctgccaatgtacatcatcagcaacggcattgatgacggcctgcacgccgaggacgatcagctgagagtgtactatatgcagaactacatcaacgaggcactgaaggcccacatcctggacggcatcaacctgtgtggctactttgcatactccttcaacgacagaaccgccccccgcttcggcctgtacaggtacgctgccgatcagttcgagcccaaggccagcatgaagcactacagaaaaatcattgatagcaacggg

SEQ ID NO: 91 - RNA, 2844 nt, synthetic construct
  source 1..2844: mol_type = other RNA
gagcctggcgacggggcccagacctgggccagattcagcagaccccccgcacccgaggccgccggcctgttccagggcaccttccccgacggatttctgtgggccgtgggaagcgctgcctaccagaccgagggcggctggcaacagcacggcaagggcgccagcatctgggacaccttcacccaccatcctctggctcctcccggagacagcagaaacgccagcctgcctctgggagcccccagccccctgcagcccgccactggagacgtggccagcgactcctacaacaacgtgttccgcgacaccgaggccctgcgcgagctgggcgtgacccactaccgctttagcatcagctgggccagagtgctgcccaacggcagcgccggcgtgcccaaccgggaaggcctgagatactatcgccgcctgctggagaggctgagagagttgggcgtgcagcccgtggtgaccctgtaccactgggatctgccccagcgcctgcaggacgcctacggcggctgggccaacagggcactcgccgaccacttccgcgactacgccgagctgtgcttccgccacttcggcggccaggtgaagtactggatcaccatcgacaacccctacgtggtggcctggcacggctacgctacaggaaggctggcccccgggatccgcggcagccccaggctgggctacctggtggcccacaatctgctgctggcacacgccaaagtgtggcacctgtataacaccagctttcgccccacccagggtggacaggtgagcattgccctgagttctcattggatcaaccccaggcgcatgaccgatcacagcatcaaggaatgccagaagagcctggacttcgtgctgggctggttcgccaagcccgtgtttatcgacggcgactaccccgagtctatgaagaacaacctcagcagcatcctgcctgacttcaccgagagcgagaagaagttcatcaagggcaccgccgacttcttcgccctgtgcttcggccccaccctgagcttccagctgctggatccccatatgaagttcagacaactcgagagtcctaatctgcgccagctgctgagctggatcgacctggaattcaaccacccacagatcttcatcgtggagaacggctggtttgtgagcggcaccactaagcgcgacgacgcaaagtatatgtattatctgaagaaattcatcatggaaaccctgaaggccatcaagctggacggcgtggacgtgatcggatacaccgcatggagcctgatggacggcttcgagtggcaccgcggttacagcatccgccggggcctgttctacgttgacttcctgagccaggacaagatgttgctgcccaagagctccgccctgttctaccagaagttgatcgagaagaacggcttcccaccactccccgagaaccagcccctggagggcaccttcccctgcgatttcgcctggggcgtggtggacaactacatccaggtggacaccaccctgagtcagttcactgacctgaacgtgtacctttgggacgtgcaccacagcaagcgcctgataaaggtcgacggcgtggtgaccaagaagcgcaaaagctactgcgtggactttgccgccatccagccccagatcgccctgctgcaggagatgcacgtgactcacttccgcttcagcctcgactgggccctgattctgcccctgggcaaccagtcacaagtgaaccacaccattctgcagtactaccgctgtatggccagcgagctggtacgcgtgaacatcacccccgttgtggccctttggcagcccatggcccccaaccagggcctgcctcgcctgctggcccgccagggagcctgggagaatccctacaccgcactggccttcgctgaatacgcccgcctgtgcttccaggagctggggcaccacgtgaaactctggatcaccatgaacgagccctacaccagaaacatgacctacagcgccggacacaatctgctgaaggcccacgctctggcctggcacgtgtacaacgagaagtttcgccacgcccagaacggcaagatcagcatcgccctgcaggccgattggatcgagcccgcctgccccttcagccagaaggacaaggaggtggctgagcgggtgctggagttcgacatcgggtggctggctgagcctatcttcggcagcggagactacccctgggtgatgcgcgattggcttaaccagaggaacaatttcctgctgccctacttcaccgaggacgagaagaagctgatccagggcacctttgacttcctggctttgagccactataccactatcctggtggacagcgagaaggaggaccccatcaagtacaacgactacttggaggtgcaggagatgaccgacatcacctggctgaacagccctagccaggtggctgtggtgccttggggcctgcgcaaggtgctgaactggctgaagttcaagtacggcgatctgcccatgtatatcatcagcaacggcatcgacgacggcctgcacgccgaggacgaccagctgagagtgtactacatgcagaactacatcaacgaggccctcaaggcccacatcctggacggcatcaacctgtgtggctactttgcctacagcttcaacgacagaaccgccccccgcttcggcctgtacaggtacgccgccgaccagttcgaacccaaggccagcatgaagcactaccgcaaaatcatcgacagcaacggattccctggacccgagacactggagcgcttctgcccagaggagttcaccgtgtgcaccgagtgcagtttcttccacacccgcaagagc

SEQ ID NO: 92 - RNA, 2844 nt, synthetic construct
  source 1..2844: mol_type = other RNA
gagcctggagatggagcccaaacatgggccagattcagcagacctcccgctcctgaagccgccggcttgtttcagggaacctttcctgacggtttcctgtgggctgtgggcagcgccgcctatcagaccgagggcggctggcaacagcacggaaaaggagccagcatctgggataccttcacccaccaccccctggccccccccggcgattcccgcaatgccagcctccctctgggagcccctagccccctgcagcctgccacaggagacgtggcctcagacagctataacaacgtgttccgcgacaccgaggcactgcgcgagctgggcgtgacccattaccgctttagcatcagctgggccagagtgctgcccaatggctctgccggcgtgcccaaccgggagggcctgaggtactaccgccgcctgctggagaggctgcgggagctgggcgtgcagcccgtggtaaccctgtaccactgggatctgccccagcgcctgcaggacgcttacggcggctgggccaaccgcgctctcgcagaccacttccgcgactacgccgagctgtgctttcgccactttggcggccaggtgaagtattggatcaccatcgataacccttacgtggtggcctggcacggatacgctacaggccgcctggcccccggcatccgcggcagccccagactgggctacctggtggcccacaatctgctgctggcccacgccaaggtgtggcacctgtacaacaccagcttccgccccacccagggtggacaggtctctattgccctgagctctcactggattaaccccaggaggatgaccgatcacagcatcaaggaatgccagaagagcctggacttcgttctgggctggttcgccaagcccgtgtttatcgacggcgactaccccgagagcatgaagaacaacctgtctagcatcctgcccgacttcaccgagagcgaaaaaaaattcatcaagggcaccgccgatttcttcgccctgtgtttcggcccaaccctgagcttccaactgctggatccccacatgaagttcagacaactcgagagtcccaatctgcgccagctgctgagctggatcgatctggaattcaaccacccccagatattcatagtggagaacggctggtttgtaagcggcactactaagcgcgatgatgcaaagtacatgtactatctgaagaagttcatcatggaaaccctgaaggccatcaagctggatggcgtggacgtgatcggatacaccgcatggagcctgatggacggcttcgagtggcaccgcggttactcaatccgcagggggttgttctacgtcgacttcctgagtcaggacaagatgttgctgccaaagagtagcgcccttttctaccagaagttgattgagaagaacggcttcccaccactccccgagaaccagcccctggagggcacctttccctgcgatttcgcttggggcgtggtggataattatattcaggtggacaccaccctgtcacagttcactgacctgaacgtgtacctgtgggacgtgcaccattccaagcgcctgatcaaggtggacggcgtggtgaccaagaagcgcaaatcctactgcgttgactttgccgccattcagccacagatcgccctgctgcaggagatgcacgtcacccacttccgcttcagcctggactgggccctcatcctgccactgggcaaccagtcccaggtgaaccacaccattctgcagtactaccgctgtatggccagcgagctggtacgcgtgaacatcacccccgtggtggccctgtggcagcccatggcccccaaccagggcctgccacgcctgctggccaggcagggggcctgggagaacccctacaccgcactcgctttcgccgaatatgccaggctgtgcttccaggagctggggcaccacgtgaagctctggatcaccatgaacgaaccctacaccagaaacatgacctactctgccggacacaatctgctgaaggcccacgccctggcctggcacgtctacaacgagaagttccgccacgcccaaaatggaaagatctctatagccctgcaggccgattggatcgagcccgcctgccccttctcacagaaggacaaggaggtggccgagcgcgtgctggagttcgacatcggctggctggccgagcccatcttcggcagcggagactacccctgggtgatgcgcgattggcttaaccagcgcaacaactttctgctgccctacttcaccgaggacgagaagaagctgatccagggcaccttcgacttcctggccctgagccactatactaccatcctggtcgacagcgagaaggaggacccaatcaagtacaacgactacctggaggtgcaggagatgaccgacatcacctggctgaacagccctagccaggtcgccgtggtgccttggggcctgcgcaaggtgctgaactggctgaagttcaagtatggcgatctgccaatgtacatcatcagcaacggcattgatgacggcctgcacgccgaggacgatcagctgagagtgtactatatgcagaactacatcaacgaggcactgaaggcccacatcctggacggcatcaacctgtgtggctactttgcatactccttcaacgacagaaccgccccccgcttcggcctgtacaggtacgctgccgatcagttcgagcccaaggccagcatgaagcactacagaaaaatcattgatagcaacgggttcccaggccccgagaccctggagcgcttctgccccgaggagttcaccgtgtgcaccgagtgcagttttttccacacccgcaagagc

SEQ ID NO: 93 - RNA, 2844 nt, synthetic construct
  source 1..2844: mol_type = other RNA
gagcctggcgacggggcccagacctgggccagattcagcagaccccccgcacccgaggccgccggcctgttccagggcaccttccccgacggatttctgtgggccgtgggaagcgctgcctaccagaccgagggcggctggcaacagcacggcaagggcgccagcatctgggacaccttcacccaccatcctctggctcctcccggagacagcagaaacgccagcctgcctctgggagcccccagccccctgcagcccgccactggagacgtggccagcgactcctacaacaacgtgttccgcgacaccgaggccctgcgcgagctgggcgtgacccactaccgctttagcatcagctgggccagagtgctgcccaacggcagcgccggcgtgcccaaccgggaaggcctgagatactatcgccgcctgctggagaggctgagagagttgggcgtgcagcccgtggtgaccctgtaccactgggatctgccccagcgcctgcaggacgcctacggcggctgggccaacagggcactcgccgaccacttccgcgactacgccgagctgtgcttccgccacttcggcggccaggtgaagtactggatcaccatcgacaacccctacgtggtggcctggcacggctacgctacaggaaggctggcccccgggatccgcggcagccccaggctgggctacctggtggcccacaatctgctgctggcacacgccaaagtgtggcacctgtataacaccagctttcgccccacccagggtggacaggtgagcattgccctgagttctcattggatcaaccccaggcgcatgaccgatcacagcatcaaggaatgccagaagagcctggacttcgtgctgggctggttcgccaagcccgtgtttatcgacggcgactaccccgagtctatgaagaacaacctcagcagcatcctgcctgacgtcaccgagagcgagaagaagttcatcaagggcaccgccgacttcttcgccctgagcttcggccccaccctgagcttccagctgctggatccccatatgaagttcagacaactcgagagtcctaatctgcgccagctgctgagctggatcgacctggaattcaaccacccacagatcttcatcgtggagaacggctggtttgtgagcggcaccactaagcgcgacgacgcaaagtatatgtattatctgaagaaattcatcatggaaaccctgaaggccatcaagctggacggcgtggacgtgatcggatacaccgcatggagcctgatggacggcttcgagtggcaccgcggttacagcatccgccggggcctgttctacgttgacttcctgagccaggacaagatgttgctgcccaagagctccgccctgttctaccagaagttgatcgagaagaacggcttcccaccactccccgagaaccagcccctggagggcaccttcccctgcgatttcgcctggggcgtggtggacaactacatccaggtggacaccaccctgagtcagttcactgacctgaacgtgtacctttgggacgtgcaccacagcaagcgcctgataaaggtcgacggcgtggtgaccaagaagcgcaaaagctactgcgtggactttgccgccatccagccccagatcgccctgctgcaggagatgcacgtgactcacttccgcttcagcctcgactgggccctgattctgcccctgggcaaccagtcacaagtgaaccacaccattctgcagtactaccgctgtatggccagcgagctggtacgcgtgaacatcacccccgttgtggccctttggcagcccatggcccccaaccagggcctgcctcgcctgctggcccgccagggagcctgggagaatccctacaccgcactggccttcgctgaatacgcccgcctgtgcttccaggagctggggcaccacgtgaaactctggatcaccatgaacgagccctacaccagaaacatgacctacagcgccggacacaatctgctgaaggcccacgctctggcctggcacgtgtacaacgagaagtttcgccacgcccagaacggcaagatcagcatcgccctgcaggccgattggatcgagcccgcctgccccttcagccagaaggacaaggaggtggctgagcgggtgctggagttcgacatcgggtggctggctgagcctatcttcggcagcggagactacccctgggtgatgcgcgattggcttaaccagaggaacaatttcctgctgccctacttcaccgaggacgagaagaagctgatccagggcacctttgacttcctggctttgagccactataccactatcctggtggacagcgagaaggaggaccccatcaagtacaacgactacttggaggtgcaggagatgaccgacatcacctggctgaacagccctagccaggtggctgtggtgccttggggcctgcgcaaggtgctgaactggctgaagttcaagtacggcgatctgcccatgtatatcatcagcaacggcatcgacgacggcctgcacgccgaggacgaccagctgagagtgtactacatgcagaactacatcaacgaggccctcaaggcccacatcctggacggcatcaacctgtgtggctactttgcctacagcttcaacgacagaaccgccccccgcttcggcctgtacaggtacgccgccgaccagttcgaacccaaggccagcatgaagcactaccgcaaaatcatcgacagcaacggattccctggacccgagacactggagcgcttctgcccagaggagttcaccgtgtgcaccgagtgcagtttcttccacacccgcaagagc

SEQ ID NO: 94 - RNA, 2844 nt, synthetic construct
  source 1..2844: mol_type = other RNA
gagcctggagatggagcccaaacatgggccagattcagcagacctcccgctcctgaagccgccggcttgtttcagggaacctttcctgacggtttcctgtgggctgtgggcagcgccgcctatcagaccgagggcggctggcaacagcacggaaaaggagccagcatctgggataccttcacccaccaccccctggccccccccggcgattcccgcaatgccagcctccctctgggagcccctagccccctgcagcctgccacaggagacgtggcctcagacagctataacaacgtgttccgcgacaccgaggcactgcgcgagctgggcgtgacccattaccgctttagcatcagctgggccagagtgctgcccaatggctctgccggcgtgcccaaccgggagggcctgaggtactaccgccgcctgctggagaggctgcgggagctgggcgtgcagcccgtggtaaccctgtaccactgggatctgccccagcgcctgcaggacgcttacggcggctgggccaaccgcgctctcgcagaccacttccgcgactacgccgagctgtgctttcgccactttggcggccaggtgaagtattggatcaccatcgataacccttacgtggtggcctggcacggatacgctacaggccgcctggcccccggcatccgcggcagccccagactgggctacctggtggcccacaatctgctgctggcccacgccaaggtgtggcacctgtacaacaccagcttccgccccacccagggtggacaggtctctattgccctgagctctcactggattaaccccaggaggatgaccgatcacagcatcaaggaatgccagaagagcctggacttcgttctgggctggttcgccaagcccgtgtttatcgacggcgactaccccgagagcatgaagaacaacctgtctagcatcctgcccgacgtcaccgagagcgaaaaaaaattcatcaagggcaccgccgatttcttcgccctgagcttcggcccaaccctgagcttccaactgctggatccccacatgaagttcagacaactcgagagtcccaatctgcgccagctgctgagctggatcgatctggaattcaaccacccccagatattcatagtggagaacggctggtttgtaagcggcactactaagcgcgatgatgcaaagtacatgtactatctgaagaagttcatcatggaaaccctgaaggccatcaagctggatggcgtggacgtgatcggatacaccgcatggagcctgatggacggcttcgagtggcaccgcggttactcaatccgcagggggttgttctacgtcgacttcctgagtcaggacaagatgttgctgccaaagagtagcgcccttttctaccagaagttgattgagaagaacggcttcccaccactccccgagaaccagcccctggagggcacctttccctgcgatttcgcttggggcgtggtggataattatattcaggtggacaccaccctgtcacagttcactgacctgaacgtgtacctgtgggacgtgcaccattccaagcgcctgatcaaggtggacggcgtggtgaccaagaagcgcaaatcctactgcgttgactttgccgccattcagccacagatcgccctgctgcaggagatgcacgtcacccacttccgcttcagcctggactgggccctcatcctgccactgggcaaccagtcccaggtgaaccacaccattctgcagtactaccgctgtatggccagcgagctggtacgcgtgaacatcacccccgtggtggccctgtggcagcccatggcccccaaccagggcctgccacgcctgctggccaggcagggggcctgggagaacccctacaccgcactcgctttcgccgaatatgccaggctgtgcttccaggagctggggcaccacgtgaagctctggatcaccatgaacgaaccctacaccagaaacatgacctactctgccggacacaatctgctgaaggcccacgccctggcctggcacgtctacaacgagaagttccgccacgcccaaaatggaaagatctctatagccctgcaggccgattggatcgagcccgcctgccccttctcacagaaggacaaggaggtggccgagcgcgtgctggagttcgacatcggctggctggccgagcccatcttcggcagcggagactacccctgggtgatgcgcgattggcttaaccagcgcaacaactttctgctgccctacttcaccgaggacgagaagaagctgatccagggcaccttcgacttcctggccctgagccactatactaccatcctggtcgacagcgagaaggaggacccaatcaagtacaacgactacctggaggtgcaggagatgaccgacatcacctggctgaacagccctagccaggtcgccgtggtgccttggggcctgcgcaaggtgctgaactggctgaagttcaagtatggcgatctgccaatgtacatcatcagcaacggcattgatgacggcctgcacgccgaggacgatcagctgagagtgtactatatgcagaactacatcaacgaggcactgaaggcccacatcctggacggcatcaacctgtgtggctactttgcatactccttcaacgacagaaccgccccccgcttcggcctgtacaggtacgctgccgatcagttcgagcccaaggccagcatgaagcactacagaaaaatcattgatagcaacgggttcccaggccccgagaccctggagcgcttctgccccgaggagttcaccgtgtgcaccgagtgcagttttttccacacccgcaagagc

SEQ ID NO: 95 - RNA, 2946 nt, synthetic construct
  source 1..2946: mol_type = other RNA
atgcccgccagcgccccgccgcgccgcccgcggccgccgccgccgtcgctgtcgctgctgctggtgctgctgggcctgggcggccgccgcctgcgtgcggagccgggcgacggcgcgcagacctgggcccgtttctcgcggcctcctgcccccgaggccgcgggcctcttccagggcaccttccccgacggcttcctctgggccgtgggcagcgccgcctaccagaccgagggcggctggcagcagcacggcaagggtgcgtccatctgggacacgttcacccaccaccccctggcacccccgggagactcccggaacgccagtctgccgttgggcgccccgtcgccgctgcagcccgccaccggggacgtagccagcgacagctacaacaacgtcttccgcgacacggaggcgctgcgcgagctcggggtcactcactaccgcttctccatctcgtgggcgcgagtgctccccaatggcagcgcgggcgtccccaaccgcgaggggctgcgctactaccggcgcctgctggagcggctgcgggagctgggcgtgcagcccgtggtcaccctgtaccactgggatctgccccagcgcctgcaggacgcctacggcggctgggccaaccgcgccctggccgaccacttcagggattacgcggagctctgcttccgccacttcggcggtcaggtcaagtactggatcaccatcgacaacccctacgtggtggcctggcacggctacgccaccgggcgcctggcccccggcatccggggcagcccgcggctcgggtacctggtggcgcacaacctcctcctggctcatgccaaagtctggcatctctacaatacttctttccgtcccactcagggaggtcaggtgtccattgccctaagctctcactggatcaatcctcgaagaatgaccgaccacagcatcaaagaatgtcaaaaatctctggactttgtactaggttggtttgccaaacccgtatttattgatggtgactatcccgagagcatgaagaataacctttcatctattctgcctgattttactgaatctgagaaaaagttcatcaaaggaactgctgacttttttgctctttgctttggacccaccttgagttttcaacttttggaccctcacatgaagttccgccaattggaatctcccaacctgaggcaactgctttcctggattgaccttgaatttaaccatcctcaaatatttattgtggaaaatggctggtttgtctcagggaccaccaagagagatgatgccaaatatatgtattacctcaaaaagttcatcatggaaaccttaaaagccatcaagctggatggggtggatgtcatcgggtataccgcatggtccctcatggatggtttcgagtggcacagaggttacagcatcaggcgtggactcttctatgttgactttctaagccaggacaagatgttgttgccaaagtcttcagccttgttctaccaaaagctgatagagaaaaatggcttccctcctttacctgaaaatcagcccctagaagggacatttccctgtgactttgcttggggagttgttgacaactacattcaagtagataccactctgtctcagtttaccgacctgaatgtttacctgtgggatgtccaccacagtaaaaggcttattaaagtggatggggttgtgaccaagaagaggaaatcctactgtgttgactttgctgccatccagccccagatcgctttactccaggaaatgcacgttacacattttcgcttctccctggactgggccctgattctccctctgggtaaccagtcccaggtgaaccacaccatcctgcagtactatcgctgcatggccagcgagcttgtccgtgtcaacatcaccccagtggtggccctgtggcagcctatggccccgaaccaaggactgccgcgcctcctggccaggcagggcgcctgggagaacccctacactgccctggcctttgcagagtatgcccgactgtgctttcaagagctcggccatcacgtcaagctttggataacgatgaatgagccgtatacaaggaatatgacatacagtgctggccacaaccttctgaaggcccatgccctggcttggcatgtgtacaatgaaaagtttaggcatgctcagaatgggaaaatatccatagccttgcaggctgattggatagaaccagcctgccctttctcccaaaaggacaaagaggtggccgagagagttttggaatttgacattggctggctggctgagcccattttcggctctggagattatccatgggtgatgagggactggctgaaccaaagaaacaattttcttcttccttatttcactgaagatgaaaaaaagctaatccagggtacctttgactttttggctttaagccattataccaccatccttgtagactcagaaaaagaagatccaataaaatacaatgattacctagaagtgcaagaaatgaccgacatcacgtggctcaactcccccagtcaggtggcggtagtgccctgggggttgcgcaaagtgctgaactggctgaagttcaagtacggagacctccccatgtacataatatccaacggaatcgatgacgggctgcatgctgaggacgaccagctgagggtgtattatatgcagaattacataaacgaagctctcaaagcccacatactggatggtatcaatctttgcggatactttgcttattcgtttaacgaccgcacagctccgaggtttggcctctatcgttatgctgcagatcagtttgagcccaaggcatccatgaaacattacaggaaaattattgacagcaatggtttcccgggcccagaaactctggaaagattttgtccagaagaattcaccgtgtgtactgagtgcagtttttttcacacccgaaagtcttga

SEQ ID NO: 96 - RNA, 2946 nt, synthetic construct
  source 1..2946: mol_type = other RNA
atgcccgctagcgccccaccgagaagaccgcggccgccaccgccatcgctgtcgctgctgctggtgctgctgggactgggcggaagaagactgcgtgcggagcctggcgacggggcccagacctgggccagattcagcagaccccccgcacccgaggccgccggcctgttccagggcaccttccccgacggatttctgtgggccgtgggaagcgctgcctaccagaccgagggcggctggcaacagcacggcaagggcgccagcatctgggacaccttcacccaccatcctctggctcctcccggagacagcagaaacgccagcctgcctctgggagcccccagccccctgcagcccgccactggagacgtggccagcgactcctacaacaacgtgttccgcgacaccgaggccctgcgcgagctgggcgtgacccactaccgctttagcatcagctgggccagagtgctgcccaacggcagcgccggcgtgcccaaccgggaaggcctgagatactatcgccgcctgctggagaggctgagagagttgggcgtgcagcccgtggtgaccctgtaccactgggatctgccccagcgcctgcaggacgcctacggcggctgggccaacagggcactcgccgaccacttccgcgactacgccgagctgtgcttccgccacttcggcggccaggtgaagtactggatcaccatcgacaacccctacgtggtggcctggcacggctacgctacaggaaggctggcccccgggatccgcggcagccccaggctgggctacctggtggcccacaatctgctgctggcacacgccaaagtgtggcacctgtataacaccagctttcgccccacccagggtggacaggtgagcattgccctgagttctcattggatcaaccccaggcgcatgaccgatcacagcatcaaggaatgccagaagagcctggacttcgtgctgggctggttcgccaagcccgtgtttatcgacggcgactaccccgagtctatgaagaacaacctcagcagcatcctgcctgacttcaccgagagcgagaagaagttcatcaagggcaccgccgacttcttcgccctgtgcttcggccccaccctgagcttccagctgctggatccccatatgaagttcagacaactcgagagtcctaatctgcgccagctgctgagctggatcgacctggaattcaaccacccacagatcttcatcgtggagaacggctggtttgtgagcggcaccactaagcgcgacgacgcaaagtatatgtattatctgaagaaattcatcatggaaaccctgaaggccatcaagctggacggcgtggacgtgatcggatacaccgcatggagcctgatggacggcttcgagtggcaccgcggttacagcatccgccggggcctgttctacgttgacttcctgagccaggacaagatgttgctgcccaagagctccgccctgttctaccagaagttgatcgagaagaacggcttcccaccactccccgagaaccagcccctggagggcaccttcccctgcgatttcgcctggggcgtggtggacaactacatccaggtggacaccaccctgagtcagttcactgacctgaacgtgtacctttgggacgtgcaccacagcaagcgcctgataaaggtcgacggcgtggtgaccaagaagcgcaaaagctactgcgtggactttgccgccatccagccccagatcgccctgctgcaggagatgcacgtgactcacttccgcttcagcctcgactgggccctgattctgcccctgggcaaccagtcacaagtgaaccacaccattctgcagtactaccgctgtatggccagcgagctggtacgcgtgaacatcacccccgttgtggccctttggcagcccatggcccccaaccagggcctgcctcgcctgctggcccgccagggagcctgggagaatccctacaccgcactggccttcgctgaatacgcccgcctgtgcttccaggagctggggcaccacgtgaaactctggatcaccatgaacgagccctacaccagaaacatgacctacagcgccggacacaatctgctgaaggcccacgctctggcctggcacgtgtacaacgagaagtttcgccacgcccagaacggcaagatcagcatcgccctgcaggccgattggatcgagcccgcctgccccttcagccagaaggacaaggaggtggctgagcgggtgctggagttcgacatcgggtggctggctgagcctatcttcggcagcggagactacccctgggtgatgcgcgattggcttaaccagaggaacaatttcctgctgccctacttcaccgaggacgagaagaagctgatccagggcacctttgacttcctggctttgagccactataccactatcctggtggacagcgagaaggaggaccccatcaagtacaacgactacttggaggtgcaggagatgaccgacatcacctggctgaacagccctagccaggtggctgtggtgccttggggcctgcgcaaggtgctgaactggctgaagttcaagtacggcgatctgcccatgtatatcatcagcaacggcatcgacgacggcctgcacgccgaggacgaccagctgagagtgtactacatgcagaactacatcaacgaggccctcaaggcccacatcctggacggcatcaacctgtgtggctactttgcctacagcttcaacgacagaaccgccccccgcttcggcctgtacaggtacgccgccgaccagttcgaacccaaggccagcatgaagcactaccgcaaaatcatcgacagcaacggattccctggacccgagacactggagcgcttctgcccagaggagttcaccgtgtgcaccgagtgcagtttcttccacacccgcaagagctga

SEQ ID NO: 97 - RNA, 2946 nt, synthetic construct
  source 1..2946: mol_type = other RNA
atgcccgctagcgccccaccgagaagaccgcggccgccaccgccatcgctgtcgctgctgctggtgctgctgggactgggcggaagaagactgcgtgcggagcctggagatggagcccaaacatgggccagattcagcagacctcccgctcctgaagccgccggcttgtttcagggaacctttcctgacggtttcctgtgggctgtgggcagcgccgcctatcagaccgagggcggctggcaacagcacggaaaaggagccagcatctgggataccttcacccaccaccccctggccccccccggcgattcccgcaatgccagcctccctctgggagcccctagccccctgcagcctgccacaggagacgtggcctcagacagctataacaacgtgttccgcgacaccgaggcactgcgcgagctgggcgtgacccattaccgctttagcatcagctgggccagagtgctgcccaatggctctgccggcgtgcccaaccgggagggcctgaggtactaccgccgcctgctggagaggctgcgggagctgggcgtgcagcccgtggtaaccctgtaccactgggatctgccccagcgcctgcaggacgcttacggcggctgggccaaccgcgctctcgcagaccacttccgcgactacgccgagctgtgctttcgccactttggcggccaggtgaagtattggatcaccatcgataacccttacgtggtggcctggcacggatacgctacaggccgcctggcccccggcatccgcggcagccccagactgggctacctggtggcccacaatctgctgctggcccacgccaaggtgtggcacctgtacaacaccagcttccgccccacccagggtggacaggtctctattgccctgagctctcactggattaaccccaggaggatgaccgatcacagcatcaaggaatgccagaagagcctggacttcgttctgggctggttcgccaagcccgtgtttatcgacggcgactaccccgagagcatgaagaacaacctgtctagcatcctgcccgacttcaccgagagcgaaaaaaaattcatcaagggcaccgccgatttcttcgccctgtgtttcggcccaaccctgagcttccaactgctggatccccacatgaagttcagacaactcgagagtcccaatctgcgccagctgctgagctggatcgatctggaattcaaccacccccagatattcatagtggagaacggctggtttgtaagcggcactactaagcgcgatgatgcaaagtacatgtactatctgaagaagttcatcatggaaaccctgaaggccatcaagctggatggcgtggacgtgatcggatacaccgcatggagcctgatggacggcttcgagtggcaccgcggttactcaatccgcagggggttgttctacgtcgacttcctgagtcaggacaagatgttgctgccaaagagtagcgcccttttctaccagaagttgattgagaagaacggcttcccaccactccccgagaaccagcccctggagggcacctttccctgcgatttcgcttggggcgtggtggataattatattcaggtggacaccaccctgtcacagttcactgacctgaacgtgtacctgtgggacgtgcaccattccaagcgcctgatcaaggtggacggcgtggtgaccaagaagcgcaaatcctactgcgttgactttgccgccattcagccacagatcgccctgctgcaggagatgcacgtcacccacttccgcttcagcctggactgggccctcatcctgccactgggcaaccagtcccaggtgaaccacaccattctgcagtactaccgctgtatggccagcgagctggtacgcgtgaacatcacccccgtggtggccctgtggcagcccatggcccccaaccagggcctgccacgcctgctggccaggcagggggcctgggagaacccctacaccgcactcgctttcgccgaatatgccaggctgtgcttccaggagctggggcaccacgtgaagctctggatcaccatgaacgaaccctacaccagaaacatgacctactctgccggacacaatctgctgaaggcccacgccctggcctggcacgtctacaacgagaagttccgccacgcccaaaatggaaagatctctatagccctgcaggccgattggatcgagcccgcctgccccttctcacagaaggacaaggaggtggccgagcgcgtgctggagttcgacatcggctggctggccgagcccatcttcggcagcggagactacccctgggtgatgcgcgattggcttaaccagcgcaacaactttctgctgccctacttcaccgaggacgagaagaagctgatccagggcaccttcgacttcctggccctgagccactatactaccatcctggtcgacagcgagaaggaggacccaatcaagtacaacgactacctggaggtgcaggagatgaccgacatcacctggctgaacagccctagccaggtcgccgtggtgccttggggcctgcgcaaggtgctgaactggctgaagttcaagtatggcgatctgccaatgtacatcatcagcaacggcattgatgacggcctgcacgccgaggacgatcagctgagagtgtactatatgcagaactacatcaacgaggcactgaaggcccacatcctggacggcatcaacctgtgtggctactttgcatactccttcaacgacagaaccgccccccgcttcggcctgtacaggtacgctgccgatcagttcgagcccaaggccagcatgaagcactacagaaaaatcattgatagcaacgggttcccaggccccgagaccctggagcgcttctgccccgaggagttcaccgtgtgcaccgagtgcagttttttccacacccgcaagagctga

SEQ ID NO: 98 - RNA, 2946 nt, synthetic construct
  source 1..2946: mol_type = other RNA
atgcccgctagcgccccaccgagaagaccgcggccgccaccgccatcgctgtcgctgctgctggtgctgctgggactgggcggaagaagactgcgtgcggagcctggcgacggggcccagacctgggccagattcagcagaccccccgcacccgaggccgccggcctgttccagggcaccttccccgacggatttctgtgggccgtgggaagcgctgcctaccagaccgagggcggctggcaacagcacggcaagggcgccagcatctgggacaccttcacccaccatcctctggctcctcccggagacagcagaaacgccagcctgcctctgggagcccccagccccctgcagcccgccactggagacgtggccagcgactcctacaacaacgtgttccgcgacaccgaggccctgcgcgagctgggcgtgacccactaccgctttagcatcagctgggccagagtgctgcccaacggcagcgccggcgtgcccaaccgggaaggcctgagatactatcgccgcctgctggagaggctgagagagttgggcgtgcagcccgtggtgaccctgtaccactgggatctgccccagcgcctgcaggacgcctacggcggctgggccaacagggcactcgccgaccacttccgcgactacgccgagctgtgcttccgccacttcggcggccaggtgaagtactggatcaccatcgacaacccctacgtggtggcctggcacggctacgctacaggaaggctggcccccgggatccgcggcagccccaggctgggctacctggtggcccacaatctgctgctggcacacgccaaagtgtggcacctgtataacaccagctttcgccccacccagggtggacaggtgagcattgccctgagttctcattggatcaaccccaggcgcatgaccgatcacagcatcaaggaatgccagaagagcctggacttcgtgctgggctggttcgccaagcccgtgtttatcgacggcgactaccccgagtctatgaagaacaacctcagcagcatcctgcctgacgtcaccgagagcgagaagaagttcatcaagggcaccgccgacttcttcgccctgagcttcggccccaccctgagcttccagctgctggatccccatatgaagttcagacaactcgagagtcctaatctgcgccagctgctgagctggatcgacctggaattcaaccacccacagatcttcatcgtggagaacggctggtttgtgagcggcaccactaagcgcgacgacgcaaagtatatgtattatctgaagaaattcatcatggaaaccctgaaggccatcaagctggacggcgtggacgtgatcggatacaccgcatggagcctgatggacggcttcgagtggcaccgcggttacagcatccgccggggcctgttctacgttgacttcctgagccaggacaagatgttgctgcccaagagctccgccctgttctaccagaagttgatcgagaagaacggcttcccaccactccccgagaaccagcccctggagggcaccttcccctgcgatttcgcctggggcgtggtggacaactacatccaggtggacaccaccctgagtcagttcactgacctgaacgtgtacctttgggacgtgcaccacagcaagcgcctgataaaggtcgacggcgtggtgaccaagaagcgcaaaagctactgcgtggactttgccgccatccagccccagatcgccctgctgcaggagatgcacgtgactcacttccgcttcagcctcgactgggccctgattctgcccctgggcaaccagtcacaagtgaaccacaccattctgcagtactaccgctgtatggccagcgagctggtacgcgtgaacatcacccccgttgtggccctttggcagcccatggcccccaaccagggcctgcctcgcctgctggcccgccagggagcctgggagaatccctacaccgcactggccttcgctgaatacgcccgcctgtgcttccaggagctggggcaccacgtgaaactctggatcaccatgaacgagccctacaccagaaacatgacctacagcgccggacacaatctgctgaaggcccacgctctggcctggcacgtgtacaacgagaagtttcgccacgcccagaacggcaagatcagcatcgccctgcaggccgattggatcgagcccgcctgccccttcagccagaaggacaaggaggtggctgagcgggtgctggagttcgacatcgggtggctggctgagcctatcttcggcagcggagactacccctgggtgatgcgcgattggcttaaccagaggaacaatttcctgctgccctacttcaccgaggacgagaagaagctgatccagggcacctttgacttcctggctttgagccactataccactatcctggtggacagcgagaaggaggaccccatcaagtacaacgactacttggaggtgcaggagatgaccgacatcacctggctgaacagccctagccaggtggctgtggtgccttggggcctgcgcaaggtgctgaactggctgaagttcaagtacggcgatctgcccatgtatatcatcagcaacggcatcgacgacggcctgcacgccgaggacgaccagctgagagtgtactacatgcagaactacatcaacgaggccctcaaggcccacatcctggacggcatcaacctgtgtggctactttgcctacagcttcaacgacagaaccgccccccgcttcggcctgtacaggtacgccgccgaccagttcgaacccaaggccagcatgaagcactaccgcaaaatcatcgacagcaacggattccctggacccgagacactggagcgcttctgcccagaggagttcaccgtgtgcaccgagtgcagtttcttccacacccgcaagagctga

SEQ ID NO: 99 - RNA, 2946 nt, synthetic construct
  source 1..2946: mol_type = other RNA
atgcccgctagcgccccaccgagaagaccgcggccgccaccgccatcgctgtcgctgctgctggtgctgctgggactgggcggaagaagactgcgtgcggagcctggagatggagcccaaacatgggccagattcagcagacctcccgctcctgaagccgccggcttgtttcagggaacctttcctgacggtttcctgtgggctgtgggcagcgccgcctatcagaccgagggcggctggcaacagcacggaaaaggagccagcatctgggataccttcacccaccaccccctggccccccccggcgattcccgcaatgccagcctccctctgggagcccctagccccctgcagcctgccacaggagacgtggcctcagacagctataacaacgtgttccgcgacaccgaggcactgcgcgagctgggcgtgacccattaccgctttagcatcagctgggccagagtgctgcccaatggctctgccggcgtgcccaaccgggagggcctgaggtactaccgccgcctgctggagaggctgcgggagctgggcgtgcagcccgtggtaaccctgtaccactgggatctgccccagcgcctgcaggacgcttacggcggctgggccaaccgcgctctcgcagaccacttccgcgactacgccgagctgtgctttcgccactttggcggccaggtgaagtattggatcaccatcgataacccttacgtggtggcctggcacggatacgctacaggccgcctggcccccggcatccgcggcagccccagactgggctacctggtggcccacaatctgctgctggcccacgccaaggtgtggcacctgtacaacaccagcttccgccccacccagggtggacaggtctctattgccctgagctctcactggattaaccccaggaggatgaccgatcacagcatcaaggaatgccagaagagcctggacttcgttctgggctggttcgccaagcccgtgtttatcgacggcgactaccccgagagcatgaagaacaacctgtctagcatcctgcccgacgtcaccgagagcgaaaaaaaattcatcaagggcaccgccgatttcttcgccctgagcttcggcccaaccctgagcttccaactgctggatccccacatgaagttcagacaactcgagagtcccaatctgcgccagctgctgagctggatcgatctggaattcaaccacccccagatattcatagtggagaacggctggtttgtaagcggcactactaagcgcgatgatgcaaagtacatgtactatctgaagaagttcatcatggaaaccctgaaggccatcaagctggatggcgtggacgtgatcggatacaccgcatggagcctgatggacggcttcgagtggcaccgcggttactcaatccgcagggggttgttctacgtcgacttcctgagtcaggacaagatgttgctgccaaagagtagcgcccttttctaccagaagttgattgagaagaacggcttcccaccactccccgagaaccagcccctggagggcacctttccctgcgatttcgcttggggcgtggtggataattatattcaggtggacaccaccctgtcacagttcactgacctgaacgtgtacctgtgggacgtgcaccattccaagcgcctgatcaaggtggacggcgtggtgaccaagaagcgcaaatcctactgcgttgactttgccgccattcagccacagatcgccctgctgcaggagatgcacgtcacccacttccgcttcagcctggactgggccctcatcctgccactgggcaaccagtcccaggtgaaccacaccattctgcagtactaccgctgtatggccagcgagctggtacgcgtgaacatcacccccgtggtggccctgtggcagcccatggcccccaaccagggcctgccacgcctgctggccaggcagggggcctgggagaacccctacaccgcactcgctttcgccgaatatgccaggctgtgcttccaggagctggggcaccacgtgaagctctggatcaccatgaacgaaccctacaccagaaacatgacctactctgccggacacaatctgctgaaggcccacgccctggcctggcacgtctacaacgagaagttccgccacgcccaaaatggaaagatctctatagccctgcaggccgattggatcgagcccgcctgccccttctcacagaaggacaaggaggtggccgagcgcgtgctggagttcgacatcggctggctggccgagcccatcttcggcagcggagactacccctgggtgatgcgcgattggcttaaccagcgcaacaactttctgctgccctacttcaccgaggacgagaagaagctgatccagggcaccttcgacttcctggccctgagccactatactaccatcctggtcgacagcgagaaggaggacccaatcaagtacaacgactacctggaggtgcaggagatgaccgacatcacctggctgaacagccctagccaggtcgccgtggtgccttggggcctgcgcaaggtgctgaactggctgaagttcaagtatggcgatctgccaatgtacatcatcagcaacggcattgatgacggcctgcacgccgaggacgatcagctgagagtgtactatatgcagaactacatcaacgaggcactgaaggcccacatcctggacggcatcaacctgtgtggctactttgcatactccttcaacgacagaaccgccccccgcttcggcctgtacaggtacgctgccgatcagttcgagcccaaggccagcatgaagcactacagaaaaatcattgatagcaacgggttcccaggccccgagaccctggagcgcttctgccccgaggagttcaccgtgtgcaccgagtgcagttttttccacacccgcaagagctga

SEQ ID NO: 100 - RNA, 3249 nt, synthetic construct
  source 1..3249: mol_type = other RNA
gggagacataaaccctggcgcgctcgcggcccggcactcttctggtccccacagactcagagagaacccaccatgcccgctagcgccccaccgagaagaccgcggccgccaccgccatcgctgtcgctgctgctggtgctgctgggactgggcggaagaagactgcgtgcggagcctggcgacggggcccagacctgggccagattcagcagaccccccgcacccgaggccgccggcctgttccagggcaccttccccgacggatttctgtgggccgtgggaagcgctgcctaccagaccgagggcggctggcaacagcacggcaagggcgccagcatctgggacaccttcacccaccatcctctggctcctcccggagacagcagaaacgccagcctgcctctgggagcccccagccccctgcagcccgccactggagacgtggccagcgactcctacaacaacgtgttccgcgacaccgaggccctgcgcgagctgggcgtgacccactaccgctttagcatcagctgggccagagtgctgcccaacggcagcgccggcgtgcccaaccgggaaggcctgagatactatcgccgcctgctggagaggctgagagagttgggcgtgcagcccgtggtgaccctgtaccactgggatctgccccagcgcctgcaggacgcctacggcggctgggccaacagggcactcgccgaccacttccgcgactacgccgagctgtgcttccgccacttcggcggccaggtgaagtactggatcaccatcgacaacccctacgtggtggcctggcacggctacgctacaggaaggctggcccccgggatccgcggcagccccaggctgggctacctggtggcccacaatctgctgctggcacacgccaaagtgtggcacctgtataacaccagctttcgccccacccagggtggacaggtgagcattgccctgagttctcattggatcaaccccaggcgcatgaccgatcacagcatcaaggaatgccagaagagcctggacttcgtgctgggctggttcgccaagcccgtgtttatcgacggcgactaccccgagtctatgaagaacaacctcagcagcatcctgcctgacttcaccgagagcgagaagaagttcatcaagggcaccgccgacttcttcgccctgtgcttcggccccaccctgagcttccagctgctggatccccatatgaagttcagacaactcgagagtcctaatctgcgccagctgctgagctggatcgacctggaattcaaccacccacagatcttcatcgtggagaacggctggtttgtgagcggcaccactaagcgcgacgacgcaaagtatatgtattatctgaagaaattcatcatggaaaccctgaaggccatcaagctggacggcgtggacgtgatcggatacaccgcatggagcctgatggacggcttcgagtggcaccgcggttacagcatccgccggggcctgttctacgttgacttcctgagccaggacaagatgttgctgcccaagagctccgccctgttctaccagaagttgatcgagaagaacggcttcccaccactccccgagaaccagcccctggagggcaccttcccctgcgatttcgcctggggcgtggtggacaactacatccaggtggacaccaccctgagtcagttcactgacctgaacgtgtacctttgggacgtgcaccacagcaagcgcctgataaaggtcgacggcgtggtgaccaagaagcgcaaaagctactgcgtggactttgccgccatccagccccagatcgccctgctgcaggagatgcacgtgactcacttccgcttcagcctcgactgggccctgattctgcccctgggcaaccagtcacaagtgaaccacaccattctgcagtactaccgctgtatggccagcgagctggtacgcgtgaacatcacccccgttgtggccctttggcagcccatggcccccaaccagggcctgcctcgcctgctggcccgccagggagcctgggagaatccctacaccgcactggccttcgctgaatacgcccgcctgtgcttccaggagctggggcaccacgtgaaactctggatcaccatgaacgagccctacaccagaaacatgacctacagcgccggacacaatctgctgaaggcccacgctctggcctggcacgtgtacaacgagaagtttcgccacgcccagaacggcaagatcagcatcgccctgcaggccgattggatcgagcccgcctgccccttcagccagaaggacaaggaggtggctgagcgggtgctggagttcgacatcgggtggctggctgagcctatcttcggcagcggagactacccctgggtgatgcgcgattggcttaaccagaggaacaatttcctgctgccctacttcaccgaggacgagaagaagctgatccagggcacctttgacttcctggctttgagccactataccactatcctggtggacagcgagaaggaggaccccatcaagtacaacgactacttggaggtgcaggagatgaccgacatcacctggctgaacagccctagccaggtggctgtggtgccttggggcctgcgcaaggtgctgaactggctgaagttcaagtacggcgatctgcccatgtatatcatcagcaacggcatcgacgacggcctgcacgccgaggacgaccagctgagagtgtactacatgcagaactacatcaacgaggccctcaaggcccacatcctggacggcatcaacctgtgtggctactttgcctacagcttcaacgacagaaccgccccccgcttcggcctgtacaggtacgccgccgaccagttcgaacccaaggccagcatgaagcactaccgcaaaatcatcgacagcaacggattccctggacccgagacactggagcgcttctgcccagaggagttcaccgtgtgcaccgagtgcagtttcttccacacccgcaagagctgagctggagcctcggtggccatgcttcttgccccttgggcctccccccagcccctcctccccttcctgcacccgtacccccgtggtctttgaataaagtctgagtgggcggcaaaaaaaaaaaaaaaaaaaaaaaaaaaaaaaaaaaaaaaaaaaaaaaaaaaaaaaaaaaaaaaaaaaaaaaaaaaaaaaaaaaaaaaaaaaaaaaaaaaaaaaaaaaaaaaaaaaaaaaaa

SEQ ID NO: 101 - RNA, 3249 nt, synthetic construct
  source 1..3249: mol_type = other RNA
gggagacataaaccctggcgcgctcgcggcccggcactcttctggtccccacagactcagagagaacccaccatgcccgctagcgccccaccgagaagaccgcggccgccaccgccatcgctgtcgctgctgctggtgctgctgggactgggcggaagaagactgcgtgcggagcctggagatggagcccaaacatgggccagattcagcagacctcccgctcctgaagccgccggcttgtttcagggaacctttcctgacggtttcctgtgggctgtgggcagcgccgcctatcagaccgagggcggctggcaacagcacggaaaaggagccagcatctgggataccttcacccaccaccccctggccccccccggcgattcccgcaatgccagcctccctctgggagcccctagccccctgcagcctgccacaggagacgtggcctcagacagctataacaacgtgttccgcgacaccgaggcactgcgcgagctgggcgtgacccattaccgctttagcatcagctgggccagagtgctgcccaatggctctgccggcgtgcccaaccgggagggcctgaggtactaccgccgcctgctggagaggctgcgggagctgggcgtgcagcccgtggtaaccctgtaccactgggatctgccccagcgcctgcaggacgcttacggcggctgggccaaccgcgctctcgcagaccacttccgcgactacgccgagctgtgctttcgccactttggcggccaggtgaagtattggatcaccatcgataacccttacgtggtggcctggcacggatacgctacaggccgcctggcccccggcatccgcggcagccccagactgggctacctggtggcccacaatctgctgctggcccacgccaaggtgtggcacctgtacaacaccagcttccgccccacccagggtggacaggtctctattgccctgagctctcactggattaaccccaggaggatgaccgatcacagcatcaaggaatgccagaagagcctggacttcgttctgggctggttcgccaagcccgtgtttatcgacggcgactaccccgagagcatgaagaacaacctgtctagcatcctgcccgacttcaccgagagcgaaaaaaaattcatcaagggcaccgccgatttcttcgccctgtgtttcggcccaaccctgagcttccaactgctggatccccacatgaagttcagacaactcgagagtcccaatctgcgccagctgctgagctggatcgatctggaattcaaccacccccagatattcatagtggagaacggctggtttgtaagcggcactactaagcgcgatgatgcaaagtacatgtactatctgaagaagttcatcatggaaaccctgaaggccatcaagctggatggcgtggacgtgatcggatacaccgcatggagcctgatggacggcttcgagtggcaccgcggttactcaatccgcagggggttgttctacgtcgacttcctgagtcaggacaagatgttgctgccaaagagtagcgcccttttctaccagaagttgattgagaagaacggcttcccaccactccccgagaaccagcccctggagggcacctttccctgcgatttcgcttggggcgtggtggataattatattcaggtggacaccaccctgtcacagttcactgacctgaacgtgtacctgtgggacgtgcaccattccaagcgcctgatcaaggtggacggcgtggtgaccaagaagcgcaaatcctactgcgttgactttgccgccattcagccacagatcgccctgctgcaggagatgcacgtcacccacttccgcttcagcctggactgggccctcatcctgccactgggcaaccagtcccaggtgaaccacaccattctgcagtactaccgctgtatggccagcgagctggtacgcgtgaacatcacccccgtggtggccctgtggcagcccatggcccccaaccagggcctgccacgcctgctggccaggcagggggcctgggagaacccctacaccgcactcgctttcgccgaatatgccaggctgtgcttccaggagctggggcaccacgtgaagctctggatcaccatgaacgaaccctacaccagaaacatgacctactctgccggacacaatctgctgaaggcccacgccctggcctggcacgtctacaacgagaagttccgccacgcccaaaatggaaagatctctatagccctgcaggccgattggatcgagcccgcctgccccttctcacagaaggacaaggaggtggccgagcgcgtgctggagttcgacatcggctggctggccgagcccatcttcggcagcggagactacccctgggtgatgcgcgattggcttaaccagcgcaacaactttctgctgccctacttcaccgaggacgagaagaagctgatccagggcaccttcgacttcctggccctgagccactatactaccatcctggtcgacagcgagaaggaggacccaatcaagtacaacgactacctggaggtgcaggagatgaccgacatcacctggctgaacagccctagccaggtcgccgtggtgccttggggcctgcgcaaggtgctgaactggctgaagttcaagtatggcgatctgccaatgtacatcatcagcaacggcattgatgacggcctgcacgccgaggacgatcagctgagagtgtactatatgcagaactacatcaacgaggcactgaaggcccacatcctggacggcatcaacctgtgtggctactttgcatactccttcaacgacagaaccgccccccgcttcggcctgtacaggtacgctgccgatcagttcgagcccaaggccagcatgaagcactacagaaaaatcattgatagcaacgggttcccaggccccgagaccctggagcgcttctgccccgaggagttcaccgtgtgcaccgagtgcagttttttccacacccgcaagagctgagctggagcctcggtggccatgcttcttgccccttgggcctccccccagcccctcctccccttcctgcacccgtacccccgtggtctttgaataaagtctgagtgggcggcaaaaaaaaaaaaaaaaaaaaaaaaaaaaaaaaaaaaaaaaaaaaaaaaaaaaaaaaaaaaaaaaaaaaaaaaaaaaaaaaaaaaaaaaaaaaaaaaaaaaaaaaaaaaaaaaaaaaaaaaa

SEQ ID NO: 102 - RNA, 3249 nt, synthetic construct
  source 1..3249: mol_type = other RNA
gggagacataaaccctggcgcgctcgcggcccggcactcttctggtccccacagactcagagagaacccaccatgcccgctagcgccccaccgagaagaccgcggccgccaccgccatcgctgtcgctgctgctggtgctgctgggactgggcggaagaagactgcgtgcggagcctggcgacggggcccagacctgggccagattcagcagaccccccgcacccgaggccgccggcctgttccagggcaccttccccgacggatttctgtgggccgtgggaagcgctgcctaccagaccgagggcggctggcaacagcacggcaagggcgccagcatctgggacaccttcacccaccatcctctggctcctcccggagacagcagaaacgccagcctgcctctgggagcccccagccccctgcagcccgccactggagacgtggccagcgactcctacaacaacgtgttccgcgacaccgaggccctgcgcgagctgggcgtgacccactaccgctttagcatcagctgggccagagtgctgcccaacggcagcgccggcgtgcccaaccgggaaggcctgagatactatcgccgcctgctggagaggctgagagagttgggcgtgcagcccgtggtgaccctgtaccactgggatctgccccagcgcctgcaggacgcctacggcggctgggccaacagggcactcgccgaccacttccgcgactacgccgagctgtgcttccgccacttcggcggccaggtgaagtactggatcaccatcgacaacccctacgtggtggcctggcacggctacgctacaggaaggctggcccccgggatccgcggcagccccaggctgggctacctggtggcccacaatctgctgctggcacacgccaaagtgtggcacctgtataacaccagctttcgccccacccagggtggacaggtgagcattgccctgagttctcattggatcaaccccaggcgcatgaccgatcacagcatcaaggaatgccagaagagcctggacttcgtgctgggctggttcgccaagcccgtgtttatcgacggcgactaccccgagtctatgaagaacaacctcagcagcatcctgcctgacgtcaccgagagcgagaagaagttcatcaagggcaccgccgacttcttcgccctgagcttcggccccaccctgagcttccagctgctggatccccatatgaagttcagacaactcgagagtcctaatctgcgccagctgctgagctggatcgacctggaattcaaccacccacagatcttcatcgtggagaacggctggtttgtgagcggcaccactaagcgcgacgacgcaaagtatatgtattatctgaagaaattcatcatggaaaccctgaaggccatcaagctggacggcgtggacgtgatcggatacaccgcatggagcctgatggacggcttcgagtggcaccgcggttacagcatccgccggggcctgttctacgttgacttcctgagccaggacaagatgttgctgcccaagagctccgccctgttctaccagaagttgatcgagaagaacggcttcccaccactccccgagaaccagcccctggagggcaccttcccctgcgatttcgcctggggcgtggtggacaactacatccaggtggacaccaccctgagtcagttcactgacctgaacgtgtacctttgggacgtgcaccacagcaagcgcctgataaaggtcgacggcgtggtgaccaagaagcgcaaaagctactgcgtggactttgccgccatccagccccagatcgccctgctgcaggagatgcacgtgactcacttccgcttcagcctcgactgggccctgattctgcccctgggcaaccagtcacaagtgaaccacaccattctgcagtactaccgctgtatggccagcgagctggtacgcgtgaacatcacccccgttgtggccctttggcagcccatggcccccaaccagggcctgcctcgcctgctggcccgccagggagcctgggagaatccctacaccgcactggccttcgctgaatacgcccgcctgtgcttccaggagctggggcaccacgtgaaactctggatcaccatgaacgagccctacaccagaaacatgacctacagcgccggacacaatctgctgaaggcccacgctctggcctggcacgtgtacaacgagaagtttcgccacgcccagaacggcaagatcagcatcgccctgcaggccgattggatcgagcccgcctgccccttcagccagaaggacaaggaggtggctgagcgggtgctggagttcgacatcgggtggctggctgagcctatcttcggcagcggagactacccctgggtgatgcgcgattggcttaaccagaggaacaatttcctgctgccctacttcaccgaggacgagaagaagctgatccagggcacctttgacttcctggctttgagccactataccactatcctggtggacagcgagaaggaggaccccatcaagtacaacgactacttggaggtgcaggagatgaccgacatcacctggctgaacagccctagccaggtggctgtggtgccttggggcctgcgcaaggtgctgaactggctgaagttcaagtacggcgatctgcccatgtatatcatcagcaacggcatcgacgacggcctgcacgccgaggacgaccagctgagagtgtactacatgcagaactacatcaacgaggccctcaaggcccacatcctggacggcatcaacctgtgtggctactttgcctacagcttcaacgacagaaccgccccccgcttcggcctgtacaggtacgccgccgaccagttcgaacccaaggccagcatgaagcactaccgcaaaatcatcgacagcaacggattccctggacccgagacactggagcgcttctgcccagaggagttcaccgtgtgcaccgagtgcagtttcttccacacccgcaagagctgagctggagcctcggtggccatgcttcttgccccttgggcctccccccagcccctcctccccttcctgcacccgtacccccgtggtctttgaataaagtctgagtgggcggcaaaaaaaaaaaaaaaaaaaaaaaaaaaaaaaaaaaaaaaaaaaaaaaaaaaaaaaaaaaaaaaaaaaaaaaaaaaaaaaaaaaaaaaaaaaaaaaaaaaaaaaaaaaaaaaaaaaaaaaaa

SEQ ID NO: 103 - RNA, 3249 nt, synthetic construct
  source 1..3249: mol_type = other RNA
gggagacataaaccctggcgcgctcgcggcccggcactcttctggtccccacagactcagagagaacccaccatgcccgctagcgccccaccgagaagaccgcggccgccaccgccatcgctgtcgctgctgctggtgctgctgggactgggcggaagaagactgcgtgcggagcctggagatggagcccaaacatgggccagattcagcagacctcccgctcctgaagccgccggcttgtttcagggaacctttcctgacggtttcctgtgggctgtgggcagcgccgcctatcagaccgagggcggctggcaacagcacggaaaaggagccagcatctgggataccttcacccaccaccccctggccccccccggcgattcccgcaatgccagcctccctctgggagcccctagccccctgcagcctgccacaggagacgtggcctcagacagctataacaacgtgttccgcgacaccgaggcactgcgcgagctgggcgtgacccattaccgctttagcatcagctgggccagagtgctgcccaatggctctgccggcgtgcccaaccgggagggcctgaggtactaccgccgcctgctggagaggctgcgggagctgggcgtgcagcccgtggtaaccctgtaccactgggatctgccccagcgcctgcaggacgcttacggcggctgggccaaccgcgctctcgcagaccacttccgcgactacgccgagctgtgctttcgccactttggcggccaggtgaagtattggatcaccatcgataacccttacgtggtggcctggcacggatacgctacaggccgcctggcccccggcatccgcggcagccccagactgggctacctggtggcccacaatctgctgctggcccacgccaaggtgtggcacctgtacaacaccagcttccgccccacccagggtggacaggtctctattgccctgagctctcactggattaaccccaggaggatgaccgatcacagcatcaaggaatgccagaagagcctggacttcgttctgggctggttcgccaagcccgtgtttatcgacggcgactaccccgagagcatgaagaacaacctgtctagcatcctgcccgacgtcaccgagagcgaaaaaaaattcatcaagggcaccgccgatttcttcgccctgagcttcggcccaaccctgagcttccaactgctggatccccacatgaagttcagacaactcgagagtcccaatctgcgccagctgctgagctggatcgatctggaattcaaccacccccagatattcatagtggagaacggctggtttgtaagcggcactactaagcgcgatgatgcaaagtacatgtactatctgaagaagttcatcatggaaaccctgaaggccatcaagctggatggcgtggacgtgatcggatacaccgcatggagcctgatggacggcttcgagtggcaccgcggttactcaatccgcagggggttgttctacgtcgacttcctgagtcaggacaagatgttgctgccaaagagtagcgcccttttctaccagaagttgattgagaagaacggcttcccaccactccccgagaaccagcccctggagggcacctttccctgcgatttcgcttggggcgtggtggataattatattcaggtggacaccaccctgtcacagttcactgacctgaacgtgtacctgtgggacgtgcaccattccaagcgcctgatcaaggtggacggcgtggtgaccaagaagcgcaaatcctactgcgttgactttgccgccattcagccacagatcgccctgctgcaggagatgcacgtcacccacttccgcttcagcctggactgggccctcatcctgccactgggcaaccagtcccaggtgaaccacaccattctgcagtactaccgctgtatggccagcgagctggtacgcgtgaacatcacccccgtggtggccctgtggcagcccatggcccccaaccagggcctgccacgcctgctggccaggcagggggcctgggagaacccctacaccgcactcgctttcgccgaatatgccaggctgtgcttccaggagctggggcaccacgtgaagctctggatcaccatgaacgaaccctacaccagaaacatgacctactctgccggacacaatctgctgaaggcccacgccctggcctggcacgtctacaacgagaagttccgccacgcccaaaatggaaagatctctatagccctgcaggccgattggatcgagcccgcctgccccttctcacagaaggacaaggaggtggccgagcgcgtgctggagttcgacatcggctggctggccgagcccatcttcggcagcggagactacccctgggtgatgcgcgattggcttaaccagcgcaacaactttctgctgccctacttcaccgaggacgagaagaagctgatccagggcaccttcgacttcctggccctgagccactatactaccatcctggtcgacagcgagaaggaggacccaatcaagtacaacgactacctggaggtgcaggagatgaccgacatcacctggctgaacagccctagccaggtcgccgtggtgccttggggcctgcgcaaggtgctgaactggctgaagttcaagtatggcgatctgccaatgtacatcatcagcaacggcattgatgacggcctgcacgccgaggacgatcagctgagagtgtactatatgcagaactacatcaacgaggcactgaaggcccacatcctggacggcatcaacctgtgtggctactttgcatactccttcaacgacagaaccgccccccgcttcggcctgtacaggtacgctgccgatcagttcgagcccaaggccagcatgaagcactacagaaaaatcattgatagcaacgggttcccaggccccgagaccctggagcgcttctgccccgaggagttcaccgtgtgcaccgagtgcagttttttccacacccgcaagagctgagctggagcctcggtggccatgcttcttgccccttgggcctccccccagcccctcctccccttcctgcacccgtacccccgtggtctttgaataaagtctgagtgggcggcaaaaaaaaaaaaaaaaaaaaaaaaaaaaaaaaaaaaaaaaaaaaaaaaaaaaaaaaaaaaaaaaaaaaaaaaaaaaaaaaaaaaaaaaaaaaaaaaaaaaaaaaaaaaaaaaaaaaaaaaa

SEQ ID NO: 104 - RNA, 1482 nt, synthetic construct
  source 1..1482: mol_type = other RNA
ctgttccagggcaccttccccgacggatttctgtgggccgtgggaagcgctgcctaccagaccgagggcggctggcaacagcacggcaagggcgccagcatctgggacaccttcacccaccatcctctggctcctcccggagacagcagaaacgccagcctgcctctgggagcccccagccccctgcagcccgccactggagacgtggccagcgactcctacaacaacgtgttccgcgacaccgaggccctgcgcgagctgggcgtgacccactaccgctttagcatcagctgggccagagtgctgcccaacggcagcgccggcgtgcccaaccgggaaggcctgagatactatcgccgcctgctggagaggctgagagagttgggcgtgcagcccgtggtgaccctgtaccactgggatctgccccagcgcctgcaggacgcctacggcggctgggccaacagggcactcgccgaccacttccgcgactacgccgagctgtgcttccgccacttcggcggccaggtgaagtactggatcaccatcgacaacccctacgtggtggcctggcacggctacgctacaggaaggctggcccccgggatccgcggcagccccaggctgggctacctggtggcccacaatctgctgctggcacacgccaaagtgtggcacctgtataacaccagctttcgccccacccagggtggacaggtgagcattgccctgagttctcattggatcaaccccaggcgcatgaccgatcacagcatcaaggaatgccagaagagcctggacttcgtgctgggctggttcgccaagcccgtgtttatcgacggcgactaccccgagtctatgaagaacaacctcagcagcatcctgcctgacttcaccgagagcgagaagaagttcatcaagggcaccgccgacttcttcgccctgtgcttcggccccaccctgagcttccagctgctggatccccatatgaagttcagacaactcgagagtcctaatctgcgccagctgctgagctggatcgacctggaattcaaccacccacagatcttcatcgtggagaacggctggtttgtgagcggcaccactaagcgcgacgacgcaaagtatatgtattatctgaagaaattcatcatggaaaccctgaaggccatcaagctggacggcgtggacgtgatcggatacaccgcatggagcctgatggacggcttcgagtggcaccgcggttacagcatccgccggggcctgttctacgttgacttcctgagccaggacaagatgttgctgcccaagagctccgccctgttctaccagaagttgatcgagaagaacggcttcccaccactccccgagaaccagcccctggagggcaccttcccctgcgatttcgcctggggcgtggtggacaactacatccaggtgagccagctgacaaaacctatcagcagcctgacaaagccttaccat

SEQ ID NO: 105 - RNA, 1482 nt, synthetic construct
  source 1..1482: mol_type = other RNA
ttgtttcagggaacctttcctgacggtttcctgtgggctgtgggcagcgccgcctatcagaccgagggcggctggcaacagcacggaaaaggagccagcatctgggataccttcacccaccaccccctggccccccccggcgattcccgcaatgccagcctccctctgggagcccctagccccctgcagcctgccacaggagacgtggcctcagacagctataacaacgtgttccgcgacaccgaggcactgcgcgagctgggcgtgacccattaccgctttagcatcagctgggccagagtgctgcccaatggctctgccggcgtgcccaaccgggagggcctgaggtactaccgccgcctgctggagaggctgcgggagctgggcgtgcagcccgtggtaaccctgtaccactgggatctgccccagcgcctgcaggacgcttacggcggctgggccaaccgcgctctcgcagaccacttccgcgactacgccgagctgtgctttcgccactttggcggccaggtgaagtattggatcaccatcgataacccttacgtggtggcctggcacggatacgctacaggccgcctggcccccggcatccgcggcagccccagactgggctacctggtggcccacaatctgctgctggcccacgccaaggtgtggcacctgtacaacaccagcttccgccccacccagggtggacaggtctctattgccctgagctctcactggattaaccccaggaggatgaccgatcacagcatcaaggaatgccagaagagcctggacttcgttctgggctggttcgccaagcccgtgtttatcgacggcgactaccccgagagcatgaagaacaacctgtctagcatcctgcccgacttcaccgagagcgaaaaaaaattcatcaagggcaccgccgatttcttcgccctgtgtttcggcccaaccctgagcttccaactgctggatccccacatgaagttcagacaactcgagagtcccaatctgcgccagctgctgagctggatcgatctggaattcaaccacccccagatattcatagtggagaacggctggtttgtaagcggcactactaagcgcgatgatgcaaagtacatgtactatctgaagaagttcatcatggaaaccctgaaggccatcaagctggatggcgtggacgtgatcggatacaccgcatggagcctgatggacggcttcgagtggcaccgcggttactcaatccgcagggggttgttctacgtcgacttcctgagtcaggacaagatgttgctgccaaagagtagcgcccttttctaccagaagttgattgagaagaacggcttcccaccactccccgagaaccagcccctggagggcacctttccctgcgatttcgcttggggcgtggtggataattatattcaggtgagccagctgacaaaacctatcagcagcctgacaaagccttaccat

SEQ ID NO: 106 - RNA, 1482 nt, synthetic construct
  source 1..1482: mol_type = other RNA
ctgttccagggcaccttccccgacggatttctgtgggccgtgggaagcgctgcctaccagaccgagggcggctggcaacagcacggcaagggcgccagcatctgggacaccttcacccaccatcctctggctcctcccggagacagcagaaacgccagcctgcctctgggagcccccagccccctgcagcccgccactggagacgtggccagcgactcctacaacaacgtgttccgcgacaccgaggccctgcgcgagctgggcgtgacccactaccgctttagcatcagctgggccagagtgctgcccaacggcagcgccggcgtgcccaaccgggaaggcctgagatactatcgccgcctgctggagaggctgagagagttgggcgtgcagcccgtggtgaccctgtaccactgggatctgccccagcgcctgcaggacgcctacggcggctgggccaacagggcactcgccgaccacttccgcgactacgccgagctgtgcttccgccacttcggcggccaggtgaagtactggatcaccatcgacaacccctacgtggtggcctggcacggctacgctacaggaaggctggcccccgggatccgcggcagccccaggctgggctacctggtggcccacaatctgctgctggcacacgccaaagtgtggcacctgtataacaccagctttcgccccacccagggtggacaggtgagcattgccctgagttctcattggatcaaccccaggcgcatgaccgatcacagcatcaaggaatgccagaagagcctggacttcgtgctgggctggttcgccaagcccgtgtttatcgacggcgactaccccgagtctatgaagaacaacctcagcagcatcctgcctgacgtcaccgagagcgagaagaagttcatcaagggcaccgccgacttcttcgccctgagcttcggccccaccctgagcttccagctgctggatccccatatgaagttcagacaactcgagagtcctaatctgcgccagctgctgagctggatcgacctggaattcaaccacccacagatcttcatcgtggagaacggctggtttgtgagcggcaccactaagcgcgacgacgcaaagtatatgtattatctgaagaaattcatcatggaaaccctgaaggccatcaagctggacggcgtggacgtgatcggatacaccgcatggagcctgatggacggcttcgagtggcaccgcggttacagcatccgccggggcctgttctacgttgacttcctgagccaggacaagatgttgctgcccaagagctccgccctgttctaccagaagttgatcgagaagaacggcttcccaccactccccgagaaccagcccctggagggcaccttcccctgcgatttcgcctggggcgtggtggacaactacatccaggtgagccagctgacaaaacctatcagcagcctgacaaagccttaccat

SEQ ID NO: 107 - RNA, 1482 nt, synthetic construct
  source 1..1482: mol_type = other RNA
ttgtttcagggaacctttcctgacggtttcctgtgggctgtgggcagcgccgcctatcagaccgagggcggctggcaacagcacggaaaaggagccagcatctgggataccttcacccaccaccccctggccccccccggcgattcccgcaatgccagcctccctctgggagcccctagccccctgcagcctgccacaggagacgtggcctcagacagctataacaacgtgttccgcgacaccgaggcactgcgcgagctgggcgtgacccattaccgctttagcatcagctgggccagagtgctgcccaatggctctgccggcgtgcccaaccgggagggcctgaggtactaccgccgcctgctggagaggctgcgggagctgggcgtgcagcccgtggtaaccctgtaccactgggatctgccccagcgcctgcaggacgcttacggcggctgggccaaccgcgctctcgcagaccacttccgcgactacgccgagctgtgctttcgccactttggcggccaggtgaagtattggatcaccatcgataacccttacgtggtggcctggcacggatacgctacaggccgcctggcccccggcatccgcggcagccccagactgggctacctggtggcccacaatctgctgctggcccacgccaaggtgtggcacctgtacaacaccagcttccgccccacccagggtggacaggtctctattgccctgagctctcactggattaaccccaggaggatgaccgatcacagcatcaaggaatgccagaagagcctggacttcgttctgggctggttcgccaagcccgtgtttatcgacggcgactaccccgagagcatgaagaacaacctgtctagcatcctgcccgacgtcaccgagagcgaaaaaaaattcatcaagggcaccgccgatttcttcgccctgagcttcggcccaaccctgagcttccaactgctggatccccacatgaagttcagacaactcgagagtcccaatctgcgccagctgctgagctggatcgatctggaattcaaccacccccagatattcatagtggagaacggctggtttgtaagcggcactactaagcgcgatgatgcaaagtacatgtactatctgaagaagttcatcatggaaaccctgaaggccatcaagctggatggcgtggacgtgatcggatacaccgcatggagcctgatggacggcttcgagtggcaccgcggttactcaatccgcagggggttgttctacgtcgacttcctgagtcaggacaagatgttgctgccaaagagtagcgcccttttctaccagaagttgattgagaagaacggcttcccaccactccccgagaaccagcccctggagggcacctttccctgcgatttcgcttggggcgtggtggataattatattcaggtgagccagctgacaaaacctatcagcagcctgacaaagccttaccat

SEQ ID NO: 108 - RNA, 1548 nt, synthetic construct
  source 1..1548: mol_type = other RNA
gagcctggcgacggggcccagacctgggccagattcagcagaccccccgcacccgaggccgccggcctgttccagggcaccttccccgacggatttctgtgggccgtgggaagcgctgcctaccagaccgagggcggctggcaacagcacggcaagggcgccagcatctgggacaccttcacccaccatcctctggctcctcccggagacagcagaaacgccagcctgcctctgggagcccccagccccctgcagcccgccactggagacgtggccagcgactcctacaacaacgtgttccgcgacaccgaggccctgcgcgagctgggcgtgacccactaccgctttagcatcagctgggccagagtgctgcccaacggcagcgccggcgtgcccaaccgggaaggcctgagatactatcgccgcctgctggagaggctgagagagttgggcgtgcagcccgtggtgaccctgtaccactgggatctgccccagcgcctgcaggacgcctacggcggctgggccaacagggcactcgccgaccacttccgcgactacgccgagctgtgcttccgccacttcggcggccaggtgaagtactggatcaccatcgacaacccctacgtggtggcctggcacggctacgctacaggaaggctggcccccgggatccgcggcagccccaggctgggctacctggtggcccacaatctgctgctggcacacgccaaagtgtggcacctgtataacaccagctttcgccccacccagggtggacaggtgagcattgccctgagttctcattggatcaaccccaggcgcatgaccgatcacagcatcaaggaatgccagaagagcctggacttcgtgctgggctggttcgccaagcccgtgtttatcgacggcgactaccccgagtctatgaagaacaacctcagcagcatcctgcctgacttcaccgagagcgagaagaagttcatcaagggcaccgccgacttcttcgccctgtgcttcggccccaccctgagcttccagctgctggatccccatatgaagttcagacaactcgagagtcctaatctgcgccagctgctgagctggatcgacctggaattcaaccacccacagatcttcatcgtggagaacggctggtttgtgagcggcaccactaagcgcgacgacgcaaagtatatgtattatctgaagaaattcatcatggaaaccctgaaggccatcaagctggacggcgtggacgtgatcggatacaccgcatggagcctgatggacggcttcgagtggcaccgcggttacagcatccgccggggcctgttctacgttgacttcctgagccaggacaagatgttgctgcccaagagctccgccctgttctaccagaagttgatcgagaagaacggcttcccaccactccccgagaaccagcccctggagggcaccttcccctgcgatttcgcctggggcgtggtggacaactacatccaggtgagccagctgacaaaacctatcagcagcctgacaaagccttaccat

SEQ ID NO: 109 - RNA, 1548 nt, synthetic construct
  source 1..1548: mol_type = other RNA
gagcctggagatggagcccaaacatgggccagattcagcagacctcccgctcctgaagccgccggcttgtttcagggaacctttcctgacggtttcctgtgggctgtgggcagcgccgcctatcagaccgagggcggctggcaacagcacggaaaaggagccagcatctgggataccttcacccaccaccccctggccccccccggcgattcccgcaatgccagcctccctctgggagcccctagccccctgcagcctgccacaggagacgtggcctcagacagctataacaacgtgttccgcgacaccgaggcactgcgcgagctgggcgtgacccattaccgctttagcatcagctgggccagagtgctgcccaatggctctgccggcgtgcccaaccgggagggcctgaggtactaccgccgcctgctggagaggctgcgggagctgggcgtgcagcccgtggtaaccctgtaccactgggatctgccccagcgcctgcaggacgcttacggcggctgggccaaccgcgctctcgcagaccacttccgcgactacgccgagctgtgctttcgccactttggcggccaggtgaagtattggatcaccatcgataacccttacgtggtggcctggcacggatacgctacaggccgcctggcccccggcatccgcggcagccccagactgggctacctggtggcccacaatctgctgctggcccacgccaaggtgtggcacctgtacaacaccagcttccgccccacccagggtggacaggtctctattgccctgagctctcactggattaaccccaggaggatgaccgatcacagcatcaaggaatgccagaagagcctggacttcgttctgggctggttcgccaagcccgtgtttatcgacggcgactaccccgagagcatgaagaacaacctgtctagcatcctgcccgacttcaccgagagcgaaaaaaaattcatcaagggcaccgccgatttcttcgccctgtgtttcggcccaaccctgagcttccaactgctggatccccacatgaagttcagacaactcgagagtcccaatctgcgccagctgctgagctggatcgatctggaattcaaccacccccagatattcatagtggagaacggctggtttgtaagcggcactactaagcgcgatgatgcaaagtacatgtactatctgaagaagttcatcatggaaaccctgaaggccatcaagctggatggcgtggacgtgatcggatacaccgcatggagcctgatggacggcttcgagtggcaccgcggttactcaatccgcagggggttgttctacgtcgacttcctgagtcaggacaagatgttgctgccaaagagtagcgcccttttctaccagaagttgattgagaagaacggcttcccaccactccccgagaaccagcccctggagggcacctttccctgcgatttcgcttggggcgtggtggataattatattcaggtgagccagctgacaaaacctatcagcagcctgacaaagccttaccat

SEQ ID NO: 110 - RNA, 1548 nt, synthetic construct
  source 1..1548: mol_type = other RNA
gagcctggcgacggggcccagacctgggccagattcagcagaccccccgcacccgaggccgccggcctgttccagggcaccttccccgacggatttctgtgggccgtgggaagcgctgcctaccagaccgagggcggctggcaacagcacggcaagggcgccagcatctgggacaccttcacccaccatcctctggctcctcccggagacagcagaaacgccagcctgcctctgggagcccccagccccctgcagcccgccactggagacgtggccagcgactcctacaacaacgtgttccgcgacaccgaggccctgcgcgagctgggcgtgacccactaccgctttagcatcagctgggccagagtgctgcccaacggcagcgccggcgtgcccaaccgggaaggcctgagatactatcgccgcctgctggagaggctgagagagttgggcgtgcagcccgtggtgaccctgtaccactgggatctgccccagcgcctgcaggacgcctacggcggctgggccaacagggcactcgccgaccacttccgcgactacgccgagctgtgcttccgccacttcggcggccaggtgaagtactggatcaccatcgacaacccctacgtggtggcctggcacggctacgctacaggaaggctggcccccgggatccgcggcagccccaggctgggctacctggtggcccacaatctgctgctggcacacgccaaagtgtggcacctgtataacaccagctttcgccccacccagggtggacaggtgagcattgccctgagttctcattggatcaaccccaggcgcatgaccgatcacagcatcaaggaatgccagaagagcctggacttcgtgctgggctggttcgccaagcccgtgtttatcgacggcgactaccccgagtctatgaagaacaacctcagcagcatcctgcctgacgtcaccgagagcgagaagaagttcatcaagggcaccgccgacttcttcgccctgagcttcggccccaccctgagcttccagctgctggatccccatatgaagttcagacaactcgagagtcctaatctgcgccagctgctgagctggatcgacctggaattcaaccacccacagatcttcatcgtggagaacggctggtttgtgagcggcaccactaagcgcgacgacgcaaagtatatgtattatctgaagaaattcatcatggaaaccctgaaggccatcaagctggacggcgtggacgtgatcggatacaccgcatggagcctgatggacggcttcgagtggcaccgcggttacagcatccgccggggcctgttctacgttgacttcctgagccaggacaagatgttgctgcccaagagctccgccctgttctaccagaagttgatcgagaagaacggcttcccaccactccccgagaaccagcccctggagggcaccttcccctgcgatttcgcctggggcgtggtggacaactacatccaggtgagccagctgacaaaacctatcagcagcctgacaaagccttaccat

SEQ ID NO: 111 - RNA, 1548 nt, synthetic construct
  source 1..1548: mol_type = other RNA
gagcctggagatggagcccaaacatgggccagattcagcagacctcccgctcctgaagccgccggcttgtttcagggaacctttcctgacggtttcctgtgggctgtgggcagcgccgcctatcagaccgagggcggctggcaacagcacggaaaaggagccagcatctgggataccttcacccaccaccccctggccccccccggcgattcccgcaatgccagcctccctctgggagcccctagccccctgcagcctgccacaggagacgtggcctcagacagctataacaacgtgttccgcgacaccgaggcactgcgcgagctgggcgtgacccattaccgctttagcatcagctgggccagagtgctgcccaatggctctgccggcgtgcccaaccgggagggcctgaggtactaccgccgcctgctggagaggctgcgggagctgggcgtgcagcccgtggtaaccctgtaccactgggatctgccccagcgcctgcaggacgcttacggcggctgggccaaccgcgctctcgcagaccacttccgcgactacgccgagctgtgctttcgccactttggcggccaggtgaagtattggatcaccatcgataacccttacgtggtggcctggcacggatacgctacaggccgcctggcccccggcatccgcggcagccccagactgggctacctggtggcccacaatctgctgctggcccacgccaaggtgtggcacctgtacaacaccagcttccgccccacccagggtggacaggtctctattgccctgagctctcactggattaaccccaggaggatgaccgatcacagcatcaaggaatgccagaagagcctggacttcgttctgggctggttcgccaagcccgtgtttatcgacggcgactaccccgagagcatgaagaacaacctgtctagcatcctgcccgacgtcaccgagagcgaaaaaaaattcatcaagggcaccgccgatttcttcgccctgagcttcggcccaaccctgagcttccaactgctggatccccacatgaagttcagacaactcgagagtcccaatctgcgccagctgctgagctggatcgatctggaattcaaccacccccagatattcatagtggagaacggctggtttgtaagcggcactactaagcgcgatgatgcaaagtacatgtactatctgaagaagttcatcatggaaaccctgaaggccatcaagctggatggcgtggacgtgatcggatacaccgcatggagcctgatggacggcttcgagtggcaccgcggttactcaatccgcagggggttgttctacgtcgacttcctgagtcaggacaagatgttgctgccaaagagtagcgcccttttctaccagaagttgattgagaagaacggcttcccaccactccccgagaaccagcccctggagggcacctttccctgcgatttcgcttggggcgtggtggataattatattcaggtgagccagctgacaaaacctatcagcagcctgacaaagccttaccat

SEQ ID NO: 112 - RNA, 1650 nt, synthetic construct
  source 1..1650: mol_type = other RNA
atgcccgctagcgccccaccgagaagaccgcggccgccaccgccatcgctgtcgctgctgctggtgctgctgggactgggcggaagaagactgcgtgcggagcctggcgacggggcccagacctgggccagattcagcagaccccccgcacccgaggccgccggcctgttccagggcaccttccccgacggatttctgtgggccgtgggaagcgctgcctaccagaccgagggcggctggcaacagcacggcaagggcgccagcatctgggacaccttcacccaccatcctctggctcctcccggagacagcagaaacgccagcctgcctctgggagcccccagccccctgcagcccgccactggagacgtggccagcgactcctacaacaacgtgttccgcgacaccgaggccctgcgcgagctgggcgtgacccactaccgctttagcatcagctgggccagagtgctgcccaacggcagcgccggcgtgcccaaccgggaaggcctgagatactatcgccgcctgctggagaggctgagagagttgggcgtgcagcccgtggtgaccctgtaccactgggatctgccccagcgcctgcaggacgcctacggcggctgggccaacagggcactcgccgaccacttccgcgactacgccgagctgtgcttccgccacttcggcggccaggtgaagtactggatcaccatcgacaacccctacgtggtggcctggcacggctacgctacaggaaggctggcccccgggatccgcggcagccccaggctgggctacctggtggcccacaatctgctgctggcacacgccaaagtgtggcacctgtataacaccagctttcgccccacccagggtggacaggtgagcattgccctgagttctcattggatcaaccccaggcgcatgaccgatcacagcatcaaggaatgccagaagagcctggacttcgtgctgggctggttcgccaagcccgtgtttatcgacggcgactaccccgagtctatgaagaacaacctcagcagcatcctgcctgacttcaccgagagcgagaagaagttcatcaagggcaccgccgacttcttcgccctgtgcttcggccccaccctgagcttccagctgctggatccccatatgaagttcagacaactcgagagtcctaatctgcgccagctgctgagctggatcgacctggaattcaaccacccacagatcttcatcgtggagaacggctggtttgtgagcggcaccactaagcgcgacgacgcaaagtatatgtattatctgaagaaattcatcatggaaaccctgaaggccatcaagctggacggcgtggacgtgatcggatacaccgcatggagcctgatggacggcttcgagtggcaccgcggttacagcatccgccggggcctgttctacgttgacttcctgagccaggacaagatgttgctgcccaagagctccgccctgttctaccagaagttgatcgagaagaacggcttcccaccactccccgagaaccagcccctggagggcaccttcccctgcgatttcgcctggggcgtggtggacaactacatccaggtgagccagctgacaaaacctatcagcagcctgacaaagccttaccattga

SEQ ID NO: 113 - RNA, 1650 nt, synthetic construct
  source 1..1650: mol_type = other RNA
atgcccgctagcgccccaccgagaagaccgcggccgccaccgccatcgctgtcgctgctgctggtgctgctgggactgggcggaagaagactgcgtgcggagcctggagatggagcccaaacatgggccagattcagcagacctcccgctcctgaagccgccggcttgtttcagggaacctttcctgacggtttcctgtgggctgtgggcagcgccgcctatcagaccgagggcggctggcaacagcacggaaaaggagccagcatctgggataccttcacccaccaccccctggccccccccggcgattcccgcaatgccagcctccctctgggagcccctagccccctgcagcctgccacaggagacgtggcctcagacagctataacaacgtgttccgcgacaccgaggcactgcgcgagctgggcgtgacccattaccgctttagcatcagctgggccagagtgctgcccaatggctctgccggcgtgcccaaccgggagggcctgaggtactaccgccgcctgctggagaggctgcgggagctgggcgtgcagcccgtggtaaccctgtaccactgggatctgccccagcgcctgcaggacgcttacggcggctgggccaaccgcgctctcgcagaccacttccgcgactacgccgagctgtgctttcgccactttggcggccaggtgaagtattggatcaccatcgataacccttacgtggtggcctggcacggatacgctacaggccgcctggcccccggcatccgcggcagccccagactgggctacctggtggcccacaatctgctgctggcccacgccaaggtgtggcacctgtacaacaccagcttccgccccacccagggtggacaggtctctattgccctgagctctcactggattaaccccaggaggatgaccgatcacagcatcaaggaatgccagaagagcctggacttcgttctgggctggttcgccaagcccgtgtttatcgacggcgactaccccgagagcatgaagaacaacctgtctagcatcctgcccgacttcaccgagagcgaaaaaaaattcatcaagggcaccgccgatttcttcgccctgtgtttcggcccaaccctgagcttccaactgctggatccccacatgaagttcagacaactcgagagtcccaatctgcgccagctgctgagctggatcgatctggaattcaaccacccccagatattcatagtggagaacggctggtttgtaagcggcactactaagcgcgatgatgcaaagtacatgtactatctgaagaagttcatcatggaaaccctgaaggccatcaagctggatggcgtggacgtgatcggatacaccgcatggagcctgatggacggcttcgagtggcaccgcggttactcaatccgcagggggttgttctacgtcgacttcctgagtcaggacaagatgttgctgccaaagagtagcgcccttttctaccagaagttgattgagaagaacggcttcccaccactccccgagaaccagcccctggagggcacctttccctgcgatttcgcttggggcgtggtggataattatattcaggtgagccagctgacaaaacctatcagcagcctgacaaagccttaccattga

SEQ ID NO: 114 - RNA, 1650 nt, synthetic construct
  source 1..1650: mol_type = other RNA
atgcccgctagcgccccaccgagaagaccgcggccgccaccgccatcgctgtcgctgctgctggtgctgctgggactgggcggaagaagactgcgtgcggagcctggcgacggggcccagacctgggccagattcagcagaccccccgcacccgaggccgccggcctgttccagggcaccttccccgacggatttctgtgggccgtgggaagcgctgcctaccagaccgagggcggctggcaacagcacggcaagggcgccagcatctgggacaccttcacccaccatcctctggctcctcccggagacagcagaaacgccagcctgcctctgggagcccccagccccctgcagcccgccactggagacgtggccagcgactcctacaacaacgtgttccgcgacaccgaggccctgcgcgagctgggcgtgacccactaccgctttagcatcagctgggccagagtgctgcccaacggcagcgccggcgtgcccaaccgggaaggcctgagatactatcgccgcctgctggagaggctgagagagttgggcgtgcagcccgtggtgaccctgtaccactgggatctgccccagcgcctgcaggacgcctacggcggctgggccaacagggcactcgccgaccacttccgcgactacgccgagctgtgcttccgccacttcggcggccaggtgaagtactggatcaccatcgacaacccctacgtggtggcctggcacggctacgctacaggaaggctggcccccgggatccgcggcagccccaggctgggctacctggtggcccacaatctgctgctggcacacgccaaagtgtggcacctgtataacaccagctttcgccccacccagggtggacaggtgagcattgccctgagttctcattggatcaaccccaggcgcatgaccgatcacagcatcaaggaatgccagaagagcctggacttcgtgctgggctggttcgccaagcccgtgtttatcgacggcgactaccccgagtctatgaagaacaacctcagcagcatcctgcctgacgtcaccgagagcgagaagaagttcatcaagggcaccgccgacttcttcgccctgagcttcggccccaccctgagcttccagctgctggatccccatatgaagttcagacaactcgagagtcctaatctgcgccagctgctgagctggatcgacctggaattcaaccacccacagatcttcatcgtggagaacggctggtttgtgagcggcaccactaagcgcgacgacgcaaagtatatgtattatctgaagaaattcatcatggaaaccctgaaggccatcaagctggacggcgtggacgtgatcggatacaccgcatggagcctgatggacggcttcgagtggcaccgcggttacagcatccgccggggcctgttctacgttgacttcctgagccaggacaagatgttgctgcccaagagctccgccctgttctaccagaagttgatcgagaagaacggcttcccaccactccccgagaaccagcccctggagggcaccttcccctgcgatttcgcctggggcgtggtggacaactacatccaggtgagccagctgacaaaacctatcagcagcctgacaaagccttaccattga

SEQ ID NO: 115 - RNA, 1650 nt, synthetic construct
  source 1..1650: mol_type = other RNA
atgcccgctagcgccccaccgagaagaccgcggccgccaccgccatcgctgtcgctgctgctggtgctgctgggactgggcggaagaagactgcgtgcggagcctggagatggagcccaaacatgggccagattcagcagacctcccgctcctgaagccgccggcttgtttcagggaacctttcctgacggtttcctgtgggctgtgggcagcgccgcctatcagaccgagggcggctggcaacagcacggaaaaggagccagcatctgggataccttcacccaccaccccctggccccccccggcgattcccgcaatgccagcctccctctgggagcccctagccccctgcagcctgccacaggagacgtggcctcagacagctataacaacgtgttccgcgacaccgaggcactgcgcgagctgggcgtgacccattaccgctttagcatcagctgggccagagtgctgcccaatggctctgccggcgtgcccaaccgggagggcctgaggtactaccgccgcctgctggagaggctgcgggagctgggcgtgcagcccgtggtaaccctgtaccactgggatctgccccagcgcctgcaggacgcttacggcggctgggccaaccgcgctctcgcagaccacttccgcgactacgccgagctgtgctttcgccactttggcggccaggtgaagtattggatcaccatcgataacccttacgtggtggcctggcacggatacgctacaggccgcctggcccccggcatccgcggcagccccagactgggctacctggtggcccacaatctgctgctggcccacgccaaggtgtggcacctgtacaacaccagcttccgccccacccagggtggacaggtctctattgccctgagctctcactggattaaccccaggaggatgaccgatcacagcatcaaggaatgccagaagagcctggacttcgttctgggctggttcgccaagcccgtgtttatcgacggcgactaccccgagagcatgaagaacaacctgtctagcatcctgcccgacgtcaccgagagcgaaaaaaaattcatcaagggcaccgccgatttcttcgccctgagcttcggcccaaccctgagcttccaactgctggatccccacatgaagttcagacaactcgagagtcccaatctgcgccagctgctgagctggatcgatctggaattcaaccacccccagatattcatagtggagaacggctggtttgtaagcggcactactaagcgcgatgatgcaaagtacatgtactatctgaagaagttcatcatggaaaccctgaaggccatcaagctggatggcgtggacgtgatcggatacaccgcatggagcctgatggacggcttcgagtggcaccgcggttactcaatccgcagggggttgttctacgtcgacttcctgagtcaggacaagatgttgctgccaaagagtagcgcccttttctaccagaagttgattgagaagaacggcttcccaccactccccgagaaccagcccctggagggcacctttccctgcgatttcgcttggggcgtggtggataattatattcaggtgagccagctgacaaaacctatcagcagcctgacaaagccttaccattga

SEQ ID NO: 116 - RNA, 1953 nt, synthetic construct
  source 1..1953: mol_type = other RNA
gggagacataaaccctggcgcgctcgcggcccggcactcttctggtccccacagactcagagagaacccaccatgcccgctagcgccccaccgagaagaccgcggccgccaccgccatcgctgtcgctgctgctggtgctgctgggactgggcggaagaagactgcgtgcggagcctggcgacggggcccagacctgggccagattcagcagaccccccgcacccgaggccgccggcctgttccagggcaccttccccgacggatttctgtgggccgtgggaagcgctgcctaccagaccgagggcggctggcaacagcacggcaagggcgccagcatctgggacaccttcacccaccatcctctggctcctcccggagacagcagaaacgccagcctgcctctgggagcccccagccccctgcagcccgccactggagacgtggccagcgactcctacaacaacgtgttccgcgacaccgaggccctgcgcgagctgggcgtgacccactaccgctttagcatcagctgggccagagtgctgcccaacggcagcgccggcgtgcccaaccgggaaggcctgagatactatcgccgcctgctggagaggctgagagagttgggcgtgcagcccgtggtgaccctgtaccactgggatctgccccagcgcctgcaggacgcctacggcggctgggccaacagggcactcgccgaccacttccgcgactacgccgagctgtgcttccgccacttcggcggccaggtgaagtactggatcaccatcgacaacccctacgtggtggcctggcacggctacgctacaggaaggctggcccccgggatccgcggcagccccaggctgggctacctggtggcccacaatctgctgctggcacacgccaaagtgtggcacctgtataacaccagctttcgccccacccagggtggacaggtgagcattgccctgagttctcattggatcaaccccaggcgcatgaccgatcacagcatcaaggaatgccagaagagcctggacttcgtgctgggctggttcgccaagcccgtgtttatcgacggcgactaccccgagtctatgaagaacaacctcagcagcatcctgcctgacttcaccgagagcgagaagaagttcatcaagggcaccgccgacttcttcgccctgtgcttcggccccaccctgagcttccagctgctggatccccatatgaagttcagacaactcgagagtcctaatctgcgccagctgctgagctggatcgacctggaattcaaccacccacagatcttcatcgtggagaacggctggtttgtgagcggcaccactaagcgcgacgacgcaaagtatatgtattatctgaagaaattcatcatggaaaccctgaaggccatcaagctggacggcgtggacgtgatcggatacaccgcatggagcctgatggacggcttcgagtggcaccgcggttacagcatccgccggggcctgttctacgttgacttcctgagccaggacaagatgttgctgcccaagagctccgccctgttctaccagaagttgatcgagaagaacggcttcccaccactccccgagaaccagcccctggagggcaccttcccctgcgatttcgcctggggcgtggtggacaactacatccaggtgagccagctgacaaaacctatcagcagcctgacaaagccttaccattgagctggagcctcggtggccatgcttcttgccccttgggcctccccccagcccctcctccccttcctgcacccgtacccccgtggtctttgaataaagtctgagtgggcggcaaaaaaaaaaaaaaaaaaaaaaaaaaaaaaaaaaaaaaaaaaaaaaaaaaaaaaaaaaaaaaaaaaaaaaaaaaaaaaaaaaaaaaaaaaaaaaaaaaaaaaaaaaaaaaaaaaaaaaaaa

SEQ ID NO: 117 - RNA, 1953 nt, synthetic construct
  source 1..1953: mol_type = other RNA
gggagacataaaccctggcgcgctcgcggcccggcactcttctggtccccacagactcagagagaacccaccatgcccgctagcgccccaccgagaagaccgcggccgccaccgccatcgctgtcgctgctgctggtgctgctgggactgggcggaagaagactgcgtgcggagcctggagatggagcccaaacatgggccagattcagcagacctcccgctcctgaagccgccggcttgtttcagggaacctttcctgacggtttcctgtgggctgtgggcagcgccgcctatcagaccgagggcggctggcaacagcacggaaaaggagccagcatctgggataccttcacccaccaccccctggccccccccggcgattcccgcaatgccagcctccctctgggagcccctagccccctgcagcctgccacaggagacgtggcctcagacagctataacaacgtgttccgcgacaccgaggcactgcgcgagctgggcgtgacccattaccgctttagcatcagctgggccagagtgctgcccaatggctctgccggcgtgcccaaccgggagggcctgaggtactaccgccgcctgctggagaggctgcgggagctgggcgtgcagcccgtggtaaccctgtaccactgggatctgccccagcgcctgcaggacgcttacggcggctgggccaaccgcgctctcgcagaccacttccgcgactacgccgagctgtgctttcgccactttggcggccaggtgaagtattggatcaccatcgataacccttacgtggtggcctggcacggatacgctacaggccgcctggcccccggcatccgcggcagccccagactgggctacctggtggcccacaatctgctgctggcccacgccaaggtgtggcacctgtacaacaccagcttccgccccacccagggtggacaggtctctattgccctgagctctcactggattaaccccaggaggatgaccgatcacagcatcaaggaatgccagaagagcctggacttcgttctgggctggttcgccaagcccgtgtttatcgacggcgactaccccgagagcatgaagaacaacctgtctagcatcctgcccgacttcaccgagagcgaaaaaaaattcatcaagggcaccgccgatttcttcgccctgtgtttcggcccaaccctgagcttccaactgctggatccccacatgaagttcagacaactcgagagtcccaatctgcgccagctgctgagctggatcgatctggaattcaaccacccccagatattcatagtggagaacggctggtttgtaagcggcactactaagcgcgatgatgcaaagtacatgtactatctgaagaagttcatcatggaaaccctgaaggccatcaagctggatggcgtggacgtgatcggatacaccgcatggagcctgatggacggcttcgagtggcaccgcggttactcaatccgcagggggttgttctacgtcgacttcctgagtcaggacaagatgttgctgccaaagagtagcgcccttttctaccagaagttgattgagaagaacggcttcccaccactccccgagaaccagcccctggagggcacctttccctgcgatttcgcttggggcgtggtggataattatattcaggtgagccagctgacaaaacctatcagcagcctgacaaagccttaccattgagctggagcctcggtggccatgcttcttgccccttgggcctccccccagcccctcctccccttcctgcacccgtacccccgtggtctttgaataaagtctgagtgggcggcaaaaaaaaaaaaaaaaaaaaaaaaaaaaaaaaaaaaaaaaaaaaaaaaaaaaaaaaaaaaaaaaaaaaaaaaaaaaaaaaaaaaaaaaaaaaaaaaaaaaaaaaaaaaaaaaaaaaaaaaa

SEQ ID NO: 118 - RNA, 1953 nt, synthetic construct
  source 1..1953: mol_type = other RNA
gggagacataaaccctggcgcgctcgcggcccggcactcttctggtccccacagactcagagagaacccaccatgcccgctagcgccccaccgagaagaccgcggccgccaccgccatcgctgtcgctgctgctggtgctgctgggactgggcggaagaagactgcgtgcggagcctggcgacggggcccagacctgggccagattcagcagaccccccgcacccgaggccgccggcctgttccagggcaccttccccgacggatttctgtgggccgtgggaagcgctgcctaccagaccgagggcggctggcaacagcacggcaagggcgccagcatctgggacaccttcacccaccatcctctggctcctcccggagacagcagaaacgccagcctgcctctgggagcccccagccccctgcagcccgccactggagacgtggccagcgactcctacaacaacgtgttccgcgacaccgaggccctgcgcgagctgggcgtgacccactaccgctttagcatcagctgggccagagtgctgcccaacggcagcgccggcgtgcccaaccgggaaggcctgagatactatcgccgcctgctggagaggctgagagagttgggcgtgcagcccgtggtgaccctgtaccactgggatctgccccagcgcctgcaggacgcctacggcggctgggccaacagggcactcgccgaccacttccgcgactacgccgagctgtgcttccgccacttcggcggccaggtgaagtactggatcaccatcgacaacccctacgtggtggcctggcacggctacgctacaggaaggctggcccccgggatccgcggcagccccaggctgggctacctggtggcccacaatctgctgctggcacacgccaaagtgtggcacctgtataacaccagctttcgccccacccagggtggacaggtgagcattgccctgagttctcattggatcaaccccaggcgcatgaccgatcacagcatcaaggaatgccagaagagcctggacttcgtgctgggctggttcgccaagcccgtgtttatcgacggcgactaccccgagtctatgaagaacaacctcagcagcatcctgcctgacgtcaccgagagcgagaagaagttcatcaagggcaccgccgacttcttcgccctgagcttcggccccaccctgagcttccagctgctggatccccatatgaagttcagacaactcgagagtcctaatctgcgccagctgctgagctggatcgacctggaattcaaccacccacagatcttcatcgtggagaacggctggtttgtgagcggcaccactaagcgcgacgacgcaaagtatatgtattatctgaagaaattcatcatggaaaccctgaaggccatcaagctggacggcgtggacgtgatcggatacaccgcatggagcctgatggacggcttcgagtggcaccgcggttacagcatccgccggggcctgttctacgttgacttcctgagccaggacaagatgttgctgcccaagagctccgccctgttctaccagaagttgatcgagaagaacggcttcccaccactccccgagaaccagcccctggagggcaccttcccctgcgatttcgcctggggcgtggtggacaactacatccaggtgagccagctgacaaaacctatcagcagcctgacaaagccttaccattgagctggagcctcggtggccatgcttcttgccccttgggcctccccccagcccctcctccccttcctgcacccgtacccccgtggtctttgaataaagtctgagtgggcggcaaaaaaaaaaaaaaaaaaaaaaaaaaaaaaaaaaaaaaaaaaaaaaaaaaaaaaaaaaaaaaaaaaaaaaaaaaaaaaaaaaaaaaaaaaaaaaaaaaaaaaaaaaaaaaaaaaaaaaaaa

SEQ ID NO: 119 - RNA, 1953 nt, synthetic construct
  source 1..1953: mol_type = other RNA
gggagacataaaccctggcgcgctcgcggcccggcactcttctggtccccacagactcagagagaacccaccatgcccgctagcgccccaccgagaagaccgcggccgccaccgccatcgctgtcgctgctgctggtgctgctgggactgggcggaagaagactgcgtgcggagcctggagatggagcccaaacatgggccagattcagcagacctcccgctcctgaagccgccggcttgtttcagggaacctttcctgacggtttcctgtgggctgtgggcagcgccgcctatcagaccgagggcggctggcaacagcacggaaaaggagccagcatctgggataccttcacccaccaccccctggccccccccggcgattcccgcaatgccagcctccctctgggagcccctagccccctgcagcctgccacaggagacgtggcctcagacagctataacaacgtgttccgcgacaccgaggcactgcgcgagctgggcgtgacccattaccgctttagcatcagctgggccagagtgctgcccaatggctctgccggcgtgcccaaccgggagggcctgaggtactaccgccgcctgctggagaggctgcgggagctgggcgtgcagcccgtggtaaccctgtaccactgggatctgccccagcgcctgcaggacgcttacggcggctgggccaaccgcgctctcgcagaccacttccgcgactacgccgagctgtgctttcgccactttggcggccaggtgaagtattggatcaccatcgataacccttacgtggtggcctggcacggatacgctacaggccgcctggcccccggcatccgcggcagccccagactgggctacctggtggcccacaatctgctgctggcccacgccaaggtgtggcacctgtacaacaccagcttccgccccacccagggtggacaggtctctattgccctgagctctcactggattaaccccaggaggatgaccgatcacagcatcaaggaatgccagaagagcctggacttcgttctgggctggttcgccaagcccgtgtttatcgacggcgactaccccgagagcatgaagaacaacctgtctagcatcctgcccgacgtcaccgagagcgaaaaaaaattcatcaagggcaccgccgatttcttcgccctgagcttcggcccaaccctgagcttccaactgctggatccccacatgaagttcagacaactcgagagtcccaatctgcgccagctgctgagctggatcgatctggaattcaaccacccccagatattcatagtggagaacggctggtttgtaagcggcactactaagcgcgatgatgcaaagtacatgtactatctgaagaagttcatcatggaaaccctgaaggccatcaagctggatggcgtggacgtgatcggatacaccgcatggagcctgatggacggcttcgagtggcaccgcggttactcaatccgcagggggttgttctacgtcgacttcctgagtcaggacaagatgttgctgccaaagagtagcgcccttttctaccagaagttgattgagaagaacggcttcccaccactccccgagaaccagcccctggagggcacctttccctgcgatttcgcttggggcgtggtggataattatattcaggtgagccagctgacaaaacctatcagcagcctgacaaagccttaccattgagctggagcctcggtggccatgcttcttgccccttgggcctccccccagcccctcctccccttcctgcacccgtacccccgtggtctttgaataaagtctgagtgggcggcaaaaaaaaaaaaaaaaaaaaaaaaaaaaaaaaaaaaaaaaaaaaaaaaaaaaaaaaaaaaaaaaaaaaaaaaaaaaaaaaaaaaaaaaaaaaaaaaaaaaaaaaaaaaaaaaaaaaaaaaa

SEQ ID NO: 120 - RNA, 2937 nt, synthetic construct
  source 1..2937: mol_type = other RNA
gagcctggcgacggggcccagacctgggccagattcagcagaccccccgcacccgaggccgccggcctgttccagggcaccttccccgacggatttctgtgggccgtgggaagcgctgcctaccagaccgagggcggctggcaacagcacggcaagggcgccagcatctgggacaccttcacccaccatcctctggctcctcccggagacagcagaaacgccagcctgcctctgggagcccccagccccctgcagcccgccactggagacgtggccagcgactcctacaacaacgtgttccgcgacaccgaggccctgcgcgagctgggcgtgacccactaccgctttagcatcagctgggccagagtgctgcccaacggcagcgccggcgtgcccaaccgggaaggcctgagatactatcgccgcctgctggagaggctgagagagttgggcgtgcagcccgtggtgaccctgtaccactgggatctgccccagcgcctgcaggacgcctacggcggctgggccaacagggcactcgccgaccacttccgcgactacgccgagctgtgcttccgccacttcggcggccaggtgaagtactggatcaccatcgacaacccctacgtggtggcctggcacggctacgctacaggaaggctggcccccgggatccgcggcagccccaggctgggctacctggtggcccacaatctgctgctggcacacgccaaagtgtggcacctgtataacaccagctttcgccccacccagggtggacaggtgagcattgccctgagttctcattggatcaaccccaggcgcatgaccgatcacagcatcaaggaatgccagaagagcctggacttcgtgctgggctggttcgccaagcccgtgtttatcgacggcgactaccccgagtctatgaagaacaacctcagcagcatcctgcctgacttcaccgagagcgagaagaagttcatcaagggcaccgccgacttcttcgccctgtgcttcggccccaccctgagcttccagctgctggatccccatatgaagttcagacaactcgagagtcctaatctgcgccagctgctgagctggatcgacctggaattcaaccacccacagatcttcatcgtggagaacggctggtttgtgagcggcaccactaagcgcgacgacgcaaagtatatgtattatctgaagaaattcatcatggaaaccctgaaggccatcaagctggacggcgtggacgtgatcggatacaccgcatggagcctgatggacggcttcgagtggcaccgcggttacagcatccgccggggcctgttctacgttgacttcctgagccaggacaagatgttgctgcccaagagctccgccctgttctaccagaagttgatcgagaagaacggcttcccaccactccccgagaaccagcccctggagggcaccttcccctgcgatttcgcctggggcgtggtggacaactacatccaggtggacaccaccctgagtcagttcactgacctgaacgtgtacctttgggacgtgcaccacagcaagcgcctgataaaggtcgacggcgtggtgaccaagaagcgcaaaagctactgcgtggactttgccgccatccagccccagatcgccctgctgcaggagatgcacgtgactcacttccgcttcagcctcgactgggccctgattctgcccctgggcaaccagtcacaagtgaaccacaccattctgcagtactaccgctgtatggccagcgagctggtacgcgtgaacatcacccccgttgtggccctttggcagcccatggcccccaaccagggcctgcctcgcctgctggcccgccagggagcctgggagaatccctacaccgcactggccttcgctgaatacgcccgcctgtgcttccaggagctggggcaccacgtgaaactctggatcaccatgaacgagccctacaccagaaacatgacctacagcgccggacacaatctgctgaaggcccacgctctggcctggcacgtgtacaacgagaagtttcgccacgcccagaacggcaagatcagcatcgccctgcaggccgattggatcgagcccgcctgccccttcagccagaaggacaaggaggtggctgagcgggtgctggagttcgacatcgggtggctggctgagcctatcttcggcagcggagactacccctgggtgatgcgcgattggcttaaccagaggaacaatttcctgctgccctacttcaccgaggacgagaagaagctgatccagggcacctttgacttcctggctttgagccactataccactatcctggtggacagcgagaaggaggaccccatcaagtacaacgactacttggaggtgcaggagatgaccgacatcacctggctgaacagccctagccaggtggctgtggtgccttggggcctgcgcaaggtgctgaactggctgaagttcaagtacggcgatctgcccatgtatatcatcagcaacggcatcgacgacggcctgcacgccgaggacgaccagctgagagtgtactacatgcagaactacatcaacgaggccctcaaggcccacatcctggacggcatcaacctgtgtggctactttgcctacagcttcaacgacagaaccgccccccgcttcggcctgtacaggtacgccgccgaccagttcgaacccaaggccagcatgaagcactaccgcaaaatcatcgacagcaacggattccctggacccgagacactggagcgcttctgcccagaggagttcaccgtgtgcaccgagtgcagtttcttccacacccgcaagagcctgctggctttcattgcttttctgttttttgcttccattatttctctctccctcatcttttactacagcaagaaaggaagaagaagctacaaa

SEQ ID NO: 121 - RNA, 2937 nt, synthetic construct
  source 1..2937: mol_type = other RNA
gagcctggagatggagcccaaacatgggccagattcagcagacctcccgctcctgaagccgccggcttgtttcagggaacctttcctgacggtttcctgtgggctgtgggcagcgccgcctatcagaccgagggcggctggcaacagcacggaaaaggagccagcatctgggataccttcacccaccaccccctggccccccccggcgattcccgcaatgccagcctccctctgggagcccctagccccctgcagcctgccacaggagacgtggcctcagacagctataacaacgtgttccgcgacaccgaggcactgcgcgagctgggcgtgacccattaccgctttagcatcagctgggccagagtgctgcccaatggctctgccggcgtgcccaaccgggagggcctgaggtactaccgccgcctgctggagaggctgcgggagctgggcgtgcagcccgtggtaaccctgtaccactgggatctgccccagcgcctgcaggacgcttacggcggctgggccaaccgcgctctcgcagaccacttccgcgactacgccgagctgtgctttcgccactttggcggccaggtgaagtattggatcaccatcgataacccttacgtggtggcctggcacggatacgctacaggccgcctggcccccggcatccgcggcagccccagactgggctacctggtggcccacaatctgctgctggcccacgccaaggtgtggcacctgtacaacaccagcttccgccccacccagggtggacaggtctctattgccctgagctctcactggattaaccccaggaggatgaccgatcacagcatcaaggaatgccagaagagcctggacttcgttctgggctggttcgccaagcccgtgtttatcgacggcgactaccccgagagcatgaagaacaacctgtctagcatcctgcccgacttcaccgagagcgaaaaaaaattcatcaagggcaccgccgatttcttcgccctgtgtttcggcccaaccctgagcttccaactgctggatccccacatgaagttcagacaactcgagagtcccaatctgcgccagctgctgagctggatcgatctggaattcaaccacccccagatattcatagtggagaacggctggtttgtaagcggcactactaagcgcgatgatgcaaagtacatgtactatctgaagaagttcatcatggaaaccctgaaggccatcaagctggatggcgtggacgtgatcggatacaccgcatggagcctgatggacggcttcgagtggcaccgcggttactcaatccgcagggggttgttctacgtcgacttcctgagtcaggacaagatgttgctgccaaagagtagcgcccttttctaccagaagttgattgagaagaacggcttcccaccactccccgagaaccagcccctggagggcacctttccctgcgatttcgcttggggcgtggtggataattatattcaggtggacaccaccctgtcacagttcactgacctgaacgtgtacctgtgggacgtgcaccattccaagcgcctgatcaaggtggacggcgtggtgaccaagaagcgcaaatcctactgcgttgactttgccgccattcagccacagatcgccctgctgcaggagatgcacgtcacccacttccgcttcagcctggactgggccctcatcctgccactgggcaaccagtcccaggtgaaccacaccattctgcagtactaccgctgtatggccagcgagctggtacgcgtgaacatcacccccgtggtggccctgtggcagcccatggcccccaaccagggcctgccacgcctgctggccaggcagggggcctgggagaacccctacaccgcactcgctttcgccgaatatgccaggctgtgcttccaggagctggggcaccacgtgaagctctggatcaccatgaacgaaccctacaccagaaacatgacctactctgccggacacaatctgctgaaggcccacgccctggcctggcacgtctacaacgagaagttccgccacgcccaaaatggaaagatctctatagccctgcaggccgattggatcgagcccgcctgccccttctcacagaaggacaaggaggtggccgagcgcgtgctggagttcgacatcggctggctggccgagcccatcttcggcagcggagactacccctgggtgatgcgcgattggcttaaccagcgcaacaactttctgctgccctacttcaccgaggacgagaagaagctgatccagggcaccttcgacttcctggccctgagccactatactaccatcctggtcgacagcgagaaggaggacccaatcaagtacaacgactacctggaggtgcaggagatgaccgacatcacctggctgaacagccctagccaggtcgccgtggtgccttggggcctgcgcaaggtgctgaactggctgaagttcaagtatggcgatctgccaatgtacatcatcagcaacggcattgatgacggcctgcacgccgaggacgatcagctgagagtgtactatatgcagaactacatcaacgaggcactgaaggcccacatcctggacggcatcaacctgtgtggctactttgcatactccttcaacgacagaaccgccccccgcttcggcctgtacaggtacgctgccgatcagttcgagcccaaggccagcatgaagcactacagaaaaatcattgatagcaacgggttcccaggccccgagaccctggagcgcttctgccccgaggagttcaccgtgtgcaccgagtgcagttttttccacacccgcaagagcctgctggctttcattgcttttctgttttttgcttccattatttctctctccctcatcttttactacagcaagaaaggaagaagaagctacaaa

SEQ ID NO: 122 - RNA, 2937 nt, synthetic construct
  source 1..2937: mol_type = other RNA
gagcctggcgacggggcccagacctgggccagattcagcagaccccccgcacccgaggccgccggcctgttccagggcaccttccccgacggatttctgtgggccgtgggaagcgctgcctaccagaccgagggcggctggcaacagcacggcaagggcgccagcatctgggacaccttcacccaccatcctctggctcctcccggagacagcagaaacgccagcctgcctctgggagcccccagccccctgcagcccgccactggagacgtggccagcgactcctacaacaacgtgttccgcgacaccgaggccctgcgcgagctgggcgtgacccactaccgctttagcatcagctgggccagagtgctgcccaacggcagcgccggcgtgcccaaccgggaaggcctgagatactatcgccgcctgctggagaggctgagagagttgggcgtgcagcccgtggtgaccctgtaccactgggatctgccccagcgcctgcaggacgcctacggcggctgggccaacagggcactcgccgaccacttccgcgactacgccgagctgtgcttccgccacttcggcggccaggtgaagtactggatcaccatcgacaacccctacgtggtggcctggcacggctacgctacaggaaggctggcccccgggatccgcggcagccccaggctgggctacctggtggcccacaatctgctgctggcacacgccaaagtgtggcacctgtataacaccagctttcgccccacccagggtggacaggtgagcattgccctgagttctcattggatcaaccccaggcgcatgaccgatcacagcatcaaggaatgccagaagagcctggacttcgtgctgggctggttcgccaagcccgtgtttatcgacggcgactaccccgagtctatgaagaacaacctcagcagcatcctgcctgacgtcaccgagagcgagaagaagttcatcaagggcaccgccgacttcttcgccctgagcttcggccccaccctgagcttccagctgctggatccccatatgaagttcagacaactcgagagtcctaatctgcgccagctgctgagctggatcgacctggaattcaaccacccacagatcttcatcgtggagaacggctggtttgtgagcggcaccactaagcgcgacgacgcaaagtatatgtattatctgaagaaattcatcatggaaaccctgaaggccatcaagctggacggcgtggacgtgatcggatacaccgcatggagcctgatggacggcttcgagtggcaccgcggttacagcatccgccggggcctgttctacgttgacttcctgagccaggacaagatgttgctgcccaagagctccgccctgttctaccagaagttgatcgagaagaacggcttcccaccactccccgagaaccagcccctggagggcaccttcccctgcgatttcgcctggggcgtggtggacaactacatccaggtggacaccaccctgagtcagttcactgacctgaacgtgtacctttgggacgtgcaccacagcaagcgcctgataaaggtcgacggcgtggtgaccaagaagcgcaaaagctactgcgtggactttgccgccatccagccccagatcgccctgctgcaggagatgcacgtgactcacttccgcttcagcctcgactgggccctgattctgcccctgggcaaccagtcacaagtgaaccacaccattctgcagtactaccgctgtatggccagcgagctggtacgcgtgaacatcacccccgttgtggccctttggcagcccatggcccccaaccagggcctgcctcgcctgctggcccgccagggagcctgggagaatccctacaccgcactggccttcgctgaatacgcccgcctgtgcttccaggagctggggcaccacgtgaaactctggatcaccatgaacgagccctacaccagaaacatgacctacagcgccggacacaatctgctgaaggcccacgctctggcctggcacgtgtacaacgagaagtttcgccacgcccagaacggcaagatcagcatcgccctgcaggccgattggatcgagcccgcctgccccttcagccagaaggacaaggaggtggctgagcgggtgctggagttcgacatcgggtggctggctgagcctatcttcggcagcggagactacccctgggtgatgcgcgattggcttaaccagaggaacaatttcctgctgccctacttcaccgaggacgagaagaagctgatccagggcacctttgacttcctggctttgagccactataccactatcctggtggacagcgagaaggaggaccccatcaagtacaacgactacttggaggtgcaggagatgaccgacatcacctggctgaacagccctagccaggtggctgtggtgccttggggcctgcgcaaggtgctgaactggctgaagttcaagtacggcgatctgcccatgtatatcatcagcaacggcatcgacgacggcctgcacgccgaggacgaccagctgagagtgtactacatgcagaactacatcaacgaggccctcaaggcccacatcctggacggcatcaacctgtgtggctactttgcctacagcttcaacgacagaaccgccccccgcttcggcctgtacaggtacgccgccgaccagttcgaacccaaggccagcatgaagcactaccgcaaaatcatcgacagcaacggattccctggacccgagacactggagcgcttctgcccagaggagttcaccgtgtgcaccgagtgcagtttcttccacacccgcaagagcctgctggctttcattgcttttctgttttttgcttccattatttctctctccctcatcttttactacagcaagaaaggaagaagaagctacaaa

SEQ ID NO: 123 - RNA, 2937 nt, synthetic construct
  source 1..2937: mol_type = other RNA
gagcctggagatggagcccaaacatgggccagattcagcagacctcccgctcctgaagccgccggcttgtttcagggaacctttcctgacggtttcctgtgggctgtgggcagcgccgcctatcagaccgagggcggctggcaacagcacggaaaaggagccagcatctgggataccttcacccaccaccccctggccccccccggcgattcccgcaatgccagcctccctctgggagcccctagccccctgcagcctgccacaggagacgtggcctcagacagctataacaacgtgttccgcgacaccgaggcactgcgcgagctgggcgtgacccattaccgctttagcatcagctgggccagagtgctgcccaatggctctgccggcgtgcccaaccgggagggcctgaggtactaccgccgcctgctggagaggctgcgggagctgggcgtgcagcccgtggtaaccctgtaccactgggatctgccccagcgcctgcaggacgcttacggcggctgggccaaccgcgctctcgcagaccacttccgcgactacgccgagctgtgctttcgccactttggcggccaggtgaagtattggatcaccatcgataacccttacgtggtggcctggcacggatacgctacaggccgcctggcccccggcatccgcggcagccccagactgggctacctggtggcccacaatctgctgctggcccacgccaaggtgtggcacctgtacaacaccagcttccgccccacccagggtggacaggtctctattgccctgagctctcactggattaaccccaggaggatgaccgatcacagcatcaaggaatgccagaagagcctggacttcgttctgggctggttcgccaagcccgtgtttatcgacggcgactaccccgagagcatgaagaacaacctgtctagcatcctgcccgacgtcaccgagagcgaaaaaaaattcatcaagggcaccgccgatttcttcgccctgagcttcggcccaaccctgagcttccaactgctggatccccacatgaagttcagacaactcgagagtcccaatctgcgccagctgctgagctggatcgatctggaattcaaccacccccagatattcatagtggagaacggctggtttgtaagcggcactactaagcgcgatgatgcaaagtacatgtactatctgaagaagttcatcatggaaaccctgaaggccatcaagctggatggcgtggacgtgatcggatacaccgcatggagcctgatggacggcttcgagtggcaccgcggttactcaatccgcagggggttgttctacgtcgacttcctgagtcaggacaagatgttgctgccaaagagtagcgcccttttctaccagaagttgattgagaagaacggcttcccaccactccccgagaaccagcccctggagggcacctttccctgcgatttcgcttggggcgtggtggataattatattcaggtggacaccaccctgtcacagttcactgacctgaacgtgtacctgtgggacgtgcaccattccaagcgcctgatcaaggtggacggcgtggtgaccaagaagcgcaaatcctactgcgttgactttgccgccattcagccacagatcgccctgctgcaggagatgcacgtcacccacttccgcttcagcctggactgggccctcatcctgccactgggcaaccagtcccaggtgaaccacaccattctgcagtactaccgctgtatggccagcgagctggtacgcgtgaacatcacccccgtggtggccctgtggcagcccatggcccccaaccagggcctgccacgcctgctggccaggcagggggcctgggagaacccctacaccgcactcgctttcgccgaatatgccaggctgtgcttccaggagctggggcaccacgtgaagctctggatcaccatgaacgaaccctacaccagaaacatgacctactctgccggacacaatctgctgaaggcccacgccctggcctggcacgtctacaacgagaagttccgccacgcccaaaatggaaagatctctatagccctgcaggccgattggatcgagcccgcctgccccttctcacagaaggacaaggaggtggccgagcgcgtgctggagttcgacatcggctggctggccgagcccatcttcggcagcggagactacccctgggtgatgcgcgattggcttaaccagcgcaacaactttctgctgccctacttcaccgaggacgagaagaagctgatccagggcaccttcgacttcctggccctgagccactatactaccatcctggtcgacagcgagaaggaggacccaatcaagtacaacgactacctggaggtgcaggagatgaccgacatcacctggctgaacagccctagccaggtcgccgtggtgccttggggcctgcgcaaggtgctgaactggctgaagttcaagtatggcgatctgccaatgtacatcatcagcaacggcattgatgacggcctgcacgccgaggacgatcagctgagagtgtactatatgcagaactacatcaacgaggcactgaaggcccacatcctggacggcatcaacctgtgtggctactttgcatactccttcaacgacagaaccgccccccgcttcggcctgtacaggtacgctgccgatcagttcgagcccaaggccagcatgaagcactacagaaaaatcattgatagcaacgggttcccaggccccgagaccctggagcgcttctgccccgaggagttcaccgtgtgcaccgagtgcagttttttccacacccgcaagagcctgctggctttcattgcttttctgttttttgcttccattatttctctctccctcatcttttactacagcaagaaaggaagaagaagctacaaa

SEQ ID NO: 124 - RNA, 3039 nt, synthetic construct
  source 1..3039: mol_type = other RNA
atgcccgctagcgccccaccgagaagaccgcggccgccaccgccatcgctgtcgctgctgctggtgctgctgggactgggcggaagaagactgcgtgcggagcctggcgacggggcccagacctgggccagattcagcagaccccccgcacccgaggccgccggcctgttccagggcaccttccccgacggatttctgtgggccgtgggaagcgctgcctaccagaccgagggcggctggcaacagcacggcaagggcgccagcatctgggacaccttcacccaccatcctctggctcctcccggagacagcagaaacgccagcctgcctctgggagcccccagccccctgcagcccgccactggagacgtggccagcgactcctacaacaacgtgttccgcgacaccgaggccctgcgcgagctgggcgtgacccactaccgctttagcatcagctgggccagagtgctgcccaacggcagcgccggcgtgcccaaccgggaaggcctgagatactatcgccgcctgctggagaggctgagagagttgggcgtgcagcccgtggtgaccctgtaccactgggatctgccccagcgcctgcaggacgcctacggcggctgggccaacagggcactcgccgaccacttccgcgactacgccgagctgtgcttccgccacttcggcggccaggtgaagtactggatcaccatcgacaacccctacgtggtggcctggcacggctacgctacaggaaggctggcccccgggatccgcggcagccccaggctgggctacctggtggcccacaatctgctgctggcacacgccaaagtgtggcacctgtataacaccagctttcgccccacccagggtggacaggtgagcattgccctgagttctcattggatcaaccccaggcgcatgaccgatcacagcatcaaggaatgccagaagagcctggacttcgtgctgggctggttcgccaagcccgtgtttatcgacggcgactaccccgagtctatgaagaacaacctcagcagcatcctgcctgacttcaccgagagcgagaagaagttcatcaagggcaccgccgacttcttcgccctgtgcttcggccccaccctgagcttccagctgctggatccccatatgaagttcagacaactcgagagtcctaatctgcgccagctgctgagctggatcgacctggaattcaaccacccacagatcttcatcgtggagaacggctggtttgtgagcggcaccactaagcgcgacgacgcaaagtatatgtattatctgaagaaattcatcatggaaaccctgaaggccatcaagctggacggcgtggacgtgatcggatacaccgcatggagcctgatggacggcttcgagtggcaccgcggttacagcatccgccggggcctgttctacgttgacttcctgagccaggacaagatgttgctgcccaagagctccgccctgttctaccagaagttgatcgagaagaacggcttcccaccactccccgagaaccagcccctggagggcaccttcccctgcgatttcgcctggggcgtggtggacaactacatccaggtggacaccaccctgagtcagttcactgacctgaacgtgtacctttgggacgtgcaccacagcaagcgcctgataaaggtcgacggcgtggtgaccaagaagcgcaaaagctactgcgtggactttgccgccatccagccccagatcgccctgctgcaggagatgcacgtgactcacttccgcttcagcctcgactgggccctgattctgcccctgggcaaccagtcacaagtgaaccacaccattctgcagtactaccgctgtatggccagcgagctggtacgcgtgaacatcacccccgttgtggccctttggcagcccatggcccccaaccagggcctgcctcgcctgctggcccgccagggagcctgggagaatccctacaccgcactggccttcgctgaatacgcccgcctgtgcttccaggagctggggcaccacgtgaaactctggatcaccatgaacgagccctacaccagaaacatgacctacagcgccggacacaatctgctgaaggcccacgctctggcctggcacgtgtacaacgagaagtttcgccacgcccagaacggcaagatcagcatcgccctgcaggccgattggatcgagcccgcctgccccttcagccagaaggacaaggaggtggctgagcgggtgctggagttcgacatcgggtggctggctgagcctatcttcggcagcggagactacccctgggtgatgcgcgattggcttaaccagaggaacaatttcctgctgccctacttcaccgaggacgagaagaagctgatccagggcacctttgacttcctggctttgagccactataccactatcctggtggacagcgagaaggaggaccccatcaagtacaacgactacttggaggtgcaggagatgaccgacatcacctggctgaacagccctagccaggtggctgtggtgccttggggcctgcgcaaggtgctgaactggctgaagttcaagtacggcgatctgcccatgtatatcatcagcaacggcatcgacgacggcctgcacgccgaggacgaccagctgagagtgtactacatgcagaactacatcaacgaggccctcaaggcccacatcctggacggcatcaacctgtgtggctactttgcctacagcttcaacgacagaaccgccccccgcttcggcctgtacaggtacgccgccgaccagttcgaacccaaggccagcatgaagcactaccgcaaaatcatcgacagcaacggattccctggacccgagacactggagcgcttctgcccagaggagttcaccgtgtgcaccgagtgcagtttcttccacacccgcaagagcctgctggctttcattgcttttctgttttttgcttccattatttctctctccctcatcttttactacagcaagaaaggaagaagaagctacaaatga

SEQ ID NO: 125 - RNA, 3039 nt, synthetic construct
  source 1..3039: mol_type = other RNA
atgcccgctagcgccccaccgagaagaccgcggccgccaccgccatcgctgtcgctgctgctggtgctgctgggactgggcggaagaagactgcgtgcggagcctggagatggagcccaaacatgggccagattcagcagacctcccgctcctgaagccgccggcttgtttcagggaacctttcctgacggtttcctgtgggctgtgggcagcgccgcctatcagaccgagggcggctggcaacagcacggaaaaggagccagcatctgggataccttcacccaccaccccctggccccccccggcgattcccgcaatgccagcctccctctgggagcccctagccccctgcagcctgccacaggagacgtggcctcagacagctataacaacgtgttccgcgacaccgaggcactgcgcgagctgggcgtgacccattaccgctttagcatcagctgggccagagtgctgcccaatggctctgccggcgtgcccaaccgggagggcctgaggtactaccgccgcctgctggagaggctgcgggagctgggcgtgcagcccgtggtaaccctgtaccactgggatctgccccagcgcctgcaggacgcttacggcggctgggccaaccgcgctctcgcagaccacttccgcgactacgccgagctgtgctttcgccactttggcggccaggtgaagtattggatcaccatcgataacccttacgtggtggcctggcacggatacgctacaggccgcctggcccccggcatccgcggcagccccagactgggctacctggtggcccacaatctgctgctggcccacgccaaggtgtggcacctgtacaacaccagcttccgccccacccagggtggacaggtctctattgccctgagctctcactggattaaccccaggaggatgaccgatcacagcatcaaggaatgccagaagagcctggacttcgttctgggctggttcgccaagcccgtgtttatcgacggcgactaccccgagagcatgaagaacaacctgtctagcatcctgcccgacttcaccgagagcgaaaaaaaattcatcaagggcaccgccgatttcttcgccctgtgtttcggcccaaccctgagcttccaactgctggatccccacatgaagttcagacaactcgagagtcccaatctgcgccagctgctgagctggatcgatctggaattcaaccacccccagatattcatagtggagaacggctggtttgtaagcggcactactaagcgcgatgatgcaaagtacatgtactatctgaagaagttcatcatggaaaccctgaaggccatcaagctggatggcgtggacgtgatcggatacaccgcatggagcctgatggacggcttcgagtggcaccgcggttactcaatccgcagggggttgttctacgtcgacttcctgagtcaggacaagatgttgctgccaaagagtagcgcccttttctaccagaagttgattgagaagaacggcttcccaccactccccgagaaccagcccctggagggcacctttccctgcgatttcgcttggggcgtggtggataattatattcaggtggacaccaccctgtcacagttcactgacctgaacgtgtacctgtgggacgtgcaccattccaagcgcctgatcaaggtggacggcgtggtgaccaagaagcgcaaatcctactgcgttgactttgccgccattcagccacagatcgccctgctgcaggagatgcacgtcacccacttccgcttcagcctggactgggccctcatcctgccactgggcaaccagtcccaggtgaaccacaccattctgcagtactaccgctgtatggccagcgagctggtacgcgtgaacatcacccccgtggtggccctgtggcagcccatggcccccaaccagggcctgccacgcctgctggccaggcagggggcctgggagaacccctacaccgcactcgctttcgccgaatatgccaggctgtgcttccaggagctggggcaccacgtgaagctctggatcaccatgaacgaaccctacaccagaaacatgacctactctgccggacacaatctgctgaaggcccacgccctggcctggcacgtctacaacgagaagttccgccacgcccaaaatggaaagatctctatagccctgcaggccgattggatcgagcccgcctgccccttctcacagaaggacaaggaggtggccgagcgcgtgctggagttcgacatcggctggctggccgagcccatcttcggcagcggagactacccctgggtgatgcgcgattggcttaaccagcgcaacaactttctgctgccctacttcaccgaggacgagaagaagctgatccagggcaccttcgacttcctggccctgagccactatactaccatcctggtcgacagcgagaaggaggacccaatcaagtacaacgactacctggaggtgcaggagatgaccgacatcacctggctgaacagccctagccaggtcgccgtggtgccttggggcctgcgcaaggtgctgaactggctgaagttcaagtatggcgatctgccaatgtacatcatcagcaacggcattgatgacggcctgcacgccgaggacgatcagctgagagtgtactatatgcagaactacatcaacgaggcactgaaggcccacatcctggacggcatcaacctgtgtggctactttgcatactccttcaacgacagaaccgccccccgcttcggcctgtacaggtacgctgccgatcagttcgagcccaaggccagcatgaagcactacagaaaaatcattgatagcaacgggttcccaggccccgagaccctggagcgcttctgccccgaggagttcaccgtgtgcaccgagtgcagttttttccacacccgcaagagcctgctggctttcattgcttttctgttttttgcttccattatttctctctccctcatcttttactacagcaagaaaggaagaagaagctacaaatga

SEQ ID NO: 126 - RNA, 3039 nt, synthetic construct
  source 1..3039: mol_type = other RNA
atgcccgctagcgccccaccgagaagaccgcggccgccaccgccatcgctgtcgctgctgctggtgctgctgggactgggcggaagaagactgcgtgcggagcctggcgacggggcccagacctgggccagattcagcagaccccccgcacccgaggccgccggcctgttccagggcaccttccccgacggatttctgtgggccgtgggaagcgctgcctaccagaccgagggcggctggcaacagcacggcaagggcgccagcatctgggacaccttcacccaccatcctctggctcctcccggagacagcagaaacgccagcctgcctctgggagcccccagccccctgcagcccgccactggagacgtggccagcgactcctacaacaacgtgttccgcgacaccgaggccctgcgcgagctgggcgtgacccactaccgctttagcatcagctgggccagagtgctgcccaacggcagcgccggcgtgcccaaccgggaaggcctgagatactatcgccgcctgctggagaggctgagagagttgggcgtgcagcccgtggtgaccctgtaccactgggatctgccccagcgcctgcaggacgcctacggcggctgggccaacagggcactcgccgaccacttccgcgactacgccgagctgtgcttccgccacttcggcggccaggtgaagtactggatcaccatcgacaacccctacgtggtggcctggcacggctacgctacaggaaggctggcccccgggatccgcggcagccccaggctgggctacctggtggcccacaatctgctgctggcacacgccaaagtgtggcacctgtataacaccagctttcgccccacccagggtggacaggtgagcattgccctgagttctcattggatcaaccccaggcgcatgaccgatcacagcatcaaggaatgccagaagagcctggacttcgtgctgggctggttcgccaagcccgtgtttatcgacggcgactaccccgagtctatgaagaacaacctcagcagcatcctgcctgacgtcaccgagagcgagaagaagttcatcaagggcaccgccgacttcttcgccctgagcttcggccccaccctgagcttccagctgctggatccccatatgaagttcagacaactcgagagtcctaatctgcgccagctgctgagctggatcgacctggaattcaaccacccacagatcttcatcgtggagaacggctggtttgtgagcggcaccactaagcgcgacgacgcaaagtatatgtattatctgaagaaattcatcatggaaaccctgaaggccatcaagctggacggcgtggacgtgatcggatacaccgcatggagcctgatggacggcttcgagtggcaccgcggttacagcatccgccggggcctgttctacgttgacttcctgagccaggacaagatgttgctgcccaagagctccgccctgttctaccagaagttgatcgagaagaacggcttcccaccactccccgagaaccagcccctggagggcaccttcccctgcgatttcgcctggggcgtggtggacaactacatccaggtggacaccaccctgagtcagttcactgacctgaacgtgtacctttgggacgtgcaccacagcaagcgcctgataaaggtcgacggcgtggtgaccaagaagcgcaaaagctactgcgtggactttgccgccatccagccccagatcgccctgctgcaggagatgcacgtgactcacttccgcttcagcctcgactgggccctgattctgcccctgggcaaccagtcacaagtgaaccacaccattctgcagtactaccgctgtatggccagcgagctggtacgcgtgaacatcacccccgttgtggccctttggcagcccatggcccccaaccagggcctgcctcgcctgctggcccgccagggagcctgggagaatccctacaccgcactggccttcgctgaatacgcccgcctgtgcttccaggagctggggcaccacgtgaaactctggatcaccatgaacgagccctacaccagaaacatgacctacagcgccggacacaatctgctgaaggcccacgctctggcctggcacgtgtacaacgagaagtttcgccacgcccagaacggcaagatcagcatcgccctgcaggccgattggatcgagcccgcctgccccttcagccagaaggacaaggaggtggctgagcgggtgctggagttcgacatcgggtggctggctgagcctatcttcggcagcggagactacccctgggtgatgcgcgattggcttaaccagaggaacaatttcctgctgccctacttcaccgaggacgagaagaagctgatccagggcacctttgacttcctggctttgagccactataccactatcctggtggacagcgagaaggaggaccccatcaagtacaacgactacttggaggtgcaggagatgaccgacatcacctggctgaacagccctagccaggtggctgtggtgccttggggcctgcgcaaggtgctgaactggctgaagttcaagtacggcgatctgcccatgtatatcatcagcaacggcatcgacgacggcctgcacgccgaggacgaccagctgagagtgtactacatgcagaactacatcaacgaggccctcaaggcccacatcctggacggcatcaacctgtgtggctactttgcctacagcttcaacgacagaaccgccccccgcttcggcctgtacaggtacgccgccgaccagttcgaacccaaggccagcatgaagcactaccgcaaaatcatcgacagcaacggattccctggacccgagacactggagcgcttctgcccagaggagttcaccgtgtgcaccgagtgcagtttcttccacacccgcaagagcctgctggctttcattgcttttctgttttttgcttccattatttctctctccctcatcttttactacagcaagaaaggaagaagaagctacaaatga

SEQ ID NO: 127 - RNA, 3039 nt, synthetic construct
  source 1..3039: mol_type = other RNA
atgcccgctagcgccccaccgagaagaccgcggccgccaccgccatcgctgtcgctgctgctggtgctgctgggactgggcggaagaagactgcgtgcggagcctggagatggagcccaaacatgggccagattcagcagacctcccgctcctgaagccgccggcttgtttcagggaacctttcctgacggtttcctgtgggctgtgggcagcgccgcctatcagaccgagggcggctggcaacagcacggaaaaggagccagcatctgggataccttcacccaccaccccctggccccccccggcgattcccgcaatgccagcctccctctgggagcccctagccccctgcagcctgccacaggagacgtggcctcagacagctataacaacgtgttccgcgacaccgaggcactgcgcgagctgggcgtgacccattaccgctttagcatcagctgggccagagtgctgcccaatggctctgccggcgtgcccaaccgggagggcctgaggtactaccgccgcctgctggagaggctgcgggagctgggcgtgcagcccgtggtaaccctgtaccactgggatctgccccagcgcctgcaggacgcttacggcggctgggccaaccgcgctctcgcagaccacttccgcgactacgccgagctgtgctttcgccactttggcggccaggtgaagtattggatcaccatcgataacccttacgtggtggcctggcacggatacgctacaggccgcctggcccccggcatccgcggcagccccagactgggctacctggtggcccacaatctgctgctggcccacgccaaggtgtggcacctgtacaacaccagcttccgccccacccagggtggacaggtctctattgccctgagctctcactggattaaccccaggaggatgaccgatcacagcatcaaggaatgccagaagagcctggacttcgttctgggctggttcgccaagcccgtgtttatcgacggcgactaccccgagagcatgaagaacaacctgtctagcatcctgcccgacgtcaccgagagcgaaaaaaaattcatcaagggcaccgccgatttcttcgccctgagcttcggcccaaccctgagcttccaactgctggatccccacatgaagttcagacaactcgagagtcccaatctgcgccagctgctgagctggatcgatctggaattcaaccacccccagatattcatagtggagaacggctggtttgtaagcggcactactaagcgcgatgatgcaaagtacatgtactatctgaagaagttcatcatggaaaccctgaaggccatcaagctggatggcgtggacgtgatcggatacaccgcatggagcctgatggacggcttcgagtggcaccgcggttactcaatccgcagggggttgttctacgtcgacttcctgagtcaggacaagatgttgctgccaaagagtagcgcccttttctaccagaagttgattgagaagaacggcttcccaccactccccgagaaccagcccctggagggcacctttccctgcgatttcgcttggggcgtggtggataattatattcaggtggacaccaccctgtcacagttcactgacctgaacgtgtacctgtgggacgtgcaccattccaagcgcctgatcaaggtggacggcgtggtgaccaagaagcgcaaatcctactgcgttgactttgccgccattcagccacagatcgccctgctgcaggagatgcacgtcacccacttccgcttcagcctggactgggccctcatcctgccactgggcaaccagtcccaggtgaaccacaccattctgcagtactaccgctgtatggccagcgagctggtacgcgtgaacatcacccccgtggtggccctgtggcagcccatggcccccaaccagggcctgccacgcctgctggccaggcagggggcctgggagaacccctacaccgcactcgctttcgccgaatatgccaggctgtgcttccaggagctggggcaccacgtgaagctctggatcaccatgaacgaaccctacaccagaaacatgacctactctgccggacacaatctgctgaaggcccacgccctggcctggcacgtctacaacgagaagttccgccacgcccaaaatggaaagatctctatagccctgcaggccgattggatcgagcccgcctgccccttctcacagaaggacaaggaggtggccgagcgcgtgctggagttcgacatcggctggctggccgagcccatcttcggcagcggagactacccctgggtgatgcgcgattggcttaaccagcgcaacaactttctgctgccctacttcaccgaggacgagaagaagctgatccagggcaccttcgacttcctggccctgagccactatactaccatcctggtcgacagcgagaaggaggacccaatcaagtacaacgactacctggaggtgcaggagatgaccgacatcacctggctgaacagccctagccaggtcgccgtggtgccttggggcctgcgcaaggtgctgaactggctgaagttcaagtatggcgatctgccaatgtacatcatcagcaacggcattgatgacggcctgcacgccgaggacgatcagctgagagtgtactatatgcagaactacatcaacgaggcactgaaggcccacatcctggacggcatcaacctgtgtggctactttgcatactccttcaacgacagaaccgccccccgcttcggcctgtacaggtacgctgccgatcagttcgagcccaaggccagcatgaagcactacagaaaaatcattgatagcaacgggttcccaggccccgagaccctggagcgcttctgccccgaggagttcaccgtgtgcaccgagtgcagttttttccacacccgcaagagcctgctggctttcattgcttttctgttttttgcttccattatttctctctccctcatcttttactacagcaagaaaggaagaagaagctacaaatga

SEQ ID NO: 128 - RNA, 3342 nt, synthetic construct
  source 1..3342: mol_type = other RNA
gggagacataaaccctggcgcgctcgcggcccggcactcttctggtccccacagactcagagagaacccaccatgcccgctagcgccccaccgagaagaccgcggccgccaccgccatcgctgtcgctgctgctggtgctgctgggactgggcggaagaagactgcgtgcggagcctggcgacggggcccagacctgggccagattcagcagaccccccgcacccgaggccgccggcctgttccagggcaccttccccgacggatttctgtgggccgtgggaagcgctgcctaccagaccgagggcggctggcaacagcacggcaagggcgccagcatctgggacaccttcacccaccatcctctggctcctcccggagacagcagaaacgccagcctgcctctgggagcccccagccccctgcagcccgccactggagacgtggccagcgactcctacaacaacgtgttccgcgacaccgaggccctgcgcgagctgggcgtgacccactaccgctttagcatcagctgggccagagtgctgcccaacggcagcgccggcgtgcccaaccgggaaggcctgagatactatcgccgcctgctggagaggctgagagagttgggcgtgcagcccgtggtgaccctgtaccactgggatctgccccagcgcctgcaggacgcctacggcggctgggccaacagggcactcgccgaccacttccgcgactacgccgagctgtgcttccgccacttcggcggccaggtgaagtactggatcaccatcgacaacccctacgtggtggcctggcacggctacgctacaggaaggctggcccccgggatccgcggcagccccaggctgggctacctggtggcccacaatctgctgctggcacacgccaaagtgtggcacctgtataacaccagctttcgccccacccagggtggacaggtgagcattgccctgagttctcattggatcaaccccaggcgcatgaccgatcacagcatcaaggaatgccagaagagcctggacttcgtgctgggctggttcgccaagcccgtgtttatcgacggcgactaccccgagtctatgaagaacaacctcagcagcatcctgcctgacttcaccgagagcgagaagaagttcatcaagggcaccgccgacttcttcgccctgtgcttcggccccaccctgagcttccagctgctggatccccatatgaagttcagacaactcgagagtcctaatctgcgccagctgctgagctggatcgacctggaattcaaccacccacagatcttcatcgtggagaacggctggtttgtgagcggcaccactaagcgcgacgacgcaaagtatatgtattatctgaagaaattcatcatggaaaccctgaaggccatcaagctggacggcgtggacgtgatcggatacaccgcatggagcctgatggacggcttcgagtggcaccgcggttacagcatccgccggggcctgttctacgttgacttcctgagccaggacaagatgttgctgcccaagagctccgccctgttctaccagaagttgatcgagaagaacggcttcccaccactccccgagaaccagcccctggagggcaccttcccctgcgatttcgcctggggcgtggtggacaactacatccaggtggacaccaccctgagtcagttcactgacctgaacgtgtacctttgggacgtgcaccacagcaagcgcctgataaaggtcgacggcgtggtgaccaagaagcgcaaaagctactgcgtggactttgccgccatccagccccagatcgccctgctgcaggagatgcacgtgactcacttccgcttcagcctcgactgggccctgattctgcccctgggcaaccagtcacaagtgaaccacaccattctgcagtactaccgctgtatggccagcgagctggtacgcgtgaacatcacccccgttgtggccctttggcagcccatggcccccaaccagggcctgcctcgcctgctggcccgccagggagcctgggagaatccctacaccgcactggccttcgctgaatacgcccgcctgtgcttccaggagctggggcaccacgtgaaactctggatcaccatgaacgagccctacaccagaaacatgacctacagcgccggacacaatctgctgaaggcccacgctctggcctggcacgtgtacaacgagaagtttcgccacgcccagaacggcaagatcagcatcgccctgcaggccgattggatcgagcccgcctgccccttcagccagaaggacaaggaggtggctgagcgggtgctggagttcgacatcgggtggctggctgagcctatcttcggcagcggagactacccctgggtgatgcgcgattggcttaaccagaggaacaatttcctgctgccctacttcaccgaggacgagaagaagctgatccagggcacctttgacttcctggctttgagccactataccactatcctggtggacagcgagaaggaggaccccatcaagtacaacgactacttggaggtgcaggagatgaccgacatcacctggctgaacagccctagccaggtggctgtggtgccttggggcctgcgcaaggtgctgaactggctgaagttcaagtacggcgatctgcccatgtatatcatcagcaacggcatcgacgacggcctgcacgccgaggacgaccagctgagagtgtactacatgcagaactacatcaacgaggccctcaaggcccacatcctggacggcatcaacctgtgtggctactttgcctacagcttcaacgacagaaccgccccccgcttcggcctgtacaggtacgccgccgaccagttcgaacccaaggccagcatgaagcactaccgcaaaatcatcgacagcaacggattccctggacccgagacactggagcgcttctgcccagaggagttcaccgtgtgcaccgagtgcagtttcttccacacccgcaagagcctgctggctttcattgcttttctgttttttgcttccattatttctctctccctcatcttttactacagcaagaaaggaagaagaagctacaaatgagctggagcctcggtggccatgcttcttgccccttgggcctccccccagcccctcctccccttcctgcacccgtacccccgtggtctttgaataaagtctgagtgggcggcaaaaaaaaaaaaaaaaaaaaaaaaaaaaaaaaaaaaaaaaaaaaaaaaaaaaaaaaaaaaaaaaaaaaaaaaaaaaaaaaaaaaaaaaaaaaaaaaaaaaaaaaaaaaaaaaaaaaaaaaa

SEQ ID NO: 129 - RNA, 3342 nt, synthetic construct
  source 1..3342: mol_type = other RNA
gggagacataaaccctggcgcgctcgcggcccggcactcttctggtccccacagactcagagagaacccaccatgcccgctagcgccccaccgagaagaccgcggccgccaccgccatcgctgtcgctgctgctggtgctgctgggactgggcggaagaagactgcgtgcggagcctggagatggagcccaaacatgggccagattcagcagacctcccgctcctgaagccgccggcttgtttcagggaacctttcctgacggtttcctgtgggctgtgggcagcgccgcctatcagaccgagggcggctggcaacagcacggaaaaggagccagcatctgggataccttcacccaccaccccctggccccccccggcgattcccgcaatgccagcctccctctgggagcccctagccccctgcagcctgccacaggagacgtggcctcagacagctataacaacgtgttccgcgacaccgaggcactgcgcgagctgggcgtgacccattaccgctttagcatcagctgggccagagtgctgcccaatggctctgccggcgtgcccaaccgggagggcctgaggtactaccgccgcctgctggagaggctgcgggagctgggcgtgcagcccgtggtaaccctgtaccactgggatctgccccagcgcctgcaggacgcttacggcggctgggccaaccgcgctctcgcagaccacttccgcgactacgccgagctgtgctttcgccactttggcggccaggtgaagtattggatcaccatcgataacccttacgtggtggcctggcacggatacgctacaggccgcctggcccccggcatccgcggcagccccagactgggctacctggtggcccacaatctgctgctggcccacgccaaggtgtggcacctgtacaacaccagcttccgccccacccagggtggacaggtctctattgccctgagctctcactggattaaccccaggaggatgaccgatcacagcatcaaggaatgccagaagagcctggacttcgttctgggctggttcgccaagcccgtgtttatcgacggcgactaccccgagagcatgaagaacaacctgtctagcatcctgcccgacttcaccgagagcgaaaaaaaattcatcaagggcaccgccgatttcttcgccctgtgtttcggcccaaccctgagcttccaactgctggatccccacatgaagttcagacaactcgagagtcccaatctgcgccagctgctgagctggatcgatctggaattcaaccacccccagatattcatagtggagaacggctggtttgtaagcggcactactaagcgcgatgatgcaaagtacatgtactatctgaagaagttcatcatggaaaccctgaaggccatcaagctggatggcgtggacgtgatcggatacaccgcatggagcctgatggacggcttcgagtggcaccgcggttactcaatccgcagggggttgttctacgtcgacttcctgagtcaggacaagatgttgctgccaaagagtagcgcccttttctaccagaagttgattgagaagaacggcttcccaccactccccgagaaccagcccctggagggcacctttccctgcgatttcgcttggggcgtggtggataattatattcaggtggacaccaccctgtcacagttcactgacctgaacgtgtacctgtgggacgtgcaccattccaagcgcctgatcaaggtggacggcgtggtgaccaagaagcgcaaatcctactgcgttgactttgccgccattcagccacagatcgccctgctgcaggagatgcacgtcacccacttccgcttcagcctggactgggccctcatcctgccactgggcaaccagtcccaggtgaaccacaccattctgcagtactaccgctgtatggccagcgagctggtacgcgtgaacatcacccccgtggtggccctgtggcagcccatggcccccaaccagggcctgccacgcctgctggccaggcagggggcctgggagaacccctacaccgcactcgctttcgccgaatatgccaggctgtgcttccaggagctggggcaccacgtgaagctctggatcaccatgaacgaaccctacaccagaaacatgacctactctgccggacacaatctgctgaaggcccacgccctggcctggcacgtctacaacgagaagttccgccacgcccaaaatggaaagatctctatagccctgcaggccgattggatcgagcccgcctgccccttctcacagaaggacaaggaggtggccgagcgcgtgctggagttcgacatcggctggctggccgagcccatcttcggcagcggagactacccctgggtgatgcgcgattggcttaaccagcgcaacaactttctgctgccctacttcaccgaggacgagaagaagctgatccagggcaccttcgacttcctggccctgagccactatactaccatcctggtcgacagcgagaaggaggacccaatcaagtacaacgactacctggaggtgcaggagatgaccgacatcacctggctgaacagccctagccaggtcgccgtggtgccttggggcctgcgcaaggtgctgaactggctgaagttcaagtatggcgatctgccaatgtacatcatcagcaacggcattgatgacggcctgcacgccgaggacgatcagctgagagtgtactatatgcagaactacatcaacgaggcactgaaggcccacatcctggacggcatcaacctgtgtggctactttgcatactccttcaacgacagaaccgccccccgcttcggcctgtacaggtacgctgccgatcagttcgagcccaaggccagcatgaagcactacagaaaaatcattgatagcaacgggttcccaggccccgagaccctggagcgcttctgccccgaggagttcaccgtgtgcaccgagtgcagttttttccacacccgcaagagcctgctggctttcattgcttttctgttttttgcttccattatttctctctccctcatcttttactacagcaagaaaggaagaagaagctacaaatgagctggagcctcggtggccatgcttcttgccccttgggcctccccccagcccctcctccccttcctgcacccgtacccccgtggtctttgaataaagtctgagtgggcggcaaaaaaaaaaaaaaaaaaaaaaaaaaaaaaaaaaaaaaaaaaaaaaaaaaaaaaaaaaaaaaaaaaaaaaaaaaaaaaaaaaaaaaaaaaaaaaaaaaaaaaaaaaaaaaaaaaaaaaaaa

SEQ ID NO: 130 - RNA, 3342 nt, synthetic construct
  source 1..3342: mol_type = other RNA
gggagacataaaccctggcgcgctcgcggcccggcactcttctggtccccacagactcagagagaacccaccatgcccgctagcgccccaccgagaagaccgcggccgccaccgccatcgctgtcgctgctgctggtgctgctgggactgggcggaagaagactgcgtgcggagcctggcgacggggcccagacctgggccagattcagcagaccccccgcacccgaggccgccggcctgttccagggcaccttccccgacggatttctgtgggccgtgggaagcgctgcctaccagaccgagggcggctggcaacagcacggcaagggcgccagcatctgggacaccttcacccaccatcctctggctcctcccggagacagcagaaacgccagcctgcctctgggagcccccagccccctgcagcccgccactggagacgtggccagcgactcctacaacaacgtgttccgcgacaccgaggccctgcgcgagctgggcgtgacccactaccgctttagcatcagctgggccagagtgctgcccaacggcagcgccggcgtgcccaaccgggaaggcctgagatactatcgccgcctgctggagaggctgagagagttgggcgtgcagcccgtggtgaccctgtaccactgggatctgccccagcgcctgcaggacgcctacggcggctgggccaacagggcactcgccgaccacttccgcgactacgccgagctgtgcttccgccacttcggcggccaggtgaagtactggatcaccatcgacaacccctacgtggtggcctggcacggctacgctacaggaaggctggcccccgggatccgcggcagccccaggctgggctacctggtggcccacaatctgctgctggcacacgccaaagtgtggcacctgtataacaccagctttcgccccacccagggtggacaggtgagcattgccctgagttctcattggatcaaccccaggcgcatgaccgatcacagcatcaaggaatgccagaagagcctggacttcgtgctgggctggttcgccaagcccgtgtttatcgacggcgactaccccgagtctatgaagaacaacctcagcagcatcctgcctgacgtcaccgagagcgagaagaagttcatcaagggcaccgccgacttcttcgccctgagcttcggccccaccctgagcttccagctgctggatccccatatgaagttcagacaactcgagagtcctaatctgcgccagctgctgagctggatcgacctggaattcaaccacccacagatcttcatcgtggagaacggctggtttgtgagcggcaccactaagcgcgacgacgcaaagtatatgtattatctgaagaaattcatcatggaaaccctgaaggccatcaagctggacggcgtggacgtgatcggatacaccgcatggagcctgatggacggcttcgagtggcaccgcggttacagcatccgccggggcctgttctacgttgacttcctgagccaggacaagatgttgctgcccaagagctccgccctgttctaccagaagttgatcgagaagaacggcttcccaccactccccgagaaccagcccctggagggcaccttcccctgcgatttcgcctggggcgtggtggacaactacatccaggtggacaccaccctgagtcagttcactgacctgaacgtgtacctttgggacgtgcaccacagcaagcgcctgataaaggtcgacggcgtggtgaccaagaagcgcaaaagctactgcgtggactttgccgccatccagccccagatcgccctgctgcaggagatgcacgtgactcacttccgcttcagcctcgactgggccctgattctgcccctgggcaaccagtcacaagtgaaccacaccattctgcagtactaccgctgtatggccagcgagctggtacgcgtgaacatcacccccgttgtggccctttggcagcccatggcccccaaccagggcctgcctcgcctgctggcccgccagggagcctgggagaatccctacaccgcactggccttcgctgaatacgcccgcctgtgcttccaggagctggggcaccacgtgaaactctggatcaccatgaacgagccctacaccagaaacatgacctacagcgccggacacaatctgctgaaggcccacgctctggcctggcacgtgtacaacgagaagtttcgccacgcccagaacggcaagatcagcatcgccctgcaggccgattggatcgagcccgcctgccccttcagccagaaggacaaggaggtggctgagcgggtgctggagttcgacatcgggtggctggctgagcctatcttcggcagcggagactacccctgggtgatgcgcgattggcttaaccagaggaacaatttcctgctgccctacttcaccgaggacgagaagaagctgatccagggcacctttgacttcctggctttgagccactataccactatcctggtggacagcgagaaggaggaccccatcaagtacaacgactacttggaggtgcaggagatgaccgacatcacctggctgaacagccctagccaggtggctgtggtgccttggggcctgcgcaaggtgctgaactggctgaagttcaagtacggcgatctgcccatgtatatcatcagcaacggcatcgacgacggcctgcacgccgaggacgaccagctgagagtgtactacatgcagaactacatcaacgaggccctcaaggcccacatcctggacggcatcaacctgtgtggctactttgcctacagcttcaacgacagaaccgccccccgcttcggcctgtacaggtacgccgccgaccagttcgaacccaaggccagcatgaagcactaccgcaaaatcatcgacagcaacggattccctggacccgagacactggagcgcttctgcccagaggagttcaccgtgtgcaccgagtgcagtttcttccacacccgcaagagcctgctggctttcattgcttttctgttttttgcttccattatttctctctccctcatcttttactacagcaagaaaggaagaagaagctacaaatgagctggagcctcggtggccatgcttcttgccccttgggcctccccccagcccctcctccccttcctgcacccgtacccccgtggtctttgaataaagtctgagtgggcggcaaaaaaaaaaaaaaaaaaaaaaaaaaaaaaaaaaaaaaaaaaaaaaaaaaaaaaaaaaaaaaaaaaaaaaaaaaaaaaaaaaaaaaaaaaaaaaaaaaaaaaaaaaaaaaaaaaaaaaaaa

SEQ ID NO: 131 - RNA, 3342 nt, synthetic construct
  source 1..3342: mol_type = other RNA
gggagacataaaccctggcgcgctcgcggcccggcactcttctggtccccacagactcagagagaacccaccatgcccgctagcgccccaccgagaagaccgcggccgccaccgccatcgctgtcgctgctgctggtgctgctgggactgggcggaagaagactgcgtgcggagcctggagatggagcccaaacatgggccagattcagcagacctcccgctcctgaagccgccggcttgtttcagggaacctttcctgacggtttcctgtgggctgtgggcagcgccgcctatcagaccgagggcggctggcaacagcacggaaaaggagccagcatctgggataccttcacccaccaccccctggccccccccggcgattcccgcaatgccagcctccctctgggagcccctagccccctgcagcctgccacaggagacgtggcctcagacagctataacaacgtgttccgcgacaccgaggcactgcgcgagctgggcgtgacccattaccgctttagcatcagctgggccagagtgctgcccaatggctctgccggcgtgcccaaccgggagggcctgaggtactaccgccgcctgctggagaggctgcgggagctgggcgtgcagcccgtggtaaccctgtaccactgggatctgccccagcgcctgcaggacgcttacggcggctgggccaaccgcgctctcgcagaccacttccgcgactacgccgagctgtgctttcgccactttggcggccaggtgaagtattggatcaccatcgataacccttacgtggtggcctggcacggatacgctacaggccgcctggcccccggcatccgcggcagccccagactgggctacctggtggcccacaatctgctgctggcccacgccaaggtgtggcacctgtacaacaccagcttccgccccacccagggtggacaggtctctattgccctgagctctcactggattaaccccaggaggatgaccgatcacagcatcaaggaatgccagaagagcctggacttcgttctgggctggttcgccaagcccgtgtttatcgacggcgactaccccgagagcatgaagaacaacctgtctagcatcctgcccgacgtcaccgagagcgaaaaaaaattcatcaagggcaccgccgatttcttcgccctgagcttcggcccaaccctgagcttccaactgctggatccccacatgaagttcagacaactcgagagtcccaatctgcgccagctgctgagctggatcgatctggaattcaaccacccccagatattcatagtggagaacggctggtttgtaagcggcactactaagcgcgatgatgcaaagtacatgtactatctgaagaagttcatcatggaaaccctgaaggccatcaagctggatggcgtggacgtgatcggatacaccgcatggagcctgatggacggcttcgagtggcaccgcggttactcaatccgcagggggttgttctacgtcgacttcctgagtcaggacaagatgttgctgccaaagagtagcgcccttttctaccagaagttgattgagaagaacggcttcccaccactccccgagaaccagcccctggagggcacctttccctgcgatttcgcttggggcgtggtggataattatattcaggtggacaccaccctgtcacagttcactgacctgaacgtgtacctgtgggacgtgcaccattccaagcgcctgatcaaggtggacggcgtggtgaccaagaagcgcaaatcctactgcgttgactttgccgccattcagccacagatcgccctgctgcaggagatgcacgtcacccacttccgcttcagcctggactgggccctcatcctgccactgggcaaccagtcccaggtgaaccacaccattctgcagtactaccgctgtatggccagcgagctggtacgcgtgaacatcacccccgtggtggccctgtggcagcccatggcccccaaccagggcctgccacgcctgctggccaggcagggggcctgggagaacccctacaccgcactcgctttcgccgaatatgccaggctgtgcttccaggagctggggcaccacgtgaagctctggatcaccatgaacgaaccctacaccagaaacatgacctactctgccggacacaatctgctgaaggcccacgccctggcctggcacgtctacaacgagaagttccgccacgcccaaaatggaaagatctctatagccctgcaggccgattggatcgagcccgcctgccccttctcacagaaggacaaggaggtggccgagcgcgtgctggagttcgacatcggctggctggccgagcccatcttcggcagcggagactacccctgggtgatgcgcgattggcttaaccagcgcaacaactttctgctgccctacttcaccgaggacgagaagaagctgatccagggcaccttcgacttcctggccctgagccactatactaccatcctggtcgacagcgagaaggaggacccaatcaagtacaacgactacctggaggtgcaggagatgaccgacatcacctggctgaacagccctagccaggtcgccgtggtgccttggggcctgcgcaaggtgctgaactggctgaagttcaagtatggcgatctgccaatgtacatcatcagcaacggcattgatgacggcctgcacgccgaggacgatcagctgagagtgtactatatgcagaactacatcaacgaggcactgaaggcccacatcctggacggcatcaacctgtgtggctactttgcatactccttcaacgacagaaccgccccccgcttcggcctgtacaggtacgctgccgatcagttcgagcccaaggccagcatgaagcactacagaaaaatcattgatagcaacgggttcccaggccccgagaccctggagcgcttctgccccgaggagttcaccgtgtgcaccgagtgcagttttttccacacccgcaagagcctgctggctttcattgcttttctgttttttgcttccattatttctctctccctcatcttttactacagcaagaaaggaagaagaagctacaaatgagctggagcctcggtggccatgcttcttgccccttgggcctccccccagcccctcctccccttcctgcacccgtacccccgtggtctttgaataaagtctgagtgggcggcaaaaaaaaaaaaaaaaaaaaaaaaaaaaaaaaaaaaaaaaaaaaaaaaaaaaaaaaaaaaaaaaaaaaaaaaaaaaaaaaaaaaaaaaaaaaaaaaaaaaaaaaaaaaaaaaaaaaaaaaa

SEQ ID NO: 132 - RNA, 2946 nt, synthetic construct
  source 1..2946: mol_type = other RNA
atgcccgccagcgcccccccccgccgcccccgcccccccccccccagcctgagcctgctgctggtgctgctgggcctgggcggccgccgcctgcgcgccgagcccggcgacggcgcccagacctgggcccgcttcagccgcccccccgcccccgaggccgccggcctgttccagggcaccttccccgacggcttcctgtgggccgtgggcagcgccgcctaccagaccgagggcggctggcagcagcacggcaagggcgccagcatctgggacaccttcacccaccaccccctggccccccccggcgacagccgcaacgccagcctgcccctgggcgcccccagccccctgcagcccgccaccggcgacgtggccagcgacagctacaacaacgtgttccgcgacaccgaggccctgcgcgagctgggcgtgacccactaccgcttcagcatcagctgggcccgcgtgctgcccaacggcagcgccggcgtgcccaaccgcgagggcctgcgctactaccgccgcctgctggagcgcctgcgcgagctgggcgtgcagcccgtggtgaccctgtaccactgggacctgccccagcgcctgcaggacgcctacggcggctgggccaaccgcgccctggccgaccacttccgcgactacgccgagctgtgcttccgccacttcggcggccaggtgaagtactggatcaccatcgacaacccctacgtggtggcctggcacggctacgccaccggccgcctggcccccggcatccgcggcagcccccgcctgggctacctggtggcccacaacctgctgctggcccacgccaaggtgtggcacctgtacaacaccagcttccgccccacccagggcggccaggtgagcatcgccctgagcagccactggatcaacccccgccgcatgaccgaccacagcatcaaggagtgccagaagagcctggacttcgtgctgggctggttcgccaagcccgtgttcatcgacggcgactaccccgagagcatgaagaacaacctgagcagcatcctgcccgacttcaccgagagcgagaagaagttcatcaagggcaccgccgacttcttcgccctgtgcttcggccccaccctgagcttccagctgctggacccccacatgaagttccgccagctggagagccccaacctgcgccagctgctgagctggatcgacctggagttcaaccacccccagatcttcatcgtggagaacggctggttcgtgagcggcaccaccaagcgcgacgacgccaagtacatgtactacctgaagaagttcatcatggagaccctgaaggccatcaagctggacggcgtggacgtgatcggctacaccgcctggagcctgatggacggcttcgagtggcaccgcggctacagcatccgccgcggcctgttctacgtggacttcctgagccaggacaagatgctgctgcccaagagcagcgccctgttctaccagaagctgatcgagaagaacggcttcccccccctgcccgagaaccagcccctggagggcaccttcccctgcgacttcgcctggggcgtggtggacaactacatccaggtggacaccaccctgagccagttcaccgacctgaacgtgtacctgtgggacgtgcaccacagcaagcgcctgatcaaggtggacggcgtggtgaccaagaagcgcaagagctactgcgtggacttcgccgccatccagccccagatcgccctgctgcaggagatgcacgtgacccacttccgcttcagcctggactgggccctgatcctgcccctgggcaaccagagccaggtgaaccacaccatcctgcagtactaccgctgcatggccagcgagctggtgcgcgtgaacatcacccccgtggtggccctgtggcagcccatggcccccaaccagggcctgccccgcctgctggcccgccagggcgcctgggagaacccctacaccgccctggccttcgccgagtacgcccgcctgtgcttccaggagctgggccaccacgtgaagctgtggatcaccatgaacgagccctacacccgcaacatgacctacagcgccggccacaacctgctgaaggcccacgccctggcctggcacgtgtacaacgagaagttccgccacgcccagaacggcaagatcagcatcgccctgcaggccgactggatcgagcccgcctgccccttcagccagaaggacaaggaggtggccgagcgcgtgctggagttcgacatcggctggctggccgagcccatcttcggcagcggcgactacccctgggtgatgcgcgactggctgaaccagcgcaacaacttcctgctgccctacttcaccgaggacgagaagaagctgatccagggcaccttcgacttcctggccctgagccactacaccaccatcctggtggacagcgagaaggaggaccccatcaagtacaacgactacctggaggtgcaggagatgaccgacatcacctggctgaacagccccagccaggtggccgtggtgccctggggcctgcgcaaggtgctgaactggctgaagttcaagtacggcgacctgcccatgtacatcatcagcaacggcatcgacgacggcctgcacgccgaggacgaccagctgcgcgtgtactacatgcagaactacatcaacgaggccctgaaggcccacatcctggacggcatcaacctgtgcggctacttcgcctacagcttcaacgaccgcaccgccccccgcttcggcctgtaccgctacgccgccgaccagttcgagcccaaggccagcatgaagcactaccgcaagatcatcgacagcaacggcttccccggccccgagaccctggagcgcttctgccccgaggagttcaccgtgtgcaccgagtgcagcttcttccacacccgcaagagctag

SEQ ID NO: 133 - RNA, 2946 nt, synthetic construct
  source 1..2946: mol_type = other RNA
atgccggcgtcggcgccgccgcgtcgaccgcgtccgccgccgccgtcgctatcgctattattagtactactaggtctaggtggtcgtcgtctacgtgcggaaccgggtgatggtgcgcaaacgtgggcgcgattttcgcgaccgccggcgccggaagcggcgggtttatttcaaggtacgtttccggatggttttttatgggcggtaggttcggcggcgtatcaaacggaaggtggttggcaacaacatggtaaaggtgcgtcgatatgggatacgtttacgcatcatccgttagcgccgccgggtgattcgcgaaatgcgtcgctaccgctaggtgcgccgtcgccgttacaaccggcgacgggtgatgttgcgtcggattcgtataataatgtatttcgtgatacggaagcgctacgtgaactaggtgttacgcattatcgtttttcgatatcgtgggcgcgtgtattaccgaatggttcggcgggtgtaccgaatcgtgaaggtttacgatattatcgacgtttattagaacgtctacgtgaactaggtgttcaaccggtagttacgctatatcattgggatctaccgcaacgtttacaagatgcgtatggtggttgggcgaatcgagcgctagcggatcattttcgtgattatgcggaactatgttttcgacattttggtggtcaagtaaaatattggataacgatagataatccgtatgttgtagcgtggcatggttatgcgacgggtcgtctagcgccgggtatacgtggttcgccgcgattaggttatttagtagcgcataatctattattagcgcatgcgaaagtttggcatctatataatacgtcgtttcgtccgacgcaaggtggtcaagtttcgatagcgttatcgtcgcattggataaatccgcgtcgtatgacggatcattcgataaaagaatgtcaaaaatcgctagattttgtactaggttggtttgcgaaaccggtttttatagatggtgattatccggaatcgatgaaaaataatctatcgtcgatattaccggattttacggaatcggaaaaaaaatttataaaaggtacggcggatttttttgcgttatgttttggtccgacgttatcgtttcaactattagatccgcatatgaaatttcgacaattagaatcgccgaatttacgtcaactattatcgtggatagatttagaatttaatcatccgcaaatatttatagtagaaaatggttggtttgtttcgggtacgacgaaacgtgatgatgcgaaatatatgtattatttaaaaaaatttataatggaaacgttaaaagcgataaaattagatggtgtagatgtaataggttatacggcgtggtcgttaatggatggttttgaatggcatcgaggttattcgatacgtcgtggtctattttatgttgattttctatcgcaagataaaatgttattaccgaaatcgtcggcgttattttatcaaaaattaatagaaaaaaatggttttccgccgctaccggaaaatcaaccgttagaaggtacgtttccgtgtgattttgcgtggggtgtagtagataattatatacaagtagatacgacgttatcgcaatttacggatctaaatgtatatctatgggatgttcatcattcgaaacgtttaataaaagtagatggtgttgtaacgaaaaaacgtaaatcgtattgtgtagattttgcggcgatacaaccgcaaatagcgctattacaagaaatgcatgtaacgcattttcgtttttcgttagattgggcgttaatactaccgttaggtaatcaatcgcaagttaatcatacgatattacaatattatcgttgtatggcgtcggaattagttcgagttaatataacgccggtagttgcgttatggcaaccgatggcgccgaatcaaggtttaccgcgattactagcgcgacaaggtgcgtgggaaaatccgtatacggcgttagcgtttgcggaatatgcgcgattatgttttcaagaattaggtcatcatgtaaaattatggataacgatgaatgaaccgtatacgcgaaatatgacgtattcggcgggtcataatctattaaaagcgcatgcgctagcgtggcatgtatataatgaaaaatttcgacatgcgcaaaatggtaaaatatcgatagcgttacaagcggattggatagaaccggcgtgtccgttttcgcaaaaagataaagaagtagcggaacgtgtattagaatttgatataggttggctagcggaaccgatatttggttcgggtgattatccgtgggtaatgcgtgattggttaaatcaacgtaataattttttattaccgtattttacggaagatgaaaaaaaattaatacaaggtacgtttgattttctagcgttatcgcattatacgacgatactagttgattcggaaaaagaagatccgataaaatataatgattatttagaagtacaagaaatgacggatataacgtggctaaattcgccgtcgcaagtagcggttgttccgtggggtttacgaaaagtattaaattggctaaaatttaaatatggtgatttaccgatgtatataatatcgaatggtatagatgatggtttacatgcggaagatgatcaattacgagtatattatatgcaaaattatataaatgaagcgctaaaagcgcatatattagatggtataaatctatgtggttattttgcgtattcgtttaatgatcgaacggcgccgcgttttggtttatatcgatatgcggcggatcaatttgaaccgaaagcgtcgatgaaacattatcgaaaaataatagattcgaatggttttccgggtccggaaacgttagaacgtttttgtccggaagaatttacggtatgtacggaatgttcgttttttcatacgcgaaaatcgtag

SEQ ID NO: 134 - RNA, 2946 nt, synthetic construct
  source 1..2946: mol_type = other RNA
atgcccgcatctgcaccacccagacgccctaggcctcccccaccctcgttgagcctgctgctggtgctcctggggctcggcggacggaggttgagggcagaacctggagatggtgctcaaacctgggctagattcagtaggcctccagcccctgaggccgctggcctattccaggggacttttcccgacggatttctgtgggcagtgggcagcgccgcttaccagacagaaggcggatggcagcagcacggcaaaggcgcatccatttgggatacttttacgcaccacccattggctccacccggagactctaggaacgcctctctacccctgggagcgccaagccccctgcagccggctacgggagacgttgcctctgactcctataacaacgtgttccgggataccgaggccctgcgggagttgggggtgacacattaccggttcagtatttcatgggcacgggtcctgccgaatggatcagcaggcgtgcccaaccgagagggcctgaggtattacagacggcttctcgagcggttgagggaactgggagtccagccagtcgtaaccttgtaccactgggatctgccacagaggttacaagatgcttatggcggatgggctaatcgggcacttgcagatcacttccgggattatgcagaactctgtttcagacattttggtggtcaagtaaaatactggattaccatcgataatccatacgtggtagcttggcacggttatgccactggacggctggctccagggatacgcggatcccctcgcctcgggtatctcgtggcccataacttactcctggcgcacgccaaggtctggcatctctacaatacgagctttcggcctactcaaggagggcaggtctcaattgccctgtcttcacactggattaatcctcggcgaatgaccgaccactctataaaggagtgccaaaagtctcttgatttcgttctcggctggtttgccaagcctgtgttcatcgatggggattacccagagtctatgaagaataacctgagcagcattttgcccgattttaccgaatcagagaagaaattcataaagggtactgccgacttttttgccctgtgctttggtccgactttatcattccaactgctcgatccgcacatgaaattccggcagctggagagccctaatctgaggcagctgttgtcttggatagacctggaatttaaccatccacagatctttattgtagagaatggctggttcgtgtccggtactaccaagagggacgatgccaagtacatgtattatctgaaaaagttcatcatggaaactctgaaggctatcaaattggacggagtggatgtcattggctacaccgcttggtctttgatggatgggtttgaatggcaccggggatattctatacgccgaggcctgttttatgtcgatttcctgagccaggacaagatgctgctgcccaagagctcagcgctcttttaccagaagcttatagagaagaacggatttccaccattacctgaaaatcagccactggaagggacattcccttgcgatttcgcgtggggggtcgttgacaactatatacaggtcgataccactcttagccaatttacagacttaaatgtgtacctctgggatgttcatcattcaaagcgtctcatcaaggtggacggagtcgtgactaagaaaaggaaaagctactgtgtggactttgcagctatacagccacaaatcgcactgctacaagagatgcacgttactcatttcaggtttagcttagactgggctctgatattgcccctcgggaaccaatctcaagtcaatcacaccattttgcagtattacaggtgtatggctagcgaactcgtgcgtgtcaacattactccagtggttgccctctggcagccgatggctcccaaccaaggcctgccccgactcctggccaggcagggcgcttgggaaaatccgtatacagcactggctttcgctgagtacgcaaggctctgcttccaggaattaggacatcacgtgaaactctggattacgatgaatgagccctataccagaaacatgacttacagcgcaggccacaatcttttaaaggcccacgcactcgcctggcatgtctataatgagaagtttaggcacgctcagaatggaaagatctccatcgccctccaggctgattggatagagcccgcatgcccattctctcagaaggacaaagaggtggctgaaagggtgctagagtttgatattggttggctggccgagcctatattcgggtccggggattacccctgggtgatgcgcgactggctgaatcagcggaacaatttcctgctcccatacttcaccgaggatgaaaaaaagctcattcagggtacattcgattttctcgcgttgtcccactacacgacaatactcgtggactctgagaaagaagacccaatcaagtataatgattatctagaggttcaggagatgactgacatcacctggttgaattctccttctcaggtggccgtggtgccctggggactccgaaaagtgttgaattggttaaaattcaagtacggcgatctaccgatgtatatcattagtaatggcattgacgatggcctgcacgccgaagatgaccaactcagggtatactatatgcagaattacatcaacgaggctctgaaggcacacattttggacgggatcaacctatgtggctacttcgcctactccttcaatgataggactgctcctcgatttggcctgtataggtatgccgctgaccagttcgaacctaaggcatcgatgaagcattatcgtaaaattatcgacagcaacgggttcccagggccagagaccttggaaaggttctgcccagaggagtttaccgtatgtaccgaatgctccttttttcatactagaaagtcatag

SEQ ID NO: 135 - RNA, 2946 nt, synthetic construct
  source 1..2946: mol_type = other RNA
atgcctgcctctgcaccgccgcgccggcctagaccaccgcccccatccctgagcctgttgcttgtgctactgggtttgggcggtcggcgtctccgcgccgagccgggcgacggtgcccaaacctgggccaggttttcccggcctcctgccccggaggcagctggcctgttccagggtacattccctgatggttttctctgggcagtcggctctgctgcatatcagacagagggcgggtggcaacagcacggcaagggtgcaagcatttgggatacattcacacaccaccctttggcacccccaggcgactccaggaacgccagcctgcccctgggtgctccaagcccccttcagcctgcgactggagacgttgcctctgacagctataataacgtctttcgagatacggaggcactcagagagctgggcgttacccactaccggttcagtatatcttgggcccgggtcctccccaacggaagcgccggggtgcctaatcgtgagggcctgagatactaccggaggctcctagaaagacttcgagaattgggggtccagcccgttgtcaccttgtatcactgggatctgccacagcgcttgcaggacgcttacgggggttgggccaatagagccctggctgatcattttagagattatgcggaactctgcttcagacacttcggaggccaggtgaaatattggatcacgatcgataatccatacgtggtggcctggcatggatatgctaccgggagactggcgccgggaatccgcgggtctccccggctcggatatttagtcgcacacaatctgctgctggcccacgccaaagtgtggcacctctacaatacctcctttaggccgacgcagggaggccaggtcagcatcgcactgagctctcattggataaatccacggaggatgaccgaccactccatcaaggagtgccaaaagagtctggattttgtgcttggatggttcgcaaaaccagtctttatcgacggcgattaccctgaaagtatgaaaaacaacctgagctctattctgcccgatttcactgagagtgaaaagaaatttataaagggaactgcggatttttttgctctatgtttcggacctaccctctcgttccaactgctggatcctcatatgaagttccggcagctagagtccccgaacctgagacaactcttgagttggatagacctggagtttaaccatccccagattttcatcgttgaaaatggctggttcgtatctggtacgacgaaacgtgatgacgccaagtatatgtactacctgaaaaaatttattatggagacccttaaagcgatcaagttggatggcgtcgacgttatcggatacacagcatggtccctcatggatggttttgagtggcacagaggttacagtattcgacgagggctcttctacgtcgactttctgagtcaggataagatgcttctgccgaaatctagcgctctgttctaccagaagcttatcgaaaagaatggcttccctcctctgcccgagaatcagcccctggagggtacattcccatgcgacttcgcctggggcgtggtggataactatattcaggtcgacactacgctgagtcagtttaccgacctgaacgtctacctgtgggatgtgcaccatagcaagcggttgatcaaggtggatggggtagtgacaaaaaaacgaaagtcttattgcgtcgatttcgctgcgattcagcctcagatcgcgcttttacaggagatgcatgttacacactttcgatttagcttagactgggccttgattctgcccctgggcaaccaatctcaggttaatcataccatcctgcagtattaccggtgcatggcttcagagttggttagggtcaatattactcccgtggtggctctctggcagcccatggcccccaaccagggtctgcctagactcctggcccgacaaggcgcctgggaaaatccgtacaccgcactggcattcgccgaatatgcacgtttgtgttttcaggagctggggcatcatgttaagttatggatcaccatgaatgagccatataccaggaacatgacctattccgccggacacaacctcctgaaggcacatgccctggcctggcatgtgtataatgagaagtttaggcacgcccagaatggtaaaatctctatcgcgctgcaggccgactggatcgaacctgcctgtccattcagccagaaggacaaagaagtcgccgaaagagtgttggaattcgatattggctggcttgctgagccgatttttgggagcggtgattacccctgggtaatgcgggactggctgaatcaaaggaacaactttttacttccttactttaccgaggatgaaaagaagctgatccagggtaccttcgatttccttgccctcagtcactacaccacgatcctggtggattcggaaaaagaggatccaatcaaatataatgattacctggaggtgcaggagatgacagatatcacttggctcaactcaccttcacaggtcgccgttgtcccttggggtttgcgtaaagtcctgaattggctaaaattcaagtatggcgatcttcccatgtacattatctctaatggcatagatgatggtcttcacgcagaagacgaccagctcagagtttattatatgcagaactacataaatgaagctcttaaagctcacatcctggatgggatcaacttgtgtggctacttcgcctacagctttaacgataggacggccccccgtttcgggttgtaccgctatgctgccgatcagttcgagcccaaggcaagcatgaagcactaccgtaagatcatagattccaatgggtttccaggcccggaaacactggagcggttctgtccagaggagttcacggtatgcacagagtgttctttcttccacacgaggaaatcctag

SEQ ID NO: 136 - RNA, 2946 nt, synthetic construct
  source 1..2946: mol_type = other RNA
atgcccgccagcgcccccccccggcggccccggccccccccccccagtctctctctgctcctggtgctgctggggctgggaggtcggaggttgagagctgagccaggcgatggggctcagacatgggcacgttttagccgtcccccagcccctgaggctgctgggctattccagggtacttttcctgatggattcctgtgggccgttggcagcgccgcttaccagaccgagggcggctggcaacaacatgggaaaggcgcttccatttgggatacattcacccatcatcccctggccccccccggggattcgcgcaatgcatcgttgcccctgggtgctcctagcccactgcagcctgcaaccggagatgtggcatcagactcatataataacgtgttccgcgacaccgaagcgcttagggagttgggcgtgactcattacaggttttccattagttgggccagggtcctaccgaacggttctgccggcgtgccaaatcgggaggggctacggtactataggagactgctggaaagactacgcgagttgggggtccagcccgttgtcaccctttaccactgggacctcccccagcgcctgcaagacgcctatgggggctgggcaaacagagcactagccgaccactttcgggactacgccgaactttgcttccgacacttcgggggacaggtcaaatattggattacgattgataatccctatgtcgtggcgtggcacggctatgccacagggaggctggcaccgggcatcagaggatcgccgaggttggggtatctagtggcccacaaccttctgctcgcacacgccaaggtctggcacctgtacaacacttccttccgacccacacaggggggccaggtttcaattgctctgagctcccattggattaatcctcgcaggatgactgatcattctattaaagagtgccagaagtccttagacttcgttctgggctggtttgctaaacctgtgtttatcgacggagattacccagaatcgatgaagaacaacttgtctagcattctgcctgacttcacagagagcgagaagaagttcataaaaggaaccgcagattttttcgcactgtgcttcgggcccaccctgtcctttcagcttctcgaccctcatatgaaattccgccagctcgagtctccaaatctgaggcagctgttgagctggatcgaccttgaattcaaccacccacagattttcatcgtcgagaacggctggttcgtgagcgggacgacaaaaagggacgacgctaagtacatgtactacctgaagaaatttatcatggagactttaaaggcgatcaagctagatggcgttgatgtgattggttacacggcctggtcacttatggacggttttgaatggcacagaggctatagcattcgccgcggtctgttttatgtcgattttctgagccaggacaagatgctcctgccgaagagctctgcacttttttatcaaaagctgattgagaagaatgggtttccccctctgcccgaaaaccaaccccttgaaggaactttcccatgtgacttcgcctggggcgtggtggacaactacatccaggtggataccaccctcagccaatttaccgatctcaacgtttatctgtgggacgtgcaccattctaagagattaattaaggtcgacggcgtggtcaccaagaagcggaagagctactgcgtggattttgctgccatccagccccaaatagccttgcttcaagaaatgcacgttactcatttccgattctcgctcgattgggccctgattctgccactgggtaatcagagtcaggtgaatcacaccattttgcagtattaccgctgcatggcatctgagcttgtcagggtgaacatcacgcccgtggtagcactatggcaacccatggcaccaaaccagggcctgcctcgcctgctcgccagacagggggcatgggagaatccttacaccgcgctggcttttgcggaatatgcgaggctgtgtttccaggaattggggcaccatgtcaaattgtggatcactatgaacgagccctacacaagaaatatgacttatagtgccgggcataacctcttaaaggctcacgctctggcttggcacgtttacaatgagaagtttcgtcatgctcagaatggtaaaatcagcatagcgttacaggccgattggatagagcccgcctgcccattctcgcaaaaggataaggaagtcgctgagagggtcctcgagttcgacatcggctggctcgctgagcctatcttcggtagcggggactacccctgggtgatgcgagactggctcaatcagaggaacaatttcctgctaccctattttaccgaggatgagaaaaagttgatacagggcacatttgattttttggcactgtcccattataccacgattctcgtcgactccgagaaagaggatcccattaaatacaacgattatctcgaagtgcaggagatgaccgatatcacctggttaaactccccctcgcaagtggcagtggtaccttggggcctgaggaaagtgctcaactggctgaaattcaagtatggggatctcccaatgtacattatctctaacggcatagatgatggtctccatgccgaagacgatcagcttcgcgtttactatatgcaaaactacataaatgaggccttgaaggctcatattctggacgggatcaatctatgtgggtacttcgcctacagtttcaatgaccgcaccgccccacgcttcgggctgtacaggtacgccgcagatcagtttgagcctaaagccagcatgaaacattaccgcaaaatcattgactctaatggtttccccggacccgagaccctcgaacgcttttgccccgaggaattcaccgtgtgcacagaatgttctttttttcacacacgaaagtcatag

SEQ ID NO: 137 - RNA, 2946 nt, synthetic construct
  source 1..2946: mol_type = other RNA
atgcctgccagcgccccaccccggcggccccggcccccaccacccagcctgagcctgctgctggtgctgctgggcctgggcggccgccgcctgcgggcagagcctggagatggagcccagacctgggcccgcttcagccggcccccagcccctgaggccgccggcctcttccagggcaccttcccagatggcttcctgtgggccgtgggcagcgctgcctaccagacagagggcggctggcagcagcacggcaaaggagccagcatctgggacaccttcacccaccaccccctggcccctcctggggacagcagaaatgccagcctgcccctgggcgcccccagccccctgcagcctgccactggagatgtggccagtgacagctacaacaacgtgttccgggacacagaggccctgcgggagctgggcgtgacccactaccgcttcagcatctcctgggcccgggtgctgcccaatggatctgctggggtgcccaaccgggagggcctgcgctactaccgccgcctgctggagcggctgcgggagctgggcgtgcagcctgtggtgaccctgtaccactgggacctgccccagaggctgcaggatgcctacggcggctgggccaacagagccctggccgaccacttccgggactatgcagagctgtgcttccgccactttggaggccaggtgaagtactggatcaccatcgacaacccctacgtggtggcctggcacggctacgccaccggccgcctggcccctggcatccggggcagcccccggctgggctacctggtggcccacaacctgctgctggcccacgccaaggtgtggcacctgtacaacaccagcttccggcccacccagggcggccaggtgtccatcgccctgagcagccactggatcaaccccaggaggatgacagaccacagcatcaaggagtgccagaagagcctggactttgtgctgggctggtttgccaagcctgtgttcattgatggagactacccagagagcatgaagaacaacctgagcagcatcctgcctgacttcacagaaagtgagaagaagttcatcaagggcacagctgacttctttgccctgtgcttcggccccaccctgtccttccagctgctggacccccacatgaagttccggcagctggagagccccaacctgcggcagctgctgtcctggattgacctggagttcaaccacccccagatcttcatcgtggagaatggctggtttgtgtctggcaccaccaagagagatgatgccaagtacatgtactacctgaagaagttcatcatggagaccctgaaggccatcaagctggatggagtggatgtgattggctacacagcctggagcctgatggatggctttgagtggcaccggggctacagcatcagaagaggcctcttctacgtggacttcctgagccaggacaagatgctgctgcccaagagcagcgccctcttctaccagaagctgattgagaagaatggcttcccccccctgcctgagaaccagcccctggagggcaccttcccctgtgactttgcctggggcgtggtggacaactacatccaggtggacaccaccctgagccagttcacagacctgaatgtgtacctgtgggatgtgcaccacagcaagaggctcatcaaggtggatggagtggtgaccaagaagaggaagagctactgtgtggactttgctgccatccagccccagatcgccctgctgcaggagatgcacgtgacccacttccgcttcagcctggactgggccctgatcctgcccctgggcaaccagagccaggtgaaccacaccatcctgcagtactaccgctgcatggccagcgagctggtgcgggtgaacatcacccctgtggtggccctgtggcagcccatggcccccaaccagggcctgccccggctgctggcccggcagggcgcctgggagaacccctacacagccctggcctttgctgaatatgcccggctgtgcttccaggagctgggccaccacgtgaagctgtggatcaccatgaatgagccctacaccaggaacatgacctacagcgctggccacaacctgctgaaggcccacgccctggcctggcacgtgtacaatgagaagttcagacatgcccagaatggcaagatcagcatcgccctgcaggccgactggattgaaccagcctgccccttcagccagaaggacaaggaggtggccgagcgggtgctggagtttgatattggctggctggccgagcccatctttggaagtggggactacccctgggtgatgagggactggctgaaccagaggaacaacttcctgctgccctacttcacagaagatgagaagaagctgatccagggcacctttgacttcctggccctgagccactacaccaccatcctggtggacagcgagaaggaggaccccatcaagtacaatgactacctggaggtgcaggagatgacagacatcacctggctgaacagccccagccaggtggccgtggtgccctggggcctgaggaaggtgctgaactggctgaagttcaagtatggagacctgcccatgtacatcatcagcaatggaattgatgatggcctgcatgctgaagatgaccagctgcgggtgtactacatgcagaactacatcaatgaggccctgaaggcccacatcctggatggcatcaacctgtgtggctactttgcctacagcttcaatgacagaacagcccccaggtttggcctgtaccgctatgctgctgaccagtttgagcccaaggcctccatgaagcactacaggaagatcatcgacagcaatggcttccctggccctgagaccctggagcgcttctgcccagaggagttcaccgtgtgcacagagtgcagcttcttccacaccaggaagagctag

SEQ ID NO: 138 - RNA, 2946 nt, synthetic construct
  source 1..2946: mol_type = other RNA
atgcccgccagcgccccccccagaagacccagaccccccccccccagcctgagcctgctgctggtgctgctgggcctgggcggcagaagactgagagccgagcccggcgacggcgcccagacctgggccagattcagcagaccccccgcccccgaggccgccggcctgttccagggcaccttccccgacggcttcctgtgggccgtgggcagcgccgcctaccagaccgagggcggctggcagcagcacggcaagggcgccagcatctgggacaccttcacccaccaccccctggccccccccggcgacagcagaaacgccagcctgcccctgggcgcccccagccccctgcagcccgccaccggcgacgtggccagcgacagctacaacaacgtgttcagagacaccgaggccctgagagagctgggcgtgacccactacagattcagcatcagctgggccagagtgctgcccaacggcagcgccggcgtgcccaacagagagggcctgagatactacagaagactgctggagagactgagagagctgggcgtgcagcccgtggtgaccctgtaccactgggacctgccccagagactgcaggacgcctacggcggctgggccaacagagccctggccgaccacttcagagactacgccgagctgtgcttcagacacttcggcggccaggtgaagtactggatcaccatcgacaacccctacgtggtggcctggcacggctacgccaccggcagactggcccccggcatcagaggcagccccagactgggctacctggtggcccacaacctgctgctggcccacgccaaggtgtggcacctgtacaacaccagcttcagacccacccagggcggccaggtgagcatcgccctgagcagccactggatcaaccccagaagaatgaccgaccacagcatcaaggagtgccagaagagcctggacttcgtgctgggctggttcgccaagcccgtgttcatcgacggcgactaccccgagagcatgaagaacaacctgagcagcatcctgcccgacttcaccgagagcgagaagaagttcatcaagggcaccgccgacttcttcgccctgtgcttcggccccaccctgagcttccagctgctggacccccacatgaagttcagacagctggagagccccaacctgagacagctgctgagctggatcgacctggagttcaaccacccccagatcttcatcgtggagaacggctggttcgtgagcggcaccaccaagagagacgacgccaagtacatgtactacctgaagaagttcatcatggagaccctgaaggccatcaagctggacggcgtggacgtgatcggctacaccgcctggagcctgatggacggcttcgagtggcacagaggctacagcatcagaagaggcctgttctacgtggacttcctgagccaggacaagatgctgctgcccaagagcagcgccctgttctaccagaagctgatcgagaagaacggcttcccccccctgcccgagaaccagcccctggagggcaccttcccctgcgacttcgcctggggcgtggtggacaactacatccaggtggacaccaccctgagccagttcaccgacctgaacgtgtacctgtgggacgtgcaccacagcaagagactgatcaaggtggacggcgtggtgaccaagaagagaaagagctactgcgtggacttcgccgccatccagccccagatcgccctgctgcaggagatgcacgtgacccacttcagattcagcctggactgggccctgatcctgcccctgggcaaccagagccaggtgaaccacaccatcctgcagtactacagatgcatggccagcgagctggtgagagtgaacatcacccccgtggtggccctgtggcagcccatggcccccaaccagggcctgcccagactgctggccagacagggcgcctgggagaacccctacaccgccctggccttcgccgagtacgccagactgtgcttccaggagctgggccaccacgtgaagctgtggatcaccatgaacgagccctacaccagaaacatgacctacagcgccggccacaacctgctgaaggcccacgccctggcctggcacgtgtacaacgagaagttcagacacgcccagaacggcaagatcagcatcgccctgcaggccgactggatcgagcccgcctgccccttcagccagaaggacaaggaggtggccgagagagtgctggagttcgacatcggctggctggccgagcccatcttcggcagcggcgactacccctgggtgatgagagactggctgaaccagagaaacaacttcctgctgccctacttcaccgaggacgagaagaagctgatccagggcaccttcgacttcctggccctgagccactacaccaccatcctggtggacagcgagaaggaggaccccatcaagtacaacgactacctggaggtgcaggagatgaccgacatcacctggctgaacagccccagccaggtggccgtggtgccctggggcctgagaaaggtgctgaactggctgaagttcaagtacggcgacctgcccatgtacatcatcagcaacggcatcgacgacggcctgcacgccgaggacgaccagctgagagtgtactacatgcagaactacatcaacgaggccctgaaggcccacatcctggacggcatcaacctgtgcggctacttcgcctacagcttcaacgacagaaccgcccccagattcggcctgtacagatacgccgccgaccagttcgagcccaaggccagcatgaagcactacagaaagatcatcgacagcaacggcttccccggccccgagaccctggagagattctgccccgaggagttcaccgtgtgcaccgagtgcagcttcttccacaccagaaagagctag